European Patent Application EP 4 702 981 A1, published March 4, 2026. Title: Targeted Antibacterial Treatment. Applicant: University of Copenhagen. Application EP. The sequence listing filed with the application follows.

SEQUENCE LISTING (16 sequences)

SEQ ID NO: 1 - DNA, 110 bp, synthetic construct
  source 1..110: mol_type = other DNA
tggccactttcggacaagcggcacattgtgcctattgcgaattaggcacaatgtgcctaatctaacgtcatgccagccacaacggcgaggcgccaagaaggatagaagcc

SEQ ID NO: 2 - DNA, 222 bp, synthetic construct
  source 1..222: mol_type = other DNA
atgaagcctgacgcctctaaccacaacccagacccgcgctacctgcgcgggctgctcaagaaagccggcatcagccagcggcgcgcagccgagctgctcggcctcagtgacagggtgatgcgctattacctgagcgaggacatcaaggagggctaccgccccgcgccgtataccgtccagttcgccctggagtgcctggcgaacgacccgccatctgcgtga

SEQ ID NO: 3 - protein, 73 aa, synthetic construct
MKPDASNHNPDPRYLRGLLKKAGISQRRAAELLGLSDRVMRYYLSEDIKEGYRPAPYTVQFALECLANDPPSA

SEQ ID NO: 4 - DNA, 972 bp, synthetic construct
  source 1..972: mol_type = other DNA
atgagttcagtacaaaccgttcgtgggccggtggacacagccgatctgggaaaggtgttgatgcacgagcatgtcttcgttctgggggaggagatgcgtcagaactatcccgactacccggagccttgggacgaggaggctcgagtagccgatgcggtgaccaagctgtccgaactgaagtcgcgagggatcagcacgatcgtcgatcccacggtcatcggactcggtcgctacatcccgcgtattgcgcggatcaacgagcaggtcgatctcaacatcatcgtcgccaccggcgtctacacgtacaacgacattccgttccaattccattacaccggtccaggtttgctgttcgacgtgcgcgagcctatggttgatctatttgtgaaggacatcaaggacggcattgccggcacagacatccgcgcgtcattcctcaagtgcgccatcgaagaacctggtctgactcccggtgtcgagcgtgtgatgcgagcggtcggtcaggcgcaggtcgaaaccggggtaccgatcacggttcacacgaacccgcacacggaatcgggcctcgttgcgcagaaggttctggccgaggaaggtgcagatctgagcaaggtcgtcatcgggcactcgggtgattcgaccgacctggactacctgtgtgcacttgccgatgcgggttcgctactcgggatggaccgtttcggtctcgatgttctgctgccgttcgaggagcgggtgaacactgtcgtggaactggcccgccgtggctatgccgagaaaatggttctggcacatgatgcctcgtgcttcatcgactggttctcgagtgaggccaaggcggccgcagtaccgaactggaacttcacccacatcagcgatcaggtcattcccacgctgctcgagcgcggcgtcaccgaggatcagatcaacaccatgctggtggataatccacgtcggtacttcgagagctga

SEQ ID NO: 5 - DNA, 810 bp, synthetic construct
  source 1..810: mol_type = other DNA
atgatcaccacaaagactgtcaatggcgtgcagatcgccttcgatgaccaggggcatgaaccaggcccggtgttcgtcacgctgagcggttgggcgcacgatcttcgcgcgtatgacggcatgctgccgtatctacgggcagcgcagcggacggtccgcgtatgttggcgcgggcatgggcccgatcggaatctagttggcgacttcggtattgacgagatggcggcagacacgatcggcctgctggatgcgcttgaggtggacagtttcgtaccaatcgcccacgcgcacggtggatgggcggcgctcgagatcgctgatcggctcggcgctcagcgggtcccggccgtgatgatcctcgatctcatcatgacgccagcaccgcgggagttcgttgccgcgctgcacggtatccaggatccagagcgctggaaggaagggcgtgatggcctcgttcagtcgtggctggcggggaccaccaatcaagcggtgctggatcacgtgcgatacgacagcggcggtcacggttttgacatgtgggctcgtgctggccgggtgattgacgaggcctaccgaacctggggatcgccgatgcggcgcatggaggctctggcggaaccgtgcgcgatccggcacgtgttctcacatcccaagatcggggagtacgacgcacttcacgacgatttcgccgcccgccatccatggtttagctaccgtcgtctcgggggcgaaacacacttccccggcattgagctgcctcaacaggtggcggccgaagcgatcgatctgcttgctggcgcgcgcatctga

SEQ ID NO: 6 - protein, 323 aa, synthetic construct
MSSVQTVRGPVDTADLGKVLMHEHVFVLGEEMRQNYPDYPEPWDEEARVADAVTKLSELKSRGISTIVDPTVIGLGRYIPRIARINEQVDLNIIVATGVYTYNDIPFQFHYTGPGLLFDVREPMVDLFVKDIKDGIAGTDIRASFLKCAIEEPGLTPGVERVMRAVGQAQVETGVPITVHTNPHTESGLVAQKVLAEEGADLSKVVIGHSGDSTDLDYLCALADAGSLLGMDRFGLDVLLPFEERVNTVVELARRGYAEKMVLAHDASCFIDWFSSEAKAAAVPNWNFTHISDQVIPTLLERGVTEDQINTMLVDNPRRYFES

SEQ ID NO: 7 - protein, 269 aa, synthetic construct
MITTKTVNGVQIAFDDQGHEPGPVFVTLSGWAHDLRAYDGMLPYLRAAQRTVRVCWRGHGPDRNLVGDFGIDEMAADTIGLLDALEVDSFVPIAHAHGGWAALEIADRLGAQRVPAVMILDLIMTPAPREFVAALHGIQDPERWKEGRDGLVQSWLAGTTNQAVLDHVRYDSGGHGFDMWARAGRVIDEAYRTWGSPMRRMEALAEPCAIRHVFSHPKIGEYDALHDDFAARHPWFSYRRLGGETHFPGIELPQQVAAEAIDLLAGARI

SEQ ID NO: 8 - DNA, 207 bp, synthetic construct
  source 1..207: mol_type = other DNA
atgaaaatcaccaacgacaccaccacctacgaagtggccgaactgatgggttcggaggctgacgaactcgatggacgtatcatgatggggctgctcagccgcgaatgcgtggtagacactgacgacctgagcgaggatcaatggctggctctgatcgacgagtcgcagaaggttcgccgcgagcagttcgaaagcgatgaagcctga

SEQ ID NO: 9 - protein, 68 aa, synthetic construct
MKITNDTTTYEVAELMGSEADELDGRIMMGLLSRECVVDTDDLSEDQWLALIDESQKVRREQFESDEA

SEQ ID NO: 10 - DNA, 36415 bp, synthetic construct
  source 1..36415: mol_type = other DNA
tgtggggaggtgactgttttgacacatgccaaaagagggagggataggccagagcccctatagcactagggctccagccggacagacgctgtgggacagtttggaaaaaatcgatcaggattgagcaaggaatgcaaaatattgatcgttaattggcgcggaatgagcgctaaaccatccatcgcccaagccagacaacgcgcccaatgatatccaagtcagaaagctggtccttggggacgaccatgtccttatacgccttgttttcgctgatgatcgcgatagagccatcgaactgccgttgtaagcgcttggcgtagagctgatccccgacccgaatcacatagatcgcttcatcccgcacggttctaaggtcatggtcgataacaacggcgtcgccatccgacaggaggggttccatggagtcgcccccgacccttactgccgacatcctggttggctctaaccccttcttgctcaagctgtagcgcgtaaaggcaagctgcgtaagaacgtgtgcgccttcgctccagcttccatgtcccgcgctgaccctcgcgtcatacagggggacgtagacatattggtccgatcccgtagcctcctgctcttccggcttctgactgccctcgccggtcataagccagcccaggctcacgcctgccgccttggccaaggaaatgagcactctccgggtgggttccccgcctttcaagtacctctgcaacccgccttgggagattccagcattcctcgctaaagcacttgcgctccctgctatagcgacaatggagcgcagcctttcgatgaaggcagcgtcattttcaggttcggttgcggaacttgaaaggctggcggtgcgctcgctacgcgttttcatgtagacctaactatttgatttaattgatattaattctatagaggtcgaaatctacctcctatagaacttgaaaaccgctatagagcttgtttttcaacttctatagcgctatgtttatgccctaagtcacgttagacacccctaaaaaaaaccaccctgccaggtggtgagatggaacgtaggcatgaacagaacccgaaatcccccgcgacaacaacgtcccgctgggagtggatcaaatacccagctccgcgccagggggtcgtccctggccgaggtggcccgctccctcgacgtatccagcccggcagtcaaaaacgccaagctgaatccctacccctcgggtagagcgcgccatcgctgctgtactcgacctcagccccctagtgctgtggcctgagcgctggctcgacgacgagaatccgaagcggcaacggcccaatcgctcggagaccttgcaggcatatgtcagacatatgccaagtgctgaggaaaataccagatacgctgaccaagcgcagcgtaaagccgacgcgggggcttgaacatggcccgccgcaaagacgaccgcaccctggacatcttcgatgttccgcagccagcccgcgctatacccggcgagtgcaactatgccgcccaggtcagcgagctggtcagcgaaattctgaaggccgccaacctcgaccgttacgaggtcgccgcccgcatgtcgcgcctatctggcgatgacgtgagcaagaacatgctcgacgcctggtcgagtcccgcccgagctgatcacaacttgcctttctaccgcgccgccctcctggaggacgtctgcgcgagccacctgctgaccaactggctggtcgatgtgcggggcggccgcgtggcctatggccgagacgcactgctcgccgagctgggccgcctggagcggacccgcgaggaagcgggtcggcaggcgcgtgagctgaaacgaatcctgggggagccgtgatgacaaacaccgacctcaaaccgctgctcgacaacctgcggaacgccaccgagttctggaacctagtcaaagaggccagcgctacggacgaaagcaccgttcacaaccgctcctaccgggacgcactcgactggctcgaatcggcggccttggccctcggtgacgccctgatcgcccagcgcaaagctgtcgggggcgaccatgaatgaatggttctccgcacagaaactggtcggcctgcccggactgcctggcacggttcaaggcatcaatagtcgcgccatccgcgactcatggcagcaaagaaaacacatgggtagaggcggtgggcgtgagtaccacatttccagcctacccgacgaaacccgcgccgcactgctgaacgccgccctgggcgaggtggccaccaaggtggtccgccaggagacgcagctggccctggtcgaaaccaaccgccagcagctggtcgccgatgctcggcagggggtgctgcacgccctggacctgatgatggcccgcaccggctacagccggaagcgctccatcaccctgatgctggacatggcgcgcctcggccaggtcgagccgcagctgctcgcgatgctcaagatggcccgcgatcctcgcggccgcccgagcgcggatggcctgccgagcgtgcgcagcctggagcgtttcctggaccaggccgagcgcggcgccctggtgccgaaggtccgccgcccggacatgagcgttcccgactgggcgccggccttcatgacgatctaccaggggccggagaagcgcagcgcccgcgctgcccatgcactgctggagaagcactggcaggggcaaatgcccagcctggaccaggtttatgcgttcctgcgtaaggtcggcaacgtcagtcgcgaggtcgggcgcatgggtgagcatgaaataaaggcgctgcgcccgttcattcgccgcgacttcaccaagttgctgccgaccgacgtctattcctgcgacggccacacgttcgacgccgaggtccagcacccgatgcacggccggcctttccggccggaaatcaccaccatcattgacatccgtacccgccgcattccgggatggtccaccggcctggccgagtcggccctggtggtggtcgatgccctgcgcgacgcctgcaccaagggcggcatcccggccatcttctacgttgacaacggctcgggctacgtcaaccacatgatgcgcgacgaggcggtcggccttatgggccgcctgggcatcgatatgaagaacagcctgccctacaacagccaggcgcggggcgtgattgagcgcgtccaccagagcctgtggattcgggccgccaaggaactgcccggctacatcggcgccgacatggaccgccaggccaagctggccaccttcaagctgacgcgccgggccatcgccaagggcggcaccatgccgctgatgtcttgggaatcttttgtcgcgttctgcgaacagcagattgccgaatacaacgaccggccgcacagcagcttgccgcgcatcgttgacccgaacaccggccgccgccggcacatgacccccaacgaggcctgggcgctgcacgaagcggagggtttcagcccgatgcgcgtcaccgacgacgaggcccggccgctgttccggccccaggtgctgcgcaccgtccgccgctgcgaactggagttcatcggcaaccgctacttcgcccgcgagctggaggaattccacggcgaccaggtggccgtgggctacgacatccacgacgccagcagggtgtgggtctacgacggcgagggccgcttcctctgcaccgcagagctgaacggcaacagccgcgactacatgccggcttcgtatgtcgagcgtgcccgcgagaaacgcgcagaggcccgcgagaagcgcgccctggctcacctcgacgagattcgcgccgagcgtgacggcgggtatgccctggaaatggatgcgccgctgtccatccccggcctcggcacgatcacccctgagcaactccggtcgcgcagcgccgcgaccctcgaaatgcaggccgagcggatcgacgaaccgcgcccggccgcagccaccgcccaagccaccaccgcccaggtcttcaccctgccgaccgctcccgcccagcgctaccggcagtggtgcgagctggccgagcggcaacgctccgggctgcccatcgagccggacgccgcccagtggttcgaggtttaccccaaatccaaagaattcgccgcccagcagcggcaagcatgaaaggagctgtattcatgaccaccccgaaaaccacccaactggccaatggcatggccgacatcgccaacatcgccctttgcgatatcgccctggagaaagcgctgtcgcgtacctccacgttgcccggcctggtctgcttctacggcccgtccggcttcggcaaatccgtttcggccgcctgggtcgccaatcgccgccgcgcctactacgtccaggccaaaagcgtctggacccgcaagcacacgctgaagtcgatcctgggtgaaatgggcatcaagccggctggcacgatcccggaaatggccgaccagatcgccgaggaactggccgccagcggccgcccgctgatcatcgacgaaatggaccacctggtcgccgctggccaggtcgagctgattcgtgatctgtacgagtccagccaagcctccatcttgctgatcggcgaggaaatgctgccgaccaagctgaagaagttcgaacgcttccatggccgcgtgctgagctgggttccggcccagccagtctccctggaggacgcccgcaacctggcgccggtctacagccccggagtggctatcgctgacgacctgctcgcgcacttggtgaagaagtcactgggctctgtccgtcgcgtcgcggtgaacctggagcagttggccgaggccgccaccgttcagggccggcgcgagctggaactggccgacctccagcgcctgaacctggagctgtataccggcgcggccccgaacccgaggacgtcgaaatgagcctcggcaaaaacccggctcacctgtccatggtcgggggcaagagcccccgccagcagatgtgggaagtcatccgggccaaccgcgaagagttcaccgtctaccgcgtggcgcgccgctccaaccagcacgacaagaccgtcgagaagtatgtcgcctgcctgcgcctgggcggctacgtcgaggcgatccgtggattcaagcgcggcgaagaggtcgttttccagctggtccgcgacaacggcgtcgaggcaccgaacctgaacgccgatggcaagccatcccagcagggctacaccaccgaggcggtctggcggacgttgcgcatcctcggtccagcgaccccggagcagatcgccgcatcggtggcggcctctggcgcgactgtgtcgcccagcaccgttcagcgctacttcatcgatctgcagaacgccggatacctgacccgcaacggccgccactacgccctcaagccgggccgctacaccggtccacggccgcccatcgtccagcgcgagacgcgccgccaggtctacgacccgaaccttgaccaggtcatgtggagttcgcacggcgagtaccagcacaaccggagtcgttcgcggggcgcttcccaggctggcgtggcggataccgaagagaacaacgaatcaggcggctgaagccgtgatgaagacggtgccgaggggtggcctcccctcgacacctaccaccacccggaaggagaggagccatgcaaatgcatgcacagcaaggcggtagcgccgcgaaggctagcacaagccactttcgcggcactacgaacattgaggagtacatccgcgacatggcgagccgtgggttcagtcgtcgggccgtgagtaaggccctgggtatgcagtcgcggaagttcaaggaactcctggaactcctgccagaaatggactgggtgcctccttgtcagtcgtgggaccgcctgcgcgctgaccaggagaagaagggacgcaagtgtccgatgacagaggggcgtctgcgctcgattgtcgcggcgaggcgcgccgcgatggcaaaacacacccgctacaccgcgtttggtgtaacagccaccttgccggagctggtgagccagttcggccaggtcaccgccgccaccgtgcgcatgcggttggccaagggaatgcctctggagcaggcccttgcctccgtgcgcagcgatccttgtggaaggaaggtcgcagatagccatccctggaaacaggaggcgcaccagggggctatcaatcaccttgagcgtcaaaccgctgcaatgcaggaacgcgttcagggggagcgcctggaccgggcggcctcactgctgagccaggaggtgccgccatgcgccgaacactgatccccatcggcatcttcctggccctcggcctactgctgatcctggccggtgatgccctgatgctcggccgccgcctcattgcctggcagtgggggtgctgatggaacgcgcaatcgatctgtcggcctggggcgagcgtccgcccgtcttcgtccaactgctggccgccgaggtggcccgcagcagccagacgaaagccggcgaggcaatcggcatgagccgttcgaccgtcagcaccatcctcgccaaccgctacccgtcgccctcgacgatccgcgtcgagcgccgcgtcctggccgcgctgagccgtattgagtgcccggccttgggcgaggcggtgacctcggtcgagtgcagcgagtacctccagcggccggcgccgctgaacaaccccgtcgcgatgcgctgctggaaagcgtgccgcgcctgtccacgcaacccgcataccgcccccatgaaacgagaggaacaaggccatgagaaccgcattgcccttgaaagtcttgacgcctgacttggcccagagcctgcgcaccttcaacgacgccgcccggctgctccagcgcatgggggtccgccttcatcgcctggagccgacagaggggcgcgtgaccatcgccgcagatgacgcccgccagctcctggagaaaggctacctgatgggcttccagcgcgacgcctcggccggcagcacccgttacatcacccgcttccagggcatcaccctggcctggagcgaaccgatcagctaccgcgacttcgccggcagcaaatccgtaattcactgaacaggagaacgccaacatggcaccgaagaaacgtctgaaatccgctgccgccgtctacgtcccgcagacccgcgaacaggtcatcagcgatatcaagaacatcggcgacctccagcgcgagctggcccgtctggaaaccgcaatgaacgatgaaatcggccagatcaccgagcgctattcggagccggccgaagacctgaagaagcgcctggcggtcctccagggcggagtccagtcctggtgcgaggccaaccgtgccgagctgaccgacaacaacaaggtcaagtacgcgaacctcacaaccggcgaggtccagtggcgcatccgtcccccgtccgtgactgtgcgcggcgccgatgcggtcctggagctactgcgcagcaaggggctaatccgcttcatccgcaccaaggaagaggtgaacaaggaagcgatcctcaacgaacccgaggccgtccaggggctgccggggctgaccctgaacaccggcatcgaggacttcgccatcgtgcctttcgaagcggaggtgcagtgacatggccgacaccatcgctttctgctgggcctctggcctgatccagttcggtgaccaggtgcccgagggcgccatcgagatcgcccgtggggacgaccaggtcgttcgcgaaaacctcgtgaccaattcgcggcacgcttacgacaacgtgtcgctcctggttccgggcgtacccgaagcggcaaaccaaaccgagggcggggacgcactggagtgcttcatccgtcttctcgccaagtacgacagcgccgctttccaggtcgcttatgtggaggacgtgtgacatggcacgcaaccgcgcgcaacagctgtgcatcgcaccttggactatcagcgcttcctgttaccccaggctgatgcactcaagctgatagacatcatgagtcgagccgcagaggttcaggccgactacgcctctggagctggattcaagtacaccgtcggcgaagtgccggaagtcgagttgacgatagtacgccccagtcaattggtcatgccgcaggccgagccggccccagctacaccacgcgctcgccggaagtctccggcccaggtcacgcacgatgccattcggctgttggaggggctctgatcatgaccaagacgttcgccatgtgccgcatcgacggcctgatcgagctgcgggaggaacacccaggcgagggctacttcgcccttgccgtgggcgacttggccagcgtgcgggcggcggtctttgcaaccgctgagccgcaccaggtcggcaagaaagtcgcccggcgcgtgccgggtgtgagccccgacgccaccgaccgcgaaaacctgggctccatcgcccggtacatccagaccctgggccagcaggatcggcccggcttccgtgcgctgggggtgtgaaatgcagcagtccaaccccttcaatcaccccggacagagctacggcgccgtagacgtcgatagccgactccgcgccgttgccggcttcgacctggagcaatgccgcgccgcgctcgcggtcaccggcctccagaagatcgtcgagcagaaaattcgcacccgcatccgccagctggaaaagcaggcatccgcacagaaggaggcatagccatggccgtatacaccatcaccctaagcgacaccgaaggcggaatagatttctccatgcaaggcccgccgctgcacgactccgaagcatcgaagatcgcctacgcccttatgcaatcgaccatgtccctcggccgagaactcgcaaagcagaacggagttggtaacgccgtttcctgcgcctgcgacgagtgcctggcacggcgcgctcgcggtgaggaaccgcagcaggaaatccactacaccacggccaagaaccgcaccgtccactgagcgaaaccgccccggcctggccgggacggtctgccggacgtggtggtccggtactgatgagcagccacccatgacgaacgaaaccaagacagaccgccagcgccgcctggcgcgggaacgccaacgagcgaagcgcgagcgcgatgccctgcgccgcgctgcgctgggcggtcgccgcttcaacatggacatgtaccagggaacggctgatgcactcgatctgatctgcgcggccggtggcttcgccgagccggccgaggcggtcaccttgctcctacacaacgttgccgaaattgcagaacgtgacgcgtcacgctttgccgaattgatccaaaagagaagccatccagggaggaccaagcgatgagcctacgcgccgtcaacctcgcaaaaatccacatcgccaaggcccagctgggcatggacgatgacacctatcgcgcattgctcgctcgcgtcgcgggcgtgcgctcggccaaggacttagggccgcgccagattgaccaggtactggtcgaactccagcgtctgggctggaaaccgaagagcaaccggcaaggccgggcgacgccaaaagtgccgcaaaaccggcaaaccgtgctgcgcaaaatcaccgcgctcctggccagcgcccatcgcccctggagctacgccgaccatatggcccggcgcatgttccaggtcgagcgggtcgagtggctggacgacagccagctctaccggctgatgcaggcgcttatcatcgacaggagccgccatggccaggtctgaggtggatcttcgggaggtccaggacatgctgccggataccgtccgcgacatggccggacgcatcggcctgccggccacgctggtggtagtcgagcagctcggcggcacgtcctggcggatagccgagggccgggcgcggaggggcgaagcgcgccgggctgcgctggccgagctggtgggcagcgacatcgaggagcagctccacacgcactatcggggcgaagaaatttacgtggctcgctgccacaaggcgctggtacggtggcgcgatctggagatcgtcgagcgcttcgaacagggcttgcgtgacgggcaaaccgcccgtagcctgctcagcgatctagcccgccaatacaacttgtccgaccgctggatatgggagattgtcaaccggccgagcgagccggcaccgcagcaatccaccctgttccactaagccggggcgcaacgccccggccggcgtctccgcgccgaccctgtctcagccgttgaaccccttccgctaatcccgcgtcgcactcaccgccacgatggcggcatgagcacatctagccccccaacgtctctacgcagcccccgcgactacgccgccgccatcctggccgagcccagccgcgagcgtcgtaacgctctgctggaagcctgcccggtcaactggcagccacttgttcgggcgcacgtcgaggacgccttcgcgaaggtcaaggcgtatcgccagatgatggaccaccgcgccgagtcgatccggcgcggcccgcctccagctccccgcgtcaccgacaccgatttccgcatatccaactacaccaaatccgccccggaggtaggcaatgcgcacctatcagcaattcgggcagcgctcgcaacggaagcaccaaatgcctgatcccgcatccacctcggccggcagcgccgcgctgctgaaaatgtttggcatccatatcagcgcgggcgccctggccgccgccctgggcttcctggtcctgtggcccaggaccatgaaagaggggtttgcccggctgttctgcaccatcgtcgcgtccagcgtcttcggcccgatcctggtcgtttacctgcactccaaccgccccgagctgttcgagtccgcccaggtggtggccgggctctaccagttagagccggcagtcggcctgctgttcgtttccgctccgctcctggtgattgccggtctgcccgcctggtggctgatcggggcggccctgcgcctgtttgagcgggacggcgattcatggctgggcgcgttcgcccagtgggtaaaacgcaaactggagaacacctgatggcccttcaacctcgcggcatccgcaacaacaaccccggcaacatcgtctggtcggcacgcaacaactggcagggccagctcccgcacaacccgaaggtcgagccgcgtttcgcccgtttcgataccgcacataacggaatccgcgccttggcaaagctgctgctgaactatcgcaaggtccacggcctgcgcaccgtcgaatcgttgatcgcacgctgggcgccgtccaacgagaacgacacccgcgcatatgccacggccgtggcccgagccatgggggttccaccgcaggccggcctgcacatggaccaggacaccctggccgccctggtgaccgcgatcattcggcacgaaaacgggcagcagccctacagcgccgagcagatcgcccaggccgtgcgggaggtgctgtgatgcaacgcctgcggttggcagcaactaaaggccgcactctggttggcgtgatcctgatcgagaccggcctagccctggtgcgggctggtaccgggctgctgccgaggtcttccgaatgacctggcgcctcggcttggccctggccctgttcctggtgatggttgcgaccagcgcctggtggagtggtcgcgtggcgggcctggccgatgggcgcgccgcctgcgccgacgcacagacccgcgcctaccgcgacgtcctggagcaatcggcggcacaactgaaggcggtccaggacaccagcgcggctcttttccagcgcctggcccagcgggccgacagcgaccaacaaactactcgggagcttcgccatgccctggccgaaaccgctgctgatcgcgctgcctgccgctttcctgctggcgtcatgcagcagctcgaaaccgcccgtcaacgtgccgcccaggccactaccggcggccttggctcaaccgtgcccgaccccggtggcggtgactgatgacagccccgatgccaccgcaattgccctcaaacaactctacgaccaatacggcctctgcgccggactgcactgggacaccgtgcggcaccttcaaaaggactgatccgatgaccgaaaagaaagcctctcccgagttcgaactgctgcaacgcatcgacggccgcctggagcgcttcgaggaccgattcccgcagatcgagcgtaaggccgtgctgtacggctcggcggccggcgcgctggcgggtggcctggttgcctgcggcctgctcgcggcgcgtatcaagctcggtatctgaggtagtcatggcgcacccgaaggaaacccgcgacgccctgcgccgcgcctacgtcctcgaccgccagtccctggaggtcgcggccgccatgttcggcgtctcctacggcaccgcccgccgctggaaacagcaggcggaagccgagggggacgactgggacaaggcgcaatcggcgcagttgctggccggtggtgggctggaggacgtggcgcgccaggtgctggccggcctggtgacccagttccaggccacgatggaagccatccaggtagacgcggacatcaagcccgccgtgaaagtgcagctgctcgccagcctggccgatgcctacaacaagacggtcagcgcgtccaagcgcgttctgcccgaaacatcagcgctggccaccgctatggaggtgctccagcgcctggccagcttcatccgtgagcggttcccgcagcacgcccaggcattcgccgaggtgctggagccgtttggagaggtgattgcgaaggagctgggctgaccaacctattcgctgaaggggtcgtaccgactgacaaccacgggtccgctatcaggaatcttttcgacatgaacaacagaattgcaggggtgacatttcaaggccttgtaccagccatcattgcaaggctgaagaatggtcttgattcctttttggtagcaatcggcacatatgtgatgcagaggttcggtgccttgaacctctggctttatgcgatacacaagtccacccgcttccgtctggtggagctggtagcgctctttctcctgttcccagcgtttgaactgagcaatttcggcttccagctcgcctatgcggcgggtcagcgtcgtctgatccgcatgggcgctgttcagctgggattgcagcccgagcagcacgccgttcagttcgaccaccttggtcgttacagccgcatccgtcttgagcgtgagcatgctctgcgtaatgtcagtggccgccttgatgccgccgtaggcaccagcaatccagtccatcatgaccaggttccttctggggagaaatcgacccatgaagggtagcaccagagacttcctggcggatattgcccagctcgcgggggagttccgccgccagatcgaggccgaggtcgcaggcttcgaccccgacccgaaggccagcgccgtccggcgtgaacgggccagcgcggactatgagtatttcgcccggacctacttcccgcactacgtgaagcgcggtaacgcgctgctccacgactacctctacaagcggttgcccgagctggtggaccacccggacggccagcacgaagccattgcggcgccgcgtggtaatgccaagtccaccctggtgagccagatattcgtgatctggtgcgtactcaccggccgcaagcattaccccctgatcatcatggatgccttcgaacaggccgccacgatgctggaggcgatcaaggcggagctggagttcaacccgcgcctggccatggacttcccccagggcgccggcaagggccgcgtttggcaggtcggcaccatcgttacggcgaacgatgccaaggtccaggtcttcggctccggcaagcggatgcgcggccttcgacacggcccgcaccgtcctgacctggtgatcggcgacgacctggagaacgacgagaacgtccgcagcccggagcagcgcgacaagctggaaaactggctgaagaaaaccgttctgtccctcggctcggccgacgacaccatggacgtgatcatcatcgggaccatccttcactacgactcggtcctgtcgcgcctgctgaaaaacccgctgtggaagcggcgcaagttcaaggcgatcatcgaatggccgcaccgcatggacctgtgggagaagtgggaggaacttctgctcaactccgacgacgagggcgccgccgctctggccttctaccaggaacgcgccgccgccatggaggacggcgcgatcatctgctggccggatgggcagcccctctacaagcttatggtgaaacgtgcccgcgatgggcactcggcgttcgactcggaacagcagaacgacccagtccagggcgagaacgcccccttcgccgcctgcatcacgttctgggtcaaccgcctggcgcagtggatgttctacggcgcgtgcgacccgtccctgggtaagcaaggttccagccgcgaccccagcgccatcctggtgggtgggttcaaccgggagacaggcgtcctggacgtggtcgaggccgccatccgcaaacgcctgccggacaagatcatcgaggacatcatcgccatgcagcgggcctatcactgcctggtgtggggcgttgaggcggtccagttccaggagttcctgcgcaccgagctggtgaagcgctccgccaaggctggctgcccagtacctgcccgagcgatcacgccacacgccgacaagctactgcgcatcgaaagcctccagccgcacatggccaacggcctgatccgtctgcatccaagccagaccgtcctggaacaacagctgcgccacttcccggccgcagaccacgacgatggccccgacgccctacacatgctctggatgctggccacgacggggttcgcgccgatagaggcgactttggtcaaacgccggcatgaatacgcgcccggccttgacgattcttttgacactggcggccgcttcggcggcgcatggtaggtacaacacatggcacaaatcgttgacgtctacggcaacccgatccgaactcagcagttgcgcgagccgcagacctcgcgcctggccggcctggcgaaggagttcgcccagcacccggccaaggggctgacgccggccaagctggctcgcatcctggtcgaggccgaacagggcaacctccaagcccaagccgaactgttcatggacatggaggaacgcgacgcccacctgttcgccgaaatgagcaagcgaaagcgcgcaatccttggcctggattgggcggtcgagcccccgcgtaacgcctcggcggccgagaaagccgatgccgactacctgcacgagctgttgctcgacctggaagggctggaggacttgctgctcgatgcgctggacggcatcggccacggctacagctgcatcgagctggagtgggcgttacaagggcgcgagtggatgccgctggcgttccaccaccgaccgcagagctggttccagctcaaccccgaagaccagaacgagctgcggctgcgcgacaacagcccggccggcgaagccttgcagcccttcggctggatcattcaccggccgcgtgcgcgctccggctatgtggcccgcagcggcctgttccgcgtgctggcctggccgtacctgttccgccactacgccacctccgacctggcggaaatgctggaaatctatggcctgccgatccggctggggaaatatccgccaggtactgccgacgaggagaaggcaaccttgctgcgggccgttaccggcctgggacatgctgccgcagggatcatccccgaaaccatggccatcgacttccagcaggccgcgcagggtagcagcgagccgttcctggcgatgatgcggcaaagcgaagacgccatatccaaggcggtcctgggcggcaccctgaccagcaccaccagccagtcaggcggcggcgcttttgctttgggccaggtgcataacgaggttcggcacgacttgctggcatccgatgcccgccagttggcggcaacgttgtcccgcgatctgctctggccgctcctggtgctgaatcgccctggtagtcccgacgtgcgccgggcgccgcgcctagtcttcgacctgcgcgagcaagccgacatcaccagcatggcgcagtcgattccggcactggtcaacgtggggctggagattcccagcgcctgggtctatgacaagctcggcatcccgcagcctgccaagaatgagccagttctgcgttcggctgcgcagcctgcgatcctgagccgacagcatggacaacgggtggcggccttggccaccatcgttggcccacgctatggcgatcagcaggcgctggacaaggcgctggctgacctgccggcgaaggacatgcaaaaccaggccaacgacctgctcgccccgctcctggaagcggtcaaccgcggagacagcgaaaccgaactactcggcgccctcgccgaagcgttcccggacatggatgacagcgccctgacggacgcgctccaccggctgctgttcgccgccgatacctggggccgtctccacggcaacctggaccggatcgactgatggccgctccgaccgaagccgatctgcgggccatcttcgccctgcggccggccgccgctatcgagtatctggagcgcaagggcttcgcgatcacttggaactggcatgacgttgacgcggccacccacgcccgcgctctgaccgttgccagagcagcacgcctggacgtgctccaggacattcgcgacgccctggtcgagaacctggagcgcggcgagacgctacgagatttcaagcgcaacctgcggccgaccctggaggcgaagggctggtggggtcgccaggtggtagtcgcgccggatggcggcgccgaggtcgcacaactgggcagcccgcgccgcctggataccatctaccagaccaacatgcaggcggcctacatggcagggcgctacgcggccgcctacgaagccagggaaacccacccttactggatgtatgtggcggtgatggatggcgttacccggcccagccatgccgccctgcatgggaaagtgttcaggtgggacgatccgatctggcagcacatcaccccgcccaatggctacaactgccggtgccggatcgttgccttgacggaggccgctgtccgccgtcgcggcctgaccgtcgaatccagtcagggcaagaccggccaggtcaccgtcgaaaccggcgtggaccggcgcacaggggagattcgcgaacagaccctgaccaccctggagacgaccgaccgggccgggcggaagatccaatttcgccccgatgccgggttcgacggcagccccgtacagagtcacctgatggaccaggtgctgtacgacaaggccgagcgcaccctgggagccccagccgcaatcgacgaggtgcggggtgtgctgctggacccggtccgccagcgcgcctgggcggccttcgtagatcgcgccgcgtccccccaggggcagaccatgtccatcggcgtgctcgatccgaccgatatcacctacgccctagcccagggcgcccagttgcgggccggcgtggtcgccaccagcgataccgcaattcgcaacagtgctgtcgctcgcgagcagctcgccagcctgccgcagcgcttcgcccagcctgacctggtgctgtgggagcgcggcagcgagtcgttggtcttcatcgtccaggccgatagcgcggccctggctatccgtctgcgcggcgagatatacgggcccggccaactggaaaatgtcggccaggttatggaaatcaccatggatagcatccaggatggcctggcgacgggccgctacaggagagtgcgctagtgacaactaggatcgacgtcgagctggacgaccaggaggttcgccagcgcctggcgctgctgatgcgctcggtgaccgatacgctgccggtcatgcgtggcatcgctgccgagctgctcgcggaaactgagttcgcctttatggacgaggggccgggctggccgcagctcagccccgtgactgtcgccgctcgcgaggctaaggggcgtggtccacacccgatcctccaggtcacaaacgccctggctcgctcggtcacgacctgggcggatcgcaacgaggcgggaatcgggtccaacttggtctatgcggccatccaccaatttggtggcgacgccggccggggtcaccaggtcgaaattcctgcacggcggtatctgcctttcgacgaaaacggccaactggcggccggcgctcggcagtcaattctggagatcgtcctaacagccttgagccgaaatcggtagtggccactttcggacaagcggcacattgtgcctattgcgaattaggcacaatgtgcctaatctaacgtcatgccagccacaacggcgaggcgccaagaaggatagaagccatgaaaatcaccaacgacaccaccacctacgaagtggccgaactgatgggttcggaggctgacgaactcgatggacgtatcatgatggggctgctcagccgcgaatgcgtggtagacactgacgacctgagcgaggatcaatggctggctctgatcgacgagtcgcagaaggttcgccgcgagcagttcgaaagcgatgaagcctgacgcctctaaccacaacccagacccgcgctacctgcgcgggctgctcaagaaagccggcatcagccagcggcgcgcagccgagctgctcggcctcagtgacagggtgatgcgctattacctgagcgaggacatcaaggagggctaccgccccgcgccgtataccgtccagttcgccctggagtgcctggcgaacgacccgccatctgcgtgatcacctgatccgcccgcaaacgcgctacacgcgccgaaacggggttagacgctacctcgctcagagtcggtgcgttaaccccgttagagccccgttagaaatcgctccagcgccattcttgtgccagggtttggccagaagatggcgccggacggtttccgcagtcgttgaaccccttcatgtgaccgctgctttctaccgtcgccaccattggcggcatggaaaagaaccgcctactcgttgccatcgccgcctgctcgttccagcttccccagctggaggatggcagcgcctggattcaagtcactccagctggtgagttccggcccacggacgggcgccccatggacgtgccggcctggcggatcgatgccgccagcgccgccgccgtgatcgaccgggccagggcacgcaagacaccgcctgtcctggactatgagcaccagaccctcaagaaagaggaaaacggccagccggcgcctgctgccggccgcttcctcgatttcgaatggcgcgaaggctccggcctgtggggccgtgtcgaatacaccgcccgcgccgcacggatgatcgaggacggtgagtacctctacttctcgccggtcttcagctacgccccggacggcacggtcctgtcgattctgatgggcgccatcaccaacgaccccgccatcgatggcatggagccgctcgcccgccgagcggcggccacctttggcctttaccccacccaagaggaaacctccgtggatgaactcctgaaagccatcatcgaggcgctgtcgctcaaggaaggggcgaccgaggccgaagccatcgccgccctgaccgcgctcaagccggccttggacgcacaggcggccagcctggccacgctgcgcgaaaccctcggcttggccaaggacgctagcgtcgagcagatcgccgccgccaccagccaactgaagaaggccgacccgagccagaaacccgacccggccaagttcgtgcccttggaagctgtgacggacctccaggagcaaatcgccgctctgaccgcacgcctcaatggtggcgagctggacaggctggtcggtgctgcgctccaggacggtcgcctgctgccctccctggagcagtgggcacgcgacctgggcggtaaggacatcggccagctcaaggcgtacctggacaaggccgcgccgattgccgcgctgacccgcctgcaaggccgccagccggagggcgacacccacaacctcaccgacgccgagatggaggccgcccgtctgaccgggatcagccccgccgactacgccaaggcaaaaggagcctgacccatggccatcattactccggcgctgattagcgcactgaaaacctcgttccagaagcatttccaggacgccctggcgacggcacccagcacctacctccaggttgccacggtgattccgtccaccaccgccagcaacacctatggctggctggggcagttccccaagctgcgcgagtggatcggtcagcgtgtcatcaaggacatggcggcccagggctaccagatcaccaacaagctcttcgaatcgaccgtgggcgtaaaacgtaccgacatcgaggacgacaacctcggcgtctacggaccgctcatgcaggaaatggggcgcgctgccggcgcgcatcccgacgagctggtcttcgccctgctcaaggccggcaacgccaatctctgctacgacggtcaaaacttcttcgacaccgatcacccggtctatccgaacgtggatggcaccggcacggcgaccaccgttagcaacctgttcgcgccggccgctgatccgggggcggcctggtatctgctcgacaccagccgcagcctcaagccgttgatctaccaggagcgcatgaagccgtcgttcacttcgatgaccaaggaagacgacgagcaggtcttcatggccgacgagtaccgctacggcgtgcgctcccgctgcaatgtcggcttcggtttctggcaactggcagcgatgtccaccgaagagctgaacacggcgaacttcgagaaagtttacgacgccatgcgcaaccagaaggccgacggcggccgtccgctggacattcgcccgaacctgctggtggtgccgaccactctgcgctccaaggccaaggaagtggtcggggtgcaacgtctggccaatggcgcggacaaccccaacttcgaactggtccaggtactcgataccgcctggctcaactgatagccccagacggaacgcctgccaggccaaggatggccaccttcttccagctacaggagacacgacatggcacgccagaactctgcggccaagaccaccgccaaatccaagaccgatccggcgaccgaaaagcccaaggacgaagctctgccgggctccacggatgccacttcgtccaccgcacccgaggcgcccaccgccaaaccagccagcacctcggacgagatcgagggcgtcttcattcgggccaccgttgagcgccgctgtcgagcgggcttctgcttcgacaaggaaggccaaggcttcgctgaaggcgtgctgagcgacaagcagttggaggctctggagtcggacccgctgctcaaggtcgagcgctgcaccttttccggcaaccaggagggcgagtgatgaatcacgccattgcccagttggacatcgccgcgcagatcgccgagcacaacgctccaatcagcgaggctcagggtgacgccgctcaggccgagttgcagaaccaggttgccgccgactgccgcgaggcgctcgacgtcctggaacaattggagtcgccgctgtgagctactgcacgctggccgacctgatcgagcagtacagcgagcaaaaaatccgcgaggtgagtgaccgcgtcaataaaccggccacaaccatcgacacggtgatcgtggatcgcgccatcgccgacgccgactcagaaatcgacctgcatctgcacggccgataccagttgccgctcgccagcgtgccaacggcgctcaagcgcattgcctgtggcctggcctacgccaatctgcacatcgttctaaaggaagagaacccggtctacaaaacggccgagcatctgcgaaagctgctgtcgggcatcgccaacggcaagttgagtctggccctggatgctgacggcaagccggcgcccgtagccaacacggtgcagataagcgaaggccgcaacgactggggggccgactggtgagcgacccgttcgactacctgttcctggaaccgttgctgatcgagcgtatccgctcagaggttcctgggctggccatcgtttccggggtgcccgatctggcggccttgagtgagcaggaccagcccgcccccagcgtctatgtcgtctatctcggcgacgagataggcaccggagcggatcaccaggggggcaggcgcgccattcaggctatcggccagcaatgggcggttgtgctggtggtgcattacgccgactcgtcgaactccggcgaaggagcgcgccgagaggcaggaccgctgctgggacggctggtcaaggcactgaccggatgggctccagccatcgatgtggctccgttggcgcgcagcgcccgacagtctcccgtcacctacgccagcggctacttctatttccccctggtgttcaccgccaggttcgtctacccgagggtcaagtcatggaaaccgtaaaagtcacgatcactgctgagaaccccaaccacacccacgcgggcaagccggtggccaagggcgacgagatcgaagtcagccgcgccgatgccgagtttctgctgcgccgtcaattgatcaccaagattcccgccgagcccaaggccgacgagaaacgcgacaagtaacgcgcaacatctgattcctacggaggcctcacatggcacaggaaacgtatttctacgggcaaggtgagattgacgccgcgcctatcgtcaacggcgtcctcggcaaatggcgctggattcaggatgtctcggccatgagcatccagctcgcagtcgagaaggtcgagcacaaggaaagctacagcggccagaaagccctggtccgaagcttccccatcggcaagaccgccaccgtcagcatgaccttgcacagcatcgacccggataacctggcgctcaccctctatggcaaggtcgtgactaaggcggccggctctgtgacggctgaggcgctccccgccgacctggtagctggtgatgtaatccgcctggccaatccgggcgtcagcgagctggtcatcaccgacagcgcgagcagtccggcgcccctcgatccgcagtattacgccctgcgagccgatggcgcctacggcgaggtccaactgctgggtctgccgacgccggccccgacccagccgttcaaggcggcctatgagtacgcggcgactcgccaggtgggcatgttcaccgcgccgcagccgaccatcgccctgcgctacaagggcatcaacctggccgaaggcggcgcgccggtcatcgtcgagctgttcaaggtcgcgaccgacccgctccaggaactggcattgatcagcgacggcaacaccgtcgccggtatgcagatcagcggcggaatcctgctggacaccagcaagccggataccggcgacctgggccgcttcggtcgcattatccagctggggtaaatcatggccaggaagaagcctgttaaccctcgcggccagccggccgactcggcgcccgacgacagcctgagcgtgctgtttcctgaccgtcagttggcggtcgggggcgtcgaggtgacggtgcgcgagctgaccttcagcgagcaactgcgccataaccacctgttggccccgctggccgatgccctggcggcagttcccccggagcagctcgacggacctgagtcgatcaacgtcatcttcgacgctctggcccggcacgccgacgcgctgcgcgagttgctcgcgatcagttgcggccaatccgtggactgggtggacgcgctgccggcagacgacggcgaagcactggtgttgacctggtggacggtgaacagtggttttttcgtgcgaaggctctggcggcctcgcctactggcgatggcattgggcaaccgacgccctggagccgagtcttctccgatctcgtccgcgccggccactgccgcgaaaccctaggcacctataccggccggcaactgattctgtactggaacgaagcgcaggcagctgaacggcgagaacaggcgcgccacgttcggtcggtgatgttcggaatggctggtggcaaggacgccagcgccttcctcaacgatttggaatcctgatggccactaatcagcaactctcgatagcactacgcatccaggctgacctggctgaagcgcagaacgcgctcagacaactaacgggcaacctccagcaggttgaccggggggcggtgcagaccaggagcgagctgtctgcgatgggtgggcagttggacagccttcgcgcacaggtgcttgggtttgtcggagcttgggctagcttgagtgcgctgggcggcctggtgaccatggttgaccaatatgggcaaatggccgaccgcatccagatggtcaccagcagcacggccgaatatgaacaagtgcaggcccggctgctggagacggccagccgcacctatcggccgctggcggaagcccaagagttgtacatccgcaccgccgacagcctgaagtcgttgcggtacaccaccgaacaagcgctggacatcaccgattcgttttccttcttgctggtaaccaacgccgcgtcggcggaccgtgcggcgagcgccatcgacgcctactcgaaatcgatccagaccggcaaggtcagctctgacgcctggcagtcgatcatggccgccatgcccagcctggtgaacgccctggcagagtccaccggcaagagcaccgaggaaatccgcaagctaggcatcgagggcagcctgtcgttgcgcgacctgaatgaagggctgcgcaagaccgtggcggcgaaccgcgaggcggcggacaacatgggcacctcggtccaggacgcgctggtcagcctgaacaacgccctgagcgcctacctgggcgagctgaaccgcacctatgacatcaccggtagcgtgtcctcggcgctgaacgtgctggccgagaacatggaggttatcgtcaaactgtttggggtcgcggcggtggcggggctgacccgctacgtggccagcctaacgctggccacccaggcgaaactggcggcagtgctggccgctcgggcgcaagccgctgaagaactgcgggcagcccaggctcaggtcgcttcgacggcagcggcagcggccaatgccagggcacaggcgggcctgacggtgagccatgctcaggcggcggcggccgaggcggcgcataccgccgcgacccagcgccttgctgctgcgcagttggcggccggcaccgcgatgcgcgggatgctggccgtgatcggtggtccggccggcatcgcgatgctggtggccggagcggcggcaagcttcttcctgtttcgcgatagcgcccaggcggtcaagagtagcctagatgacctgagtgagccgctggaccaggtcgtcgagcgcatgggcaagctgagcgagattgagcaagatcgcgaactgacccggctttccgagcagatcgacggattgcggcagacggctgtggaagccgcccgcgaaatgcgagaggtggccagcaccgccctctatggtgccaggctggatcgtatcccgtctgccgaagcacagcaggccctccagcctctaatcgatgcgtcggctgacgctgcgcgaggcgtggaggtggactggaagtcggtgatggactccctggctgccagcggcgctgttcccgattcactcaagcgcaagctgctggacatggcggctggtcaggcagaggcaggccgtactgctaccgagctggggcagcgtcatgcggaactcaaggcacgcctggagggttcgactgccgccatcaatgagaacagcgatgcactgagtaaagggtcggacaaggcagccgagtatatccagtccctgcgcctggccatcgccgacctggaagatccatcggtcctgggcaaggccggccgtcgcctccagcagttcggggccgacctcaatgccgagcagagtgccgaaatactccgcctggagaccctgaaggccaataccgaaaaggcggcccaggcccgcgaggatgcacggcgcaaggctgaatccagtgcgcgacaacaagcctccacggctgagcagttggcgaagagccaggaaggctatgttgcggggctggaaaagcaagcccgcaccctgggtctcaccagcgcagaggtgcgggcctacgagctggccgagaagggtttgaccggagccctccaagctcgggcagcggcagcacttgccgccctcgcggcggacgagaagaagcggcaagccgacgccactgcgcgcaccaacgccggactggaggccgaatatctgcgggcgaccggccgcaccgttgacgcggggctgctggagattcggacgaaatttgacgcgatgcgtcgtgacttcgaaaaggcgggcaacgacgccggcctggcctggatcgacaagctaatccccgtcgccgaggccaaggtccgcctggatgacgtcaagcagcagatggacgatttgctggccgaccagcaacgggccgagtcgtccgttaacgtccagcaggatgccggcatcatcaacgaaatggacgcccggcagcgcatcctggacattcaccgagcgacctacgagaagctccagcagattcggccgatcctagagcagatggcccgccagcctggcgaggtcggccgagccgctgccgaatcgctcgcccaactggacgccgaggcggcgcgactccagcagaccacgacgctgctcgaaaccaccctacgggacggcctcaccagcggctttaccgacgccatcaaagggctcgcttccgggaccatggacttgcgcgacgccatcacgtcgctgggtgaagctgtactcaatgccttggtgaacatggcggcgcagaacctcgcgcagtcgttgtccagcggcatcatggggctgtttggtggcggccagcaggacaccagcatgactaccggcgcggcggctgtgaccgcgtcggccggtgccctatcgactgcgggcgcctcgctgctgaccggggccgctgctatccagacggccgctgcgtcgctggcagccgccaatggcgtccaagggctgggcgctgctgcgggtggtgcgggtgcggcaggagcggcagcgggcggcggcagttggtggtcctccatcgccggcgtgttcggtttcgccaccggcggccacatcaagggaccaggaacaggcacaagcgacagtatcccgattctggcatccaacgacgagtttatgacccgcgccgcagttgtacgacagcctggcgccctggcatttctcgaacagttcaaccgctacggcatggccgcgctggccggctgggcgaaccctgtccgtcacgcaaccggcggacagatcggcattcccgctcccaatctgccggctcccgtccgtggcggcgcgaacctgcccgagccctccaaaaacttcagtacctcggtcgctaactcgatctacctgcacgccgttcaggaccccgaccagatggcggccgaaatgtgggccggcaagggcggcgaccattacatcgtctggctgaacaagaaccgccaggccgtcaagcaaatactcggaaactaggaattcatggctactgaaatcggcaccgccacgaaccaccagaacctggtcgagcgcctcgtccagttcctcaccgcgaacccagacctggtcgcggctgggcaggcctacgagaaggttttcgacaacaccatccccgcgtccggcacggccatcgccgtgcgccaggtgaccctgcgcgccccgggcctgggcggcaccgacagcatctacatggggattcagagctacggcgataccgccctggactactacaaccttcgcctgatgggcggcacggcgttcaatcctggagcaatcccgcctggcggcgactactggaccgcgtttgccaactacagtccgcgggttcaggcgctgctgtggaaccagcccatgccgtactggttcttcgccaacggccgacgcttctgggtcgtcgtgaaagtctcgacgatctacgagtcggccggcgccggcttcatcctgccaccctgtccgccgtcgcagtatccgtacccgcttgccgtcgtgggctcctaccgtggtgacgttgcaactcgctggtcagacgtcagcgaccggcacagaggcatcagcagcccctacgagcgtagctgctatctccgcgatcccgccgggcgctggctcggtttcactgtcgcaggccgttcaagcaacgagtccgactacaacaatcggaccctgctgccgcttggctgcggtcgctatgcgggtggtagcgacactgtgatcaaccagctccgcgactctttcagcaagttcccgctgaaagctttgcagttcgtcacccgcgaaaccgaggggcgccgctatctgggcgatttcgacggcgccttctacgtgccgacgctcaactccggcgccgaagacgtgattgtcgaggacggtgtggaccacgtcgtttttcaaaccgcttggcgtagcggtaacccttggctctacgcgatcaggaaggactgaaatggcttacttcacaggaacagcgaacaacccggccgacttgctcgccaagctgcgcgtccacgccgagtcgctcggctgggtcaccgaccgcgcctcggcatcggaatggctttgtcacaacgccgacggctactggtcgttcaacgccggttccaatcaatggcagctcgcgggcaatacggggttcgacgacgggcttgcgtggaatgcgcagcccggcaactcggtgcagaacaacccgtattcgtcgaaagaagcaaccatagcgcagctcagcgccgggccattcacgcgctatcacctgttcgccaccgctgcctatctgcacctgcacgtcgaaatcgctgccggtcagtttcgtccagtgatgatcggctccctcaacaagcgtggcgtcggctatacgggcggccagtatgtttgcggctcgttcctctacagctctggccaggcgctcacaaacaactggtcatcgcatccattcgatggttaccacattcgatacagcggcggcggcagcatgctgcggctagacagcctcgacggtggcccatcgccggagtggttgccgttcgactacacaacgaacgtctcccggcgcgtcgtcggccccggtcgcggaaactacagcagtcagtaccatcccgacgtggggctgatcgacgcgagcgcaaacgagctgaacagctcgaccacccctgtgccctgcgccatctatgcgttcggcgctcagcagcgctcgcggtacgtgggcgaggtgccggactttggcatatgcaacatggcgttcctcgcgcctggcgatccgctggtgatcggcagcgacacttggcgcgtctatccgttgctccaacgcggaagcgctaccgatttcggcaacaccagcgcctgggtcggctactgcttccgggtgcttgagtaatggcgacgtttccggggttccaggtgccaaagccgctcgtggggatcgttgccggcatcacgccgaatatcgacgccctggagctgaaccaggacatcagcctggcagcggtcgcggcctcgacctgggccggcgcctacgcggcgcatcagccggtagaggtgatccattcgacgtaccaggctgtccaccaaagcgctctggaagagaactactacaaccgcctgtggctgatccctacgaccatggagctgggcaacgtcgtcagcacccaggtacgaccggcatcagtctggaacgcttatttcagtccgcgcacgctgaccgccatcgagcgggaagatgcagacggcatcacgctatccggccaggcgtcgccgccgctgggttttgccgccctggaggaacgcacttggaccgtcagcattggcacggacggcccgcccgtcgtcaatgcgcggatcgtctggacgctccagggcgagccggacctggtcctggtcatcaccggcaatcgcatcatcgcctggaccttcgcgccggactggggcgacagcatcgtcgagcgcctgagcgcctcgacaaatatcctgcaaagcgaatcagccgtgacccagcgccgggctatgcgcctggcgccgcgccgggagttcgaagcgaacatgtacgcggtagaccgcgagcggcagctcctggacatgacgctgtttggctggggcgcgcgaatttgggcgctgccgatttggcctgatatccaactgctccaagaaccgctggcggccggctcgctgaacattccgtgcgacacggtcggcctcgacttccgcgacggcggtctggcgatgctgcgcggcgaggacgccttcacctatgaagtcgtcgaggtcaaggcagtgaccgccgccggcctggacctggtccgccccgtccaggccacctgggtaactggctcgcgactgtacccggtgcgcaccgcgcagctgaccgaacagcccacgctgacccggctgaccgataccgcgcagtctgcgcgggtgtcgttcctgataatggagcccagcgcctggcccgaggtaatgccggcgacgacctacagggggcggccagtgctggagcagcgcccggacgaaagcgaagacctcacctccagctatcagcgcctgctgtccaccctggacaacggcagcgcgattccccgcgtgaccgacgtcgccgggatggcgctgcccgtcatcggtcatcgctggatcggcatgggccgagccgagcggtcggcgttccgcagcctggtctatgcgctgcgaggccagcagaagccgctatgggtgccgacccacgccgacgacctgaccctagtcgccaccgtctcgcagctgtccactgcgctggacgtgcgcaatatcggctatgcccgtttcgccaatgggcgaccgggtcgtcgcgatatccgcatcgagctgtacgacggcaccgtctatcaccgccgcattctcaccagcaccgagctggacgccgacaccgagcgcttggccatcgacgccgccctgggccgcctggtcgagccgaccgatgtagcgcgcatctgtttcatggcgctctgtagcgccgccagcgacgtggtcgagattgagcacgtcaccgatagcgagggcgtcgcaaccgccgcgctgacattcaaaggggttcgtgacgatgagttttaacagccgcgaaagctcgctcgcggatgggcagccggtgcggctgtaccagttcagccgtggcgcgatccgctggagctacaacagcagcgaccgggacatcacctaccagaaccagattttccgcaccgtgccgggcggcatcaccgacaacgggatcatctgttccggcgacccgcagtccgatcagttcatcatcaccgcgccggccgacctcgatgtcgcgctgctgtacaaggccaaatcgccgagtgatgccatcgatctggtcgtctacgacatgcactacggcgatgtcgaggcagcggtttcctgggtgggggagattggcgacgtggactggccgaccgtggacagcagtcgcataacgtgcgtgtccgaagacgagctgatggaccagccaggcttgatcgataccagttgccgcacctgcacggcgaccttgggcgaccaccgctgcaaggtaaacctcattccgtatcgagtgacgctgacaccgcagagcgtgtccgcgtgggtgatttccagcggagtggtcgccggctatgccgacggctggtttaccggtggctatgtggagtggcaggtggacggcgacaactacgaccgccgctacatcgagcggcacgccggggccgatctgcacatcctgggcggcaccgagggcgtcccggcgggggggcaactgcgggtctatccaggctgcgatctgctcgatgaaacctgcgccggaaagttcgacaacatcctgaatttccggggctttaacaagatgcaaggcaagtcgccattcgatggcgaccaggtctggtgaggtaggccatggacccgatcacaatcaatctcgtcattctggctgcgtcgttcatcctatccagagccttggcgccgaagccgcaaaagcccaagccaacagcgtttgaagacatcgatttcccgcgctgcgacgagggcgacgaactggccgccgtgttcggtcagtgctggaggaagtcctggatggtgctgaccgtaggcaactaccgaacgaaggcgatcaagacaaaggggagcaagaaatgatcgttacggctcagcacttacatacggtcccgacctggaccactcggcagggctactgccatcgccaggcgcgggagttcttcaagcgccatcacctcgactggatggcgttcttacgggacggcatcgaggccgatcagttgattgcgaccggcgacgcgctcgcgctcaagctggttgagcacgcacgccaggaggtggctgatgggcgctaaacccaaggctcaaacggtcggctttcgatacttcttcgacatccatttcaccctaggcaagaaaatcgacgagctgtgcgcgctccgggcaagcggaaaaaccgcgtggaaaggatcgatcactactaacggtcaggtacgcatcaacgccccgaaactgttcggcggcgacaagggcgaaggtgggctcgatggaacgttggatatcctgttcggcgaagaagaccagggtgtcctgccgcgcctggcggccatgctcggcggcctggtgccggcgttccgtggcgtaaccacagggttctattccggcttggtaacctccatgaacccctacccgaagacatgggaatttttggtccggggaggaaaccgcttgtgggacggcaatccctggtatcccgaaaagcagttcatctggctagcggacggtcagatcaaggcgatgaacccggcgcacatcctttatctcgtctacaccggccgggacttccggggactggcccgcacgcgaatggacgaggcgagctggcgggccgctgctgacaagctgtatgccgagggtttcgggctgtgctttgaatggaccaggtccgacacgttcgccaacttctgcgagacggtgaaatcgcatatcggcgctgaggtttacccgaaccgtcagacgggacagatcagcatccggctcctgcgggacgactataacgtcgcagacctgccgctgttcgacgaggacagcggcctcctggaaatcactcaggagaagaccggctcgacctccctggcgccgagccagcttatcgtgaaatacatcgaccagatcgacggggcgcagcgccaaatcatcgtcaacaacaacgcggtcgctgcgtcgcaggggcggcgctcgtctgaggaaatcgagttcctgggcgtgcctaccggggagctggccgggcgagtcggtgagcgggaaatgcgtctgaagacaaccggcctgaagcgctataagggcgtgttcgaccgccgcgcccgtagcctgaaccctggccagccgttccgcatccgttcgacccggcgcggcatccctgaaaccgtcgttcgggtcggccggatcgaggacaacttcctcggcgacggcaagatcaccctgaccgtcgtccaggatcagttcaatctgccggcgacaaccggcgtggcgccgccaccaccgggctggattccgcccgaccggacgcctcgggcgatcactgtgcgccgcctgatcgaggcaccctatcgcgaactggccggcgtgatcgatccggcaaatctccagctcctggacgtgagcgcgtcctacttggccgcgctggccgaggcgccgaccagcctgtcgcagagctacacactgaccgaccgcgtcggcagctctggcgcgttcgttgatcgcggaaccggcgactggtgcccgaccggactactcgccgccgagctgccgctggcggccggtccgaacgtcgtcacgttgacgaacgccagccggctggaggacgtcactgtcggccaggccgcagtcgtggacgacgagatagtccgggtcgatgcggtcaactacgccagcggcacggtcaccctcgcgcgcggctgcgccgataccgtaccggccaagcatctggccggggctcgggtctggttctacgacacgttcgaagctgtggacgaaacggtctacagccagggcgtgacgctccaggcccggctgctgacgaacaccagcgagggccaactggccccggcgctggccgccaccgacagcctcaccctgaccgggcgccaaggtaagccgtatccgcccggccagttccgcatcaacggcagcgcgtacccaacgaaagtctacggggcgctgtcggtgagctgggcgaagcgcgaccggatcggccaggccgaccagttgatcgataccacggtcggcaacatcggacccgaagatggggcgacggttacgctcctggtctacagcggtacgacgctgaagcgtacctatgccggtctcacatccagtaactggtcctatccgctggccgaagacatggcggatggcccgctccaggacgtgcgccttgtcctgcgcagtgtccgcgacggcatcgattcttggcagcagcacgacatcacgattgaacgccacggcctcggtttccggcttggcgaagaactaggaggcgtatccgcatgagcctgacaatggggccgaacactggcttactgatcaacggcgcccccggtgaggggcattacagcgaactgatccgcatgttgcgctgggatgacttcctgcgccaaccggtcgtaaaggggcgggtcgcaacgctgccgacttccggccaggccgagggcgacacttacattttcaccggggccggggcgaaccagaaccgcttggcccgctggtgggcgactggtgcgtcaacgccaatctgggagtacatgccgccacggctgggctggcgtgtccaggtcgcaaacgagacaaccccggcaggccaggtcaagacctacgagtattccggcagcgcctggactgagctggtgggcggaatggccgacgcgccgagcgacgggaagcgctatgcccgactaaacaacgcgtgggcaggcttggggactgctgccgtcgccgatattcttgggccggtctctcaggctggcggtgtgccaactggtgcgatctacgagggcggcagtaacgcgaacggaagttacgtcaggctcgcagacggaacgcaaatttgctccagcagccttttaacgtttactgcgggttcaacgtcggtgggtgcgtcttggacgtttccggccagctttgtgtcgccgtcgctgatgtttggcaccgttgtagcatcgggagccggcgcagactatgaccccggcgtcgctgcgaggaacctgggagctgtttacttcaatgcgtcaacaaactctgctgcactggggtttctttgcatctcgtctgcatcgttcaccgctggcgcccaaactcgaaataaccgtgctgtcgcaattgggaggtggttctgatgatcatcacgttgtcgccgtatgtcgcgctgcccggcagcgatgaacatctgatgctgagcaggactggcgatgtactcaccgtgaacggccagtcgttcgatttcacaccgctcccggagggcggcgagttgccggccgaggctatcgggtcggagtggttcgctggccccgtcgttcgccgtgaggggcgtctagagttcagcctgcggctgccgctggctgacggcgctagtgcagccgctcgctttcctgaaccaatgctgatcgaggccgacggccctgtggagttgccgcaatgactattgactggagcatgttgaagtcacccgaagaccagcaggttgagcagcgggaggccatcagagcgcagcgccgccaggcctatcgcaccgagtccgacccgctgcgcctggaggccgagtttgacgccatcaccgctggcaccaagccggacctggcggcatgggttgcagctgtccaggcgatcaaagcgcggtatccactacctgaataggtagttgtgatggcgttctcgtttttgccacgttccgacagtctgatgtcgagtagtagataggaaccttgggatggacgaggtactgaggcaaaggttgcgggctgaactactggaagtggggtttctcaaccagtgctgccttgatctcatggaaagcatggaggctgagttcagtctcactaaggaccagcgcgagtgcattgagcagctcagccaattcctacgggagggcatcggcaaactgaccgctctgtctgaacgggtagccgacggcgatatcgtcgtcctgtgctgatcttttgaaattcttttgccgctggcgaaacggttagggcgcgtcatttattgcgcaaatcggcgccaaatttcgcgccgcgctaca

SEQ ID NO: 11 - DNA, 49033 bp, synthetic construct
  source 1..49033: mol_type = other DNA
tgcgcaagccagttgcagctggcttgcgcgtatagcaatacgtggagacctgagtatgagttacagagagagcattcgcaagtccgtgcgctttgaggtgttcaagcgcgacaacttcacttgccagtactgcggcgccaaggcgcctgacgtggtcctgcatgtcgatcacatcaacccggtgagcaagggcggcgacaacgagatcatcaacctggtgaccgcctgcctgccctgcaatctcggcaagtcggatcgcctgctgtcggacacctcaatgctggatcgtcagcgggcccagttggaagacctgaacgagcgccgcgagcagctggaaatgatgctggcctggcgcgatgagctccagtctttcggtgaagagaccgtacagctgattgccgatcgcatcaccgcgcgcatggtcggccactcggtcaacgagcacggcaagacggtaatccgcaaatggatcaagaagttctccgtcgaggagatcctggacgccctggacatcgccgccgacaagctcagcactgcgcccgatcaggaggaagtgctggagtgcttcgatgccattcctcgcatttgcgtcacccggcgccttcccgaagcaaagcagaaaatgctctacgccagaggaatcctgcgccgccggatttatgtcaacgaagctcacgtcatgccgctgatggccaaggccatcgaggcgggtctcgaggtggaagagctgatcgaatttgcgaaacaagtgaagaactggaccgaattccgggcagagatggaggaaatcgcaaatggctagggcccgcaacatcaaacccggaatcatggcaaacgaagacctagcagagctagatcctctcgctcgcctgctgttcatctacctctggatgttggccgatcgggaagggcgccttgaggatcgcccgaaacggatcaaggccgaggcacttccctacgacaacgtagacgctgacttgatgctggatgatctggccaaggcagggttcatccatcgctatgaggctgccggggtcaagctgattcaggttcttaactttgccaagcatcagacacctcatgtccgtgagcaggccagttctctcccgggcgttgacgcagaacacccaaagagagaacaaggcacaaccaaggaagtgcctggtcacaaccaaggctgtgctgagcaatcgccaagatcgcctgattctctgattccggattctctgattccagaggaagagcatgtcgacgctgacgcctcgacccattccgctccgcagcaagcagcagagcaagagcctggctccggccagaccgcacagctgttccagattgatcgcatcccttacgagaagatccgcgacctgtacaaccagatcctcggtggaaagctcaagcgctgcatgggagtgacggaggctcaccggaagcacatccgcgccgcgtacaacctcaagctcgatggcgggttcccggtccgtgacggtggactgtcgttttgggaagggctgttcaacgacgttctggattgccccttcatgctgggcaacaacaaccgggggtggcgcgcagacttcgagttcctgacaaccgccagcaagatccagcgcttcatggagggcaagtacgatgccgcatgagcgtcctctggtagcgatggaagctgagcagggtgtgcttggcgcgctgatgaagaaaccggaactgtgcgaggttgttggggctttcctttccccgaccgacttcagccatgccgacaactcggtgatctacagcctgatccttgcctgtcattcgaaggccatcgtgcctgacccgctttctctggcggaggctaggtcggagcttccaagtggcgcctttacgcttgcatacgccaacgatctatggcgcgaggttgcaagcacagctagcgccgaaaacttcgccaggattgtcgtcgagcgtgcaaaggctcgggagctgtacgaagcgggcgaacggatcatgaacatcgcccttcagagagggaaaatcccggaccaggtggctgaagcgcagagcatcgttctcgatctcaacgcccaggacgagactcctgatgtggtgacactgcgcgaggcaatgctcccagtcttcgacgaaatggaagttcgctggaagggaactcagtcggtcggactgaagttcaacctgccagacctcgatgccgttatccagggattgcgtcccggcaacctggcaatcatcgctggtcggcctggcacgggtaagacggttctcggggtggggattgctgacgaaattgccgttcgcaaccggggcgccgcgttgatcttctcgctggagatgtctcaagccgaacttgcaaagcgctcgctcgcatcgctttctggtgtttcgcaagcggcgatcgactcaggcaaagcgctggagtgccaggactctattgcgcgcatgactgccgcagtggaccaagtctccaggggtgatgtgcgaatttgcgacaagggaggactgactttcagtcggatctgctccatcgcccgattccagcatcgagcaaagccgctgagcctgatcgtcatcgactatctcgggcttatcacctcagatccgagtcaccgtcatcagaaccgaaaccaagaacttggcgccataagccgagggctcaaggctctcgccaaagagcttggcattccaattgtcgcgcttgctcagctcaatcggagcatcgaaacccgggccgacgccaagccaaaaatgagcgacctgcgcgattccggcgagatcgaacaagacgccgacgtgatcatcatggctcaccgggatatgagcactgagcgtggacagaacggtatcaccgagcttgatgtcgtgaagtgtcgacacgcaaagccgggcttctgcctgttgcagttccagggtgagttcgcgcgcttcgtcagttgcgcccaggaccgggaagagcagcaggagcagacggttcgtccgcagcgtccttccgcgcgatcaatggtagctgacttcaagccgcgaggtgcccaatgaaacgctccttgaccgtaatcgtaggcgccaagcgcttcacgatgattctgatggaggactgcgacccgctcgcggtcgtgaagagcatttggccgcaggggagggttgaggcatgaagaccttcgaactgatccgcatggaaggcctgcgcacctacggtcgccagattgaggccaatacctggcgcgaagccgagatgcaatgccgcgacggcgagatcgtaaacggcgaactgatcggtgtgtacgactgtgacccggtaactgaggccgtctgcactgcgcgcaatgacgtgatgattgatagcttgggggtgtgctgtggctgaccgcactttccgcatccaaggcgctgccggcatccgtccggctttcgtcgcggcctggaacctcatccaggggctgatgaaagaagcacagggtggctacgagctggttctacgccctctcaagtcgaagcgctccattgagcagaacaagcggtactggtcccttctgcgcgagctggccgccgtcgcctgggtcgacaaccgccagttcgacgatcaggtctggcacgaacagttcaagcgctggttcatcggctgcgaggacgtgaagttgccggacggctcgaccgagttgcgcggcatcagcaccacgaagctgaccgtagacgagtttggaatctacatgaccaagatcgaagcgtgggccgccgagcaagggtggccgctgatgatgcaggaggtcgcatgagcaagttcaaggcgggcgatctcgctcttaatctgcaagacatccccagctgcatcagtgcgggagtggtagtcgagttgatgtctcgacttgcccctggtgatctgtttgccgaagacggccagacctttcaggtgattcggccagcttggtgggtgctccatgaaggagaccggctctacatacctgaacggtatctcatgcccctgcgcggcgacttccagcccgagcagcagaaggcgaagggggtggaggcatgagcaggcggcaggttgcaaaaattctggtgggccagcttctggtcatcgcactcatcatctacacgcagacctctgcggccatcagcccatggattgtctcaatggttgggacggccaccctatggcttggctacttcgcgggagaagagctatgagccgcagcttgttcttctgcgccatgcggagagttcctgttcggccaagagcgctcattgtcctgatgatcatgatcgcctttggctgggtgccgcttgtggtggccgtatgcgaggcagtcggcgaaggggttcgggcctgccggcaggaatcgtccaggctctacggcgacttcagcaaagctttcaccgactgctggaaagccttggtttcgggggagcctcaatgagcctatccgccagccagcccaaaccgaagaaatgccagaaccctgcatgcggccaggagttcacccctcgcttcagcagcacgcaaaaggtctgctcgccggcctgcgccctgtccatcaaggacaagcacgccaagccggcgcggaaggctatcgccgaccgagagcggcgggagatcaaggttcggaaggagaggctgaagagtaaggcggatcacctgcgcgaggctcagcaggcattcaacgaattcattcgcctgcgcgacgccgaccagccgtgcatcagttgtggccgccaccacgatgggcagtaccacgccgggcactaccgcacggttgccgccagcccagagcttcgcttcgagccgctcaacgtccacaagcagtgcgccccatgcaacaaccataagtcaggcgacatcgtgaactaccggatcaacctggtgcgcaagatcggcgccgagaacgtggagtggctggaaggccctcatgagcccctgaaactgaccatcgaagaaatcaaagcgctgaaggcccagttccgggcctgggtgcgcgaactgaagagggcaacggcatgaccaaagaaactctgaccatcgttctcttcagcatagggagcggtctcatcggttatgcgatcggtattgctgccgcctggctgggaaactggttcgccgacggttatcacccgctgctgctgtcgaacatggtcagcacaccaggtgctgaggatggtgagcgcgccaacgaataccccgattatctggagcctccgagaggctgtttcggcatgtgctgtgctggatgtgatgctcgctcgcaggtcaactccaggagcaaaacagtcagcgaacagacagaccaatcttacgttttaaacgccgtgctcagcgctcaaggggatgaatgatgatctacaccagcattcggtcggcagtcgtctctgccttggcggcggaaaccatcgacaacactgcaaagcaagcctggcagaagctctaccagccagggtatgccgagagtgagggtttagctgggctgatcaggggctcgaacacgtcaggcatcaagcgcatcgatgctgattgctgggtgcacgcccggctgcacagtcagctcaagcctaggcactggaacgcgcttgtggcgaagtacagcacccaccgcgagaagaagaaggccgcaatcgaggcgcttatccccctgatcgccaccccggcgccgcgcagattcctcggaatggcagtctatacctgggctatccccaagctgaagggggcagaaggcaagcgctctaccgacatgatcattctcgacgccgtgttctaccacatgaacaactgggaatctgaaggccgccccgaacagacgaggcgacgctggaggtcaggaattcacagtgtgctgaacgaaatgctcaaggaggcagagctcgatgcgggtgaaatcctgatggaggagggcatcatcgtcggagaggctgcgtaggacttgcaattagtgagcgtttgagcgaatatttccccatcctgccgatcttgcgcgttatgaggatcggtagctctgaagccctggcaaatgccggggctttttcgtttccggggtatggatgaatctcgagcatcgcataaggcgctggcttcttcaggctgggcgacgtggcaagccgatccacgcaattctcatccaccccaacgacatccaatctgcaagaaagatctgccggtttgtgccagtgaaggtgctcggcattgaagtacgccggtatggcgcaacagggagcgctgctgatttgtaatcagagggttgcgggttcgactcctgctgccggcaccacactacaaggcccaggcaatgacctgggcttttctgcatctggagtaagcaaatggacccgatgacgaccgttggcggaggtctcttcgccaagtacagcgtcgctattgccgggttctgggggtctattctgtcccttggattcctgagcggcctgaaccgctggcaagccgcgctcgctgtagcaaccggattcgggtgctcaacctattggactgctccggttgccgcatggctttcgcgtgagtacgagattccactcgatgacgcatttctgagtggtgtcgcattcaccattggtttgctggcgatgaatatcatccccggcctgaaggcggcagtaacggcaatcacagagcggttccttcctacgagaggaacctgatcatgatcatgtcgattctggcggcgctggatgcgctgctgtgtgtgcttgtcgttgtagctgctctggagttcctgcgcaccgtccagctgtctgggcagccgctattgggtatctccttctacctggtggcaggtggtgcattcggaatcctgtacggaatcatgaagggcgcaccggttaatccattttcggtgatcctccatgctgggctcgtactttacgcctggtcccggcgccggcagatattcggaagcgactggtcgtggaactgaagcgacctaaccctccagagacgatcgggcagttcgcggaaggcgaagattgggcggacgcctttgtccccgctcaggatgttctggcttgggcgaagtcagtgttaatcgatccgaacggaatcctgggcaatgaagaccacgcccacctacaagacgctcctctcgctttcctatgggctgcctccagcttcaccaagcaggggaggacggtactgggtcagtgcgaagaggtgacgttccgctgtggagcctggcagaagggtaggcaggaacagcagatgatccgttggttcggatacctgccgaggtttctgatcaccctggctgctgactactgctcccagtgctccgacgcggagttctgcgcattggtcgagcatgagctctaccacatctgccaagagcacaaccaatatggcgagcccaagttcaccgaggagggctttccaaagctgaagctccgcgggcatgacgtcgaggagttcgtcggcgtggtgaggcggtacggcccaagcaaggacgtgcagtatctcatcgacgctgctagcaggcctccagaggtggccaaaattaacatttcgagagcctgcggtacgtgcctgctgaagtcggcatagccacgacaggcccatgacaggaagaaaaacgatggcaaccctgaacagcgacgtgaaggcgttcatcgttcaggcgctggcctgtttcgatacgccatcccaggttgcggaatcggtcaagaaggaattcggcatcgaggtcagtcggcagcagatcgagtcgcacgacccgaacaaggtgtgcagcaagggccttgccgcgaagtggcggatcctcttcgaggacacccgcaagcgcttccgcgaggagatcgccgacatcccgatcgccaaccgcgcctaccgactgagggcattgggtcggatggctgagcgcgccgagggcatgcgaaacatggccctggctgcccagctttacgagcaggccgccaaggagtcgggtggcatgtacagcaacaagcaccagctcgagcactctggtcctggcggaggtccgatcccgacaatgccgaccaccatccagcttgtggcgccaggccatgaccacggcgaagattgaacttccgccaaagctgataccagtcttctcaggccctgcccggtaccgcggcgcccatggtggacgaggcagtgccaaaacgcgcacgttcgccaagatgacggcagtaagggcgtacatgtacgcggaggctggaatcagtggcgtgatcctcggggcgcgcgagtacatgaactcgcttgaagagtcctccatggaggaaatcaagcaggcaattcgatccgagccatggctggacgcgtactttgacattggtgagaagtacattcggaccaagaatcgccgaatttcgtatgtgttctgcggattgcgccataacctcgacagcatcaagtcgaaggccagaatcctgatcgcctgggttgacgaggctgaaaacgtcagcgaaacggcgtggataaagctcctgccgacggttcgtgagaacgactcggaggtctggattacctggaacccggagcgcgatggaagcgccaccgacacccggttccggaagaacatgccggcaggcgcaaaaatcgtcgagatgaactacacggacaatccgtggtttcccgatgtgctcgatcaggagcgcctgaacgaccggcagacgctggacgaccagacctatgcctggatctgggatggcgcctaccgcgagaacagcgacgctcagatccttgctggcaagtaccgggtggccgagttcgagcctggtcccgattgggatggcccttactacggcatcgactgggggttcagccaggacccgactgtcggcgtcaaatgctggatttacgaccgcaggctttggattgagcacgaagccggaaaggttggacttgagaacgacgatatcgctgagtacatgatcaggcgcttgccagggatcgaacgacatgcagtccgagccgactcggccaggccggagacgatcagccacgtcaggagtaaagggaaagatggcagtcgtgcatgtctgcccaggatcgaaggtgtcgagaaatggaaaggcagcgtcgaggacggcattgcccaccttcgcagctatgtcgagatcgtgatccatgagcgatgcacgaaaaccctccgcgaggccaggctatacagctacaaggtagaccggcagaccggggatgtgcttaccgatatcgtcgacaagaacaaccactactgggacgccacacgctacgcgttgggcccgctgatcaagcgccgcggcgcggtcggtatgctgctaccaggagcccgctgatggccatcttcatcctcacggagcgcgcaaccagccgctccatggtggtccgtgctcgctgcacgtcctgcgcccgcaccgtggcggtcgagaacgctggcgctgaagggacgatggtatggcgcgaccccaacctctcttctgtcgaactggtccgcgagacggacaagccaggcctcatcctgaaatcggactgaccatgactgacaaactcgacctcgcggtcaatcacgcgatgagcagtgctgtcgcgcgtgcgcgaatgagcctgctgaaccagggcatcggccatgacgccaagcggccgcaggcatggtgcgagtatggtttccctcaggaaatcacgttcaacgacctgtacaccatgtaccggcggggcggtattgcccatggcgcggtcgagaagatcgtcaccacgtgctggaagacaaatccgcaggtcatcgagggcgacgatcaggaccgctccaaggacgaaaccgagtgggagaggaagaacaagccgttgatcgcaggcggcaggttctggcgggctgtctccgaagccgaccggcgccgcttggtgggtcggtattccgggttgctcctgcacatcagggatagccagccgtgggatatgcctgtcacgggaaaggtcaatggcctggcgaaggtcaccccggcctgggctgggtgccttaagccgaagtcgttcgacgaaaagctagatagcgagacctacgggcagcccaccatgtgggaatacaccgaggcctcccaagccgggcgccctggcctggtgcgggatatccatccggatcgggtgtttatcctcggcgactggaccggcgatgcaatcggcttcctggagcctgcctacaactccttcatcagccttgagaaggtcgagggaggcagtggcgaatcgttcctcaagaacgccgcacgtcagctcctgctgaacttcgacaaggagattcagctcggcgagatcgccagcacctacggcgtgacgatcgatgcgctcaacgaacgcttcaacgaggcggcgcgtcagttaaaccgcggcaacgatgtcctgcttccaacccagggggcgaccgtcacgcagatggtgtccgccgtttcggaccccagcccaacctacaacgtcaacctgcaaaccgccgccgccggggtcgacatcccgaccaagattctggtgggcatgcagaccggcgagcgggcgagcagtgaggaccagaagtaccacaacgccagatgccaggcgcgccgggtgcaagaactgacgttcgagatcaacgacctgttcgggcacctgatgcgcatcggcgtggtccctctgaaggccgagttcacggcaatctgggatgacctcaccgttccaaccaaggccgagcgcctggccaactccaagaccatgagcgagatcaacagcgccgcaatcggcactggcgagccggtattcaccgcggaggagatccgcgaagaggctggctacgacccgctcgtgggcggtgacccgctgcctgataccgaaccggaggatgaagatgccgcgcgcaccgatcctaccggcgagcagcagtgacccgaccggggtagatcgactggaaaggggcgcaatgcgcgagttcgacaggcgcatgcggaaaatccgggatggctatgtcgctgccttggaccgaatcccggcccagccggtggtgaatgagcagtacacctaccgtctcgaccaggcccttctctccgcgatcttcgccgacaccaacctgatggtcgacgagatactgcaggagggcggggagcgcgacctctggttcttcgaatcctatgtcggggttgcctacatccgcggtaccgcacagacgcatgccaacctggcgcagcaatcgcctgcataccgcgccggccgggaatcgctggatgtcctgcttcgatccgacgcctaccgcgcgcggatggcactgcttcgcgcccgggagttcgaggagatgaagggcttgtccggccaagtcaaggccgacatggcgcgcattctcgccgagggcatggggcgcgggaagaatccccgcgaaatcgcacgggacctgaccgcacagaccggcatcgaggcgcgtcgcggccatcgcatcgcacgcaccgaagtcacaaccgctctccgaagggctcgctgggacgagaaagacgctgctgaggccgactacggcgttcagtcgaagctgatgcatatgtcggccctgtcccccagcaccagggcaacccatgcggccaggcacgccaggctctacacctcggacgaggtgagggactggtacagccgagacggaaactcgatcaactgcaagtgcagccaggtcgaggtactggtcgatgacgaagggaatccggttgtcccggccatcgtcgagcgcgcgcgccgcaactaccaagtcatgaaagccaaagggcgcgggccctgggcgaaagaggattgagccatgcccatgcaggtcaacatcaccacccaggtcaacagcgccagcattcggcgtgagacacacaacgggcgcgaacacctggttctgccgagctacaccctgccggccggcgtgatcatgaacggtggtctctacaccgccgagcagatcgacaagcactacccaggcctggagggaacgctggcgccgctcgggcacccgatggtcgacgggaagttcgtgtctgcgttctcgcctgaggggatcaacgccgcccacgtcggcgcctggaaccgcaacgtgaagaagtccggcaaccgggtctacatggagaagtgggtcgacgtcgagtttgccaagtccacggagggcggccgtgaactgttgcagcgcgtcgaagcgctggagaagggggaggacgtccccccgatccataccagcgttgccgcattcctcaatcgcatcgagccgaacgaaagccagcgtgcccagggcgcggagtgggtcgccgacatccagagcatggatcacgacgcgatcctgctgcacgaagtaggggcggccactcctgagcagggcgtcggcctgatggtaaacgccgaccaggctgtcccgcttcagccgaattccggcgctctggttggcgagtcctaccgggagcgggagcagcgtctcgatcgcgccgcaaaggagcgattcgcctccgggcccgaccagtacgcatgggttgccgacttcaccgattctcaggctgtgatcagccgcaatggcggtgtgaccgaggtgtacggctacaaggtcgaggcagggaagatcgtcttcgacgaatccggccagcccgttgtcaggcaagagtcctgggtcgccatggtggccaacagcatcaagaacattttcacccatcgtcaggctcggcctgatcaacctgagaaggagggcgacatgcccctgacccccgaagaaaaggccgaaatcgtgaaggaaatcggcaccaacacctccagcgccatcaaggaactggcggacactatcatcaagcctctggccgacaaggtcgacggcctggtcgccaatcacaaggcgctggccgacacgctgaccgccaaccagcgcgccgaggaagacagcatgcgcgaagcggtcaaggccaagtttggcgaggtcatcgccaacagcctggccggcgacgcgctcaaggaactgttcaagcagtgcggcgaatccgctccactgggcgccaatgctgccaccgacaaaggcggcctcaccgccgatatcgccaacctgccgaaggagtaagccatgtctcgctatcgtcgcgtgaacatcgacggcaagtcgctgttcaagaccgaaacccgcaagaccgccgcggcactcctgcccggcacgttcgccgtgatcaatggcagcgacctgttcgcccaggcaagcgccagcgttggccgcctctacgtcatcgactgcgctcaccacgaaggactcaacatccgcgatgcggttcccgccggccattcggccgtgggcaactacgtcgaagagggtcgcgaactcgccgtgctgtgcccggccggcacctacaagaaagacacgccgatcaaactcggcaccagcggccagggtgccatcgcgtcgagcgataccgacacggtcctcgggtacagccaggacgatgcagtcatcgcctccggcgaaaccgacttcatccgcatccgcttccgtgtcggcagtgtcgccgccccggcgccctaataggagtacggacacatgttcctcacccagcaagcaaccgccgcccatcctcgcctgatgggccactaccaggagttgcaggccaatcgcaacatctggaacaaccagaacgccgctatgatcgcccgccaccgcggcgccatgacccccgaaatgctggcctgcaacgcgctcgccggcctgggtcgtgagttctgggccgaggtcgacgcccagatcatccagtaccgcaaccaggaaaccggcatggagatcgtcaacgatctcctgcaggtgcagaccgtgcttccgatcggcaagaccgccaagctctacaacgtggtcggcgacatcgccgatgatgtgtcggtgagcatcgacggccaggccccgtactccttcgatcacaccgagtacaactccgatggcgaccccattccggtgttcaccgccggctacggtgtcaactggcgccatgccgccggcatgaacaccgtcggcatcgacctggttctggactcgcaggctgcgaagctccgcaagttcaacaagcggatcgttgcctacaccctggacggcgccaccaacatccaggtcgagaactacccggctcagggtctgcgcaatcaccgcaacaccatcaaggtcaacctgggctccggcgccggcggcgcgaacatcgacctgaccaccgccacgccgcagcagatcatcgacttcttcaccaaaggcgcattcggccaagctgcgcgtgccaacaaggtggacgcctacgatgttctctgggtttccccggaaatcaacgccaacctgtcccagccctacatgatcaccatgggcggcggtgccaacgcggtggtggccggcaccgtgctcgatgcggtcatgcgcttcatcccggcgcgcgcggttcgccagaccttcgccctgtcgggcaacgagttcctgggctatcagcgccgccgcgacgtggtcaccccgctggtcggcatggctaccggtgttatcccgctgccgcgcccgctgccgcaggtcaactacaacttccagatcatgagcgccatgggcatccaggtgaagaaggacgacgaaggtctgtccggcgtgatctacggcgccaacctggcgtaaggagaacgacatgcccaaatacgaggtgatcaagccctggaacggcgtttccaagggtcaggtgctggagctcgaatcacttgccgctgcgctcctgccgaacgtgcgcgaggttggcgcactcaggagcggaagcctgaccttggacgtttcggcccaggtcgacgaagcggccaggcaagctctcgccgaagcgcgtgtatccgtcgatgccatgatcgacgaagccaaggcccaggccggtaccctgaccccggccattccggacggtagcgagcgccgcgagctgatcaaagcgcgcctgaaggagctgaagatcgagttcgatggccgccagggcgaggaagcgcttgccgccctgctgccggagggcgaactggcgaagctgttcccggccaagtgaccggtgcgtgacgagaggccgcctgcgggcggcttcgtcgtttctggcctcagcgatggggtcgcttcttctggagaatgaaatgtttggcaatctgatcgactcggacatcccggcaattccgaaggctccgcccgctcccatggagttcccggcctcgttcggggctagcgatgacttcaggctctgcgatgctatccggaacaccgtggatgctgcgcaagacgcccaaggtatgacgcttcggattcttcaacgacacctcctccgtctgtgcaacctgcaggtcgagcaactggagggatgtggtgatgatcacagttgagcaggcccggcagtatctgcagagccagggcatcgacaacgtgcccgatttcatactcgcggcgtggatcgagcaattgcaggagatccagagttgcctggatgcccactacccggcatcgaccgcgctgttgatccaggcctacctgctggcgctgtttgcgctggcccaggccgacaagtacatcagcagccagacggccccatccggcgcttctcgatcgttccgctaccaggcctttgctgatcgctggaaggcgcagttggccctgctgaacgccctggacaagcacggatgtgtgacggggctgattcccccgaacccaacccagaccgcacacggcggtctttggatcgcgcgaggcggctgcatgtgtggtgactcatgagcacgacggcgaattggagttacaccaacacggcgacggttcggccattcctgcacttcgacctttcgacccaggaggccgtttacggccctgagtacgaaatcgcctgcacctggaccgccaagagcgagcagatgcgggaggagggcgggcaatctggagcgcggggggctgagttcgtatcgcgccaccagatattcaccgaggaccgccggccgaagtacctggacctgatccagttcgacggatccaacggctgggaagagattcgctcggtgacgaactgggacatgtccttcttcggtgaacagccggactttctgctggtgacctgacatggcaatccaaggaatcgaccgcgtccggcggaatcttcgtgtggctgtcgaaaacatcgccggcggtgtttccgagcgcgcagtttacgaggtactgagccagggcgccgcaatggcgcagaccatgacgccgatcgacacgtcgaatttgatcaatagtcagactgcaccccagatcagtaatgggactgctggggtggaagggcggattggatatacagcagcctacgcggcagcggtccatgatgcgccaggaactctcgccggacagccaagggcggatttcggaaagacagcggacggaaccgcctttggaggcggtactggagttgggaactactgggatccaaatgcagagccagagtttctcactaaggggttcgatcagattgaatctgcaatcccatcaattctccgcaggatctaccgcgtatgaccccctacgacgccttccaggattggctggcttcgatcctgggcgagggctaccagtacagccgtgggatgtgggtcgaccacccgtcgctcgactcggcattcatcgcagcgatccagcaaaccggcggccccccgactcaggtcgacattcgtcgcctgcggttcaaggtgatcctcctcggcccgaagggcgtccggaaacatgttgtcgacgtcggcaactcaatcgagaccctggcgcaggtagcgcttggtgacagcgtcccctgtggcgccgcatctgttcgggcaatcggcgagccgatcgggcctggatacaccaccgaaaaccgggcctggtacagcctggaccttgaagttctctattaatcaggaggccagacatggcttgcaagaagctcaaatttccgggccgcgacgtcgtgctcgagtattacatcgggtgcggcgatgcgctgccggcggagaatgactggcgccgttttgggtcgctccgcacgaaggaattcaccgtcgagtgggacaccatcgacgcgactgattccgactcggttggcgcactgcgggagaacctggccagtttccagacgctgaccatttccggtgacggtaccgtgaaggcctccggtgccggcgcgcagaacctgatcgacctgacgaagcatgtcgtgaagccggacgcgaccggcggacagcctgttgtctggatgcgcatgaccttcccggacctgaccttcaccgcattcatgctcatcagcaacctcagtcgctccgcgccgtacgacgatgtcaccacctacagcttcgaggcttcggcgaccgcttccgacttcggcctgatcgtcgaggatacccccgacgcggatgcgccggacccgaccagcattcaggtcgtgccggagaccctctcgcttaccgttggcgaaggcttcaacttcgagggcgtcgtgctgcctgttggcgctccgcaaggcctgcgctggacttccagtgcgccgaccgtggccgcagtgaacacggttaccggcgaggtgagcgcgctgtcggccggtaccgccacgatcaccgccgcttccagcgtcgccccgggcgtcaccgataccgcaaccgtcacggtcatcccgctggtgcagggcatcaccgtctcgccgacatctgtctcgatcgccgaaggtgccacccagcaactgaccgccgctgtatctccgactggcgcggctcctggcctggtctacgaaagtgcggcgccggcgattgctaccgtgagctctaccggcctggttaccggcgttgatgtgggcaccaccacggtgaaaatcaccagtgcggcgcggccgtcggtgagcgtgacagttccggtaaccgtcactgcgccgtgatcctcaccgagatcggtgagataggcgtacacacggcctcgggggagttctttctcctgcggccgtccctgtacgccatgacccagctcggtacgccggccgagattgtcgacgtcttcgcgcgcgtcatgagcgacccgatcactgagaagcatcaggcggaccagttcgcggacgccctggccgtggtggtggcctgtagtgagcaggacctgtccgacgtgtttggctactacgaccaggatcttgtctaccggccaggaactgcggacgtcgagcaccttgtgcctctcgcgcgctgcctgctgaagcacggcgtcacaggagcgcttccgccgcttccccggcgccacgacgaagagccgaactactcgggggagttcgttgcgcgggagtacgtcgcgacggcgatagcgcacctggggctgagcgagcgcgaagcttggtccatgaccatgaccggcctgatcggcgccctgcgcgcgaaataccccccaaccgaatcgaacgctccgggcgccagagccccgaccgcggcagagcatgacgcgacgatggagtggttcgacaagatcgaggccaagcgcaaggcgcgggcgaaaggagcaccctgatggctgagaatgtcggcagcatctattacaccgtcgaggcggatacctctggccttgtaaacggcacgaatgctgctgaccgttcattggatcagatgcaggcaaccatgcggcgtgctgatagcgaggcggcacgtctcaacacgactgtcaccaagctttcgtcggctattaagacgatcatcgcggcgtcagcgctccgcgagatggccagcatggtccagtcctatcaggagatggctgacagggttcgtctggcgtctgcaagccaggaagagtatgaaaacgtacaggccagactgctccgtaccgccaacgggacataccgagcgctctccgaggcgcaggaactctacatccgcacttctgcaggcctgaaagctctcggatacgacacaacgtctgcactggatgtgatggattcgctgtcgtatgcattcgtgaccaatgcgaccaaggcggatgcagcagaggcagcgatcagccagttctccaaggcaatcaacaccggcaaggtttcggctgaccaatgggaaacaatctccagcgcagttccgtctgttattgaggatatcggcgccgctgcaggtaagacgggggcggaagtcaggagtcttggtgcgcaggggcaattaacggcgcaaatgctcaccgagggtctacgtaagtccttggaagagaactcaaaggcagccgccggcatgtccaataacctgaccgatgcaggggtcaggattcggactgcatttactcaagtccttgtttcgctggaagaccagactggcgcccttcaaaccttcaccaatggtcttatttcggctgctgatgcgcttcttgagttcgggcttgactcggaaaaaatggcagcatttctcgacactgcaacagtcgcagcagcttctctggcctctgttgtggctgggcgtctagttacctccctgtatgcagcaggtgcggcccaagtgcaaagattgcgggcaacgcttgagcagatagcagctgatcggaatgctgctataggtgcactgaggcgggcagaggcagagaaggccgccgccgccgcggctgtcgctctggctcaggcggacttgaatgctgccaggggttcaaatgcccacgcaacagctctaaacgcgctgctggccgctaaagaacgcgacttggccgccacaagagcgctaacggctgctcaagcaacgctgaatggtgtagcaaccaccgggacggtggtgatgggtggacttcgatcggcaatggcgttcctcggcggaccgcttggggttgttctgctggcagcaaccgcgatcgcaacatttgcaacgaatgcacgggaggcgaaagagcctacggaccttctaaccctgtccgttgaaaaacttggacaggcacagctgaaggttgcacaactggacatcgacaagcgaatccaagcagtgagcgataagctcaaactgcttggggaaaactatgcgttcgcggcaaaagaagcccaaggctctggtcgaagggccaatcgatatgctgaagatgccgtgcgtatccagggcgcggtcgaggagcttacgcaggagcttgaccagttacagaaaaagcgttcagacgtcgacgcagccctagataaaaagagttcatccccatctggtaatggcccggatcgccaggcaaacccggaggatacaaaggctctccagaatcttcgcgacgaggctgaactatctgctctcgcgggtgaagaacgggcgaagcttgccgcgcgcaaaaagctcagtgctgatgccacaaaagaggagatcgcggaggcggagcgtctcgctgtccagatattccgcaacagcgaagcgcggaagcaagagaagaagtcagcctctgataccgcctctacggtcaaaaagtcgatggaggatcagcgtcgcgctgccttggacaatgagaagactatcggagacctttcccagcaactggcacaggctggactgaagggaaaggaactggcagaagctggggcgcaatctcgccttaatccattcgccacgccggagcaggtcgcccaggtccgcgcgctcgccgcagctctgtacgaagcgcaacaggtcgaagccaacaagcagttgctggggcaaatggaccctatcgccggcgaagaccagcgctaccagaccgaactggagaatctgaaaaagctgaacgaggccaagttgctcgaggaccagcgctacctggaactcaaggcgcaggccgagcaacagcacgatgccacgatgaagcaactggaggaggagcgattccgccgccaggctgccggcaacgagatgatcatggcaacgctggatcaggtgcagcaggccggcacgaacgctctgactgggctgataaccggggcgaacaacggtgccgatgccatgcggcaactggccggcgccatgctgaaccaggtcgttggcgccctcgtcaaggtcggcatcgaacaggcgaagaacttcatcatggggcagagcatgcaagcgaccgcaaccgcccagggcattgctcaggccggggcgttggctggcgcatatgccccagctgcagctgcggcctctgtggcctcatttggcggcgctgcgacggcaggccttgctgcaatggcagcagcaatcccagcgatgctaggcctcttcggaggacgccaatatggcggaggcgtccaggcaaatggcctgtaccgaatcaacgagaacggcgcgccagaggtattccaggctgcgaatggccggcagtacatgctgccgaatacgcgaggcgaggtgatcagcaacggcgacgccaccgcgcagggctcgccgcagatcagcctgcagatcatcaacaacggtcctccggtttccgccaccgccaccatggacgggaacaacctgcgggtaactctcgatgcggtcgagcaggactttgccaacaaggtttcgtccggccaggggctttacccgaaagcaatcgaaggcgcatatggattcaagagggcagggcgatgatcaaatggcctgatggccttcccttcccgctcagggaggggtacggcttcaagacggtagagccaatggccaggaccgtcctccagagcggccgtgcacgctaccgacggaacttcagcaatgtgccggtcaacctggaggtttcctggctgttcaccgctgagcaggcgcgtctgttcaaggggtggtaccgagacgtcctgaaagacggcgtcaagtggttcgagtgcgatttgcgtacggaagagggaatcgttccgtgcaacctgcacttcgaggggatctacgacggtggctatctcgtcgggcgcgaccactggcgcttcaacgcgaccgtcgtgatgcgagagcgctcgatcatcgatcctgggtgggctgagattctgcccgagtacatcctcctcgctgacatcttcgacatcgcgatgaacagggagtggcctcgacatggcgacggctcttgagcggttctatgcctcaggcggtgaggacctgcagctcgccacgatcgagttgtcatgcccggcgtggccggagcctattctcatctgccagggctatgacgacctaacctgcatgaccgaagacgggcggctgctgacgttcatcgctggtgcgatcgatgtatcgattccgaagcgagacaacagcggaaaccagaacgttggattcgcgatcgacaacgcgaccggattcgcccagcagcgtatcaacgaagcgctggaggctggcgagtatgtcaccctgatcctgcggatgtacctggagagcgatctcacagcgcccgctgagcggccataccgcatgagggtcaagacgccgggtttcgagggtctcactgttcaggtcgaggccggttactacgacctcatcaataccgccgcgctgcgccacatctacaacgtcagcgagttctccggactcaaatactggccttgatcccatgccgaacagatacctcaccgccatctataccgagggcgggcgggcactgccgtgcctggactgctggggcctgacgctcatagcgcgggttgagctgttcggactgccgatgctgaccgacttcgatggtgtcacgcgactcaccccggtttcgatgcagcgggcgtgcgatacggagatccagcgcgcgctcgagcaatgcgagccaggacctggggtcatcgccgcggcctatagagggcggctgctcgatcacgtaggtctgctggtcgaggtggatggacgcctgcggattctcgaaatcaacccgggaagcggggtgtcgctcaccccgctccagatgttctccgacaaatattccaaggtggtcttctaccgtgatcgaaatctacccatcgctccttgacggagaaccgctggagcggcatccgatcggtcgcaggatgacgattcatgcctggctgaccgcgaattctcctgggtaccgctgccacgatgtccacccgttctccatcggtgttgtccccgccgaggttgcgctctgcggtgacctgaccgacaagcagaaaaaggcgcatgaggagttcgtccaccccggcgagtgggccgagcgcatcatcgaccgcggcgacattgtgaggatctacaagctcccgcgcgggactgatccgttcacgattactgcggcccttttcaagggggcgcaatcggtttttcggatgctcatgcctcaattgcccggcatgccgacgaaccccgggcagggcgcgtcgctctctgaaaccagcgcgcgcgggaacaaggtaaaactcggcgatgcgatccgcgaagttgctggccgtcgtctgatttatcccgactacatcctgccgcccaggaagtatttcgccggtccgcgtgagcagtggaccgaaatgctgttgtgcattggccgtggtcggttccagatcgccgaaggtgcagcgaaaatcggtgaaacgtcgttcctggcactgggcgctgatgcctctttccagattttcgaaccagggcagaacgtcagcgggcacccggcatcggtctggtggcacctggttgaggaagttggtgcgagctcaactggtaatgccggcctggacctgaccgagagctccaatctcacgccgaacccgtcggcaactacgttcacgttttccggaacgaacatcatcatttctgccggagccgggtcgttcccctctgacttggttgcggggacgatcctccgggttgaggcgatgtacccctattcggttaacgatggcggcgggacgaatcgcgacgtcgtgacgggggatatcgctcagctcgggctggatgttggcgatgagatcgaggttgttggcaccaacggcggcctctacatcgtaaacgacatcacctccacgtcgatgacgctcaactacagcaacggttctccggcgaatgcgctccagaccgggtccggcagcgccgcaatcggcccgcgcggactgcgctatcggatcacggcgtacagcgcgcagcaactcacagtcgagcggctgaccagtgccggcggtgtagatgtggactggccaggattcaccgctctcaattcgtctacgtctcgcgtcacgatcgatccgactagcctcgaagggggctggcgcgggccattccctgcatgccctgtatcggagaagaccaacttcgtcgagatcgacgtgttttgcccggaaggcctgtgcggtgtaggcagggaagggcagatctaccagatccgcacctattacgacatccagtggcgagacatggccatcggcggcgcatggacgacggtcagtaagaaccatgctggcagttctctcgaccagcagggttttacggacggcatctcgctgccgtacatgatgcggcccgagtttcgcatcagaaaagtgttcgtcaaccagggcggcaactcaacatccgagtaccgagaccgcactcagtggtacgggatgcgcgcgcgcctccaggctccgtcgtcctacgccggcgtcactacaatggctgttcgatatcggtcgtctgaccgtatcgcggcgcagacagaaagccgcgtctcggtagaggctacccgcatgctaccgactcggcagaacggtgcatggacacccgagatagcaacgcgagacatcgtcccattcctctgctacatcgcgaaggaacgcggctacaccgatgcggatctcgatcttgaggaactcgatcggctggacgcaatctggaaggcccgcggcgacacgtttgacatgatctacgaggacggcaaggtcacggtcgcgcaggtcatggacgatgtgcttgccgccgggtatgcggagaagaccattaagcgcggcgtgatctccgcagcccgagacgaaccaaggaccacattcgggcacatgtactcgccgcagaacatggatggtccgctgaggatcagcatcagcgcgccgtctgaggacgactacgacggcgtcgatgtagagttcgtcaatgccaacggctggatcgaagataccgtccagtgccgactgcccggcgatgttggcaggaaggtcgagaagatcacggctgtcggtgtcacaaaccgcgatcgcgcctggcgctacgggatgcgccgccggatggctcagcgataccggagaactgagtattcgttcgataccggcctagacgcgctgaacagcgagttctgggattatgtggcccttgccggcgatgttcccggccctggcctggcgcagagcgcatacctgaaatcgttcgttatctctggaaactcggtcctgatcgagtccagcgagccgctcgactggtcactgctgaactcgccagcgctctacctgcggcgcccaggcggaacggtttccggtggatatccggcgtcgaggatcgacgactaccggctgagcattcccagcatcgatttcgtccctgatgtttcgtgggaaatcgaaccgccgcacctgctgctgggaaatccatacccggtgctgatcagttccatcgatcccaacggaaataccgcggcatctgttcgtgcggtgaactattctgaaagagtatacgattatgacgattcatttgcgcctgagtaatccaatttggcccccttctttaggttgtcttctgcccaaagaggttgaagatttgtatagtgattcagcctgattacctcctcgttagaggatgcagaggaaagcgggatcttgtggtcaatatgccacaaatcccgattttcccaagtcattccgggcagaaaaagagtctctatgtgcaatcgtaacgtatcccaatcgcatccaagtatctctgctgtggctgatgattttcctatgccctgtctttttagtactgttgatattctagagcgaatattgcaccttaatctaaatattggatctatgcttcttcgagttttcatatagctgttggctctagagttctctgtttctttgtttttcctgtagtaatttcttcttttttcaataagtttttgtgggttttcttcttttcttttcttccatatttctgcatgccttccttgaattttggatgcccaagactttgcatgagcctttaccctatcttgattcttcaatttccatgattttgagtattcttttagtctctctgagttattaagataatatgtcttgcttttcagtctgattttttcacgattttgttcgcgccattctcttgttctggagaggattttttcataattttgtttctcatattctttctgctttgatcggattttttcgtaattcaattctctgtatttttttcgtttttcgtttacgcatgacttgcattgagagtggagtccatcctttctttgcttattttttatgaactctgatacgtgcagttcctcgttgcagctgctgcatgtttttttgcttgtcaattcaatctcctattcttgtgttgttagcttggacctgccgagctacgcatctaagaatactgcaaagctatagattaacctggacaaccatacacaacctagcccgccatagagcgggctttttcatgcttggagaatttgcatgactacgtacgccaccagcaatccgcttggctccaaagacccgcgcgacttgtacgacaacgccgagaacttcgacgcggcgatgaacgaccgggtaaacaccacgtggaatgatcgtttcggcgttagtcgcccaacgatgaaagggtatgaggaacagttcaacggctggctggacgcccaaggcttcgaacccggagtcctggagtacgtcgacggctcaccgctgaccgtagaccgtccgacccaactgatccagcgcgacggaaacctctacagcgtcaagcgtcctgcatcgttccccgtcaatctgaccgggaactgggcgacggaccagagcctgcttgttatccaagtagaccaagggttcccgcaagaaatcggtcgcggcgtacgccgggttgactcggttgccgacctccgggccatcgcagggcgattcgccggggatgccgcgctggttgtcggatactacgcggaaaccccgggggtcggcggcggagagttccactgggattcaacctcgatagaggacgacaacggcggctcgatcatccaggcaaccggtatcaccactggccgatggaagcgcgatataacgcacggcgtgtgggccgaatggttcggcgctcgcaatgatggtactgatgctgcgggaactactgctgcggtgtgggctgcaatcatcgcactccggcacgacccggagacaatcgtgcagtacatcggcggtcccactgtcacagcgtatgcatccgggcgactgaacttcggtaacggggtctttgcactccagcctgatagtttcgatattacccaggacctcggcctgaccatcgtcgggcagggattcagaggtaagaaccaggcgatgaaggcggctactactctggtagtgagaggtacaagctctggcttcttcttcaggcactatgggaatggcggcaggaatctaacattcaacaacattgatgttgtgtatgatgacagccaattcagcggcgatatcatagaaaccacctcttctcccggccttactctgcaaagggtgcgggttggctgttatggtggatttcttgccagtcgtctcaccaccgcgagaagctgcatacgggcgacgtttgatgaattcatcaggtgcgaggatgtcgttttagatggggctcaatatgggttctactctgatgggacgataaacgttccagggctttcattcggcggctggggtgtgacttttctgaattgcacattttacgacttcgcgaagtccatggttctgcatgctggaaatcgcacaaggcacagccttaacattattgcgagctactttaaccccatcaatacatcccccgagcgctgccatgatatagataatgtcgagggactgattatcgatggttgccagcacactcctagcactggaagccagccttcacaggaatggtttagggttattggtagtactggcaggatttcctgtaacgcctttgccggactttcctcaaaacttggaaccattggtggggcgaatccgtctgctgttgagtggtcgaataaccgggtttcttgccagggcggcctaaccataaccggtggagttgttcgcggtggcgggaatgagtacagcaatgccgaccactctgtagatgtcgctccggttgcaattgtatctttagacatcgggcctgacattcataaagccggcgtcactggttactcatataggatatcggcagatagctcgatgctgagtgggagagttaactactcattcgaacaggataattccaatagtaaatactatagcgcctctactagggtagggatgtcaaactgcgatagcaggttcataactcttgctactgctggaaccaaactgtcgccttataacgctgggcgcacgtacaatgtgactgttgcaggtacgcagaccttgccaaccccgatcccaggggctgcgccaatacgcattctaaagtccggcgcaaatgctctgacgattgcaaccacctctggaacaaacttcctgatcggtgcctccgggtcaaggaccagtgcagtggcgacctctactgaggtaggttctctcatagagtttgagccgttaacgtctacggcatgggttggcagagtgctatcaggcacttggtcatttacctgacagtttcggagatggggacacaaggattcctatccttgtgtttctttctacgatagtcactattacgatatccggtctgtacctatcaaccagatcggcaattactttagggctagaacgctgatgatgcagttgtagggtttctgagaacgtggcggccataaatggggatatagcagatccgaaagagtctcgaagccacagaacacgcttgttgttaagcgcgccctctgatcggaccaatagtggcttaacgggggctgtaacttgaacattgtctcccgagtagactttctccatgctttcgaagtctatttggctaacatggattttacgtatggaactgtccgacagatccacctctgcatccgtgatgtacggacgtatcctttggaatgcagaaaggtcgccgcctccccgtttccttataatcacagcctctggttttggttcttcaggtatagatatatctggggagttagattttatacgcttcgccagtgcataaaaagaaacccaagctcctagtgtattccagtgagtgtctgtcttgtagtataaaggtgcggtggatctagattttatattaataagttcattttttggatatacaaaaatatctggagattttctgtatatgtgctgggcaatgcttgtaccggaaggtgcagcccagtcaggaaggttctcggggtatatcgtagacttgtcagggccaattaaaacatagtagcccctaacgccatttgacgaaaaccattcacgccatccgtcagaaacgtttttgataatatctgtttttgcagtgtcggagtccgtgactccgactcgttttgcggttacagagttttcgaagaaatcgccgaggaacatccatccgtctcttccaataataaccttttcaggactaatggatattcctagcttgtagaaaatcatcccgatgtagggtagtgtaaaatccatgttgtaggaaaggtccttccaccctactatagtttctggaagtggtttgtttgagctaatcgcttgctcaatgtttacggcaggagctattcctagaacagcgatagaaatgaatatgaatgaatatattttccctttcacttctataatccttagaaattgaaatataggaatacagtgcttgttgattgtagtgtagagtacattgccaagcagaatagtattgacatgtatattgcttttaaatttccgatccttccggtcgttgaaagctcgaatgagtttttctgtgaaattatcaaaaatgctgctgcaatcattccatagcacagcgagttcgcaacaacaccgattggcagaaattgtaaaagcttgtcggaaattacccctgcccacgcaagatcgcttgtcggtatttcagccaggctttccgatgagatagatctaatatcaatcatccctccaaggattgacatggcttcctgcatggatgtggctcggaaaaatacccaggttatatttacgaatagaaatgtcacaacccaagccaaaggtcttggcatagacattccgagatttttccacattctgtggatgacaagcgctccaccatgcagcgccccccatatcacaaacatccagcttgctccatgccataggccaccaagaacaaacgttgccattaggttgaagtaaactctggcggaagaacagcggtttccacctaacgggatgtaaaggtagtctcgcagatagcggcttagggtcatgtgccaacgccgccagaaatcttgaatatcaagcgccttgtagggcgagttgaagtttattgggagccaaatgttaaagagaagggccgcgcctatggccatgtcgcagtaaccgctaaagtcaaagtatagttggaatgtgtaggaaaggcttgtcgcccatgatctgaagaaatcatgattggcaccgctcgaaaatcctgcatctgcccagacagagaatgtgtcagcgatcataactttcttgaataggccgatgctgaatataaacagtccagtaagaatatttctatagcgtactgcccatgtccatttcgacttgaattgacccatcatttccttgtggtggagtattgggccggcaattagatgcgggaagaatgtaacgaataaagcgtaatttattaggtcgtattcttttgcttcgcctctgtagctatccaccaagaatgcaatttgagtgaatgtgtagaagctaataccaagaggcaagattatttcatgtagcgcaaattctgatccggccgcagcattcaggttctcaataaaaaagttcgcatatttaaagtatccaagcagagccagattcgcagtaatgcttaatgctagtattgtttttctgtatccaccaatggataaattctttgaggtcggggagatcgcgcaccctactgcaaagttgaataaaattgaccctatcaggagtggtatatagtcaacgctccagtatccatagaagaaaacactggctaatactagccatattttccccaatgagatcatccttagcttgtttagtccaaaataaacaaagaacactattggcaagtaggccagtatgaaagcagcggaactgaagatcattatgccttcctgttcgttccctgatgagggaaggtttgttagtgctgtggccacatcgagggcggcgcagatcatacccaattggagcggaacatgcccatcactgagcagcagttgctgcatatcctcccgaacgccggctcgagggccggcgtttttgttggtgcgctgaaccgcgggatgacgcgcttcggtatcacgtcgcctgtgcgcgcggcgacgttcctcgcccaggtcggccacgaaagcggccagttgacccgcttggtggagaacctcaactacagtgcccgtggcctggctgcgacctggccgagccggtacctcggcgccgacggccagcccaacgccctggcgcagcgcctggcgcgcaacccccgagccatcgccaacaacgcctacgcctcgcgcaacggcaatggcgacgaggcatcgggcgacggctggcggtaccgcgggcgcgggctgctgcagatcaccggccgggcgaactaccgcgccgccggcgacgggctgggccagccgctggagcaggaacccgagcttctcgagcaaccggagtgggcggcgatctcggcggcctggtggtgggccagtcacggcttgaacgacctggccgaccgcggcgagttcgccgccatcactcggcgcatcaacggcggcacgaacggccaggcggagcgcctggcgctgtgggagcgggcgaagagggtgctgtcgtgatctccgcccgcgttctatcggtcgcgctggcctgcctgctactgctcggcctcggcgccgccggcggtgtctggctcggcgcgcggcactaccggccgcagctcgatgctgcgctggcggatctggtcgcctgccgtgcctcccggggagagttggagtccgcagtggcggagcaggtccggcaggttgccgcgctgcgcgtggtcggcgaacagcgggcccgggatgccgcgctggctgtggatcggggacgacagcaggccgcggagcagtatgccgcggcacagcgcctgctgagccagcgaaccgccggcgagcagtgtgcggccgccgaggcggtcattgatcaggagttgggcctatgaaactgcaggcgtggcgaaagactgcaggtgcagcgattttcggcaggtgcagccgaaaggcgcaggtggtgcaggtgctggggttggtgttcgcgctggcgggatgcgccggccaggtcgagcctgagccgcgcacggtgcgcgtagaagtgccggtggcggtgccgtgccgggtgccggcggtggaggttcccgcatgggccacggcggggctgcgaaaaggcgacgatctccagaccaaggtccgtgcgctgctggccgagcggcggcagcggatcgggtatgaagcccaactgctggctgccaacagagcatgccagtaggagtagactacggccttttcctacggagcttggtgatgctggtcattcgattcaagggctggtcggtgaaactcgaccaccaggtgggcagcgctgggaagttcggcatctggtcgttccacggttcggagagcagctacgtgccggacatggagacgattctccggcatgcagcgatccggccggcggagccgaaagaaggcgggcggtagggcccggcgtagcggcttacgaggcggagcgctgatcctgtaccagtttttgtaccaatcgatgcgaattctggcgaatcatggcgcctgaaagccttgattctactgctctccagcgcgctagctatcgccaaaaaaatcgcatggtgatgttagctgtagatatcaaggcattgtcctgcggggctttgcgggatggttacgcgccttcctctgcttcctgtaccaattccgtaccagttttaaccctggtctgtagcttctccaactcgctccaatccgaggcggagttcagccacttggcataggtcgatagcagcatctgcacgctgtggcctagctgtccagcgataaacgcagggttcatgccagccatcaggcacatggtcgcgtatgtgtggcgggtgtcatactgccggcgccttcggatggatagagcatcaagcgcggcgtggaagtgctttatggtaacacttggctccttgatccacagcccgcctttgctgggcgggaatacgaacgggctgaccgcgaactccgagactgatgcgacgcgcctcaggcgcgcaatccgcttggcctctaccagggcattcaatgctcgatcattgagcagcacgtcgcgctcatgcttggtctttacgcgttcctcgatcccgcgatctatgacgatccggcacacatgaatacgtcgtgcctcttcgtctacctcgtcccatcgaagggcgaacgcctctccaggccgaagaccagtgaagaacaggaattcgtacagtgcggcgtagatccttgagtacttcccaagggtcgcgtacaggtgctggatgatgcgttctgcctcgtcccgggtgaatggatctaccagtttcttagacacccgaggcttctcaaggggcgccatcgggttcttcttgatcagaccgtccttcacagcggaatctaggatcgtcgacagcttgaacatcgcgtttcgcttcacgcctggcgacgtccactcgatgctgctgatgattcggcgcaagagggtaggggtgatctgatcaagccgggctactgctagatgtggcatccagtattggttgaggatgctcttgtagttcttgcgtgtcccaagcacgatctctcggctgtctagccagagttgagcatgctcaccgaacagggggatttggctgctgaccgattccgcaatcgcagacccggggaagaactctgcataccgggcttcatccatgatgcccagcttgattgcctggactacctgatctctaagaccggatgcagtcttaatccctttttgcgtcgcgggataggggagtgtttcgcacttccttgttccgttccacatgaagcggatacggatagagttgccgatgacttccaccccggtgggcatacccaaaggctttcgagccattcgtcgtatctccgtcgactgtagattattttcccgttgaccttgttccagacgccttctggaatctgtccctttgaccgtctggtttgtagggcgcggtaggttatcccaagcagcgccgccatgacctgttcgggcaccttgtcttcgtactcgatttgctctgcggtactcatagacaatacctctccgccccagctattgccggggagggcatgatggtaggatttagacgcccagccgggttagctcagggagagctagtggcgcccggctgggttacttgatgagttcggctgggacgttgatggtttcgcccagcttcgctcgaacgatggcgcggcaggctgctattaggtgggttggacctgccgatgctgcatcagctggcatatcgcagccgcaggctgtgaagaatcgcagcggttcgccatgccagtcgctaccgatccactcgaattcaaagcggtgcttttcaatcagtggtccgccttgagcccatgagtccgaaggttcgtatcgctcgacttcttcagtaatcgagcgagggccaaaggtgcagccatatttgcagcagtgaatgccgcctctcacgtcataacggtactgtccaatgtcatggacaatgacctcttcgccttcagccattgcaacggcccaattaagcgctgccccctcaagatcccagatcttcacttctacggtttcgctcattccccacctcccatagacttgccgatctcggcggcggcgcggacgatggctagtcgaatgcacgtgtcctgatagaagacatcgttttcagcagttctaaacatgactgtcggattgctctttgggctatggatctccagattaagcagaactgccagcctcagcgcgtcgccgtcgtcgtgtcgtgggtcccattgtcgccaccgcccagtctctgccaggattaacgggatggagatggagtggtacgggtatgagaactgatagcccgccgcccgcgccgccagttcgagtagctcgcggtcgttcattgcgtttctccttccagggctgcgtcgatttcagcgtctaggtcttcctggttgagtacgatgttctccggggtcatcccggcgaatacgccgccttgtctgatcgtttcgaggtctcgctctcgcagccaccggtagcgagcggcatccttcgccatgcgccgaatctgctctggtatgctgacattgccgccgtctggagggtccatgtagtaggtgccaggcagggcgcttgcgcactccttcaagtactgctccaacaactcgcagtgtttctgcgtgtccttgtgggcgcagttctccgccttgagccgagcgctcagcagatcaacctcggcaatcagcttgaggatggcttgtggattggcggcggcacggaatgcggagtcttcgccgccggctccggatggattggcgatgtaccgctccgccaattccttcagcttgttgatatcggtcatggcttggttcctttgatgatttcgtcaagatcgattggcacattgatgcttttcagcatctcggcgaactgcttcagtgccccacgcagaacctcgttctccgccttgatctggtctttctctcgcgtccattccagccatgcgtcaatgtcgtagtcgcctttcatgccttgacgcagcctgtcgctctccgccttgagctggtcgatctcgtccagcagggcgaggatggtcttggggttggcggcggaatcgaacaaatcccaagcagcggagatcggctcatcctcgctccgctcaattcggatcacgtcctcagcaagcctccgcagctctgcgtggtcggtcatgatctggtccgcctgctttacgctttccagcagttcgttaaaaagtggctcatccatcacttcacctctattccggctttctggagggctgctagacattccctgattcctcggttgaattcggcaagctcaggataagcatcaagtgatgagctaccatatggctttggcggcctcaccctcagagccgcgcggctggcttgccaggccttgaacgcaaggtgagccgagtagtctttgaagcagttgcgctcatcctgccattccgactcaaggccatgctcgcgcagtagccaagcttcaaactcttctctcatgtcaggcacggtcaggactcctttgggtggccacgcagacggtcggccaactccatctcggcgtaataggcgctcatgctttcggcatcgttgaggttcaacgttccgtagacatggcggttatagaattgcgtggtgcctaggcaaggcttcgacaggttcagggtgtagccgcgcttgtcggccaggaacttagcgactgcggcggatcggctcatgcctgcttggcagtgaacgatgatcggttcatcaccacactcgttcacgaagtcgtggatctgcttggcgtcaatgtggctgaacacccgaaaaccatcgcttcccaggtatccgtctacatcatcaaattccagccgcagaacgcgcttgtgatcgcaggcaaaggcataccagtcgcccttgctgccgatgctgatcacgttactcggcgtctcgatcctgctggcatccactgcggagaggaatgtcacctctcgcctgttcactgcttgctccatctgctcaactcctgtcctttcaactcggtctgctcgtataggttctggaagtccccgacgacccggaagattcccaggacgaagagaacgatgactatcactgccaatatggtttcgttgtcgttgtccacagttggtcctccgggggggcggatacggttgggttcgttggggttattcgcccgctgctttggagatcaggtgcatgagcatttcgcgcagttgctcgcgctctagcacctgtccggttttcgcgtactcgtcggcctggcgcaggatcgcgtcgatctcgatgttgaacatcggcgagagcacgtctggctcgcactgctcgagcagcaactggattgcgcgggtcgggtgcgccatcgtgatcccgagccagttgtaggccgaggcagtgcggtagtagcgaaggccggcgatctcatgccgctgaggcgggcggaagggtttcgtgcgcatatgcaatccgggtaggttgagcctacattttccagattgctgtatatgcgtacagtggttggcgatgggtggctatgcctgctccgacaggtactgcaactcccaggtcgggtggaacttccttggcttgctttcgccgtcgagcttgatcatgaggtgggcgcccttggcgcttgtgattgtccctcgctcttcggtgccgcgccctcggtaaatgacttggccgccgcgcttgcatggaacggcataggccttgcggatgaactccatgctcattgcgtccctccctcctgctcgcccagcaggtcgcgcaggtcgttcgcaatctcaagcatcttcttcgcgcgtgtcgtggctgctttcgtgcctgccggaacgttttcgcagttccaatcggactctcggcggcactcccgctctatgcgtcgcagcaagtcctcggcgaccggcacatgaccatccgggaccatgtagagtgccttggtcctgcgctcggttctctcccttgatacatgcccgcaacgaccagcgagcgatcgactgatccctaattcgctgatgaacccgacgagggacagcttatcagccattgccgttctccttgccctggttgagcaggacgcgaaggtctgccgttatccggtagcattcagtcgggaacgaggtagaccaggcgcatgcgcagtactcttctgggccgcggcatggctcgttcatcacctgcttggcgatcagtccatggcgttcagcgctttcctgtatgcctgccccatcgaagcttccgccatcgagggctccgcagatgatctcgcgcgcgaacttggccatcccctgcacaagcccctcgctgaccgtcataccgttgatgcgcgccagttcgtcgaggcaggcgttccagccgctattacgatttagccctgggacgccggcatttagaagcttccgctccggcacaaccaccacccttgcgcgcagtgtcgcgagttcggcgcgaagctcctcgatctccatctccatgccgccgcactgctggcgggcagcatctccctttgccgctgcgtcctcggccatggctagtttggcgactagggcgtcgtagtcggaggccaggacgacctcataccccattactgcctgctcgccctgggtcaaagagcgcatgctcggcacgtcgaaccgcttcacctcactcatgacctacctccttgctggctgctcggcgcttcttcatgatctctgctacgccgtcggggtacgtgatagccacggccccggctgcgagagctgctgacttcttcgacaggcagatatcgaagtgctccttgatggtcccggcatgctgaatccacttccgctgaacaccgatcttgtctgccattgcgagcagttcctcggtcgtgtccgcgagcatgtgacacatcttcatgcggccaaaggttgcgttcatgtcgtcgacgtaaacggccatcacaccccctccttgccgggcgcggcggccttccgaagtgcggcgttcaatgctctttccatcgatttgaacggggactcgcccggtcggaaagcgtcaagggcagccacgatcatttcgccagtaaccttcagcacgctgtgctgagccgagctgccgggcacgtcggcgagtatggaaagcagttggcgctcagccgtaattcgggtgtcgtggtccttgtcgctcatcatgttgagaagcggctcaatcggaaccagcttccagccctccggcacgctgtgctgagccttggcgaccgctagcgcctcgttgagccggaacccttcgtgcacccagtccgtcaacttcccttccagctccgcgaccctggccagggcgacttccagccgcttagcgttttcgtcgcgctcgtacatcactttcatgcacttttcgaagctgccaacagggtcacctttggactcactcaggcgctcgacttcgaccagggcggcgtcgcgctctttacgcatttcatcccagtccgcgaggcgctgctctgcctgctctgcccacgaatcgcgatccgcccgcagctccccgacgatgcggtcgtgctgttcgaataggtcagcggctttctcggcgtactcgacgatggaaacgtcgcaccctgtatcgcggccttcggcatcctcgaagcgcagatcaacgttgtcgccgtcgatgtcttcagcgtccatagcgccgatgttgcgcaggacgaacgcgacttctgctacctccggccgctcctcttcccctaccaggtcggtcccccacttcgctacaggcacttcgaaccggtcgttggctacatcaatggcggcacgcagggttggggccggagagggttgagtctgcgctggggagggttgcgccagggcggcgcgggccatccaccccttcttgttttcccgtatggagtggtggttttcgttcagatcatacttgtcttcaattccatactccttgcaggcccaggctaggaacttctccagctcatccccgcctgcctgctctaccggtgccttgttcagttccttgctcacaatcccttctcctgccgctcaatagcagcgatgaattcgacaatctctgtgctgaggtccatggcgccaatgctgttgtggaccccgacgtagcggtttgcgcgcttcagaaggagcaccgctgtgcgcaggccggagtcacgcttggtcttcgccttgacttccatcatccacctccgggtagacctgaacgccctcggcgccctgggcctggttgatcgctatctgcctcaccgctctcgcgaatagcagaatgtcgtctggggtcatgagctggctttcttcgggccagccggtgaccgtcacaccgccagggcggtgatgcgctgttagctggtgcatggggttattcctgttcggggagagggagtcgcggcgctaacgatgcccgaacctgatgccgtgctcggcggcgatcttgcggacagtagcgcggtcaaggtccattgcgtctgcggtggcggagatagtcatccccttgtctgcgcagtaacggactgtttgcgatagcagcctgcgattctctcggcggttgctttcgaacgcagcgtgcgcggcgtcggtctgccctggcttagcttttcgtgccgacctaccgttccactggacgtccttgtctcccgacatgccgattgggatggatgcgatctttccgccgctggctaggaacgcatctacctggctggctatttcgtctcgatgcaagtcctggctcatgctgccacccctagcaccttttccatgcgctcctcgagcagttcgtagaaggtctttactcgctcggacagcttgcgtatgtaggcctcatcgcggtggacgcgcaccatgcaaagcggcatgcctggccagtagccgaggaagtcgatccactcgcgctccgaaacccaaaggcctccatagcactgagccgcgtgctcggaaggcagctcgcctgcgatgatcacgctaaccagcttttccggtaccttggttttcacctctatcaggccgttgtcgccgaccagtccatccggcgaatagccgatcccgtggttcagaatgatcccggcctgctggatctgatctggctcggtatctgtgcgcaggcagtacaagtcgcgcacaaccggctcaagcttgtgacccctggcgctgctaccgttaccacgccatggctcggcctctgctccggtgatccgctcaccaattagacggtccatgtaagtgaaggcgccaacgccgaaccctgcctggcctttgccgttaaccatcaacacgtccagttcggagcaggttgcgattccaagacgcgcgtcaagccactcctgggagccctgctccaggtccttgaagatctgcatgattcactcctgggagcgcttggcgcgctcgcgagccttggtaagccgtgccagtgccgcatcgaagtcggcggatgggacaccctcagcagagccgtacatagcatcgaaggcttcttgcgtgtcctgaaggcattgggagagaagggttttcagttgctgcgcctgagcttgggtaatgagcttctttggcggcacagccgcgttgccgtcgtcgtcctcgccgcgagtggtgatgttcagcagtgcggacagcacgtaacgcttgccgtagctgaccgatgatccaagagactgaacggcgttcttgctgccacttgtgtctagcggaacgagcatcgtcgtctgctctcggtgtccggcgcagtgcatcagaattccagtaaccgaaacgccagtctgaacagtctcgacgcggaagctcactgcgaaaccgaaccgctgcatgatcggcttcacgatgtcgttgatgtcttcgaaggtcgcgtagttgctgcgcttttggccgttgacggtgatagcgccacgctcggcaatgctcggcaattcgctttgcatggcggccatggatgcgttgaactcagcctctgcgctgcgggactgcatccgttcgtgcatggccataagccgctccatcttctcgatgtcgcacgcagggtcagcagcggcacgctggatcacttgaaggattgttgccgactcaccagcttggattacggcagcaccttcctgccgctgtgcaatggagttgctcatgatgggcctcagtagttgattgtgatgtgaggaaccttgcgctgagcgatcagtgtgatcgcctgcttggcgcattcctcgggcatgccgccggcgatcagggccgccagggcttcgttgttgatggctttcttgtgggccttgtcggcttctcgggctgctgcctcgcgctcgatcctggcttgctcgtctgcctgccgttggcgctctgcggcagcggcttcttcggcgcgccgctgtgcatcacgctcagcctgctcggcgcgttgctgtgcttccaacttctcgcgctccgccttctcggcagcgagtcgcagttccagttcccggcgctcggcggcagcctttgcctcggtttcgcggcgagcggcggcttcgcgttcttcctgggcgcgtcgttccgctgcaaggcgctcggcctcggctgcttcgcgggcaatgcgctcctcgcgctctttctgctcgcgtgctgctgcttcggcgcgcaggcgttccagttcggcctgctcggcttcgaacttctcacgggcaaccagggcttctcggagagcgatcaaagccttatctttggcgcgagcagcctctgcctcgaactcttcccaggcttcacttatggccaggccttccaaccaagcgatgttggctttgagttcattagagtccagatcgcggcattccaggcgaaggtttatcttgtcgatctcgccctgatgacgcgcaacccgcgccgcttcagcctcttcccactcggtcaacggactgcgcacttcggcctgccaggaatccaacaggtcgcgcatccgcttacgctcggcatcgatcttcttcggaacttccttcagctcagcgaccaattccttgcccacgttgtccagcgccgtcttggagcgggcgaccttgtaggcgatggaagcgatggcatcgcggcccttgcgggttgaaacgtccggcacgaagccgtcgatttcctcgcgaatcttggccaggaacgggtcaaggccattggctgccgagtagacttgcagagcggtttctttggctggtacttcgaccagttggttttctgcggacatgaatgatcctcgccgcgcatgcgcagccagtgaagggaggggttattggccagtggccgtagattctgcggtgatgatcccgccccagatcgggccggctgcgagaatgaacaggtacagcaggccgccgaagaggctgcctagccagattgctgtgcgtctggtgttcatagccctgccacctcaacaaacgccacggcgaacatgaacacgctgcccacaaaaaagccgccgaagatcaggacttgggcggcctctttcaggtctatggtgatggtcatggcgtgctctccattgcttcatcaacagctttgtctacggccttcccgaaaagccagttagacacctgatcgccacagtcatcggtaagcgacaccatcggatagaccccgtctgcgtccgccgacttgtcccgcaaccaccgatagcgcttagcatcagcctcagcagcgcgcaggcgagcgatcaggccaagtatctcctctgctggagtgttgatatttacatccgtcaacactggctcgttacagcagacttcctcgcgcgcgctcatgtattcggccccggatttgaaattgccacaacagacgaatgccctcttgtggcagtactcttccaactccgccaattgctcatcactgatcgattgcacgataggggttgtcatttcccttcctcctggcggcggtagccggcgtcaaatagcgcgtaaagcgtagggtactgatatggaactccttgaattgacatagccatatcaccgactgccttctcccgctcctcggcggcgatctgctcaggggttcggagcgggcggaaagcaggaagagatccgaatttcaaaacggcatatgacccgtactgcccctttcttttgccttcgcaccaacggaatacgacacggccctcgtcgtgagcgagtatcttggctcgaaagtacgcaatatcggcgccgtcccagatggcctcggcctcaatgccaatcggaggaaagccttggccgtcccatgaggtaggcacaagccgcggaacggaatcttcaatgagggacttgccttcttctgggttgcaatacctcatccaaaagggagggcagaagtacatcggtatctcgccatccttcagccacgggtaggcgagtttttggttgtagtgcgtcgcaccctctggtgccttgttccagtcaatgctcatactcgtctctccctaaccagtcgttcagcgttctcgatcagcgttgcttcgaatgcgcggaaccagatgcgttgtgccagttccaggtcgcctcggcgcactgcaagcagtagctgcgtcatcgggcactctttgccgtctacctcggcgagccactcgggcacgaatccagcaaagccgtagaccgtgaactccggcccgataaagggcctctctttccggtcatggaacggcacgcaatcaccgtcctcgcagttcaggagcttcccgacttgctcagtgacatactctcggtcgccgtcatcgtctggcggcagcgcgttgtcccagcgctcctgggcgtatttcaatgcagtgttcatttctcacctcagtcggtgtaggcgatgtacttgaactggcctttctcttcgttgaagtactcgaagcggccgccaaacgtcccgatcacggctttttcaacctcggcgcgcgaagtgccgatggggaaaactcccttcttgatcattgacgcgcccgaatgcggttcccatgtccagtcgattttggttgggtcaagcacccgaggcttgctttcgaggaaagccccatatccaccaatgtctaggatgatcgtgtgaatctcgcgcacacagagcggatcgtccgccgcgcgccaaccgcagtcaggacagcacatgtccgcgctcgtatgcgctgcacacggagggctaatatggcaactgcaattctcgaccctctccagctcaatcactccctcgcagccgccgcggttgcagatggagccttcctcgtatccgagttctttcatgtctcacctcgcgttcgcgtgcatgcggcagcgttccgaatcgctgtcgtcatacaggcgaaaaaatgcccggacttgccgggctaatgagcggtagggtggggatggccggagtttcaccggcggcttaattggtcactgccaataagctattaccgctattcgcatgcgatacttatccccattgaagggtggcgtccttgccggggaagtcagtcggctggaggcgctgggagtggcatccagtgcgttgggcgccagttgaaaattgatgaatgtattggatcaaaccaatcccacccagcgttcagggggccatcaccgcgctgccatgtcgcatagccgatactcccctccgtgtactttcgcatgtgagtttctctcacgccgtaatctgggcaataaccaagaaacttggtgccatcctttggagcgctatcaatcgttttccactcgctcatcttgcctccagtgtgtgtattcgccagggcgcggttaggcggttggtttgactggtcgaactgaaacaacaacccaagcatcatttccaataacaaatacacaggaagcttcttcgtaggggccgtcgtagaggttgccgtccgaaccttcttgcccgaaatcgatcttaccgttcatatcggcgattccatcccaaagcgggccagtagtcagcgcatgcgatgcccattccggggcgctcttccagtcgatatttacgctgttctccagcggaagctctggactcggcatccagtatttgaccttgtaacattggctttcgcctttacgttggcaccatgcgcctaaccattcgccttctccctcgtaagttgctccttctatttcatatcgcccacataccgggatcatgatcaggcatttgtcgccaacgtttggtagatgatcactacacttgatccactcactcatctatcacctcaccaataaatagtcagaaacagaacaacgaacagcgctgcgaactcgccaaggtctggcatggattcctctcttcccgtatcagggcaaatggattgcatcccgctgctagccaaggcttgcagggacgactttcatcgcttcagcgacaatcgagtgaactccttgtgagtcaaccgtggcgaaccccttttcggcgtggtcccactgctcatcctcgtctccggggaagttgctgcacgccactgaacagacgccaagcccgtcgggcttgaagtagaggcgcacctccgggccgtcatccccgcgatcaagcatcacgagcacctggcccaggtcttcgaactcaaacagcttcgcgaactgcttcattggtattcctcggtttggtttcccagatgcccctcggaggaagggcatcgaggaaatcggtattgctcccgcgttcgcctactgggcttctacaacccgcgggtgttgctgtcctcaccactgccgatagcagctcggactcgatgtgtttggccttgggcttccctcgctgcgccttcaatcggcttacggagcaggtcatggggactaggggtgatctcgagggttcgctgcagcccggcggcctggtgaagtgggcagctgatcgcgaggcgccgacccgtgtcgtcggctgggcttagtgcttcatgggatggttcctcctctggtgatggggtggagaactctccggtatggagcaggtcgatccctcttcggggcctggaaccgacttccctcggtccgtggtatccggcgagcctccggcttgttgccgcgttgttctgcggcgttgaggtgagtatgagactgctcatatttactgtcaatgagtattcccatatttttttatgaggtgactcatcggaggtttctcaggacgaaaaaaagcccgcgctaagcgggctcgttgggttgctggaggggcttaggaaccgattccgccgccacgccagataacgcggccgatgatcggtagatcatgaactgacgtttcgcttgcgatttcgtctgggtatgcggttttgtcagggttgtcgcttcgaatgagccaagcaccagttagctgttgattcaggcgcttgatgctgacgccgccgtctggtcgcctgatgacgtacacctgcttatcctggggctctatcttggccacgtcgaagagaaccacatcgccttcgaatatgtagggctccatgctgtcgccctctgcgtagatcacgaagaggttctctggtttggagttgacccgcttcagccaatctcgcttgaacaccaaaccttcagtggtctcaacgtgatcattgaaatatccatcgccgcactcgccgcgagcagtgtattggggaatcagggcgtagtccttttcgctcggggctcctggtggaacctcttcattgttgttcatgtttccacgcccggcggctagccatagtgcgcttacgccacaagcggcagccaactgagcaatatatgccgacccctgcgacttcccctgctcaaggttggaaattgaggtttggtccaggccgactcgttgagctaattgagcctgggtgagtttggcgtgcttgcgcgcggccttgatgcggtctttgagttccatccgaaaagtatcaggggcgttcccatatccttgcaaatgagtattcccctgggataccttatgagtattcccataaggagggatgctatgaccaccatctacaaagagctcgtcgcccattttgggactcaagacgagaccgccgcgaagctcggcgttgaccaaagcactgtgtctggatgggtccggggaaagcacgggatgtctcctgttgttgcgaagcgggctcaggttctgaccgacgggaaattcaagaaagaggacctgtgtccggctttcccgtgggaagtgctgtcggcggttgcctgacatgacagccagccaattaaacgccgagcaggaagcaagggcccgcacgttcttaggcgtctccttgcatggggatgatccgactgcaatagcccgcacgttccagacttggagcgcgatgctcgagcgctgctacatccctggatccatgagtggaaagcactaccttgggcgcggaataggcgtctgtgagcgctggttcgtcttctccaacttcgtgagagacatggggcttcgcccgaaggggacgactctcgaccgagtcgacaatgatggcgattacctcccagaaaactgccgctgggcaacccgccagcagcaggcgagaaacacccgtagaaacaaaatggttggcgatgtacttcaagtcgacgccgccattgcatcaggtgttctggcgtcgaccatctcccgtcgcatggcttctggctactcagcagaagaagccattgataactcaaagatcaccaaagtgaagctcactgcagagatggcgagagcgatcaaggatcgcctgaaaaccggtgatacccagtccaagattgctgcctgcttcggtgtctctcgccagatgatctccggaatagcctccggtcgatattggaggtctgcatgaacagcatggaaacccgcgctagaaaaaattacagcctcatcgtgcagcgacttgcatcggttggaaatgcgccggttgcgcatgcagtcggttgcgacgagtcgacgatcagccggatgaagccggagaagttcttggagttcgcccggatcttggctgtgctggacctgaaggtcgtaggcaacgagatgaagtgcttcaacgagaaggagatcgccgcgatcttgcacctggcgaagtcgaagctttccgaggtcgagagcgtcgagcagttggagtgggactgatgcgaaagcgcctcacgaataccgactacgccgcaatggctaacgctgctgaagagctggcgggtatgggttcgagtgagtggaggcgcagatacaacaaagccctgcgcgactactacagggctttgtcggtgcccc

SEQ ID NO: 12 - DNA, 36415 bp, synthetic construct
  source 1..36415: mol_type = other DNA
tgtggggaggtgactgttttgacacatgccaaaagagggagggataggccagagcccctatagcactagggctccagccggacagacgctgtgggacagtttggaaaaaatcgatcaggattgagcaaggaatgcaaaatattgatcgttaattggcgcggaatgagcgctaaaccatccatcgcccaagccagacaacgcgcccaatgatatccaagtcagaaagctggtccttggggacgaccatgtccttatacgccttgttttcgctgatgatcgcgatagagccatcgaactgccgttgtaagcgcttggcgtagagctgatccccgacccgaatcacatagatcgcttcatcccgcacggttctaaggtcatggtcgataacaacggcgtcgccatccgacaggaggggttccatggagtcgcccccgacccttactgccgacatcctggttggctctaaccccttcttgctcaagctgtagcgcgtaaaggcaagctgcgtaagaacgtgtgcgccttcgctccagcttccatgtcccgcgctgaccctcgcgtcatacagggggacgtagacatattggtccgatcccgtagcctcctgctcttccggcttctgactgccctcgccggtcataagccagcccaggctcacgcctgccgccttggccaaggaaatgagcactctccgggtgggttccccgcctttcaagtacctctgcaacccgccttgggagattccagcattcctcgctaaagcacttgcgctccctgctatagcgacaatggagcgcagcctttcgatgaaggcagcgtcattttcaggttcggttgcggaacttgaaaggctggcggtgcgctcgctacgcgttttcatgtagacctaactatttgatttaattgatattaattctatagaggtcgaaatctacctcctatagaacttgaaaaccgctatagagcttgtttttcaacttctatagcgctatgtttatgccctaagtcacgttagacacccctaaaaaaaaccaccctgccaggtggtgagatggaacgtaggcatgaacagaacccgaaatcccccgcgacaacaacgtcccgctgggagtggatcaaatacccagctccgcgccagggggtcgtccctggccgaggtggcccgctccctcgacgtatccagcccggcagtcaaaaacgccaagctgaatccctacccctcgggtagagcgcgccatcgctgctgtactcgacctcagccccctagtgctgtggcctgagcgctggctcgacgacgagaatccgaagcggcaacggcccaatcgctcggagaccttgcaggcatatgtcagacatatgccaagtgctgaggaaaataccagatacgctgaccaagcgcagcgtaaagccgacgcgggggcttgaacatggcccgccgcaaagacgaccgcaccctggacatcttcgatgttccgcagccagcccgcgctatacccggcgagtgcaactatgccgcccaggtcagcgagctggtcagcgaaattctgaaggccgccaacctcgaccgttacgaggtcgccgcccgcatgtcgcgcctatctggcgatgacgtgagcaagaacatgctcgacgcctggtcgagtcccgcccgagctgatcacaacttgcctttctaccgcgccgccctcctggaggacgtctgcgcgagccacctgctgaccaactggctggtcgatgtgcggggcggccgcgtggcctatggccgagacgcactgctcgccgagctgggccgcctggagcggacccgcgaggaagcgggtcggcaggcgcgtgagctgaaacgaatcctgggggagccgtgatgacaaacaccgacctcaaaccgctgctcgacaacctgcggaacgccaccgagttctggaacctagtcaaagaggccagcgctacggacgaaagcaccgttcacaaccgctccttttcggatgctcgcgagtggctcgaatcggcggccttggccctcggtgacgccctgatcgcccagcgcaaagctgtcgggggcgaccatgaatgaatggttctccgcacagaaactggtcggcctgcccggactgcctggcacggttcaaggcatcaatagtcgcgccatccgcgactcatggcagcaaagaaaacacatgggtagaggcggtgggcgtgagtaccacatttccagcctacccgacgaaacccgcgccgcactgctgaacgccgccctgggcgaggtggccaccaaggtggtccgccaggagacgcagctggccctggtcgaaaccaaccgccagcagctggtcgccgatgctcggcagggggtgctgcacgccctggacctgatgatggcccgcaccggctacagccggaagcgctccatcaccctgatgctggacatggcgcgcctcggccaggtcgagccgcagctgctcgcgatgctcaagatggcccgcgatcctcgcggccgcccgagcgcggatggcctgccgagcgtgcgcagcctggagcgtttcctggaccaggccgagcgcggcgccctggtgccgaaggtccgccgcccggacatgagcgttcccgactgggcgccggccttcatgacgatctaccaggggccggagaagcgcagcgcccgcgctgcccatgcactgctggagaagcactggcaggggcaaatgcccagcctggaccaggtttatgcgttcctgcgtaaggtcggcaacgtcagtcgcgaggtcgggcgcatgggtgagcatgaaataaaggcgctgcgcccgttcattcgccgcgacttcaccaagttgctgccgaccgacgtctattcctgcgacggccacacgttcgacgccgaggtccagcacccgatgcacggccggcctttccggccggaaatcaccaccatcattgacatccgtacccgccgcattccgggatggtccaccggcctggccgagtcggccctggtggtggtcgatgccctgcgcgacgcctgcaccaagggcggcatcccggccatcttctacgttgacaacggctcgggctacgtcaaccacatgatgcgcgacgaggcggtcggccttatgggccgcctgggcatcgatatgaagaacagcctgccctacaacagccaggcgcggggcgtgattgagcgcgtccaccagagcctgtggattcgggccgccaaggaactgcccggctacatcggcgccgacatggaccgccaggccaagctggccaccttcaagctgacgcgccgggccatcgccaagggcggcaccatgccgctgatgtcttgggaatcttttgtcgcgttctgcgaacagcagattgccgaatacaacgaccggccgcacagcagcttgccgcgcatcgttgacccgaacaccggccgccgccggcacatgacccccaacgaggcctgggcgctgcacgaagcggagggtttcagcccgatgcgcgtcaccgacgacgaggcccggccgctgttccggccccaggtgctgcgcaccgtccgccgctgcgaactggagttcatcggcaaccgctacttcgcccgcgagctggaggaattccacggcgaccaggtggccgtgggctacgacatccacgacgccagcagggtgtgggtctacgacggcgagggccgcttcctctgcaccgcagagctgaacggcaacagccgcgactacatgccggcttcgtatgtcgagcgtgcccgcgagaaacgcgcagaggcccgcgagaagcgcgccctggctcacctcgacgagattcgcgccgagcgtgacggcgggtatgccctggaaatggatgcgccgctgtccatccccggcctcggcacgatcacccctgagcaactccggtcgcgcagcgccgcgaccctcgaaatgcaggccgagcggatcgacgaaccgcgcccggccgcagccaccgcccaagccaccaccgcccaggtcttcaccctgccgaccgctcccgcccagcgctaccggcagtggtgcgagctggccgagcggcaacgctccgggctgcccatcgagccggacgccgcccagtggttcgaggtttaccccaaatccaaagaattcgccgcccagcagcggcaagcatgaaaggagctgtattcatgaccaccccgaaaaccacccaactggccaatggcatggccgacatcgccaacatcgccctttgcgatatcgccctggagaaagcgctgtcgcgtacctccacgttgcccggcctggtctgcttctacggcccgtccggcttcggcaaatccgtttcggccgcctgggtcgccaatcgccgccgcgcctactacgtccaggccaaaagcgtctggacccgcaagcacacgctgaagtcgatcctgggtgaaatgggcatcaagccggctggcacgatcccggaaatggccgaccagatcgccgaggaactggccgccagcggccgcccgctgatcatcgacgaaatggaccacctggtcgccgctggccaggtcgagctgattcgtgatctgtacgagtccagccaagcctccatcttgctgatcggcgaggaaatgctgccgaccaagctgaagaagttcgaacgcttccatggccgcgtgctgagctgggttccggcccagccagtctccctggaggacgcccgcaacctggcgccggtctacagccccggagtggctatcgctgacgacctgctcgcgcacttggtgaagaagtcactgggctctgtccgtcgcgtcgcggtgaacctggagcagttggccgaggccgccaccgttcagggccggcgcgagctggaactggccgacctccagcgcctgaacctggagctgtataccggcgcggccccgaacccgaggacgtcgaaatgagcctcggcaaaaacccggctcacctgtccatggtcgggggcaagagcccccgccagcagatgtgggaagtcatccgggccaaccgcgaagagttcaccgtctaccgcgtggcgcgccgctccaaccagcacgacaagaccgtcgagaagtatgtcgcctgcctgcgcctgggcggctacgtcgaggcgatccgtggattcaagcgcggcgaagaggtcgttttccagctggtccgcgacaacggcgtcgaggcaccgaacctgaacgccgatggcaagccatcccagcagggctacaccaccgaggcggtctggcggacgttgcgcatcctcggtccagcgaccccggagcagatcgccgcatcggtggcggcctctggcgcgactgtgtcgcccagcaccgttcagcgctacttcatcgatctgcagaacgccggatacctgacccgcaacggccgccactacgccctcaagccgggccgctacaccggtccacggccgcccatcgtccagcgcgagacgcgccgccaggtctacgacccgaaccttgaccaggtcatgtggagttcgcacggcgagtaccagcacaaccggagtcgttcgcggggcgcttcccaggctggcgtggcggataccgaagagaacaacgaatcaggcggctgaagccgtgatgaagacggtgccgaggggtggcctcccctcgacacctaccaccacccggaaggagaggagccatgcaaatgcatgcacagcaaggcggtagcgccgcgaaggctagcacaagccactttcgcggcactacgaacattgaggagtacatccgcgacatggcgagccgtgggttcagtcgtcgggccgtgagtaaggccctgggtatgcagtcgcggaagttcaaggaactcctggaactcctgccagaaatggactgggtgcctccttgtcagtcgtgggaccgcctgcgcgctgaccaggagaagaagggacgcaagtgtccgatgacagaggggcgtctgcgctcgattgtcgcggcgaggcgcgccgcgatggcaaaacacacccgctacaccgcgtttggtgtaacagccaccttgccggagctggtgagccagttcggccaggtcaccgccgccaccgtgcgcatgcggttggccaagggaatgcctctggagcaggcccttgcctccgtgcgcagcgatccttgtggaaggaaggtcgcagatagccatccctggaaacaggaggcgcaccagggggctatcaatcaccttgagcgtcaaaccgctgcaatgcaggaacgcgttcagggggagcgcctggaccgggcggcctcactgctgagccaggaggtgccgccatgcgccgaacactgatccccatcggcatcttcctggccctcggcctactgctgatcctggccggtgatgccctgatgctcggccgccgcctcattgcctggcagtgggggtgctgatggaacgcgcaatcgatctgtcggcctggggcgagcgtccgcccgtcttcgtccaactgctggccgccgaggtggcccgcagcagccagacgaaagccggcgaggcaatcggcatgagccgttcgaccgtcagcaccatcctcgccaaccgctacccgtcgccctcgacgatccgcgtcgagcgccgcgtcctggccgcgctgagccgtattgagtgcccggccttgggcgaggcggtgacctcggtcgagtgcagcgagtacctccagcggccggcgccgctgaacaaccccgtcgcgatgcgctgctggaaagcgtgccgcgcctgtccacgcaacccgcataccgcccccatgaaacgagaggaacaaggccatgagaaccgcattgcccttgaaagtcttgacgcctgacttggcccagagcctgcgcaccttcaacgacgccgcccggctgctccagcgcatgggggtccgccttcatcgcctggagccgacagaggggcgcgtgaccatcgccgcagatgacgcccgccagctcctggagaaaggctacctgatgggcttccagcgcgacgcctcggccggcagcacccgttacatcacccgcttccagggcatcaccctggcctggagcgaaccgatcagctaccgcgacttcgccggcagcaaatccgtaattcactgaacaggagaacgccaacatggcaccgaagaaacgtctgaaatccgctgccgccgtctacgtcccgcagacccgcgaacaggtcatcagcgatatcaagaacatcggcgacctccagcgcgagctggcccgtctggaaaccgcaatgaacgatgaaatcggccagatcaccgagcgctattcggagccggccgaagacctgaagaagcgcctggcggtcctccagggcggagtccagtcctggtgcgaggccaaccgtgccgagctgaccgacaacaacaaggtcaagtacgcgaacctcacaaccggcgaggtccagtggcgcatccgtcccccgtccgtgactgtgcgcggcgccgatgcggtcctggagctactgcgcagcaaggggctaatccgcttcatccgcaccaaggaagaggtgaacaaggaagcgatcctcaacgaacccgaggccgtccaggggctgccggggctgaccctgaacaccggcatcgaggacttcgccatcgtgcctttcgaagcggaggtgcagtgacatggccgacaccatcgctttctgctgggcctctggcctgatccagttcggtgaccaggtgcccgagggcgccatcgagatcgcccgtggggacgaccaggtcgttcgcgaaaacctcgtgaccaattcgcggcacgcttacgacaacgtgtcgctcctggttccgggcgtacccgaagcggcaaaccaaaccgagggcggggacgcactggagtgcttcatccgtcttctcgccaagtacgacagcgccgctttccaggtcgcttatgtggaggacgtgtgacatggcacgcaaccgcgcgcaacagctgtgcatcgcaccttggactatcagcgcttcctgttaccccaggctgatgcactcaagctgatagacatcatgagtcgagccgcagaggttcaggccgactacgcctctggagctggattcaagtacaccgtcggcgaagtgccggaagtcgagttgacgatagtacgccccagtcaattggtcatgccgcaggccgagccggccccagctacaccacgcgctcgccggaagtctccggcccaggtcacgcacgatgccattcggctgttggaggggctctgatcatgaccaagacgttcgccatgtgccgcatcgacggcctgatcgagctgcgggaggaacacccaggcgagggctacttcgcccttgccgtgggcgacttggccagcgtgcgggcggcggtctttgcaaccgctgagccgcaccaggtcggcaagaaagtcgcccggcgcgtgccgggtgtgagccccgacgccaccgaccgcgaaaacctgggctccatcgcccggtacatccagaccctgggccagcaggatcggcccggcttccgtgcgctgggggtgtgaaatgcagcagtccaaccccttcaatcaccccggacagagctacggcgccgtagacgtcgatagccgactccgcgccgttgccggcttcgacctggagcaatgccgcgccgcgctcgcggtcaccggcctccagaagatcgtcgagcagaaaattcgcacccgcatccgccagctggaaaagcaggcatccgcacagaaggaggcatagccatggccgtatacaccatcaccctaagcgacaccgaaggcggaatagatttctccatgcaaggcccgccgctgcacgactccgaagcatcgaagatcgcctacgcccttatgcaatcgaccatgtccctcggccgagaactcgcaaagcagaacggagttggtaacgccgtttcctgcgcctgcgacgagtgcctggcacggcgcgctcgcggtgaggaaccgcagcaggaaatccactacaccacggccaagaaccgcaccgtccactgagcgaaaccgccccggcctggccgggacggtctgccggacgtggtggtccggtactgatgagcagccacccatgacgaacgaaaccaagacagaccgccagcgccgcctggcgcgggaacgccaacgagcgaagcgcgagcgcgatgccctgcgccgcgctgcgctgggcggtcgccgcttcaacatggacatgtaccagggaacggctgatgcactcgatctgatctgcgcggccggtggcttcgccgagccggccgaggcggtcaccttgctcctacacaacgttgccgaaattgcagaacgtgacgcgtcacgctttgccgaattgatccaaaagagaagccatccagggaggaccaagcgatgagcctacgcgccgtcaacctcgcaaaaatccacatcgccaaggcccagctgggcatggacgatgacacctatcgcgcattgctcgctcgcgtcgcgggcgtgcgctcggccaaggacttagggccgcgccagattgaccaggtactggtcgaactccagcgtctgggctggaaaccgaagagcaaccggcaaggccgggcgacgccaaaagtgccgcaaaaccggcaaaccgtgctgcgcaaaatcaccgcgctcctggccagcgcccatcgcccctggagctacgccgaccatatggcccggcgcatgttccaggtcgagcgggtcgagtggctggacgacagccagctctaccggctgatgcaggcgcttatcatcgacaggagccgccatggccaggtctgaggtggatcttcgggaggtccaggacatgctgccggataccgtccgcgacatggccggacgcatcggcctgccggccacgctggtggtagtcgagcagctcggcggcacgtcctggcggatagccgagggccgggcgcggaggggcgaagcgcgccgggctgcgctggccgagctggtgggcagcgacatcgaggagcagctccacacgcactatcggggcgaagaaatttacgtggctcgctgccacaaggcgctggtacggtggcgcgatctggagatcgtcgagcgcttcgaacagggcttgcgtgacgggcaaaccgcccgtagcctgctcagcgatctagcccgccaatacaacttgtccgaccgctggatatgggagattgtcaaccggccgagcgagccggcaccgcagcaatccaccctgttccactaagccggggcgcaacgccccggccggcgtctccgcgccgaccctgtctcagccgttgaaccccttccgctaatcccgcgtcgcactcaccgccacgatggcggcatgagcacatctagccccccaacgtctctacgcagcccccgcgactacgccgccgccatcctggccgagcccagccgcgagcgtcgtaacgctctgctggaagcctgcccggtcaactggcagccacttgttcgggcgcacgtcgaggacgccttcgcgaaggtcaaggcgtatcgccagatgatggaccaccgcgccgagtcgatccggcgcggcccgcctccagctccccgcgtcaccgacaccgatttccgcatatccaactacaccaaatccgccccggaggtaggcaatgcgcacctatcagcaattcgggcagcgctcgcaacggaagcaccaaatgcctgatcccgcatccacctcggccggcagcgccgcgctgctgaaaatgtttggcatccatatcagcgcgggcgccctggccgccgccctgggcttcctggtcctgtggcccaggaccatgaaagaggggtttgcccggctgttctgcaccatcgtcgcgtccagcgtcttcggcccgatcctggtcgtttacctgcactccaaccgccccgagctgttcgagtccgcccaggtggtggccgggctctaccagttagagccggcagtcggcctgctgttcgtttccgctccgctcctggtgattgccggtctgcccgcctggtggctgatcggggcggccctgcgcctgtttgagcgggacggcgattcatggctgggcgcgttcgcccagtgggtaaaacgcaaactggagaacacctgatggcccttcaacctcgcggcatccgcaacaacaaccccggcaacatcgtctggtcggcacgcaacaactggcagggccagctcccgcacaacccgaaggtcgagccgcgtttcgcccgtttcgataccgcacataacggaatccgcgccttggcaaagctgctgctgaactatcgcaaggtccacggcctgcgcaccgtcgaatcgttgatcgcacgctgggcgccgtccaacgagaacgacacccgcgcatatgccacggccgtggcccgagccatgggggttccaccgcaggccggcctgcacatggaccaggacaccctggccgccctggtgaccgcgatcattcggcacgaaaacgggcagcagccctacagcgccgagcagatcgcccaggccgtgcgggaggtgctgtgatgcaacgcctgcggttggcagcaactaaaggccgcactctggttggcgtgatcctgatcgagaccggcctagccctggtgcgggctggtaccgggctgctgccgaggtcttccgaatgacctggcgcctcggcttggccctggccctgttcctggtgatggttgcgaccagcgcctggtggagtggtcgcgtggcgggcctggccgatgggcgcgccgcctgcgccgacgcacagacccgcgcctaccgcgacgtcctggagcaatcggcggcacaactgaaggcggtccaggacaccagcgcggctcttttccagcgcctggcccagcgggccgacagcgaccaacaaactactcgggagcttcgccatgccctggccgaaaccgctgctgatcgcgctgcctgccgctttcctgctggcgtcatgcagcagctcgaaaccgcccgtcaacgtgccgcccaggccactaccggcggccttggctcaaccgtgcccgaccccggtggcggtgactgatgacagccccgatgccaccgcaattgccctcaaacaactctacgaccaatacggcctctgcgccggactgcactgggacaccgtgcggcaccttcaaaaggactgatccgatgaccgaaaagaaagcctctcccgagttcgaactgctgcaacgcatcgacggccgcctggagcgcttcgaggaccgattcccgcagatcgagcgtaaggccgtgctgtacggctcggcggccggcgcgctggcgggtggcctggttgcctgcggcctgctcgcggcgcgtatcaagctcggtatctgaggtagtcatggcgcacccgaaggaaacccgcgacgccctgcgccgcgcctacgtcctcgaccgccagtccctggaggtcgcggccgccatgttcggcgtctcctacggcaccgcccgccgctggaaacagcaggcggaagccgagggggacgactgggacaaggcgcaatcggcgcagttgctggccggtggtgggctggaggacgtggcgcgccaggtgctggccggcctggtgacccagttccaggccacgatggaagccatccaggtagacgcggacatcaagcccgccgtgaaagtgcagctgctcgccagcctggccgatgcctacaacaagacggtcagcgcgtccaagcgcgttctgcccgaaacatcagcgctggccaccgctatggaggtgctccagcgcctggccagcttcatccgtgagcggttcccgcagcacgcccaggcattcgccgaggtgctggagccgtttggagaggtgattgcgaaggagctgggctgaccaacctattcgctgaaggggtcgtaccgactgacaaccacgggtccgctatcaggaatcttttcgacatgaacaacagaattgcaggggtgacatttcaaggccttgtaccagccatcattgcaaggctgaagaatggtcttgattcctttttggtagcaatcggcacatatgtgatgcagaggttcggtgccttgaacctctggctttatgcgatacacaagtccacccgcttccgtctggtggagctggtagcgctctttctcctgttcccagcgtttgaactgagcaatttcggcttccagctcgcctatgcggcgggtcagcgtcgtctgatccgcatgggcgctgttcagctgggattgcagcccgagcagcacgccgttcagttcgaccaccttggtcgttacagccgcatccgtcttgagcgtgagcatgctctgcgtaatgtcagtggccgccttgatgccgccgtaggcaccagcaatccagtccatcatgaccaggttccttctggggagaaatcgacccatgaagggtagcaccagagacttcctggcggatattgcccagctcgcgggggagttccgccgccagatcgaggccgaggtcgcaggcttcgaccccgacccgaaggccagcgccgtccggcgtgaacgggccagcgcggactatgagtatttcgcccggacctacttcccgcactacgtgaagcgcggtaacgcgctgctccacgactacctctacaagcggttgcccgagctggtggaccacccggacggccagcacgaagccattgcggcgccgcgtggtaatgccaagtccaccctggtgagccagatattcgtgatctggtgcgtactcaccggccgcaagcattaccccctgatcatcatggatgccttcgaacaggccgccacgatgctggaggcgatcaaggcggagctggagttcaacccgcgcctggccatggacttcccccagggcgccggcaagggccgcgtttggcaggtcggcaccatcgttacggcgaacgatgccaaggtccaggtcttcggctccggcaagcggatgcgcggccttcgacacggcccgcaccgtcctgacctggtgatcggcgacgacctggagaacgacgagaacgtccgcagcccggagcagcgcgacaagctggaaaactggctgaagaaaaccgttctgtccctcggctcggccgacgacaccatggacgtgatcatcatcgggaccatccttcactacgactcggtcctgtcgcgcctgctgaaaaacccgctgtggaagcggcgcaagttcaaggcgatcatcgaatggccgcaccgcatggacctgtgggagaagtgggaggaacttctgctcaactccgacgacgagggcgccgccgctctggccttctaccaggaacgcgccgccgccatggaggacggcgcgatcatctgctggccggatgggcagcccctctacaagcttatggtgaaacgtgcccgcgatgggcactcggcgttcgactcggaacagcagaacgacccagtccagggcgagaacgcccccttcgccgcctgcatcacgttctgggtcaaccgcctggcgcagtggatgttctacggcgcgtgcgacccgtccctgggtaagcaaggttccagccgcgaccccagcgccatcctggtgggtgggttcaaccgggagacaggcgtcctggacgtggtcgaggccgccatccgcaaacgcctgccggacaagatcatcgaggacatcatcgccatgcagcgggcctatcactgcctggtgtggggcgttgaggcggtccagttccaggagttcctgcgcaccgagctggtgaagcgctccgccaaggctggctgcccagtacctgcccgagcgatcacgccacacgccgacaagctactgcgcatcgaaagcctccagccgcacatggccaacggcctgatccgtctgcatccaagccagaccgtcctggaacaacagctgcgccacttcccggccgcagaccacgacgatggccccgacgccctacacatgctctggatgctggccacgacggggttcgcgccgatagaggcgactttggtcaaacgccggcatgaatacgcgcccggccttgacgattcttttgacactggcggccgcttcggcggcgcatggtaggtacaacacatggcacaaatcgttgacgtctacggcaacccgatccgaactcagcagttgcgcgagccgcagacctcgcgcctggccggcctggcgaaggagttcgcccagcacccggccaaggggctgacgccggccaagctggctcgcatcctggtcgaggccgaacagggcaacctccaagcccaagccgaactgttcatggacatggaggaacgcgacgcccacctgttcgccgaaatgagcaagcgaaagcgcgcaatccttggcctggattgggcggtcgagcccccgcgtaacgcctcggcggccgagaaagccgatgccgactacctgcacgagctgttgctcgacctggaagggctggaggacttgctgctcgatgcgctggacggcatcggccacggctacagctgcatcgagctggagtgggcgttacaagggcgcgagtggatgccgctggcgttccaccaccgaccgcagagctggttccagctcaaccccgaagaccagaacgagctgcggctgcgcgacaacagcccggccggcgaagccttgcagcccttcggctggatcattcaccggccgcgtgcgcgctccggctatgtggcccgcagcggcctgttccgcgtgctggcctggccgtacctgttccgccactacgccacctccgacctggcggaaatgctggaaatctatggcctgccgatccggctggggaaatatccgccaggtactgccgacgaggagaaggcaaccttgctgcgggccgttaccggcctgggacatgctgccgcagggatcatccccgaaaccatggccatcgacttccagcaggccgcgcagggtagcagcgagccgttcctggcgatgatgcggcaaagcgaagacgccatatccaaggcggtcctgggcggcaccctgaccagcaccaccagccagtcaggcggcggcgcttttgctttgggccaggtgcataacgaggttcggcacgacttgctggcatccgatgcccgccagttggcggcaacgttgtcccgcgatctgctctggccgctcctggtgctgaatcgccctggtagtcccgacgtgcgccgggcgccgcgcctagtcttcgacctgcgcgagcaagccgacatcaccagcatggcgcagtcgattccggcactggtcaacgtggggctggagattcccagcgcctgggtctatgacaagctcggcatcccgcagcctgccaagaatgagccagttctgcgttcggctgcgcagcctgcgatcctgagccgacagcatggacaacgggtggcggccttggccaccatcgttggcccacgctatggcgatcagcaggcgctggacaaggcgctggctgacctgccggcgaaggacatgcaaaaccaggccaacgacctgctcgccccgctcctggaagcggtcaaccgcggagacagcgaaaccgaactactcggcgccctcgccgaagcgttcccggacatggatgacagcgccctgacggacgcgctccaccggctgctgttcgccgccgatacctggggccgtctccacggcaacctggaccggatcgactgatggccgctccgaccgaagccgatctgcgggccatcttcgccctgcggccggccgccgctatcgagtatctggagcgcaagggcttcgcgatcacttggaactggcatgacgttgacgcggccacccacgcccgcgctctgaccgttgccagagcagcacgcctggacgtgctccaggacattcgcgacgccctggtcgagaacctggagcgcggcgagacgctacgagatttcaagcgcaacctgcggccgaccctggaggcgaagggctggtggggtcgccaggtggtagtcgcgccggatggcggcgccgaggtcgcacaactgggcagcccgcgccgcctggataccatctaccagaccaacatgcaggcggcctacatggcagggcgctacgcggccgcctacgaagccagggaaacccacccttactggatgtatgtggcggtgatggatggcgttacccggcccagccatgccgccctgcatgggaaagtgttcaggtgggacgatccgatctggcagcacatcaccccgcccaatggctacaactgccggtgccggatcgttgccttgacggaggccgctgtccgccgtcgcggcctgaccgtcgaatccagtcagggcaagaccggccaggtcaccgtcgaaaccggcgtggaccggcgcacaggggagattcgcgaacagaccctgaccaccctggagacgaccgaccgggccgggcggaagatccaatttcgccccgatgccgggttcgacggcagccccgtacagagtcacctgatggaccaggtgctgtacgacaaggccgagcgcaccctgggagccccagccgcaatcgacgaggtgcggggtgtgctgctggacccggtccgccagcgcgcctgggcggccttcgtagatcgcgccgcgtccccccaggggcagaccatgtccatcggcgtgctcgatccgaccgatatcacctacgccctagcccagggcgcccagttgcgggccggcgtggtcgccaccagcgataccgcaattcgcaacagtgctgtcgctcgcgagcagctcgccagcctgccgcagcgcttcgcccagcctgacctggtgctgtgggagcgcggcagcgagtcgttggtcttcatcgtccaggccgatagcgcggccctggctatccgtctgcgcggcgagatatacgggcccggccaactggaaaatgtcggccaggttatggaaatcaccatggatagcatccaggatggcctggcgacgggccgctacaggagagtgcgctagtgacaactaggatcgacgtcgagctggacgaccaggaggttcgccagcgcctggcgctgctgatgcgctcggtgaccgatacgctgccggtcatgcgtggcatcgctgccgagctgctcgcggaaactgagttcgcctttatggacgaggggccgggctggccgcagctcagccccgtgactgtcgccgctcgcgaggctaaggggcgtggtccacacccgatcctccaggtcacaaacgccctggctcgctcggtcacgacctgggcggatcgcaacgaggcgggaatcgggtccaacttggtctatgcggccatccaccaatttggtggcgacgccggccggggtcaccaggtcgaaattcctgcacggcggtatctgcctttcgacgaaaacggccaactggcggccggcgctcggcagtcaattctggagatcgtcctaacagccttgagccgaaatcggtagtggccactttcggacaagcggcacattgtgcctattgcgaattaggcacaatgtgcctaatctaacgtcatgccagccacaacggcgaggcgccaagaaggatagaagccatgaaaatcaccaacgacaccaccacctacgaagtggccgaactgatgggttcggaggctgacgaactcgatggacgtatcatgatggggctgctcagccgcgaatgcgtggtagacactgacgacctgagcgaggatcaatggctggctctgatcgacgagtcgcagaaggttcgccgcgagcagttcgaaagcgatgaagcctgacgcctctaaccacaacccagacccgcgctacctgcgcgggctgctcaagaaagccggcatcagccagcggcgcgcagccgagctgctcggcctcagtgacagggtgatgcgctattacctgagcgaggacatcaaggagggctaccgccccgcgccgtataccgtccagttcgccctggagtgcctggcgaacgacccgccatctgcgtgatcacctgatccgcccgcaaacgcgctacacgcgccgaaacggggttagacgctacctcgctcagagtcggtgcgttaaccccgttagagccccgttagaaatcgctccagcgccattcttgtgccagggtttggccagaagatggcgccggacggtttccgcagtcgttgaaccccttcatgtgaccgctgctttctaccgtcgccaccattggcggcatggaaaagaaccgcctactcgttgccatcgccgcctgctcgttccagcttccccagctggaggatggcagcgcctggattcaagtcactccagctggtgagttccggcccacggacgggcgccccatggacgtgccggcctggcggatcgatgccgccagcgccgccgccgtgatcgaccgggccagggcacgcaagacaccgcctgtcctggactatgagcaccagaccctcaagaaagaggaaaacggccagccggcgcctgctgccggccgcttcctcgatttcgaatggcgcgaaggctccggcctgtggggccgtgtcgaatacaccgcccgcgccgcacggatgatcgaggacggtgagtacctctacttctcgccggtcttcagctacgccccggacggcacggtcctgtcgattctgatgggcgccatcaccaacgaccccgccatcgatggcatggagccgctcgcccgccgagcggcggccacctttggcctttaccccacccaagaggaaacctccgtggatgaactcctgaaagccatcatcgaggcgctgtcgctcaaggaaggggcgaccgaggccgaagccatcgccgccctgaccgcgctcaagccggccttggacgcacaggcggccagcctggccacgctgcgcgaaaccctcggcttggccaaggacgctagcgtcgagcagatcgccgccgccaccagccaactgaagaaggccgacccgagccagaaacccgacccggccaagttcgtgcccttggaagctgtgacggacctccaggagcaaatcgccgctctgaccgcacgcctcaatggtggcgagctggacaggctggtcggtgctgcgctccaggacggtcgcctgctgccctccctggagcagtgggcacgcgacctgggcggtaaggacatcggccagctcaaggcgtacctggacaaggccgcgccgattgccgcgctgacccgcctgcaaggccgccagccggagggcgacacccacaacctcaccgacgccgagatggaggccgcccgtctgaccgggatcagccccgccgactacgccaaggcaaaaggagcctgacccatggccatcattactccggcgctgattagcgcactgaaaacctcgttccagaagcatttccaggacgccctggcgacggcacccagcacctacctccaggttgccacggtgattccgtccaccaccgccagcaacacctatggctggctggggcagttccccaagctgcgcgagtggatcggtcagcgtgtcatcaaggacatggcggcccagggctaccagatcaccaacaagctcttcgaatcgaccgtgggcgtaaaacgtaccgacatcgaggacgacaacctcggcgtctacggaccgctcatgcaggaaatggggcgcgctgccggcgcgcatcccgacgagctggtcttcgccctgctcaaggccggcaacgccaatctctgctacgacggtcaaaacttcttcgacaccgatcacccggtctatccgaacgtggatggcaccggcacggcgaccaccgttagcaacctgttcgcgccggccgctgatccgggggcggcctggtatctgctcgacaccagccgcagcctcaagccgttgatctaccaggagcgcatgaagccgtcgttcacttcgatgaccaaggaagacgacgagcaggtcttcatggccgacgagtaccgctacggcgtgcgctcccgctgcaatgtcggcttcggtttctggcaactggcagcgatgtccaccgaagagctgaacacggcgaacttcgagaaagtttacgacgccatgcgcaaccagaaggccgacggcggccgtccgctggacattcgcccgaacctgctggtggtgccgaccactctgcgctccaaggccaaggaagtggtcggggtgcaacgtctggccaatggcgcggacaaccccaacttcgaactggtccaggtactcgataccgcctggctcaactgatagccccagacggaacgcctgccaggccaaggatggccaccttcttccagctacaggagacacgacatggcacgccagaactctgcggccaagaccaccgccaaatccaagaccgatccggcgaccgaaaagcccaaggacgaagctctgccgggctccacggatgccacttcgtccaccgcacccgaggcgcccaccgccaaaccagccagcacctcggacgagatcgagggcgtcttcattcgggccaccgttgagcgccgctgtcgagcgggcttctgcttcgacaaggaaggccaaggcttcgctgaaggcgtgctgagcgacaagcagttggaggctctggagtcggacccgctgctcaaggtcgagcgctgcaccttttccggcaaccaggagggcgagtgatgaatcacgccattgcccagttggacatcgccgcgcagatcgccgagcacaacgctccaatcagcgaggctcagggtgacgccgctcaggccgagttgcagaaccaggttgccgccgactgccgcgaggcgctcgacgtcctggaacaattggagtcgccgctgtgagctactgcacgctggccgacctgatcgagcagtacagcgagcaaaaaatccgcgaggtgagtgaccgcgtcaataaaccggccacaaccatcgacacggtgatcgtggatcgcgccatcgccgacgccgactcagaaatcgacctgcatctgcacggccgataccagttgccgctcgccagcgtgccaacggcgctcaagcgcattgcctgtggcctggcctacgccaatctgcacatcgttctaaaggaagagaacccggtctacaaaacggccgagcatctgcgaaagctgctgtcgggcatcgccaacggcaagttgagtctggccctggatgctgacggcaagccggcgcccgtagccaacacggtgcagataagcgaaggccgcaacgactggggggccgactggtgagcgacccgttcgactacctgttcctggaaccgttgctgatcgagcgtatccgctcagaggttcctgggctggccatcgtttccggggtgcccgatctggcggccttgagtgagcaggaccagcccgcccccagcgtctatgtcgtctatctcggcgacgagataggcaccggagcggatcaccaggggggcaggcgcgccattcaggctatcggccagcaatgggcggttgtgctggtggtgcattacgccgactcgtcgaactccggcgaaggagcgcgccgagaggcaggaccgctgctgggacggctggtcaaggcactgaccggatgggctccagccatcgatgtggctccgttggcgcgcagcgcccgacagtctcccgtcacctacgccagcggctacttctatttccccctggtgttcaccgccaggttcgtctacccgagggtcaagtcatggaaaccgtaaaagtcacgatcactgctgagaaccccaaccacacccacgcgggcaagccggtggccaagggcgacgagatcgaagtcagccgcgccgatgccgagtttctgctgcgccgtcaattgatcaccaagattcccgccgagcccaaggccgacgagaaacgcgacaagtaacgcgcaacatctgattcctacggaggcctcacatggcacaggaaacgtatttctacgggcaaggtgagattgacgccgcgcctatcgtcaacggcgtcctcggcaaatggcgctggattcaggatgtctcggccatgagcatccagctcgcagtcgagaaggtcgagcacaaggaaagctacagcggccagaaagccctggtccgaagcttccccatcggcaagaccgccaccgtcagcatgaccttgcacagcatcgacccggataacctggcgctcaccctctatggcaaggtcgtgactaaggcggccggctctgtgacggctgaggcgctccccgccgacctggtagctggtgatgtaatccgcctggccaatccgggcgtcagcgagctggtcatcaccgacagcgcgagcagtccggcgcccctcgatccgcagtattacgccctgcgagccgatggcgcctacggcgaggtccaactgctgggtctgccgacgccggccccgacccagccgttcaaggcggcctatgagtacgcggcgactcgccaggtgggcatgttcaccgcgccgcagccgaccatcgccctgcgctacaagggcatcaacctggccgaaggcggcgcgccggtcatcgtcgagctgttcaaggtcgcgaccgacccgctccaggaactggcattgatcagcgacggcaacaccgtcgccggtatgcagatcagcggcggaatcctgctggacaccagcaagccggataccggcgacctgggccgcttcggtcgcattatccagctggggtaaatcatggccaggaagaagcctgttaaccctcgcggccagccggccgactcggcgcccgacgacagcctgagcgtgctgtttcctgaccgtcagttggcggtcgggggcgtcgaggtgacggtgcgcgagctgaccttcagcgagcaactgcgccataaccacctgttggccccgctggccgatgccctggcggcagttcccccggagcagctcgacggacctgagtcgatcaacgtcatcttcgacgctctggcccggcacgccgacgcgctgcgcgagttgctcgcgatcagttgcggccaatccgtggactgggtggacgcgctgccggcagacgacggcgaagcactggtgttgacctggtggacggtgaacagtggttttttcgtgcgaaggctctggcggcctcgcctactggcgatggcattgggcaaccgacgccctggagccgagtcttctccgatctcgtccgcgccggccactgccgcgaaaccctaggcacctataccggccggcaactgattctgtactggaacgaagcgcaggcagctgaacggcgagaacaggcgcgccacgttcggtcggtgatgttcggaatggctggtggcaaggacgccagcgccttcctcaacgatttggaatcctgatggccactaatcagcaactctcgatagcactacgcatccaggctgacctggctgaagcgcagaacgcgctcagacaactaacgggcaacctccagcaggttgaccggggggcggtgcagaccaggagcgagctgtctgcgatgggtgggcagttggacagccttcgcgcacaggtgcttgggtttgtcggagcttgggctagcttgagtgcgctgggcggcctggtgaccatggttgaccaatatgggcaaatggccgaccgcatccagatggtcaccagcagcacggccgaatatgaacaagtgcaggcccggctgctggagacggccagccgcacctatcggccgctggcggaagcccaagagttgtacatccgcaccgccgacagcctgaagtcgttgcggtacaccaccgaacaagcgctggacatcaccgattcgttttccttcttgctggtaaccaacgccgcgtcggcggaccgtgcggcgagcgccatcgacgcctactcgaaatcgatccagaccggcaaggtcagctctgacgcctggcagtcgatcatggccgccatgcccagcctggtgaacgccctggcagagtccaccggcaagagcaccgaggaaatccgcaagctaggcatcgagggcagcctgtcgttgcgcgacctgaatgaagggctgcgcaagaccgtggcggcgaaccgcgaggcggcggacaacatgggcacctcggtccaggacgcgctggtcagcctgaacaacgccctgagcgcctacctgggcgagctgaaccgcacctatgacatcaccggtagcgtgtcctcggcgctgaacgtgctggccgagaacatggaggttatcgtcaaactgtttggggtcgcggcggtggcggggctgacccgctacgtggccagcctaacgctggccacccaggcgaaactggcggcagtgctggccgctcgggcgcaagccgctgaagaactgcgggcagcccaggctcaggtcgcttcgacggcagcggcagcggccaatgccagggcacaggcgggcctgacggtgagccatgctcaggcggcggcggccgaggcggcgcataccgccgcgacccagcgccttgctgctgcgcagttggcggccggcaccgcgatgcgcgggatgctggccgtgatcggtggtccggccggcatcgcgatgctggtggccggagcggcggcaagcttcttcctgtttcgcgatagcgcccaggcggtcaagagtagcctagatgacctgagtgagccgctggaccaggtcgtcgagcgcatgggcaagctgagcgagattgagcaagatcgcgaactgacccggctttccgagcagatcgacggattgcggcagacggctgtggaagccgcccgcgaaatgcgagaggtggccagcaccgccctctatggtgccaggctggatcgtatcccgtctgccgaagcacagcaggccctccagcctctaatcgatgcgtcggctgacgctgcgcgaggcgtggaggtggactggaagtcggtgatggactccctggctgccagcggcgctgttcccgattcactcaagcgcaagctgctggacatggcggctggtcaggcagaggcaggccgtactgctaccgagctggggcagcgtcatgcggaactcaaggcacgcctggagggttcgactgccgccatcaatgagaacagcgatgcactgagtaaagggtcggacaaggcagccgagtatatccagtccctgcgcctggccatcgccgacctggaagatccatcggtcctgggcaaggccggccgtcgcctccagcagttcggggccgacctcaatgccgagcagagtgccgaaatactccgcctggagaccctgaaggccaataccgaaaaggcggcccaggcccgcgaggatgcacggcgcaaggctgaatccagtgcgcgacaacaagcctccacggctgagcagttggcgaagagccaggaaggctatgttgcggggctggaaaagcaagcccgcaccctgggtctcaccagcgcagaggtgcgggcctacgagctggccgagaagggtttgaccggagccctccaagctcgggcagcggcagcacttgccgccctcgcggcggacgagaagaagcggcaagccgacgccactgcgcgcaccaacgccggactggaggccgaatatctgcgggcgaccggccgcaccgttgacgcggggctgctggagattcggacgaaatttgacgcgatgcgtcgtgacttcgaaaaggcgggcaacgacgccggcctggcctggatcgacaagctaatccccgtcgccgaggccaaggtccgcctggatgacgtcaagcagcagatggacgatttgctggccgaccagcaacgggccgagtcgtccgttaacgtccagcaggatgccggcatcatcaacgaaatggacgcccggcagcgcatcctggacattcaccgagcgacctacgagaagctccagcagattcggccgatcctagagcagatggcccgccagcctggcgaggtcggccgagccgctgccgaatcgctcgcccaactggacgccgaggcggcgcgactccagcagaccacgacgctgctcgaaaccaccctacgggacggcctcaccagcggctttaccgacgccatcaaagggctcgcttccgggaccatggacttgcgcgacgccatcacgtcgctgggtgaagctgtactcaatgccttggtgaacatggcggcgcagaacctcgcgcagtcgttgtccagcggcatcatggggctgtttggtggcggccagcaggacaccagcatgactaccggcgcggcggctgtgaccgcgtcggccggtgccctatcgactgcgggcgcctcgctgctgaccggggccgctgctatccagacggccgctgcgtcgctggcagccgccaatggcgtccaagggctgggcgctgctgcgggtggtgcgggtgcggcaggagcggcagcgggcggcggcagttggtggtcctccatcgccggcgtgttcggtttcgccaccggcggccacatcaagggaccaggaacaggcacaagcgacagtatcccgattctggcatccaacgacgagtttatgacccgcgccgcagttgtacgacagcctggcgccctggcatttctcgaacagttcaaccgctacggcatggccgcgctggccggctgggcgaaccctgtccgtcacgcaaccggcggacagatcggcattcccgctcccaatctgccggctcccgtccgtggcggcgcgaacctgcccgagccctccaaaaacttcagtacctcggtcgctaactcgatctacctgcacgccgttcaggaccccgaccagatggcggccgaaatgtgggccggcaagggcggcgaccattacatcgtctggctgaacaagaaccgccaggccgtcaagcaaatactcggaaactaggaattcatggctactgaaatcggcaccgccacgaaccaccagaacctggtcgagcgcctcgtccagttcctcaccgcgaacccagacctggtcgcggctgggcaggcctacgagaaggttttcgacaacaccatccccgcgtccggcacggccatcgccgtgcgccaggtgaccctgcgcgccccgggcctgggcggcaccgacagcatctacatggggattcagagctacggcgataccgccctggactactacaaccttcgcctgatgggcggcacggcgttcaatcctggagcaatcccgcctggcggcgactactggaccgcgtttgccaactacagtccgcgggttcaggcgctgctgtggaaccagcccatgccgtactggttcttcgccaacggccgacgcttctgggtcgtcgtgaaagtctcgacgatctacgagtcggccggcgccggcttcatcctgccaccctgtccgccgtcgcagtatccgtacccgcttgccgtcgtgggctcctaccgtggtgacgttgcaactcgctggtcagacgtcagcgaccggcacagaggcatcagcagcccctacgagcgtagctgctatctccgcgatcccgccgggcgctggctcggtttcactgtcgcaggccgttcaagcaacgagtccgactacaacaatcggaccctgctgccgcttggctgcggtcgctatgcgggtggtagcgacactgtgatcaaccagctccgcgactctttcagcaagttcccgctgaaagctttgcagttcgtcacccgcgaaaccgaggggcgccgctatctgggcgatttcgacggcgccttctacgtgccgacgctcaactccggcgccgaagacgtgattgtcgaggacggtgtggaccacgtcgtttttcaaaccgcttggcgtagcggtaacccttggctctacgcgatcaggaaggactgaaatggcttacttcacaggaacagcgaacaacccggccgacttgctcgccaagctgcgcgtccacgccgagtcgctcggctgggtcaccgaccgcgcctcggcatcggaatggctttgtcacaacgccgacggctactggtcgttcaacgccggttccaatcaatggcagctcgcgggcaatacggggttcgacgacgggcttgcgtggaatgcgcagcccggcaactcggtgcagaacaacccgtattcgtcgaaagaagcaaccatagcgcagctcagcgccgggccattcacgcgctatcacctgttcgccaccgctgcctatctgcacctgcacgtcgaaatcgctgccggtcagtttcgtccagtgatgatcggctccctcaacaagcgtggcgtcggctatacgggcggccagtatgtttgcggctcgttcctctacagctctggccaggcgctcacaaacaactggtcatcgcatccattcgatggttaccacattcgatacagcggcggcggcagcatgctgcggctagacagcctcgacggtggcccatcgccggagtggttgccgttcgactacacaacgaacgtctcccggcgcgtcgtcggccccggtcgcggaaactacagcagtcagtaccatcccgacgtggggctgatcgacgcgagcgcaaacgagctgaacagctcgaccacccctgtgccctgcgccatctatgcgttcggcgctcagcagcgctcgcggtacgtgggcgaggtgccggactttggcatatgcaacatggcgttcctcgcgcctggcgatccgctggtgatcggcagcgacacttggcgcgtctatccgttgctccaacgcggaagcgctaccgatttcggcaacaccagcgcctgggtcggctactgcttccgggtgcttgagtaatggcgacgtttccggggttccaggtgccaaagccgctcgtggggatcgttgccggcatcacgccgaatatcgacgccctggagctgaaccaggacatcagcctggcagcggtcgcggcctcgacctgggccggcgcctacgcggcgcatcagccggtagaggtgatccattcgacgtaccaggctgtccaccaaagcgctctggaagagaactactacaaccgcctgtggctgatccctacgaccatggagctgggcaacgtcgtcagcacccaggtacgaccggcatcagtctggaacgcttatttcagtccgcgcacgctgaccgccatcgagcgggaagatgcagacggcatcacgctatccggccaggcgtcgccgccgctgggttttgccgccctggaggaacgcacttggaccgtcagcattggcacggacggcccgcccgtcgtcaatgcgcggatcgtctggacgctccagggcgagccggacctggtcctggtcatcaccggcaatcgcatcatcgcctggaccttcgcgccggactggggcgacagcatcgtcgagcgcctgagcgcctcgacaaatatcctgcaaagcgaatcagccgtgacccagcgccgggctatgcgcctggcgccgcgccgggagttcgaagcgaacatgtacgcggtagaccgcgagcggcagctcctggacatgacgctgtttggctggggcgcgcgaatttgggcgctgccgatttggcctgatatccaactgctccaagaaccgctggcggccggctcgctgaacattccgtgcgacacggtcggcctcgacttccgcgacggcggtctggcgatgctgcgcggcgaggacgccttcacctatgaagtcgtcgaggtcaaggcagtgaccgccgccggcctggacctggtccgccccgtccaggccacctgggtaactggctcgcgactgtacccggtgcgcaccgcgcagctgaccgaacagcccacgctgacccggctgaccgataccgcgcagtctgcgcgggtgtcgttcctgataatggagcccagcgcctggcccgaggtaatgccggcgacgacctacagggggcggccagtgctggagcagcgcccggacgaaagcgaagacctcacctccagctatcagcgcctgctgtccaccctggacaacggcagcgcgattccccgcgtgaccgacgtcgccgggatggcgctgcccgtcatcggtcatcgctggatcggcatgggccgagccgagcggtcggcgttccgcagcctggtctatgcgctgcgaggccagcagaagccgctatgggtgccgacccacgccgacgacctgaccctagtcgccaccgtctcgcagctgtccactgcgctggacgtgcgcaatatcggctatgcccgtttcgccaatgggcgaccgggtcgtcgcgatatccgcatcgagctgtacgacggcaccgtctatcaccgccgcattctcaccagcaccgagctggacgccgacaccgagcgcttggccatcgacgccgccctgggccgcctggtcgagccgaccgatgtagcgcgcatctgtttcatggcgctctgtagcgccgccagcgacgtggtcgagattgagcacgtcaccgatagcgagggcgtcgcaaccgccgcgctgacattcaaaggggttcgtgacgatgagttttaacagccgcgaaagctcgctcgcggatgggcagccggtgcggctgtaccagttcagccgtggcgcgatccgctggagctacaacagcagcgaccgggacatcacctaccagaaccagattttccgcaccgtgccgggcggcatcaccgacaacgggatcatctgttccggcgacccgcagtccgatcagttcatcatcaccgcgccggccgacctcgatgtcgcgctgctgtacaaggccaaatcgccgagtgatgccatcgatctggtcgtctacgacatgcactacggcgatgtcgaggcagcggtttcctgggtgggggagattggcgacgtggactggccgaccgtggacagcagtcgcataacgtgcgtgtccgaagacgagctgatggaccagccaggcttgatcgataccagttgccgcacctgcacggcgaccttgggcgaccaccgctgcaaggtaaacctcattccgtatcgagtgacgctgacaccgcagagcgtgtccgcgtgggtgatttccagcggagtggtcgccggctatgccgacggctggtttaccggtggctatgtggagtggcaggtggacggcgacaactacgaccgccgctacatcgagcggcacgccggggccgatctgcacatcctgggcggcaccgagggcgtcccggcgggggggcaactgcgggtctatccaggctgcgatctgctcgatgaaacctgcgccggaaagttcgacaacatcctgaatttccggggctttaacaagatgcaaggcaagtcgccattcgatggcgaccaggtctggtgaggtaggccatggacccgatcacaatcaatctcgtcattctggctgcgtcgttcatcctatccagagccttggcgccgaagccgcaaaagcccaagccaacagcgtttgaagacatcgatttcccgcgctgcgacgagggcgacgaactggccgccgtgttcggtcagtgctggaggaagtcctggatggtgctgaccgtaggcaactaccgaacgaaggcgatcaagacaaaggggagcaagaaatgatcgttacggctcagcacttacatacggtcccgacctggaccactcggcagggctactgccatcgccaggcgcgggagttcttcaagcgccatcacctcgactggatggcgttcttacgggacggcatcgaggccgatcagttgattgcgaccggcgacgcgctcgcgctcaagctggttgagcacgcacgccaggaggtggctgatgggcgctaaacccaaggctcaaacggtcggctttcgatacttcttcgacatccatttcaccctaggcaagaaaatcgacgagctgtgcgcgctccgggcaagcggaaaaaccgcgtggaaaggatcgatcactactaacggtcaggtacgcatcaacgccccgaaactgttcggcggcgacaagggcgaaggtgggctcgatggaacgttggatatcctgttcggcgaagaagaccagggtgtcctgccgcgcctggcggccatgctcggcggcctggtgccggcgttccgtggcgtaaccacagggttctattccggcttggtaacctccatgaacccctacccgaagacatgggaatttttggtccggggaggaaaccgcttgtgggacggcaatccctggtatcccgaaaagcagttcatctggctagcggacggtcagatcaaggcgatgaacccggcgcacatcctttatctcgtctacaccggccgggacttccggggactggcccgcacgcgaatggacgaggcgagctggcgggccgctgctgacaagctgtatgccgagggtttcgggctgtgctttgaatggaccaggtccgacacgttcgccaacttctgcgagacggtgaaatcgcatatcggcgctgaggtttacccgaaccgtcagacgggacagatcagcatccggctcctgcgggacgactataacgtcgcagacctgccgctgttcgacgaggacagcggcctcctggaaatcactcaggagaagaccggctcgacctccctggcgccgagccagcttatcgtgaaatacatcgaccagatcgacggggcgcagcgccaaatcatcgtcaacaacaacgcggtcgctgcgtcgcaggggcggcgctcgtctgaggaaatcgagttcctgggcgtgcctaccggggagctggccgggcgagtcggtgagcgggaaatgcgtctgaagacaaccggcctgaagcgctataagggcgtgttcgaccgccgcgcccgtagcctgaaccctggccagccgttccgcatccgttcgacccggcgcggcatccctgaaaccgtcgttcgggtcggccggatcgaggacaacttcctcggcgacggcaagatcaccctgaccgtcgtccaggatcagttcaatctgccggcgacaaccggcgtggcgccgccaccaccgggctggattccgcccgaccggacgcctcgggcgatcactgtgcgccgcctgatcgaggcaccctatcgcgaactggccggcgtgatcgatccggcaaatctccagctcctggacgtgagcgcgtcctacttggccgcgctggccgaggcgccgaccagcctgtcgcagagctacacactgaccgaccgcgtcggcagctctggcgcgttcgttgatcgcggaaccggcgactggtgcccgaccggactactcgccgccgagctgccgctggcggccggtccgaacgtcgtcacgttgacgaacgccagccggctggaggacgtcactgtcggccaggccgcagtcgtggacgacgagatagtccgggtcgatgcggtcaactacgccagcggcacggtcaccctcgcgcgcggctgcgccgataccgtaccggccaagcatctggccggggctcgggtctggttctacgacacgttcgaagctgtggacgaaacggtctacagccagggcgtgacgctccaggcccggctgctgacgaacaccagcgagggccaactggccccggcgctggccgccaccgacagcctcaccctgaccgggcgccaaggtaagccgtatccgcccggccagttccgcatcaacggcagcgcgtacccaacgaaagtctacggggcgctgtcggtgagctgggcgaagcgcgaccggatcggccaggccgaccagttgatcgataccacggtcggcaacatcggacccgaagatggggcgacggttacgctcctggtctacagcggtacgacgctgaagcgtacctatgccggtctcacatccagtaactggtcctatccgctggccgaagacatggcggatggcccgctccaggacgtgcgccttgtcctgcgcagtgtccgcgacggcatcgattcttggcagcagcacgacatcacgattgaacgccacggcctcggtttccggcttggcgaagaactaggaggcgtatccgcatgagcctgacaatggggccgaacactggcttactgatcaacggcgcccccggtgaggggcattacagcgaactgatccgcatgttgcgctgggatgacttcctgcgccaaccggtcgtaaaggggcgggtcgcaacgctgccgacttccggccaggccgagggcgacacttacattttcaccggggccggggcgaaccagaaccgcttggcccgctggtgggcgactggtgcgtcaacgccaatctgggagtacatgccgccacggctgggctggcgtgtccaggtcgcaaacgagacaaccccggcaggccaggtcaagacctacgagtattccggcagcgcctggactgagctggtgggcggaatggccgacgcgccgagcgacgggaagcgctatgcccgactaaacaacgcgtgggcaggcttggggactgctgccgtcgccgatattcttgggccggtctctcaggctggcggtgtgccaactggtgcgatctacgagggcggcagtaacgcgaacggaagttacgtcaggctcgcagacggaacgcaaatttgctccagcagccttttaacgtttactgcgggttcaacgtcggtgggtgcgtcttggacgtttccggccagctttgtgtcgccgtcgctgatgtttggcaccgttgtagcatcgggagccggcgcagactatgaccccggcgtcgctgcgaggaacctgggagctgtttacttcaatgcgtcaacaaactctgctgcactggggtttctttgcatctcgtctgcatcgttcaccgctggcgcccaaactcgaaataaccgtgctgtcgcaattgggaggtggttctgatgatcatcacgttgtcgccgtatgtcgcgctgcccggcagcgatgaacatctgatgctgagcaggactggcgatgtactcaccgtgaacggccagtcgttcgatttcacaccgctcccggagggcggcgagttgccggccgaggctatcgggtcggagtggttcgctggccccgtcgttcgccgtgaggggcgtctagagttcagcctgcggctgccgctggctgacggcgctagtgcagccgctcgctttcctgaaccaatgctgatcgaggccgacggccctgtggagttgccgcaatgactattgactggagcatgttgaagtcacccgaagaccagcaggttgagcagcgggaggccatcagagcgcagcgccgccaggcctatcgcaccgagtccgacccgctgcgcctggaggccgagtttgacgccatcaccgctggcaccaagccggacctggcggcatgggttgcagctgtccaggcgatcaaagcgcggtatccactacctgaataggtagttgtgatggcgttctcgtttttgccacgttccgacagtctgatgtcgagtagtagataggaaccttgggatggacgaggtactgaggcaaaggttgcgggctgaactactggaagtggggtttctcaaccagtgctgccttgatctcatggaaagcatggaggctgagttcagtctcactaaggaccagcgcgagtgcattgagcagctcagccaattcctacgggagggcatcggcaaactgaccgctctgtctgaacgggtagccgacggcgatatcgtcgtcctgtgctgatcttttgaaattcttttgccgctggcgaaacggttagggcgcgtcatttattgcgcaaatcggcgccaaatttcgcgccgcgctaca

SEQ ID NO: 13 - DNA, 36967 bp, synthetic construct
  source 1..36967: mol_type = other DNA
tgtggggaggtgactgttttgacacatgccaaaagagggagggataggccagagcccctatagcactagggctccagccggacagacgctgtgggacagtttggaaaaaatcgatcaggattgagcaaggaatgcaaaatattgatcgttaattggcgcggaatgagcgctaaaccatccatcgcccaagccagacaacgcgcccaatgatatccaagtcagaaagctggtccttggggacgaccatgtccttatacgccttgttttcgctgatgatcgcgatagagccatcgaactgccgttgtaagcgcttggcgtagagctgatccccgacccgaatcacatagatcgcttcatcccgcacggttctaaggtcatggtcgataacaacggcgtcgccatccgacaggaggggttccatggagtcgcccccgacccttactgccgacatcctggttggctctaaccccttcttgctcaagctgtagcgcgtaaaggcacccgccttgggagattccagcattcctcgctaaagcacttgcgctccctgctatagcgacaatggagcgcagcctttcgatgaaggcagcgtcattttcaggttcggttgcggaacttgaaaggctggcggtgcgctcgctacgcgttttcatgtagacctaactatttgatttaattgatattaattctatagaggtcgaaatctacctcctatagaacttgaaaaccgctatagagcttgtttttcaacttctatagcgctatgtttatgccctaagtcacgttagacacccctaaaaaaaaccaccctgccaggtggtgagatggaacgtaggcatgaacagaacccgaaatcccccgcgacaacaacgtcccgctgggagtggatcaaatacccagctccgcgccagggggtcgtccctggccgaggtggcccgctccctcgacgtatccagcccggcagtcaaaaacgccaagctgaatccctacccctcgggtagagcgcgccatcgctgctgtactcgacctcagccccctagtgctgtggcctgagcgctggctcgacgacgagaatccgaagcggcaacggcccaatcgctcggagaccttgcaggcatatgtcagacatatgccaagtgctgaggaaaataccagatacgctgaccaagcgcagcgtaaagccgacgcgggggcttgaacatggcccgccgcaaagacgaccgcaccctggacatcttcgatgttccgcagccagcccgcgctatacccggcgagtgcaactatgccgcccaggtcagcgagctggtcagcgaaattctgaaggccgccaacctcgaccgttacgaggtcgccgcccgcatgtcgcgcctatctggcgatgacgtgagcaagaacatgctcgacgcctggtcgagtcccgcccgagctgatcacaacttgcctttctaccgcgccgccctcctggaggacgtctgcgcgagccacctgctgaccaactggctggtcgatgtgcggggcggccgcgtggcctatggccgagacgcactgctcgccgagctgggccgcctggagcggacccgcgaggaagcgggtcggcaggcgcgtgagctgaaacgaatcctgggggagccgtgatgacaaacaccgacctcaaaccgctgctcgacaacctgcggaacgccaccgagttctggaacctagtcaaagaggccagcgctacggacgaaagcaccgttcacaaccgctccttttcggatgctcgcgagtggctcgaatcggcggccttggccctcggtgacgccctgatcgcccagcgcaaagctgtcgggggcgaccatgaatgaatggttctccgcacagaaactggtcggcctgcccggactgcctggcacggttcaaggcatcaatagtcgcgccatccgcgactcatggcagcaaagaaaacacatgggtagaggcggtgggcgtgagtaccacatttccagcctacccgacgaaacccgcgccgcactgctgaacgccgccctgggcgaggtggccaccaaggtggtccgccaggagacgcagctggccctggtcgaaaccaaccgccagcagctggtcgccgatgctcggcagggggtgctgcacgccctggacctgatgatggcccgcaccggctacagccggaagcgctccatcaccctgatgctggacatggcgcgcctcggccaggtcgagccgcagctgctcgcgatgctcaagatggcccgcgatcctcgcggccgcccgagcgcggatggcctgccgagcgtgcgcagcctggagcgtttcctggaccaggccgagcgcggcgccctggtgccgaaggtccgccgcccggacatgagcgttcccgactgggcgccggccttcatgacgatctaccaggggccggagaagcgcagcgcccgcgctgcccatgcactgctggagaagcactggcaggggcaaatgcccagcctggaccaggtttatgcgttcctgcgtaaggtcggcaacgtcagtcgcgaggtcgggcgcatgggtgagcatgaaataaaggcgctgcgcccgttcattcgccgcgacttcaccaagttgctgccgaccgacgtctattcctgcgacggccacacgttcgacgccgaggtccagcacccgatgcacggccggcctttccggccggaaatcaccaccatcattgacatccgtacccgccgcattccgggatggtccaccggcctggccgagtcggccctggtggtggtcgatgccctgcgcgacgcctgcaccaagggcggcatcccggccatcttctacgttgacaacggctcgggctacgtcaaccacatgatgcgcgacgaggcggtcggccttatgggccgcctgggcatcgatatgaagaacagcctgccctacaacagccaggcgcggggcgtgattgagcgcgtccaccagagcctgtggattcgggccgccaaggaactgcccggctacatcggcgccgacatggaccgccaggccaagctggccaccttcaagctgacgcgccgggccatcgccaagggcggcaccatgccgctgatgtcttgggaatcttttgtcgcgttctgcgaacagcagattgccgaatacaacgaccggccgcacagcagcttgccgcgcatcgttgacccgaacaccggccgccgccggcacatgacccccaacgaggcctgggcgctgcacgaagcggagggtttcagcccgatgcgcgtcaccgacgacgaggcccggccgctgttccggccccaggtgctgcgcaccgtccgccgctgcgaactggagttcatcggcaaccgctacttcgcccgcgagctggaggaattccacggcgaccaggtggccgtgggctacgacatccacgacgccagcagggtgtgggtctacgacggcgagggccgcttcctctgcaccgcagagctgaacggcaacagccgcgactacatgccggcttcgtatgtcgagcgtgcccgcgagaaacgcgcagaggcccgcgagaagcgcgccctggctcacctcgacgagattcgcgccgagcgtgacggcgggtatgccctggaaatggatgcgccgctgtccatccccggcctcggcacgatcacccctgagcaactccggtcgcgcagcgccgcgaccctcgaaatgcaggccgagcggatcgacgaaccgcgcccggccgcagccaccgcccaagccaccaccgcccaggtcttcaccctgccgaccgctcccgcccagcgctaccggcagtggtgcgagctggccgagcggcaacgctccgggctgcccatcgagccggacgccgcccagtggttcgaggtttaccccaaatccaaagaattcgccgcccagcagcggcaagcatgaaaggagctgtattcatgaccaccccgaaaaccacccaactggccaatggcatggccgacatcgccaacatcgccctttgcgatatcgccctggagaaagcgctgtcgcgtacctccacgttgcccggcctggtctgcttctacggcccgtccggcttcggcaaatccgtttcggccgcctgggtcgccaatcgccgccgcgcctactacgtccaggccaaaagcgtctggacccgcaagcacacgctgaagtcgatcctgggtgaaatgggcatcaagccggctggcacgatcccggaaatggccgaccagatcgccgaggaactggccgccagcggccgcccgctgatcatcgacgaaatggaccacctggtcgccgctggccaggtcgagctgattcgtgatctgtacgagtccagccaagcctccatcttgctgatcggcgaggaaatgctgccgaccaagctgaagaagttcgaacgcttccatggccgcgtgctgagctgggttccggcccagccagtctccctggaggacgcccgcaacctggcgccggtctacagccccggagtggctatcgctgacgacctgctcgcgcacttggtgaagaagtcactgggctctgtccgtcgcgtcgcggtgaacctggagcagttggccgaggccgccaccgttcagggccggcgcgagctggaactggccgacctccagcgcctgaacctggagctgtataccggcgcggccccgaacccgaggacgtcgaaatgagcctcggcaaaaacccggctcacctgtccatggtcgggggcaagagcccccgccagcagatgtgggaagtcatccgggccaaccgcgaagagttcaccgtctaccgcgtggcgcgccgctccaaccagcacgacaagaccgtcgagaagtatgtcgcctgcctgcgcctgggcggctacgtcgaggcgatccgtggattcaagcgcggcgaagaggtcgttttccagctggtccgcgacaacggcgtcgaggcaccgaacctgaacgccgatggcaagccatcccagcagggctacaccaccgaggcggtctggcggacgttgcgcatcctcggtccagcgaccccggagcagatcgccgcatcggtggcggcctctggcgcgactgtgtcgcccagcaccgttcagcgctacttcatcgatctgcagaacgccggatacctgacccgcaacggccgccactacgccctcaagccgggccgctacaccggtccacggccgcccatcgtccagcgcgagacgcgccgccaggtctacgacccgaaccttgaccaggtcatgtggagttcgcacggcgagtaccagcacaaccggagtcgttcgcggggcgcttcccaggctggcgtggcggataccgaagagaacaacgaatcaggcggctgaagccgtgatgaagacggtgccgaggggtggcctcccctcgacacctaccaccacccggaaggagaggagccatgcaaatgcatgcacagcaaggcggtagcgccgcgaaggctagcacaagccactttcgcggcactacgaacattgaggagtacatccgcgacatggcgagccgtgggttcagtcgtcgggccgtgagtaaggccctgggtatgcagtcgcggaagttcaaggaactcctggaactcctgccagaaatggactgggtgcctccttgtcagtcgtgggaccgcctgcgcgctgaccaggagaagaagggacgcaagtgtccgatgacagaggggcgtctgcgctcgattgtcgcggcgaggcgcgccgcgatggcaaaacacacccgctacaccgcgtttggtgtaacagccaccttgccggagctggtgagccagttcggccaggtcaccgccgccaccgtgcgcatgcggttggccaagggaatgcctctggagcaggcccttgcctccgtgcgcagcgatccttgtggaaggaaggtcgcagatagccatccctggaaacaggaggcgcaccagggggctatcaatcaccttgagcgtcaaaccgctgcaatgcaggaacgcgttcagggggagcgcctggaccgggcggcctcactgctgagccaggaggtgccgccatgcgccgaacactgatccccatcggcatcttcctggccctcggcctactgctgatcctggccggtgatgccctgatgctcggccgccgcctcattgcctggcagtgggggtgctgatggaacgcgcaatcgatctgtcggcctggggcgagcgtccgcccgtcttcgtccaactgctggccgccgaggtggcccgcagcagccagacgaaagccggcgaggcaatcggcatgagccgttcgaccgtcagcaccatcctcgccaaccgctacccgtcgccctcgacgatccgcgtcgagcgccgcgtcctggccgcgctgagccgtattgagtgcccggccttgggcgaggcggtgacctcggtcgagtgcagcgagtacctccagcggccggcgccgctgaacaaccccgtcgcgatgcgctgctggaaagcgtgccgcgcctgtccacgcaacccgcataccgcccccatgaaacgagaggaacaaggccatgagaaccgcattgcccttgaaagtcttgacgcctgacttggcccagagcctgcgcaccttcaacgacgccgcccggctgctccagcgcatgggggtccgccttcatcgcctggagccgacagaggggcgcgtgaccatcgccgcagatgacgcccgccagctcctggagaaaggctacctgatgggcttccagcgcgacgcctcggccggcagcacccgttacatcacccgcttccagggcatcaccctggcctggagcgaaccgatcagctaccgcgacttcgccggcagcaaatccgtaattcactgaacaggagaacgccaacatggcaccgaagaaacgtctgaaatccgctgccgccgtctacgtcccgcagacccgcgaacaggtcatcagcgatatcaagaacatcggcgacctccagcgcgagctggcccgtctggaaaccgcaatgaacgatgaaatcggccagatcaccgagcgctattcggagccggccgaagacctgaagaagcgcctggcggtcctccagggcggagtccagtcctggtgcgaggccaaccgtgccgagctgaccgacaacaacaaggtcaagtacgcgaacctcacaaccggcgaggtccagtggcgcatccgtcccccgtccgtgactgtgcgcggcgccgatgcggtcctggagctactgcgcagcaaggggctaatccgcttcatccgcaccaaggaagaggtgaacaaggaagcgatcctcaacgaacccgaggccgtccaggggctgccggggctgaccctgaacaccggcatcgaggacttcgccatcgtgcctttcgaagcggaggtgcagtgacatggccgacaccatcgctttctgctgggcctctggcctgatccagttcggtgaccaggtgcccgagggcgccatcgagatcgcccgtggggacgaccaggtcgttcgcgaaaacctcgtgaccaattcgcggcacgcttacgacaacgtgtcgctcctggttccgggcgtacccgaagcggcaaaccaaaccgagggcggggacgcactggagtgcttcatccgtcttctcgccaagtacgacagcgccgctttccaggtcgcttatgtggaggacgtgtgacatggcacgcaaccgcgcgcaacagctgtgcatcgcaccttggactatcagcgcttcctgttaccccaggctgatgcactcaagctgatagacatcatgagtcgagccgcagaggttcaggccgactacgcctctggagctggattcaagtacaccgtcggcgaagtgccggaagtcgagttgacgatagtacgccccagtcaattggtcatgccgcaggccgagccggccccagctacaccacgcgctcgccggaagtctccggcccaggtcacgcacgatgccattcggctgttggaggggctctgatcatgaccaagacgttcgccatgtgccgcatcgacggcctgatcgagctgcgggaggaacacccaggcgagggctacttcgcccttgccgtgggcgacttggccagcgtgcgggcggcggtctttgcaaccgctgagccgcaccaggtcggcaagaaagtcgcccggcgcgtgccgggtgtgagccccgacgccaccgaccgcgaaaacctgggctccatcgcccggtacatccagaccctgggccagcaggatcggcccggcttccgtgcgctgggggtgtgaaatgcagcagtccaaccccttcaatcaccccggacagagctacggcgccgtagacgtcgatagccgactccgcgccgttgccggcttcgacctggagcaatgccgcgccgcgctcgcggtcaccggcctccagaagatcgtcgagcagaaaattcgcacccgcatccgccagctggaaaagcaggcatccgcacagaaggaggcatagccatggccgtatacaccatcaccctaagcgacaccgaaggcggaatagatttctccatgcaaggcccgccgctgcacgactccgaagcatcgaagatcgcctacgcccttatgcaatcgaccatgtccctcggccgagaactcgcaaagcagaacggagttggtaacgccgtttcctgcgcctgcgacgagtgcctggcacggcgcgctcgcggtgaggaaccgcagcaggaaatccactacaccacggccaagaaccgcaccgtccactgagcgaaaccgccccggcctggccgggacggtctgccggacgtggtggtccggtactgatgagcagccacccatgacgaacgaaaccaagacagaccgccagcgccgcctggcgcgggaacgccaacgagcgaagcgcgagcgcgatgccctgcgccgcgctgcgctgggcggtcgccgcttcaacatggacatgtaccagggaacggctgatgcactcgatctgatctgcgcggccggtggcttcgccgagccggccgaggcggtcaccttgctcctacacaacgttgccgaaattgcagaacgtgacgcgtcacgctttgccgaattgatccaaaagagaagccatccagggaggaccaagcgatgagcctacgcgccgtcaacctcgcaaaaatccacatcgccaaggcccagctgggcatggacgatgacacctatcgcgcattgctcgctcgcgtcgcgggcgtgcgctcggccaaggacttagggccgcgccagattgaccaggtactggtcgaactccagcgtctgggctggaaaccgaagagcaaccggcaaggccgggcgacgccaaaagtgccgcaaaaccggcaaaccgtgctgcgcaaaatcaccgcgctcctggccagcgcccatcgcccctggagctacgccgaccatatggcccggcgcatgttccaggtcgagcgggtcgagtggctggacgacagccagctctaccggctgatgcaggcgcttatcatcgacaggagccgccatggccaggtctgaggtggatcttcgggaggtccaggacatgctgccggataccgtccgcgacatggccggacgcatcggcctgccggccacgctggtggtagtcgagcagctcggcggcacgtcctggcggatagccgagggccgggcgcggaggggcgaagcgcgccgggctgcgctggccgagctggtgggcagcgacatcgaggagcagctccacacgcactatcggggcgaagaaatttacgtggctcgctgccacaaggcgctggtacggtggcgcgatctggagatcgtcgagcgcttcgaacagggcttgcgtgacgggcaaaccgcccgtagcctgctcagcgatctagcccgccaatacaacttgtccgaccgctggatatgggagattgtcaaccggccgagcgagccggcaccgcagcaatccaccctgttccactaagccggggcgcaacgccccggccggcgtctccgcgccgaccctgtctcagccgttgaaccccttccgctaatcccgcgtcgcactcaccgccacgatggcggcatgagcacatctagccccccaacgtctctacgcagcccccgcgactacgccgccgccatcctggccgagcccagccgcgagcgtcgtaacgctctgctggaagcctgcccggtcaactggcagccacttgttcgggcgcacgtcgaggacgccttcgcgaaggtcaaggcgtatcgccagatgatggaccaccgcgccgagtcgatccggcgcggcccgcctccagctccccgcgtcaccgacaccgatttccgcatatccaactacaccaaatccgccccggaggtaggcaatgcgcacctatcagcaattcgggcagcgctcgcaacggaagcaccaaatgcctgatcccgcatccacctcggccggcagcgccgcgctgctgaaaatgtttggcatccatatcagcgcgggcgccctggccgccgccctgggcttcctggtcctgtggcccaggaccatgaaagaggggtttgcccggctgttctgcaccatcgtcgcgtccagcgtcttcggcccgatcctggtcgtttacctgcactccaaccgccccgagctgttcgagtccgcccaggtggtggccgggctctaccagttagagccggcagtcggcctgctgttcgtttccgctccgctcctggtgattgccggtctgcccgcctggtggctgatcggggcggccctgcgcctgtttgagcgggacggcgattcatggctgggcgcgttcgcccagtgggtaaaacgcaaactggagaacacctgatggcccttcaacctcgcggcatccgcaacaacaaccccggcaacatcgtctggtcggcacgcaacaactggcagggccagctcccgcacaacccgaaggtcgagccgcgtttcgcccgtttcgataccgcacataacggaatccgcgccttggcaaagctgctgctgaactatcgcaaggtccacggcctgcgcaccgtcgaatcgttgatcgcacgctgggcgccgtccaacgagaacgacacccgcgcatatgccacggccgtggcccgagccatgggggttccaccgcaggccggcctgcacatggaccaggacaccctggccgccctggtgaccgcgatcattcggcacgaaaacgggcagcagccctacagcgccgagcagatcgcccaggccgtgcgggaggtgctgtgatgcaacgcctgcggttggcagcaactaaaggccgcactctggttggcgtgatcctgatcgagaccggcctagccctggtgcgggctggtaccgggctgctgccgaggtcttccgaatgacctggcgcctcggcttggccctggccctgttcctggtgatggttgcgaccagcgcctggtggagtggtcgcgtggcgggcctggccgatgggcgcgccgcctgcgccgacgcacagacccgcgcctaccgcgacgtcctggagcaatcggcggcacaactgaaggcggtccaggacaccagcgcggctcttttccagcgcctggcccagcgggccgacagcgaccaacaaactactcgggagcttcgccatgccctggccgaaaccgctgctgatcgcgctgcctgccgctttcctgctggcgtcatgcagcagctcgaaaccgcccgtcaacgtgccgcccaggccactaccggcggccttggctcaaccgtgcccgaccccggtggcggtgactgatgacagccccgatgccaccgcaattgccctcaaacaactctacgaccaatacggcctctgcgccggactgcactgggacaccgtgcggcaccttcaaaaggactgatccgatgaccgaaaagaaagcctctcccgagttcgaactgctgcaacgcatcgacggccgcctggagcgcttcgaggaccgattcccgcagatcgagcgtaaggccgtgctgtacggctcggcggccggcgcgctggcgggtggcctggttgcctgcggcctgctcgcggcgcgtatcaagctcggtatctgaggtagtcatggcgcacccgaaggaaacccgcgacgccctgcgccgcgcctacgtcctcgaccgccagtccctggaggtcgcggccgccatgttcggcgtctcctacggcaccgcccgccgctggaaacagcaggcggaagccgagggggacgactgggacaaggcgcaatcggcgcagttgctggccggtggtgggctggaggacgtggcgcgccaggtgctggccggcctggtgacccagttccaggccacgatggaagccatccaggtagacgcggacatcaagcccgccgtgaaagtgcagctgctcgccagcctggccgatgcctacaacaagacggtcagcgcgtccaagcgcgttctgcccgaaacatcagcgctggccaccgctatggaggtgctccagcgcctggccagcttcatccgtgagcggttcccgcagcacgcccaggcattcgccgaggtgctggagccgtttggagaggtgattgcgaaggagctgggctgaccaacctattcgctgaaggggtcgtaccgactgacaaccacgggtccgctatcaggaatcttttcgacatgaacaacagaattgcaggggtgacatttcaaggccttgtaccagccatcattgcaaggctgaagaatggtcttgattcctttttggtagcaatcggcacatatgtgatgcagaggttcggtgccttgaacctctggctttatgcgatacacaagtccacccgcttccgtctggtggagctggtagcgctctttctcctgttcccagcgtttgaactgagcaatttcggcttccagctcgcctatgcggcgggtcagcgtcgtctgatccgcatgggcgctgttcagctgggattgcagcccgagcagcacgccgttcagttcgaccaccttggtcgttacagccgcatccgtcttgagcgtgagcatgctctgcgtaatgtcagtggccgccttgatgccgccgtaggcaccagcaatccagtccatcatgaccaggttccttctggggagaaatcgacccatgaagggtagcaccagagacttcctggcggatattgcccagctcgcgggggagttccgccgccagatcgaggccgaggtcgcaggcttcgaccccgacccgaaggccagcgccgtccggcgtgaacgggccagcgcggactatgagtatttcgcccggacctacttcccgcactacgtgaagcgcggtaacgcgctgctccacgactacctctacaagcggttgcccgagctggtggaccacccggacggccagcacgaagccattgcggcgccgcgtggtaatgccaagtccaccctggtgagccagatattcgtgatctggtgcgtactcaccggccgcaagcattaccccctgatcatcatggatgccttcgaacaggccgccacgatgctggaggcgatcaaggcggagctggagttcaacccgcgcctggccatggacttcccccagggcgccggcaagggccgcgtttggcaggtcggcaccatcgttacggcgaacgatgccaaggtccaggtcttcggctccggcaagcggatgcgcggccttcgacacggcccgcaccgtcctgacctggtgatcggcgacgacctggagaacgacgagaacgtccgcagcccggagcagcgcgacaagctggaaaactggctgaagaaaaccgttctgtccctcggctcggccgacgacaccatggacgtgatcatcatcgggaccatccttcactacgactcggtcctgtcgcgcctgctgaaaaacccgctgtggaagcggcgcaagttcaaggcgatcatcgaatggccgcaccgcatggacctgtgggagaagtgggaggaacttctgctcaactccgacgacgagggcgccgccgctctggccttctaccaggaacgcgccgccgccatggaggacggcgcgatcatctgctggccggatgggcagcccctctacaagcttatggtgaaacgtgcccgcgatgggcactcggcgttcgactcggaacagcagaacgacccagtccagggcgagaacgcccccttcgccgcctgcatcacgttctgggtcaaccgcctggcgcagtggatgttctacggcgcgtgcgacccgtccctgggtaagcaaggttccagccgcgaccccagcgccatcctggtgggtgggttcaaccgggagacaggcgtcctggacgtggtcgaggccgccatccgcaaacgcctgccggacaagatcatcgaggacatcatcgccatgcagcgggcctatcactgcctggtgtggggcgttgaggcggtccagttccaggagttcctgcgcaccgagctggtgaagcgctccgccaaggctggctgcccagtacctgcccgagcgatcacgccacacgccgacaagctactgcgcatcgaaagcctccagccgcacatggccaacggcctgatccgtctgcatccaagccagaccgtcctggaacaacagctgcgccacttcccggccgcagaccacgacgatggccccgacgccctacacatgctctggatgctggccacgacggggttcgcgccgatagaggcgactttggtcaaacgccggcatgaatacgcgcccggccttgacgattcttttgacactggcggccgcttcggcggcgcatggtaggtacaacacatggcacaaatcgttgacgtctacggcaacccgatccgaactcagcagttgcgcgagccgcagacctcgcgcctggccggcctggcgaaggagttcgcccagcacccggccaaggggctgacgccggccaagctggctcgcatcctggtcgaggccgaacagggcaacctccaagcccaagccgaactgttcatggacatggaggaacgcgacgcccacctgttcgccgaaatgagcaagcgaaagcgcgcaatccttggcctggattgggcggtcgagcccccgcgtaacgcctcggcggccgagaaagccgatgccgactacctgcacgagctgttgctcgacctggaagggctggaggacttgctgctcgatgcgctggacggcatcggccacggctacagctgcatcgagctggagtgggcgttacaagggcgcgagtggatgccgctggcgttccaccaccgaccgcagagctggttccagctcaaccccgaagaccagaacgagctgcggctgcgcgacaacagcccggccggcgaagccttgcagcccttcggctggatcattcaccggccgcgtgcgcgctccggctatgtggcccgcagcggcctgttccgcgtgctggcctggccgtacctgttccgccactacgccacctccgacctggcggaaatgctggaaatctatggcctgccgatccggctggggaaatatccgccaggtactgccgacgaggagaaggcaaccttgctgcgggccgttaccggcctgggacatgctgccgcagggatcatccccgaaaccatggccatcgacttccagcaggccgcgcagggtagcagcgagccgttcctggcgatgatgcggcaaagcgaagacgccatatccaaggcggtcctgggcggcaccctgaccagcaccaccagccagtcaggcggcggcgcttttgctttgggccaggtgcataacgaggttcggcacgacttgctggcatccgatgcccgccagttggcggcaacgttgtcccgcgatctgctctggccgctcctggtgctgaatcgccctggtagtcccgacgtgcgccgggcgccgcgcctagtcttcgacctgcgcgagcaagccgacatcaccagcatggcgcagtcgattccggcactggtcaacgtggggctggagattcccagcgcctgggtctatgacaagctcggcatcccgcagcctgccaagaatgagccagttctgcgttcggctgcgcagcctgcgatcctgagccgacagcatggacaacgggtggcggccttggccaccatcgttggcccacgctatggcgatcagcaggcgctggacaaggcgctggctgacctgccggcgaaggacatgcaaaaccaggccaacgacctgctcgccccgctcctggaagcggtcaaccgcggagacagcgaaaccgaactactcggcgccctcgccgaagcgttcccggacatggatgacagcgccctgacggacgcgctccaccggctgctgttcgccgccgatacctggggccgtctccacggcaacctggaccggatcgactgatggccgctccgaccgaagccgatctgcgggccatcttcgccctgcggccggccgccgctatcgagtatctggagcgcaagggcttcgcgatcacttggaactggcatgacgttgacgcggccacccacgcccgcgctctgaccgttgccagagcagcacgcctggacgtgctccaggacattcgcgacgccctggtcgagaacctggagcgcggcgagacgctacgagatttcaagcgcaacctgcggccgaccctggaggcgaagggctggtggggtcgccaggtggtagtcgcgccggatggcggcgccgaggtcgcacaactgggcagcccgcgccgcctggataccatctaccagaccaacatgcaggcggcctacatggcagggcgctacgcggccgcctacgaagccagggaaacccacccttactggatgtatgtggcggtgatggatggcgttacccggcccagccatgccgccctgcatgggaaagtgttcaggtgggacgatccgatctggcagcacatcaccccgcccaatggctacaactgccggtgccggatcgttgccttgacggaggccgctgtccgccgtcgcggcctgaccgtcgaatccagtcagggcaagaccggccaggtcaccgtcgaaaccggcgtggaccggcgcacaggggagattcgcgaacagaccctgaccaccctggagacgaccgaccgggccgggcggaagatccaatttcgccccgatgccgggttcgacggcagccccgtacagagtcacctgatggaccaggtgctgtacgacaaggccgagcgcaccctgggagccccagccgcaatcgacgaggtgcggggtgtgctgctggacccggtccgccagcgcgcctgggcggccttcgtagatcgcgccgcgtccccccaggggcagaccatgtccatcggcgtgctcgatccgaccgatatcacctacgccctagcccagggcgcccagttgcgggccggcgtggtcgccaccagcgataccgcaattcgcaacagtgctgtcgctcgcgagcagctcgccagcctgccgcagcgcttcgcccagcctgacctggtgctgtgggagcgcggcagcgagtcgttggtcttcatcgtccaggccgatagcgcggccctggctatccgtctgcgcggcgagatatacgggcccggccaactggaaaatgtcggccaggttatggaaatcaccatggatagcatccaggatggcctggcgacgggccgctacaggagagtgcgctagtgacaactaggatcgacgtcgagctggacgaccaggaggttcgccagcgcctggcgctgctgatgcgctcggtgaccgatacgctgccggtcatgcgtggcatcgctgccgagctgctcgcggaaactgagttcgcctttatggacgaggggccgggctggccgcagctcagccccgtgactgtcgccgctcgcgaggctaaggggcgtggtccacacccgatcctccaggtcacaaacgccctggctcgctcggtcacgacctgggcggatcgcaacgaggcgggaatcgggtccaacttggtctatgcggccatccaccaatttggtggcgacgccggccggggtcaccaggtcgaaattcctgcacggcggtatctgcctttcgacgaaaacggccaactggcggccggcgctcggcagtcaattctggagatcgtcctaacagccttgagccgaaatcggtagtggccactttcggacaagcggcacattgtgcctattgcgaattaggcacaatgtgcctaatctaacgtcatgccagccacaacggcgaggcgccaagaaggatagaagccatgagttcagtacaaaccgttcgtgggccggtggacacagccgatctgggaaaggtgttgatgcacgagcatgtcttcgttctgggggaggagatgcgtcagaactatcccgactacccggagccttgggacgaggaggctcgagtagccgatgcggtgaccaagctgtccgaactgaagtcgcgagggatcagcacgatcgtcgatcccacggtcatcggactcggtcgctacatcccgcgtattgcgcggatcaacgagcaggtcgatctcaacatcatcgtcgccaccggcgtctacacgtacaacgacattccgttccaattccattacaccggtccaggtttgctgttcgacgtgcgcgagcctatggttgatctatttgtgaaggacatcaaggacggcattgccggcacagacatccgcgcgtcattcctcaagtgcgccatcgaagaacctggtctgactcccggtgtcgagcgtgtgatgcgagcggtcggtcaggcgcaggtcgaaaccggggtaccgatcacggttcacacgaacccgcacacggaatcgggcctcgttgcgcagaaggttctggccgaggaaggtgcagatctgagcaaggtcgtcatcgggcactcgggtgattcgaccgacctggactacctgtgtgcacttgccgatgcgggttcgctactcgggatggaccgtttcggtctcgatgttctgctgccgttcgaggagcgggtgaacactgtcgtggaactggcccgccgtggctatgccgagaaaatggttctggcacatgatgcctcgtgcttcatcgactggttctcgagtgaggccaaggcggccgcagtaccgaactggaacttcacccacatcagcgatcaggtcattcccacgctgctcgagcgcggcgtcaccgaggatcagatcaacaccatgctggtggataatccacgtcggtacttcgagagctgagttatgaagcctgacgcctctaaccacaacccagacccgcgctacctgcgcgggctgctcaagaaagccggcatcagccagcggcgcgcagccgagctgctcggcctcagtgacagggtgatgcgctattacctgagcgaggacatcaaggagggctaccgccccgcgccgtataccgtccagttcgccctggagtgcctggcgaacgacccgccatctgcgtgatcacctgatccgcccgcaaacgcgctacacgcgccgaaacggggttagacgctacctcgctcagagtcggtgcgttaaccccgttagagccccgttagaaatcgctccagcgccattcttgtgccagggtttggccagaagatggcgccggacggtttccgcagtcgttgaaccccttcatgtgaccgctgctttctaccgtcgccaccattggcggcatggaaaagaaccgcctactcgttgccatcgccgcctgctcgttccagcttccccagctggaggatggcagcgcctggattcaagtcactccagctggtgagttccggcccacggacgggcgccccatggacgtgccggcctggcggatcgatgccgccagcgccgccgccgtgatcgaccgggccagggcacgcaagacaccgcctgtcctggactatgagcaccagaccctcaagaaagaggaaaacggccagccggcgcctgctgccggccgcttcctcgatttcgaatggcgcgaaggctccggcctgtggggccgtgtcgaatacaccgcccgcgccgcacggatgatcgaggacggtgagtacctctacttctcgccggtcttcagctacgccccggacggcacggtcctgtcgattctgatgggcgccatcaccaacgaccccgccatcgatggcatggagccgctcgcccgccgagcggcggccacctttggcctttaccccacccaagaggaaacctccgtggatgaactcctgaaagccatcatcgaggcgctgtcgctcaaggaaggggcgaccgaggccgaagccatcgccgccctgaccgcgctcaagccggccttggacgcacaggcggccagcctggccacgctgcgcgaaaccctcggcttggccaaggacgctagcgtcgagcagatcgccgccgccaccagccaactgaagaaggccgacccgagccagaaacccgacccggccaagttcgtgcccttggaagctgtgacggacctccaggagcaaatcgccgctctgaccgcacgcctcaatggtggcgagctggacaggctggtcggtgctgcgctccaggacggtcgcctgctgccctccctggagcagtgggcacgcgacctgggcggtaaggacatcggccagctcaaggcgtacctggacaaggccgcgccgattgccgcgctgacccgcctgcaaggccgccagccggagggcgacacccacaacctcaccgacgccgagatggaggccgcccgtctgaccgggatcagccccgccgactacgccaaggcaaaaggagcctgacccatggccatcattactccggcgctgattagcgcactgaaaacctcgttccagaagcatttccaggacgccctggcgacggcacccagcacctacctccaggttgccacggtgattccgtccaccaccgccagcaacacctatggctggctggggcagttccccaagctgcgcgagtggatcggtcagcgtgtcatcaaggacatggcggcccagggctaccagatcaccaacaagctcttcgaatcgaccgtgggcgtaaaacgtaccgacatcgaggacgacaacctcggcgtctacggaccgctcatgcaggaaatggggcgcgctgccggcgcgcatcccgacgagctggtcttcgccctgctcaaggccggcaacgccaatctctgctacgacggtcaaaacttcttcgacaccgatcacccggtctatccgaacgtggatggcaccggcacggcgaccaccgttagcaacctgttcgcgccggccgctgatccgggggcggcctggtatctgctcgacaccagccgcagcctcaagccgttgatctaccaggagcgcatgaagccgtcgttcacttcgatgaccaaggaagacgacgagcaggtcttcatggccgacgagtaccgctacggcgtgcgctcccgctgcaatgtcggcttcggtttctggcaactggcagcgatgtccaccgaagagctgaacacggcgaacttcgagaaagtttacgacgccatgcgcaaccagaaggccgacggcggccgtccgctggacattcgcccgaacctgctggtggtgccgaccactctgcgctccaaggccaaggaagtggtcggggtgcaacgtctggccaatggcgcggacaaccccaacttcgaactggtccaggtactcgataccgcctggctcaactgatagccccagacggaacgcctgccaggccaaggatggccaccttcttccagctacaggagacacgacatggcacgccagaactctgcggccaagaccaccgccaaatccaagaccgatccggcgaccgaaaagcccaaggacgaagctctgccgggctccacggatgccacttcgtccaccgcacccgaggcgcccaccgccaaaccagccagcacctcggacgagatcgagggcgtcttcattcgggccaccgttgagcgccgctgtcgagcgggcttctgcttcgacaaggaaggccaaggcttcgctgaaggcgtgctgagcgacaagcagttggaggctctggagtcggacccgctgctcaaggtcgagcgctgcaccttttccggcaaccaggagggcgagtgatgaatcacgccattgcccagttggacatcgccgcgcagatcgccgagcacaacgctccaatcagcgaggctcagggtgacgccgctcaggccgagttgcagaaccaggttgccgccgactgccgcgaggcgctcgacgtcctggaacaattggagtcgccgctgtgagctactgcacgctggccgacctgatcgagcagtacagcgagcaaaaaatccgcgaggtgagtgaccgcgtcaataaaccggccacaaccatcgacacggtgatcgtggatcgcgccatcgccgacgccgactcagaaatcgacctgcatctgcacggccgataccagttgccgctcgccagcgtgccaacggcgctcaagcgcattgcctgtggcctggcctacgccaatctgcacatcgttctaaaggaagagaacccggtctacaaaacggccgagcatctgcgaaagctgctgtcgggcatcgccaacggcaagttgagtctggccctggatgctgacggcaagccggcgcccgtagccaacacggtgcagataagcgaaggccgcaacgactggggggccgactggtgagcgacccgttcgactacctgttcctggaaccgttgctgatcgagcgtatccgctcagaggttcctgggctggccatcgtttccggggtgcccgatctggcggccttgagtgagcaggaccagcccgcccccagcgtctatgtcgtctatctcggcgacgagataggcaccggagcggatcaccaggggggcaggcgcgccattcaggctatcggccagcaatgggcggttgtgctggtggtgcattacgccgactcgtcgaactccggcgaaggagcgcgccgagaggcaggaccgctgctgggacggctggtcaaggcactgaccggatgggctccagccatcgatgtggctccgttggcgcgcagcgcccgacagtctcccgtcacctacgccagcggctacttctatttccccctggtgttcaccgccaggttcgtctacccgagggtcaagtcatggaaaccgtaaaagtcacgatcactgctgagaaccccaaccacacccacgcgggcaagccggtggccaagggcgacgagatcgaagtcagccgcgccgatgccgagtttctgctgcgccgtcaattgatcaccaagattcccgccgagcccaaggccgacgagaaacgcgacaagtaacgcgcaacatctgattcctacggaggcctcacatggcacaggaaacgtatttctacgggcaaggtgagattgacgccgcgcctatcgtcaacggcgtcctcggcaaatggcgctggattcaggatgtctcggccatgagcatccagctcgcagtcgagaaggtcgagcacaaggaaagctacagcggccagaaagccctggtccgaagcttccccatcggcaagaccgccaccgtcagcatgaccttgcacagcatcgacccggataacctggcgctcaccctctatggcaaggtcgtgactaaggcggccggctctgtgacggctgaggcgctccccgccgacctggtagctggtgatgtaatccgcctggccaatccgggcgtcagcgagctggtcatcaccgacagcgcgagcagtccggcgcccctcgatccgcagtattacgccctgcgagccgatggcgcctacggcgaggtccaactgctgggtctgccgacgccggccccgacccagccgttcaaggcggcctatgagtacgcggcgactcgccaggtgggcatgttcaccgcgccgcagccgaccatcgccctgcgctacaagggcatcaacctggccgaaggcggcgcgccggtcatcgtcgagctgttcaaggtcgcgaccgacccgctccaggaactggcattgatcagcgacggcaacaccgtcgccggtatgcagatcagcggcggaatcctgctggacaccagcaagccggataccggcgacctgggccgcttcggtcgcattatccagctggggtaaatcatggccaggaagaagcctgttaaccctcgcggccagccggccgactcggcgcccgacgacagcctgagcgtgctgtttcctgaccgtcagttggcggtcgggggcgtcgaggtgacggtgcgcgagctgaccttcagcgagcaactgcgccataaccacctgttggccccgctggccgatgccctggcggcagttcccccggagcagctcgacggacctgagtcgatcaacgtcatcttcgacgctctggcccggcacgccgacgcgctgcgcgagttgctcgcgatcagttgcggccaatccgtggactgggtggacgcgctgccggcagacgacggcgaagcactggtgttgacctggtggacggtgaacagtggttttttcgtgcgaaggctctggcggcctcgcctactggcgatggcattgggcaaccgacgccctggagccgagtcttctccgatctcgtccgcgccggccactgccgcgaaaccctaggcacctataccggccggcaactgattctgtactggaacgaagcgcaggcagctgaacggcgagaacaggcgcgccacgttcggtcggtgatgttcggaatggctggtggcaaggacgccagcgccttcctcaacgatttggaatcctgatggccactaatcagcaactctcgatagcactacgcatccaggctgacctggctgaagcgcagaacgcgctcagacaactaacgggcaacctccagcaggttgaccggggggcggtgcagaccaggagcgagctgtctgcgatgggtgggcagttggacagccttcgcgcacaggtgcttgggtttgtcggagcttgggctagcttgagtgcgctgggcggcctggtgaccatggttgaccaatatgggcaaatggccgaccgcatccagatggtcaccagcagcacggccgaatatgaacaagtgcaggcccggctgctggagacggccagccgcacctatcggccgctggcggaagcccaagagttgtacatccgcaccgccgacagcctgaagtcgttgcggtacaccaccgaacaagcgctggacatcaccgattcgttttccttcttgctggtaaccaacgccgcgtcggcggaccgtgcggcgagcgccatcgacgcctactcgaaatcgatccagaccggcaaggtcagctctgacgcctggcagtcgatcatggccgccatgcccagcctggtgaacgccctggcagagtccaccggcaagagcaccgaggaaatccgcaagctaggcatcgagggcagcctgtcgttgcgcgacctgaatgaagggctgcgcaagaccgtggcggcgaaccgcgaggcggcggacaacatgggcacctcggtccaggacgcgctggtcagcctgaacaacgccctgagcgcctacctgggcgagctgaaccgcacctatgacatcaccggtagcgtgtcctcggcgctgaacgtgctggccgagaacatggaggttatcgtcaaactgtttggggtcgcggcggtggcggggctgacccgctacgtggccagcctaacgctggccacccaggcgaaactggcggcagtgctggccgctcgggcgcaagccgctgaagaactgcgggcagcccaggctcaggtcgcttcgacggcagcggcagcggccaatgccagggcacaggcgggcctgacggtgagccatgctcaggcggcggcggccgaggcggcgcataccgccgcgacccagcgccttgctgctgcgcagttggcggccggcaccgcgatgcgcgggatgctggccgtgatcggtggtccggccggcatcgcgatgctggtggccggagcggcggcaagcttcttcctgtttcgcgatagcgcccaggcggtcaagagtagcctagatgacctgagtgagccgctggaccaggtcgtcgagcgcatgggcaagctgagcgagattgagcaagatcgcgaactgacccggctttccgagcagatcgacggattgcggcagacggctgtggaagccgcccgcgaaatgcgagaggtggccagcaccgccctctatggtgccaggctggatcgtatcccgtctgccgaagcacagcaggccctccagcctctaatcgatgcgtcggctgacgctgcgcgaggcgtggaggtggactggaagtcggtgatggactccctggctgccagcggcgctgttcccgattcactcaagcgcaagctgctggacatggcggctggtcaggcagaggcaggccgtactgctaccgagctggggcagcgtcatgcggaactcaaggcacgcctggagggttcgactgccgccatcaatgagaacagcgatgcactgagtaaagggtcggacaaggcagccgagtatatccagtccctgcgcctggccatcgccgacctggaagatccatcggtcctgggcaaggccggccgtcgcctccagcagttcggggccgacctcaatgccgagcagagtgccgaaatactccgcctggagaccctgaaggccaataccgaaaaggcggcccaggcccgcgaggatgcacggcgcaaggctgaatccagtgcgcgacaacaagcctccacggctgagcagttggcgaagagccaggaaggctatgttgcggggctggaaaagcaagcccgcaccctgggtctcaccagcgcagaggtgcgggcctacgagctggccgagaagggtttgaccggagccctccaagctcgggcagcggcagcacttgccgccctcgcggcggacgagaagaagcggcaagccgacgccactgcgcgcaccaacgccggactggaggccgaatatctgcgggcgaccggccgcaccgttgacgcggggctgctggagattcggacgaaatttgacgcgatgcgtcgtgacttcgaaaaggcgggcaacgacgccggcctggcctggatcgacaagctaatccccgtcgccgaggccaaggtccgcctggatgacgtcaagcagcagatggacgatttgctggccgaccagcaacgggccgagtcgtccgttaacgtccagcaggatgccggcatcatcaacgaaatggacgcccggcagcgcatcctggacattcaccgagcgacctacgagaagctccagcagattcggccgatcctagagcagatggcccgccagcctggcgaggtcggccgagccgctgccgaatcgctcgcccaactggacgccgaggcggcgcgactccagcagaccacgacgctgctcgaaaccaccctacgggacggcctcaccagcggctttaccgacgccatcaaagggctcgcttccgggaccatggacttgcgcgacgccatcacgtcgctgggtgaagctgtactcaatgccttggtgaacatggcggcgcagaacctcgcgcagtcgttgtccagcggcatcatggggctgtttggtggcggccagcaggacaccagcatgactaccggcgcggcggctgtgaccgcgtcggccggtgccctatcgactgcgggcgcctcgctgctgaccggggccgctgctatccagacggccgctgcgtcgctggcagccgccaatggcgtccaagggctgggcgctgctgcgggtggtgcgggtgcggcaggagcggcagcgggcggcggcagttggtggtcctccatcgccggcgtgttcggtttcgccaccggcggccacatcaagggaccaggaacaggcacaagcgacagtatcccgattctggcatccaacgacgagtttatgacccgcgccgcagttgtacgacagcctggcgccctggcatttctcgaacagttcaaccgctacggcatggccgcgctggccggctgggcgaaccctgtccgtcacgcaaccggcggacagatcggcattcccgctcccaatctgccggctcccgtccgtggcggcgcgaacctgcccgagccctccaaaaacttcagtacctcggtcgctaactcgatctacctgcacgccgttcaggaccccgaccagatggcggccgaaatgtgggccggcaagggcggcgaccattacatcgtctggctgaacaagaaccgccaggccgtcaagcaaatactcggaaactaggaattcatggctactgaaatcggcaccgccacgaaccaccagaacctggtcgagcgcctcgtccagttcctcaccgcgaacccagacctggtcgcggctgggcaggcctacgagaaggttttcgacaacaccatccccgcgtccggcacggccatcgccgtgcgccaggtgaccctgcgcgccccgggcctgggcggcaccgacagcatctacatggggattcagagctacggcgataccgccctggactactacaaccttcgcctgatgggcggcacggcgttcaatcctggagcaatcccgcctggcggcgactactggaccgcgtttgccaactacagtccgcgggttcaggcgctgctgtggaaccagcccatgccgtactggttcttcgccaacggccgacgcttctgggtcgtcgtgaaagtctcgacgatctacgagtcggccggcgccggcttcatcctgccaccctgtccgccgtcgcagtatccgtacccgcttgccgtcgtgggctcctaccgtggtgacgttgcaactcgctggtcagacgtcagcgaccggcacagaggcatcagcagcccctacgagcgtagctgctatctccgcgatcccgccgggcgctggctcggtttcactgtcgcaggccgttcaagcaacgagtccgactacaacaatcggaccctgctgccgcttggctgcggtcgctatgcgggtggtagcgacactgtgatcaaccagctccgcgactctttcagcaagttcccgctgaaagctttgcagttcgtcacccgcgaaaccgaggggcgccgctatctgggcgatttcgacggcgccttctacgtgccgacgctcaactccggcgccgaagacgtgattgtcgaggacggtgtggaccacgtcgtttttcaaaccgcttggcgtagcggtaacccttggctctacgcgatcaggaaggactgaaatggcttacttcacaggaacagcgaacaacccggccgacttgctcgccaagctgcgcgtccacgccgagtcgctcggctgggtcaccgaccgcgcctcggcatcggaatggctttgtcacaacgccgacggctactggtcgttcaacgccggttccaatcaatggcagctcgcgggcaatacggggttcgacgacgggcttgcgtggaatgcgcagcccggcaactcggtgcagaacaacccgtattcgtcgaaagaagcaaccatagcgcagctcagcgccgggccattcacgcgctatcacctgttcgccaccgctgcctatctgcacctgcacgtcgaaatcgctgccggtcagtttcgtccagtgatgatcggctccctcaacaagcgtggcgtcggctatacgggcggccagtatgtttgcggctcgttcctctacagctctggccaggcgctcacaaacaactggtcatcgcatccattcgatggttaccacattcgatacagcggcggcggcagcatgctgcggctagacagcctcgacggtggcccatcgccggagtggttgccgttcgactacacaacgaacgtctcccggcgcgtcgtcggccccggtcgcggaaactacagcagtcagtaccatcccgacgtggggctgatcgacgcgagcgcaaacgagctgaacagctcgaccacccctgtgccctgcgccatctatgcgttcggcgctcagcagcgctcgcggtacgtgggcgaggtgccggactttggcatatgcaacatggcgttcctcgcgcctggcgatccgctggtgatcggcagcgacacttggcgcgtctatccgttgctccaacgcggaagcgctaccgatttcggcaacaccagcgcctgggtcggctactgcttccgggtgcttgagtaatggcgacgtttccggggttccaggtgccaaagccgctcgtggggatcgttgccggcatcacgccgaatatcgacgccctggagctgaaccaggacatcagcctggcagcggtcgcggcctcgacctgggccggcgcctacgcggcgcatcagccggtagaggtgatccattcgacgtaccaggctgtccaccaaagcgctctggaagagaactactacaaccgcctgtggctgatccctacgaccatggagctgggcaacgtcgtcagcacccaggtacgaccggcatcagtctggaacgcttatttcagtccgcgcacgctgaccgccatcgagcgggaagatgcagacggcatcacgctatccggccaggcgtcgccgccgctgggttttgccgccctggaggaacgcacttggaccgtcagcattggcacggacggcccgcccgtcgtcaatgcgcggatcgtctggacgctccagggcgagccggacctggtcctggtcatcaccggcaatcgcatcatcgcctggaccttcgcgccggactggggcgacagcatcgtcgagcgcctgagcgcctcgacaaatatcctgcaaagcgaatcagccgtgacccagcgccgggctatgcgcctggcgccgcgccgggagttcgaagcgaacatgtacgcggtagaccgcgagcggcagctcctggacatgacgctgtttggctggggcgcgcgaatttgggcgctgccgatttggcctgatatccaactgctccaagaaccgctggcggccggctcgctgaacattccgtgcgacacggtcggcctcgacttccgcgacggcggtctggcgatgctgcgcggcgaggacgccttcacctatgaagtcgtcgaggtcaaggcagtgaccgccgccggcctggacctggtccgccccgtccaggccacctgggtaactggctcgcgactgtacccggtgcgcaccgcgcagctgaccgaacagcccacgctgacccggctgaccgataccgcgcagtctgcgcgggtgtcgttcctgataatggagcccagcgcctggcccgaggtaatgccggcgacgacctacagggggcggccagtgctggagcagcgcccggacgaaagcgaagacctcacctccagctatcagcgcctgctgtccaccctggacaacggcagcgcgattccccgcgtgaccgacgtcgccgggatggcgctgcccgtcatcggtcatcgctggatcggcatgggccgagccgagcggtcggcgttccgcagcctggtctatgcgctgcgaggccagcagaagccgctatgggtgccgacccacgccgacgacctgaccctagtcgccaccgtctcgcagctgtccactgcgctggacgtgcgcaatatcggctatgcccgtttcgccaatgggcgaccgggtcgtcgcgatatccgcatcgagctgtacgacggcaccgtctatcaccgccgcattctcaccagcaccgagctggacgccgacaccgagcgcttggccatcgacgccgccctgggccgcctggtcgagccgaccgatgtagcgcgcatctgtttcatggcgctctgtagcgccgccagcgacgtggtcgagattgagcacgtcaccgatagcgagggcgtcgcaaccgccgcgctgacattcaaaggggttcgtgacgatgagttttaacagccgcgaaagctcgctcgcggatgggcagccggtgcggctgtaccagttcagccgtggcgcgatccgctggagctacaacagcagcgaccgggacatcacctaccagaaccagattttccgcaccgtgccgggcggcatcaccgacaacgggatcatctgttccggcgacccgcagtccgatcagttcatcatcaccgcgccggccgacctcgatgtcgcgctgctgtacaaggccaaatcgccgagtgatgccatcgatctggtcgtctacgacatgcactacggcgatgtcgaggcagcggtttcctgggtgggggagattggcgacgtggactggccgaccgtggacagcagtcgcataacgtgcgtgtccgaagacgagctgatggaccagccaggcttgatcgataccagttgccgcacctgcacggcgaccttgggcgaccaccgctgcaaggtaaacctcattccgtatcgagtgacgctgacaccgcagagcgtgtccgcgtgggtgatttccagcggagtggtcgccggctatgccgacggctggtttaccggtggctatgtggagtggcaggtggacggcgacaactacgaccgccgctacatcgagcggcacgccggggccgatctgcacatcctgggcggcaccgagggcgtcccggcgggggggcaactgcgggtctatccaggctgcgatctgctcgatgaaacctgcgccggaaagttcgacaacatcctgaatttccggggctttaacaagatgcaaggcaagtcgccattcgatggcgaccaggtctggtgaggtaggccatggacccgatcacaatcaatctcgtcattctggctgcgtcgttcatcctatccagagccttggcgccgaagccgcaaaagcccaagccaacagcgtttgaagacatcgatttcccgcgctgcgacgagggcgacgaactggccgccgtgttcggtcagtgctggaggaagtcctggatggtgctgaccgtaggcaactaccgaacgaaggcgatcaagacaaaggggagcaagaaatgatcgttacggctcagcacttacatacggtcccgacctggaccactcggcagggctactgccatcgccaggcgcgggagttcttcaagcgccatcacctcgactggatggcgttcttacgggacggcatcgaggccgatcagttgattgcgaccggcgacgcgctcgcgctcaagctggttgagcacgcacgccaggaggtggctgatgggcgctaaacccaaggctcaaacggtcggctttcgatacttcttcgacatccatttcaccctaggcaagaaaatcgacgagctgtgcgcgctccgggcaagcggaaaaaccgcgtggaaaggatcgatcactactaacggtcaggtacgcatcaacgccccgaaactgttcggcggcgacaagggcgaaggtgggctcgatggaacgttggatatcctgttcggcgaagaagaccagggtgtcctgccgcgcctggcggccatgctcggcggcctggtgccggcgttccgtggcgtaaccacagggttctattccggcttggtaacctccatgaacccctacccgaagacatgggaatttttggtccggggaggaaaccgcttgtgggacggcaatccctggtatcccgaaaagcagttcatctggctagcggacggtcagatcaaggcgatgaacccggcgcacatcctttatctcgtctacaccggccgggacttccggggactggcccgcacgcgaatggacgaggcgagctggcgggccgctgctgacaagctgtatgccgagggtttcgggctgtgctttgaatggaccaggtccgacacgttcgccaacttctgcgagacggtgaaatcgcatatcggcgctgaggtttacccgaaccgtcagacgggacagatcagcatccggctcctgcgggacgactataacgtcgcagacctgccgctgttcgacgaggacagcggcctcctggaaatcactcaggagaagaccggctcgacctccctggcgccgagccagcttatcgtgaaatacatcgaccagatcgacggggcgcagcgccaaatcatcgtcaacaacaacgcggtcgctgcgtcgcaggggcggcgctcgtctgaggaaatcgagttcctgggcgtgcctaccggggagctggccgggcgagtcggtgagcgggaaatgcgtctgaagacaaccggcctgaagcgctataagggcgtgttcgaccgccgcgcccgtagcctgaaccctggccagccgttccgcatccgttcgacccggcgcggcatccctgaaaccgtcgttcgggtcggccggatcgaggacaacttcctcggcgacggcaagatcaccctgaccgtcgtccaggatcagttcaatctgccggcgacaaccggcgtggcgccgccaccaccgggctggattccgcccgaccggacgcctcgggcgatcactgtgcgccgcctgatcgaggcaccctatcgcgaactggccggcgtgatcgatccggcaaatctccagctcctggacgtgagcgcgtcctacttggccgcgctggccgaggcgccgaccagcctgtcgcagagctacacactgaccgaccgcgtcggcagctctggcgcgttcgttgatcgcggaaccggcgactggtgcccgaccggactactcgccgccgagctgccgctggcggccggtccgaacgtcgtcacgttgacgaacgccagccggctggaggacgtcactgtcggccaggccgcagtcgtggacgacgagatagtccgggtcgatgcggtcaactacgccagcggcacggtcaccctcgcgcgcggctgcgccgataccgtaccggccaagcatctggccggggctcgggtctggttctacgacacgttcgaagctgtggacgaaacggtctacagccagggcgtgacgctccaggcccggctgctgacgaacaccagcgagggccaactggccccggcgctggccgccaccgacagcctcaccctgaccgggcgccaaggtaagccgtatccgcccggccagttccgcatcaacggcagcgcgtacccaacgaaagtctacggggcgctgtcggtgagctgggcgaagcgcgaccggatcggccaggccgaccagttgatcgataccacggtcggcaacatcggacccgaagatggggcgacggttacgctcctggtctacagcggtacgacgctgaagcgtacctatgccggtctcacatccagtaactggtcctatccgctggccgaagacatggcggatggcccgctccaggacgtgcgccttgtcctgcgcagtgtccgcgacggcatcgattcttggcagcagcacgacatcacgattgaacgccacggcctcggtttccggcttggcgaagaactaggaggcgtatccgcatgagcctgacaatggggccgaacactggcttactgatcaacggcgcccccggtgaggggcattacagcgaactgatccgcatgttgcgctgggatgacttcctgcgccaaccggtcgtaaaggggcgggtcgcaacgctgccgacttccggccaggccgagggcgacacttacattttcaccggggccggggcgaaccagaaccgcttggcccgctggtgggcgactggtgcgtcaacgccaatctgggagtacatgccgccacggctgggctggcgtgtccaggtcgcaaacgagacaaccccggcaggccaggtcaagacctacgagtattccggcagcgcctggactgagctggtgggcggaatggccgacgcgccgagcgacgggaagcgctatgcccgactaaacaacgcgtgggcaggcttggggactgctgccgtcgccgatattcttgggccggtctctcaggctggcggtgtgccaactggtgcgatctacgagggcggcagtaacgcgaacggaagttacgtcaggctcgcagacggaacgcaaatttgctccagcagccttttaacgtttactgcgggttcaacgtcggtgggtgcgtcttggacgtttccggccagctttgtgtcgccgtcgctgatgtttggcaccgttgtagcatcgggagccggcgcagactatgaccccggcgtcgctgcgaggaacctgggagctgtttacttcaatgcgtcaacaaactctgctgcactggggtttctttgcatctcgtctgcatcgttcaccgctggcgcccaaactcgaaataaccgtgctgtcgcaattgggaggtggttctgatgatcatcacgttgtcgccgtatgtcgcgctgcccggcagcgatgaacatctgatgctgagcaggactggcgatgtactcaccgtgaacggccagtcgttcgatttcacaccgctcccggagggcggcgagttgccggccgaggctatcgggtcggagtggttcgctggccccgtcgttcgccgtgaggggcgtctagagttcagcctgcggctgccgctggctgacggcgctagtgcagccgctcgctttcctgaaccaatgctgatcgaggccgacggccctgtggagttgccgcaatgactattgactggagcatgttgaagtcacccgaagaccagcaggttgagcagcgggaggccatcagagcgcagcgccgccaggcctatcgcaccgagtccgacccgctgcgcctggaggccgagtttgacgccatcaccgctggcaccaagccggacctggcggcatgggttgcagctgtccaggcgatcaaagcgcggtatccactacctgaataggtagttgtgatggcgttctcgtttttgccacgttccgacagtctgatgtcgagtagtagataggaaccttgggatggacgaggtactgaggcaaaggttgcgggctgaactactggaagtggggtttctcaaccagtgctgccttgatctcatggaaagcatggaggctgagttcagtctcactaaggaccagcgcgagtgcattgagcagctcagccaattcctacgggagggcatcggcaaactgaccgctctgtctgaacgggtagccgacggcgatatcgtcgtcctgtgctgatcttttgaaattcttttgccgctggcgaaacggttagggcgcgtcatttattgcgcaaatcggcgccaaatttcgcgccgcgctaca

SEQ ID NO: 14 - DNA, 36805 bp, synthetic construct
  source 1..36805: mol_type = other DNA
tgtggggaggtgactgttttgacacatgccaaaagagggagggataggccagagcccctatagcactagggctccagccggacagacgctgtgggacagtttggaaaaaatcgatcaggattgagcaaggaatgcaaaatattgatcgttaattggcgcggaatgagcgctaaaccatccatcgcccaagccagacaacgcgcccaatgatatccaagtcagaaagctggtccttggggacgaccatgtccttatacgccttgttttcgctgatgatcgcgatagagccatcgaactgccgttgtaagcgcttggcgtagagctgatccccgacccgaatcacatagatcgcttcatcccgcacggttctaaggtcatggtcgataacaacggcgtcgccatccgacaggaggggttccatggagtcgcccccgacccttactgccgacatcctggttggctctaaccccttcttgctcaagctgtagcgcgtaaaggcacccgccttgggagattccagcattcctcgctaaagcacttgcgctccctgctatagcgacaatggagcgcagcctttcgatgaaggcagcgtcattttcaggttcggttgcggaacttgaaaggctggcggtgcgctcgctacgcgttttcatgtagacctaactatttgatttaattgatattaattctatagaggtcgaaatctacctcctatagaacttgaaaaccgctatagagcttgtttttcaacttctatagcgctatgtttatgccctaagtcacgttagacacccctaaaaaaaaccaccctgccaggtggtgagatggaacgtaggcatgaacagaacccgaaatcccccgcgacaacaacgtcccgctgggagtggatcaaatacccagctccgcgccagggggtcgtccctggccgaggtggcccgctccctcgacgtatccagcccggcagtcaaaaacgccaagctgaatccctacccctcgggtagagcgcgccatcgctgctgtactcgacctcagccccctagtgctgtggcctgagcgctggctcgacgacgagaatccgaagcggcaacggcccaatcgctcggagaccttgcaggcatatgtcagacatatgccaagtgctgaggaaaataccagatacgctgaccaagcgcagcgtaaagccgacgcgggggcttgaacatggcccgccgcaaagacgaccgcaccctggacatcttcgatgttccgcagccagcccgcgctatacccggcgagtgcaactatgccgcccaggtcagcgagctggtcagcgaaattctgaaggccgccaacctcgaccgttacgaggtcgccgcccgcatgtcgcgcctatctggcgatgacgtgagcaagaacatgctcgacgcctggtcgagtcccgcccgagctgatcacaacttgcctttctaccgcgccgccctcctggaggacgtctgcgcgagccacctgctgaccaactggctggtcgatgtgcggggcggccgcgtggcctatggccgagacgcactgctcgccgagctgggccgcctggagcggacccgcgaggaagcgggtcggcaggcgcgtgagctgaaacgaatcctgggggagccgtgatgacaaacaccgacctcaaaccgctgctcgacaacctgcggaacgccaccgagttctggaacctagtcaaagaggccagcgctacggacgaaagcaccgttcacaaccgctccttttcggatgctcgcgagtggctcgaatcggcggccttggccctcggtgacgccctgatcgcccagcgcaaagctgtcgggggcgaccatgaatgaatggttctccgcacagaaactggtcggcctgcccggactgcctggcacggttcaaggcatcaatagtcgcgccatccgcgactcatggcagcaaagaaaacacatgggtagaggcggtgggcgtgagtaccacatttccagcctacccgacgaaacccgcgccgcactgctgaacgccgccctgggcgaggtggccaccaaggtggtccgccaggagacgcagctggccctggtcgaaaccaaccgccagcagctggtcgccgatgctcggcagggggtgctgcacgccctggacctgatgatggcccgcaccggctacagccggaagcgctccatcaccctgatgctggacatggcgcgcctcggccaggtcgagccgcagctgctcgcgatgctcaagatggcccgcgatcctcgcggccgcccgagcgcggatggcctgccgagcgtgcgcagcctggagcgtttcctggaccaggccgagcgcggcgccctggtgccgaaggtccgccgcccggacatgagcgttcccgactgggcgccggccttcatgacgatctaccaggggccggagaagcgcagcgcccgcgctgcccatgcactgctggagaagcactggcaggggcaaatgcccagcctggaccaggtttatgcgttcctgcgtaaggtcggcaacgtcagtcgcgaggtcgggcgcatgggtgagcatgaaataaaggcgctgcgcccgttcattcgccgcgacttcaccaagttgctgccgaccgacgtctattcctgcgacggccacacgttcgacgccgaggtccagcacccgatgcacggccggcctttccggccggaaatcaccaccatcattgacatccgtacccgccgcattccgggatggtccaccggcctggccgagtcggccctggtggtggtcgatgccctgcgcgacgcctgcaccaagggcggcatcccggccatcttctacgttgacaacggctcgggctacgtcaaccacatgatgcgcgacgaggcggtcggccttatgggccgcctgggcatcgatatgaagaacagcctgccctacaacagccaggcgcggggcgtgattgagcgcgtccaccagagcctgtggattcgggccgccaaggaactgcccggctacatcggcgccgacatggaccgccaggccaagctggccaccttcaagctgacgcgccgggccatcgccaagggcggcaccatgccgctgatgtcttgggaatcttttgtcgcgttctgcgaacagcagattgccgaatacaacgaccggccgcacagcagcttgccgcgcatcgttgacccgaacaccggccgccgccggcacatgacccccaacgaggcctgggcgctgcacgaagcggagggtttcagcccgatgcgcgtcaccgacgacgaggcccggccgctgttccggccccaggtgctgcgcaccgtccgccgctgcgaactggagttcatcggcaaccgctacttcgcccgcgagctggaggaattccacggcgaccaggtggccgtgggctacgacatccacgacgccagcagggtgtgggtctacgacggcgagggccgcttcctctgcaccgcagagctgaacggcaacagccgcgactacatgccggcttcgtatgtcgagcgtgcccgcgagaaacgcgcagaggcccgcgagaagcgcgccctggctcacctcgacgagattcgcgccgagcgtgacggcgggtatgccctggaaatggatgcgccgctgtccatccccggcctcggcacgatcacccctgagcaactccggtcgcgcagcgccgcgaccctcgaaatgcaggccgagcggatcgacgaaccgcgcccggccgcagccaccgcccaagccaccaccgcccaggtcttcaccctgccgaccgctcccgcccagcgctaccggcagtggtgcgagctggccgagcggcaacgctccgggctgcccatcgagccggacgccgcccagtggttcgaggtttaccccaaatccaaagaattcgccgcccagcagcggcaagcatgaaaggagctgtattcatgaccaccccgaaaaccacccaactggccaatggcatggccgacatcgccaacatcgccctttgcgatatcgccctggagaaagcgctgtcgcgtacctccacgttgcccggcctggtctgcttctacggcccgtccggcttcggcaaatccgtttcggccgcctgggtcgccaatcgccgccgcgcctactacgtccaggccaaaagcgtctggacccgcaagcacacgctgaagtcgatcctgggtgaaatgggcatcaagccggctggcacgatcccggaaatggccgaccagatcgccgaggaactggccgccagcggccgcccgctgatcatcgacgaaatggaccacctggtcgccgctggccaggtcgagctgattcgtgatctgtacgagtccagccaagcctccatcttgctgatcggcgaggaaatgctgccgaccaagctgaagaagttcgaacgcttccatggccgcgtgctgagctgggttccggcccagccagtctccctggaggacgcccgcaacctggcgccggtctacagccccggagtggctatcgctgacgacctgctcgcgcacttggtgaagaagtcactgggctctgtccgtcgcgtcgcggtgaacctggagcagttggccgaggccgccaccgttcagggccggcgcgagctggaactggccgacctccagcgcctgaacctggagctgtataccggcgcggccccgaacccgaggacgtcgaaatgagcctcggcaaaaacccggctcacctgtccatggtcgggggcaagagcccccgccagcagatgtgggaagtcatccgggccaaccgcgaagagttcaccgtctaccgcgtggcgcgccgctccaaccagcacgacaagaccgtcgagaagtatgtcgcctgcctgcgcctgggcggctacgtcgaggcgatccgtggattcaagcgcggcgaagaggtcgttttccagctggtccgcgacaacggcgtcgaggcaccgaacctgaacgccgatggcaagccatcccagcagggctacaccaccgaggcggtctggcggacgttgcgcatcctcggtccagcgaccccggagcagatcgccgcatcggtggcggcctctggcgcgactgtgtcgcccagcaccgttcagcgctacttcatcgatctgcagaacgccggatacctgacccgcaacggccgccactacgccctcaagccgggccgctacaccggtccacggccgcccatcgtccagcgcgagacgcgccgccaggtctacgacccgaaccttgaccaggtcatgtggagttcgcacggcgagtaccagcacaaccggagtcgttcgcggggcgcttcccaggctggcgtggcggataccgaagagaacaacgaatcaggcggctgaagccgtgatgaagacggtgccgaggggtggcctcccctcgacacctaccaccacccggaaggagaggagccatgcaaatgcatgcacagcaaggcggtagcgccgcgaaggctagcacaagccactttcgcggcactacgaacattgaggagtacatccgcgacatggcgagccgtgggttcagtcgtcgggccgtgagtaaggccctgggtatgcagtcgcggaagttcaaggaactcctggaactcctgccagaaatggactgggtgcctccttgtcagtcgtgggaccgcctgcgcgctgaccaggagaagaagggacgcaagtgtccgatgacagaggggcgtctgcgctcgattgtcgcggcgaggcgcgccgcgatggcaaaacacacccgctacaccgcgtttggtgtaacagccaccttgccggagctggtgagccagttcggccaggtcaccgccgccaccgtgcgcatgcggttggccaagggaatgcctctggagcaggcccttgcctccgtgcgcagcgatccttgtggaaggaaggtcgcagatagccatccctggaaacaggaggcgcaccagggggctatcaatcaccttgagcgtcaaaccgctgcaatgcaggaacgcgttcagggggagcgcctggaccgggcggcctcactgctgagccaggaggtgccgccatgcgccgaacactgatccccatcggcatcttcctggccctcggcctactgctgatcctggccggtgatgccctgatgctcggccgccgcctcattgcctggcagtgggggtgctgatggaacgcgcaatcgatctgtcggcctggggcgagcgtccgcccgtcttcgtccaactgctggccgccgaggtggcccgcagcagccagacgaaagccggcgaggcaatcggcatgagccgttcgaccgtcagcaccatcctcgccaaccgctacccgtcgccctcgacgatccgcgtcgagcgccgcgtcctggccgcgctgagccgtattgagtgcccggccttgggcgaggcggtgacctcggtcgagtgcagcgagtacctccagcggccggcgccgctgaacaaccccgtcgcgatgcgctgctggaaagcgtgccgcgcctgtccacgcaacccgcataccgcccccatgaaacgagaggaacaaggccatgagaaccgcattgcccttgaaagtcttgacgcctgacttggcccagagcctgcgcaccttcaacgacgccgcccggctgctccagcgcatgggggtccgccttcatcgcctggagccgacagaggggcgcgtgaccatcgccgcagatgacgcccgccagctcctggagaaaggctacctgatgggcttccagcgcgacgcctcggccggcagcacccgttacatcacccgcttccagggcatcaccctggcctggagcgaaccgatcagctaccgcgacttcgccggcagcaaatccgtaattcactgaacaggagaacgccaacatggcaccgaagaaacgtctgaaatccgctgccgccgtctacgtcccgcagacccgcgaacaggtcatcagcgatatcaagaacatcggcgacctccagcgcgagctggcccgtctggaaaccgcaatgaacgatgaaatcggccagatcaccgagcgctattcggagccggccgaagacctgaagaagcgcctggcggtcctccagggcggagtccagtcctggtgcgaggccaaccgtgccgagctgaccgacaacaacaaggtcaagtacgcgaacctcacaaccggcgaggtccagtggcgcatccgtcccccgtccgtgactgtgcgcggcgccgatgcggtcctggagctactgcgcagcaaggggctaatccgcttcatccgcaccaaggaagaggtgaacaaggaagcgatcctcaacgaacccgaggccgtccaggggctgccggggctgaccctgaacaccggcatcgaggacttcgccatcgtgcctttcgaagcggaggtgcagtgacatggccgacaccatcgctttctgctgggcctctggcctgatccagttcggtgaccaggtgcccgagggcgccatcgagatcgcccgtggggacgaccaggtcgttcgcgaaaacctcgtgaccaattcgcggcacgcttacgacaacgtgtcgctcctggttccgggcgtacccgaagcggcaaaccaaaccgagggcggggacgcactggagtgcttcatccgtcttctcgccaagtacgacagcgccgctttccaggtcgcttatgtggaggacgtgtgacatggcacgcaaccgcgcgcaacagctgtgcatcgcaccttggactatcagcgcttcctgttaccccaggctgatgcactcaagctgatagacatcatgagtcgagccgcagaggttcaggccgactacgcctctggagctggattcaagtacaccgtcggcgaagtgccggaagtcgagttgacgatagtacgccccagtcaattggtcatgccgcaggccgagccggccccagctacaccacgcgctcgccggaagtctccggcccaggtcacgcacgatgccattcggctgttggaggggctctgatcatgaccaagacgttcgccatgtgccgcatcgacggcctgatcgagctgcgggaggaacacccaggcgagggctacttcgcccttgccgtgggcgacttggccagcgtgcgggcggcggtctttgcaaccgctgagccgcaccaggtcggcaagaaagtcgcccggcgcgtgccgggtgtgagccccgacgccaccgaccgcgaaaacctgggctccatcgcccggtacatccagaccctgggccagcaggatcggcccggcttccgtgcgctgggggtgtgaaatgcagcagtccaaccccttcaatcaccccggacagagctacggcgccgtagacgtcgatagccgactccgcgccgttgccggcttcgacctggagcaatgccgcgccgcgctcgcggtcaccggcctccagaagatcgtcgagcagaaaattcgcacccgcatccgccagctggaaaagcaggcatccgcacagaaggaggcatagccatggccgtatacaccatcaccctaagcgacaccgaaggcggaatagatttctccatgcaaggcccgccgctgcacgactccgaagcatcgaagatcgcctacgcccttatgcaatcgaccatgtccctcggccgagaactcgcaaagcagaacggagttggtaacgccgtttcctgcgcctgcgacgagtgcctggcacggcgcgctcgcggtgaggaaccgcagcaggaaatccactacaccacggccaagaaccgcaccgtccactgagcgaaaccgccccggcctggccgggacggtctgccggacgtggtggtccggtactgatgagcagccacccatgacgaacgaaaccaagacagaccgccagcgccgcctggcgcgggaacgccaacgagcgaagcgcgagcgcgatgccctgcgccgcgctgcgctgggcggtcgccgcttcaacatggacatgtaccagggaacggctgatgcactcgatctgatctgcgcggccggtggcttcgccgagccggccgaggcggtcaccttgctcctacacaacgttgccgaaattgcagaacgtgacgcgtcacgctttgccgaattgatccaaaagagaagccatccagggaggaccaagcgatgagcctacgcgccgtcaacctcgcaaaaatccacatcgccaaggcccagctgggcatggacgatgacacctatcgcgcattgctcgctcgcgtcgcgggcgtgcgctcggccaaggacttagggccgcgccagattgaccaggtactggtcgaactccagcgtctgggctggaaaccgaagagcaaccggcaaggccgggcgacgccaaaagtgccgcaaaaccggcaaaccgtgctgcgcaaaatcaccgcgctcctggccagcgcccatcgcccctggagctacgccgaccatatggcccggcgcatgttccaggtcgagcgggtcgagtggctggacgacagccagctctaccggctgatgcaggcgcttatcatcgacaggagccgccatggccaggtctgaggtggatcttcgggaggtccaggacatgctgccggataccgtccgcgacatggccggacgcatcggcctgccggccacgctggtggtagtcgagcagctcggcggcacgtcctggcggatagccgagggccgggcgcggaggggcgaagcgcgccgggctgcgctggccgagctggtgggcagcgacatcgaggagcagctccacacgcactatcggggcgaagaaatttacgtggctcgctgccacaaggcgctggtacggtggcgcgatctggagatcgtcgagcgcttcgaacagggcttgcgtgacgggcaaaccgcccgtagcctgctcagcgatctagcccgccaatacaacttgtccgaccgctggatatgggagattgtcaaccggccgagcgagccggcaccgcagcaatccaccctgttccactaagccggggcgcaacgccccggccggcgtctccgcgccgaccctgtctcagccgttgaaccccttccgctaatcccgcgtcgcactcaccgccacgatggcggcatgagcacatctagccccccaacgtctctacgcagcccccgcgactacgccgccgccatcctggccgagcccagccgcgagcgtcgtaacgctctgctggaagcctgcccggtcaactggcagccacttgttcgggcgcacgtcgaggacgccttcgcgaaggtcaaggcgtatcgccagatgatggaccaccgcgccgagtcgatccggcgcggcccgcctccagctccccgcgtcaccgacaccgatttccgcatatccaactacaccaaatccgccccggaggtaggcaatgcgcacctatcagcaattcgggcagcgctcgcaacggaagcaccaaatgcctgatcccgcatccacctcggccggcagcgccgcgctgctgaaaatgtttggcatccatatcagcgcgggcgccctggccgccgccctgggcttcctggtcctgtggcccaggaccatgaaagaggggtttgcccggctgttctgcaccatcgtcgcgtccagcgtcttcggcccgatcctggtcgtttacctgcactccaaccgccccgagctgttcgagtccgcccaggtggtggccgggctctaccagttagagccggcagtcggcctgctgttcgtttccgctccgctcctggtgattgccggtctgcccgcctggtggctgatcggggcggccctgcgcctgtttgagcgggacggcgattcatggctgggcgcgttcgcccagtgggtaaaacgcaaactggagaacacctgatggcccttcaacctcgcggcatccgcaacaacaaccccggcaacatcgtctggtcggcacgcaacaactggcagggccagctcccgcacaacccgaaggtcgagccgcgtttcgcccgtttcgataccgcacataacggaatccgcgccttggcaaagctgctgctgaactatcgcaaggtccacggcctgcgcaccgtcgaatcgttgatcgcacgctgggcgccgtccaacgagaacgacacccgcgcatatgccacggccgtggcccgagccatgggggttccaccgcaggccggcctgcacatggaccaggacaccctggccgccctggtgaccgcgatcattcggcacgaaaacgggcagcagccctacagcgccgagcagatcgcccaggccgtgcgggaggtgctgtgatgcaacgcctgcggttggcagcaactaaaggccgcactctggttggcgtgatcctgatcgagaccggcctagccctggtgcgggctggtaccgggctgctgccgaggtcttccgaatgacctggcgcctcggcttggccctggccctgttcctggtgatggttgcgaccagcgcctggtggagtggtcgcgtggcgggcctggccgatgggcgcgccgcctgcgccgacgcacagacccgcgcctaccgcgacgtcctggagcaatcggcggcacaactgaaggcggtccaggacaccagcgcggctcttttccagcgcctggcccagcgggccgacagcgaccaacaaactactcgggagcttcgccatgccctggccgaaaccgctgctgatcgcgctgcctgccgctttcctgctggcgtcatgcagcagctcgaaaccgcccgtcaacgtgccgcccaggccactaccggcggccttggctcaaccgtgcccgaccccggtggcggtgactgatgacagccccgatgccaccgcaattgccctcaaacaactctacgaccaatacggcctctgcgccggactgcactgggacaccgtgcggcaccttcaaaaggactgatccgatgaccgaaaagaaagcctctcccgagttcgaactgctgcaacgcatcgacggccgcctggagcgcttcgaggaccgattcccgcagatcgagcgtaaggccgtgctgtacggctcggcggccggcgcgctggcgggtggcctggttgcctgcggcctgctcgcggcgcgtatcaagctcggtatctgaggtagtcatggcgcacccgaaggaaacccgcgacgccctgcgccgcgcctacgtcctcgaccgccagtccctggaggtcgcggccgccatgttcggcgtctcctacggcaccgcccgccgctggaaacagcaggcggaagccgagggggacgactgggacaaggcgcaatcggcgcagttgctggccggtggtgggctggaggacgtggcgcgccaggtgctggccggcctggtgacccagttccaggccacgatggaagccatccaggtagacgcggacatcaagcccgccgtgaaagtgcagctgctcgccagcctggccgatgcctacaacaagacggtcagcgcgtccaagcgcgttctgcccgaaacatcagcgctggccaccgctatggaggtgctccagcgcctggccagcttcatccgtgagcggttcccgcagcacgcccaggcattcgccgaggtgctggagccgtttggagaggtgattgcgaaggagctgggctgaccaacctattcgctgaaggggtcgtaccgactgacaaccacgggtccgctatcaggaatcttttcgacatgaacaacagaattgcaggggtgacatttcaaggccttgtaccagccatcattgcaaggctgaagaatggtcttgattcctttttggtagcaatcggcacatatgtgatgcagaggttcggtgccttgaacctctggctttatgcgatacacaagtccacccgcttccgtctggtggagctggtagcgctctttctcctgttcccagcgtttgaactgagcaatttcggcttccagctcgcctatgcggcgggtcagcgtcgtctgatccgcatgggcgctgttcagctgggattgcagcccgagcagcacgccgttcagttcgaccaccttggtcgttacagccgcatccgtcttgagcgtgagcatgctctgcgtaatgtcagtggccgccttgatgccgccgtaggcaccagcaatccagtccatcatgaccaggttccttctggggagaaatcgacccatgaagggtagcaccagagacttcctggcggatattgcccagctcgcgggggagttccgccgccagatcgaggccgaggtcgcaggcttcgaccccgacccgaaggccagcgccgtccggcgtgaacgggccagcgcggactatgagtatttcgcccggacctacttcccgcactacgtgaagcgcggtaacgcgctgctccacgactacctctacaagcggttgcccgagctggtggaccacccggacggccagcacgaagccattgcggcgccgcgtggtaatgccaagtccaccctggtgagccagatattcgtgatctggtgcgtactcaccggccgcaagcattaccccctgatcatcatggatgccttcgaacaggccgccacgatgctggaggcgatcaaggcggagctggagttcaacccgcgcctggccatggacttcccccagggcgccggcaagggccgcgtttggcaggtcggcaccatcgttacggcgaacgatgccaaggtccaggtcttcggctccggcaagcggatgcgcggccttcgacacggcccgcaccgtcctgacctggtgatcggcgacgacctggagaacgacgagaacgtccgcagcccggagcagcgcgacaagctggaaaactggctgaagaaaaccgttctgtccctcggctcggccgacgacaccatggacgtgatcatcatcgggaccatccttcactacgactcggtcctgtcgcgcctgctgaaaaacccgctgtggaagcggcgcaagttcaaggcgatcatcgaatggccgcaccgcatggacctgtgggagaagtgggaggaacttctgctcaactccgacgacgagggcgccgccgctctggccttctaccaggaacgcgccgccgccatggaggacggcgcgatcatctgctggccggatgggcagcccctctacaagcttatggtgaaacgtgcccgcgatgggcactcggcgttcgactcggaacagcagaacgacccagtccagggcgagaacgcccccttcgccgcctgcatcacgttctgggtcaaccgcctggcgcagtggatgttctacggcgcgtgcgacccgtccctgggtaagcaaggttccagccgcgaccccagcgccatcctggtgggtgggttcaaccgggagacaggcgtcctggacgtggtcgaggccgccatccgcaaacgcctgccggacaagatcatcgaggacatcatcgccatgcagcgggcctatcactgcctggtgtggggcgttgaggcggtccagttccaggagttcctgcgcaccgagctggtgaagcgctccgccaaggctggctgcccagtacctgcccgagcgatcacgccacacgccgacaagctactgcgcatcgaaagcctccagccgcacatggccaacggcctgatccgtctgcatccaagccagaccgtcctggaacaacagctgcgccacttcccggccgcagaccacgacgatggccccgacgccctacacatgctctggatgctggccacgacggggttcgcgccgatagaggcgactttggtcaaacgccggcatgaatacgcgcccggccttgacgattcttttgacactggcggccgcttcggcggcgcatggtaggtacaacacatggcacaaatcgttgacgtctacggcaacccgatccgaactcagcagttgcgcgagccgcagacctcgcgcctggccggcctggcgaaggagttcgcccagcacccggccaaggggctgacgccggccaagctggctcgcatcctggtcgaggccgaacagggcaacctccaagcccaagccgaactgttcatggacatggaggaacgcgacgcccacctgttcgccgaaatgagcaagcgaaagcgcgcaatccttggcctggattgggcggtcgagcccccgcgtaacgcctcggcggccgagaaagccgatgccgactacctgcacgagctgttgctcgacctggaagggctggaggacttgctgctcgatgcgctggacggcatcggccacggctacagctgcatcgagctggagtgggcgttacaagggcgcgagtggatgccgctggcgttccaccaccgaccgcagagctggttccagctcaaccccgaagaccagaacgagctgcggctgcgcgacaacagcccggccggcgaagccttgcagcccttcggctggatcattcaccggccgcgtgcgcgctccggctatgtggcccgcagcggcctgttccgcgtgctggcctggccgtacctgttccgccactacgccacctccgacctggcggaaatgctggaaatctatggcctgccgatccggctggggaaatatccgccaggtactgccgacgaggagaaggcaaccttgctgcgggccgttaccggcctgggacatgctgccgcagggatcatccccgaaaccatggccatcgacttccagcaggccgcgcagggtagcagcgagccgttcctggcgatgatgcggcaaagcgaagacgccatatccaaggcggtcctgggcggcaccctgaccagcaccaccagccagtcaggcggcggcgcttttgctttgggccaggtgcataacgaggttcggcacgacttgctggcatccgatgcccgccagttggcggcaacgttgtcccgcgatctgctctggccgctcctggtgctgaatcgccctggtagtcccgacgtgcgccgggcgccgcgcctagtcttcgacctgcgcgagcaagccgacatcaccagcatggcgcagtcgattccggcactggtcaacgtggggctggagattcccagcgcctgggtctatgacaagctcggcatcccgcagcctgccaagaatgagccagttctgcgttcggctgcgcagcctgcgatcctgagccgacagcatggacaacgggtggcggccttggccaccatcgttggcccacgctatggcgatcagcaggcgctggacaaggcgctggctgacctgccggcgaaggacatgcaaaaccaggccaacgacctgctcgccccgctcctggaagcggtcaaccgcggagacagcgaaaccgaactactcggcgccctcgccgaagcgttcccggacatggatgacagcgccctgacggacgcgctccaccggctgctgttcgccgccgatacctggggccgtctccacggcaacctggaccggatcgactgatggccgctccgaccgaagccgatctgcgggccatcttcgccctgcggccggccgccgctatcgagtatctggagcgcaagggcttcgcgatcacttggaactggcatgacgttgacgcggccacccacgcccgcgctctgaccgttgccagagcagcacgcctggacgtgctccaggacattcgcgacgccctggtcgagaacctggagcgcggcgagacgctacgagatttcaagcgcaacctgcggccgaccctggaggcgaagggctggtggggtcgccaggtggtagtcgcgccggatggcggcgccgaggtcgcacaactgggcagcccgcgccgcctggataccatctaccagaccaacatgcaggcggcctacatggcagggcgctacgcggccgcctacgaagccagggaaacccacccttactggatgtatgtggcggtgatggatggcgttacccggcccagccatgccgccctgcatgggaaagtgttcaggtgggacgatccgatctggcagcacatcaccccgcccaatggctacaactgccggtgccggatcgttgccttgacggaggccgctgtccgccgtcgcggcctgaccgtcgaatccagtcagggcaagaccggccaggtcaccgtcgaaaccggcgtggaccggcgcacaggggagattcgcgaacagaccctgaccaccctggagacgaccgaccgggccgggcggaagatccaatttcgccccgatgccgggttcgacggcagccccgtacagagtcacctgatggaccaggtgctgtacgacaaggccgagcgcaccctgggagccccagccgcaatcgacgaggtgcggggtgtgctgctggacccggtccgccagcgcgcctgggcggccttcgtagatcgcgccgcgtccccccaggggcagaccatgtccatcggcgtgctcgatccgaccgatatcacctacgccctagcccagggcgcccagttgcgggccggcgtggtcgccaccagcgataccgcaattcgcaacagtgctgtcgctcgcgagcagctcgccagcctgccgcagcgcttcgcccagcctgacctggtgctgtgggagcgcggcagcgagtcgttggtcttcatcgtccaggccgatagcgcggccctggctatccgtctgcgcggcgagatatacgggcccggccaactggaaaatgtcggccaggttatggaaatcaccatggatagcatccaggatggcctggcgacgggccgctacaggagagtgcgctagtgacaactaggatcgacgtcgagctggacgaccaggaggttcgccagcgcctggcgctgctgatgcgctcggtgaccgatacgctgccggtcatgcgtggcatcgctgccgagctgctcgcggaaactgagttcgcctttatggacgaggggccgggctggccgcagctcagccccgtgactgtcgccgctcgcgaggctaaggggcgtggtccacacccgatcctccaggtcacaaacgccctggctcgctcggtcacgacctgggcggatcgcaacgaggcgggaatcgggtccaacttggtctatgcggccatccaccaatttggtggcgacgccggccggggtcaccaggtcgaaattcctgcacggcggtatctgcctttcgacgaaaacggccaactggcggccggcgctcggcagtcaattctggagatcgtcctaacagccttgagccgaaatcggtagtggccactttcggacaagcggcacattgtgcctattgcgaattaggcacaatgtgcctaatctaacgtcatgccagccacaacggcgaggcgccaagaaggatagaagccatgatcaccacaaagactgtcaatggcgtgcagatcgccttcgatgaccaggggcatgaaccaggcccggtgttcgtcacgctgagcggttgggcgcacgatcttcgcgcgtatgacggcatgctgccgtatctacgggcagcgcagcggacggtccgcgtatgttggcgcgggcatgggcccgatcggaatctagttggcgacttcggtattgacgagatggcggcagacacgatcggcctgctggatgcgcttgaggtggacagtttcgtaccaatcgcccacgcgcacggtggatgggcggcgctcgagatcgctgatcggctcggcgctcagcgggtcccggccgtgatgatcctcgatctcatcatgacgccagcaccgcgggagttcgttgccgcgctgcacggtatccaggatccagagcgctggaaggaagggcgtgatggcctcgttcagtcgtggctggcggggaccaccaatcaagcggtgctggatcacgtgcgatacgacagcggcggtcacggttttgacatgtgggctcgtgctggccgggtgattgacgaggcctaccgaacctggggatcgccgatgcggcgcatggaggctctggcggaaccgtgcgcgatccggcacgtgttctcacatcccaagatcggggagtacgacgcacttcacgacgatttcgccgcccgccatccatggtttagctaccgtcgtctcgggggcgaaacacacttccccggcattgagctgcctcaacaggtggcggccgaagcgatcgatctgcttgctggcgcgcgcatctgagttatgaagcctgacgcctctaaccacaacccagacccgcgctacctgcgcgggctgctcaagaaagccggcatcagccagcggcgcgcagccgagctgctcggcctcagtgacagggtgatgcgctattacctgagcgaggacatcaaggagggctaccgccccgcgccgtataccgtccagttcgccctggagtgcctggcgaacgacccgccatctgcgtgatcacctgatccgcccgcaaacgcgctacacgcgccgaaacggggttagacgctacctcgctcagagtcggtgcgttaaccccgttagagccccgttagaaatcgctccagcgccattcttgtgccagggtttggccagaagatggcgccggacggtttccgcagtcgttgaaccccttcatgtgaccgctgctttctaccgtcgccaccattggcggcatggaaaagaaccgcctactcgttgccatcgccgcctgctcgttccagcttccccagctggaggatggcagcgcctggattcaagtcactccagctggtgagttccggcccacggacgggcgccccatggacgtgccggcctggcggatcgatgccgccagcgccgccgccgtgatcgaccgggccagggcacgcaagacaccgcctgtcctggactatgagcaccagaccctcaagaaagaggaaaacggccagccggcgcctgctgccggccgcttcctcgatttcgaatggcgcgaaggctccggcctgtggggccgtgtcgaatacaccgcccgcgccgcacggatgatcgaggacggtgagtacctctacttctcgccggtcttcagctacgccccggacggcacggtcctgtcgattctgatgggcgccatcaccaacgaccccgccatcgatggcatggagccgctcgcccgccgagcggcggccacctttggcctttaccccacccaagaggaaacctccgtggatgaactcctgaaagccatcatcgaggcgctgtcgctcaaggaaggggcgaccgaggccgaagccatcgccgccctgaccgcgctcaagccggccttggacgcacaggcggccagcctggccacgctgcgcgaaaccctcggcttggccaaggacgctagcgtcgagcagatcgccgccgccaccagccaactgaagaaggccgacccgagccagaaacccgacccggccaagttcgtgcccttggaagctgtgacggacctccaggagcaaatcgccgctctgaccgcacgcctcaatggtggcgagctggacaggctggtcggtgctgcgctccaggacggtcgcctgctgccctccctggagcagtgggcacgcgacctgggcggtaaggacatcggccagctcaaggcgtacctggacaaggccgcgccgattgccgcgctgacccgcctgcaaggccgccagccggagggcgacacccacaacctcaccgacgccgagatggaggccgcccgtctgaccgggatcagccccgccgactacgccaaggcaaaaggagcctgacccatggccatcattactccggcgctgattagcgcactgaaaacctcgttccagaagcatttccaggacgccctggcgacggcacccagcacctacctccaggttgccacggtgattccgtccaccaccgccagcaacacctatggctggctggggcagttccccaagctgcgcgagtggatcggtcagcgtgtcatcaaggacatggcggcccagggctaccagatcaccaacaagctcttcgaatcgaccgtgggcgtaaaacgtaccgacatcgaggacgacaacctcggcgtctacggaccgctcatgcaggaaatggggcgcgctgccggcgcgcatcccgacgagctggtcttcgccctgctcaaggccggcaacgccaatctctgctacgacggtcaaaacttcttcgacaccgatcacccggtctatccgaacgtggatggcaccggcacggcgaccaccgttagcaacctgttcgcgccggccgctgatccgggggcggcctggtatctgctcgacaccagccgcagcctcaagccgttgatctaccaggagcgcatgaagccgtcgttcacttcgatgaccaaggaagacgacgagcaggtcttcatggccgacgagtaccgctacggcgtgcgctcccgctgcaatgtcggcttcggtttctggcaactggcagcgatgtccaccgaagagctgaacacggcgaacttcgagaaagtttacgacgccatgcgcaaccagaaggccgacggcggccgtccgctggacattcgcccgaacctgctggtggtgccgaccactctgcgctccaaggccaaggaagtggtcggggtgcaacgtctggccaatggcgcggacaaccccaacttcgaactggtccaggtactcgataccgcctggctcaactgatagccccagacggaacgcctgccaggccaaggatggccaccttcttccagctacaggagacacgacatggcacgccagaactctgcggccaagaccaccgccaaatccaagaccgatccggcgaccgaaaagcccaaggacgaagctctgccgggctccacggatgccacttcgtccaccgcacccgaggcgcccaccgccaaaccagccagcacctcggacgagatcgagggcgtcttcattcgggccaccgttgagcgccgctgtcgagcgggcttctgcttcgacaaggaaggccaaggcttcgctgaaggcgtgctgagcgacaagcagttggaggctctggagtcggacccgctgctcaaggtcgagcgctgcaccttttccggcaaccaggagggcgagtgatgaatcacgccattgcccagttggacatcgccgcgcagatcgccgagcacaacgctccaatcagcgaggctcagggtgacgccgctcaggccgagttgcagaaccaggttgccgccgactgccgcgaggcgctcgacgtcctggaacaattggagtcgccgctgtgagctactgcacgctggccgacctgatcgagcagtacagcgagcaaaaaatccgcgaggtgagtgaccgcgtcaataaaccggccacaaccatcgacacggtgatcgtggatcgcgccatcgccgacgccgactcagaaatcgacctgcatctgcacggccgataccagttgccgctcgccagcgtgccaacggcgctcaagcgcattgcctgtggcctggcctacgccaatctgcacatcgttctaaaggaagagaacccggtctacaaaacggccgagcatctgcgaaagctgctgtcgggcatcgccaacggcaagttgagtctggccctggatgctgacggcaagccggcgcccgtagccaacacggtgcagataagcgaaggccgcaacgactggggggccgactggtgagcgacccgttcgactacctgttcctggaaccgttgctgatcgagcgtatccgctcagaggttcctgggctggccatcgtttccggggtgcccgatctggcggccttgagtgagcaggaccagcccgcccccagcgtctatgtcgtctatctcggcgacgagataggcaccggagcggatcaccaggggggcaggcgcgccattcaggctatcggccagcaatgggcggttgtgctggtggtgcattacgccgactcgtcgaactccggcgaaggagcgcgccgagaggcaggaccgctgctgggacggctggtcaaggcactgaccggatgggctccagccatcgatgtggctccgttggcgcgcagcgcccgacagtctcccgtcacctacgccagcggctacttctatttccccctggtgttcaccgccaggttcgtctacccgagggtcaagtcatggaaaccgtaaaagtcacgatcactgctgagaaccccaaccacacccacgcgggcaagccggtggccaagggcgacgagatcgaagtcagccgcgccgatgccgagtttctgctgcgccgtcaattgatcaccaagattcccgccgagcccaaggccgacgagaaacgcgacaagtaacgcgcaacatctgattcctacggaggcctcacatggcacaggaaacgtatttctacgggcaaggtgagattgacgccgcgcctatcgtcaacggcgtcctcggcaaatggcgctggattcaggatgtctcggccatgagcatccagctcgcagtcgagaaggtcgagcacaaggaaagctacagcggccagaaagccctggtccgaagcttccccatcggcaagaccgccaccgtcagcatgaccttgcacagcatcgacccggataacctggcgctcaccctctatggcaaggtcgtgactaaggcggccggctctgtgacggctgaggcgctccccgccgacctggtagctggtgatgtaatccgcctggccaatccgggcgtcagcgagctggtcatcaccgacagcgcgagcagtccggcgcccctcgatccgcagtattacgccctgcgagccgatggcgcctacggcgaggtccaactgctgggtctgccgacgccggccccgacccagccgttcaaggcggcctatgagtacgcggcgactcgccaggtgggcatgttcaccgcgccgcagccgaccatcgccctgcgctacaagggcatcaacctggccgaaggcggcgcgccggtcatcgtcgagctgttcaaggtcgcgaccgacccgctccaggaactggcattgatcagcgacggcaacaccgtcgccggtatgcagatcagcggcggaatcctgctggacaccagcaagccggataccggcgacctgggccgcttcggtcgcattatccagctggggtaaatcatggccaggaagaagcctgttaaccctcgcggccagccggccgactcggcgcccgacgacagcctgagcgtgctgtttcctgaccgtcagttggcggtcgggggcgtcgaggtgacggtgcgcgagctgaccttcagcgagcaactgcgccataaccacctgttggccccgctggccgatgccctggcggcagttcccccggagcagctcgacggacctgagtcgatcaacgtcatcttcgacgctctggcccggcacgccgacgcgctgcgcgagttgctcgcgatcagttgcggccaatccgtggactgggtggacgcgctgccggcagacgacggcgaagcactggtgttgacctggtggacggtgaacagtggttttttcgtgcgaaggctctggcggcctcgcctactggcgatggcattgggcaaccgacgccctggagccgagtcttctccgatctcgtccgcgccggccactgccgcgaaaccctaggcacctataccggccggcaactgattctgtactggaacgaagcgcaggcagctgaacggcgagaacaggcgcgccacgttcggtcggtgatgttcggaatggctggtggcaaggacgccagcgccttcctcaacgatttggaatcctgatggccactaatcagcaactctcgatagcactacgcatccaggctgacctggctgaagcgcagaacgcgctcagacaactaacgggcaacctccagcaggttgaccggggggcggtgcagaccaggagcgagctgtctgcgatgggtgggcagttggacagccttcgcgcacaggtgcttgggtttgtcggagcttgggctagcttgagtgcgctgggcggcctggtgaccatggttgaccaatatgggcaaatggccgaccgcatccagatggtcaccagcagcacggccgaatatgaacaagtgcaggcccggctgctggagacggccagccgcacctatcggccgctggcggaagcccaagagttgtacatccgcaccgccgacagcctgaagtcgttgcggtacaccaccgaacaagcgctggacatcaccgattcgttttccttcttgctggtaaccaacgccgcgtcggcggaccgtgcggcgagcgccatcgacgcctactcgaaatcgatccagaccggcaaggtcagctctgacgcctggcagtcgatcatggccgccatgcccagcctggtgaacgccctggcagagtccaccggcaagagcaccgaggaaatccgcaagctaggcatcgagggcagcctgtcgttgcgcgacctgaatgaagggctgcgcaagaccgtggcggcgaaccgcgaggcggcggacaacatgggcacctcggtccaggacgcgctggtcagcctgaacaacgccctgagcgcctacctgggcgagctgaaccgcacctatgacatcaccggtagcgtgtcctcggcgctgaacgtgctggccgagaacatggaggttatcgtcaaactgtttggggtcgcggcggtggcggggctgacccgctacgtggccagcctaacgctggccacccaggcgaaactggcggcagtgctggccgctcgggcgcaagccgctgaagaactgcgggcagcccaggctcaggtcgcttcgacggcagcggcagcggccaatgccagggcacaggcgggcctgacggtgagccatgctcaggcggcggcggccgaggcggcgcataccgccgcgacccagcgccttgctgctgcgcagttggcggccggcaccgcgatgcgcgggatgctggccgtgatcggtggtccggccggcatcgcgatgctggtggccggagcggcggcaagcttcttcctgtttcgcgatagcgcccaggcggtcaagagtagcctagatgacctgagtgagccgctggaccaggtcgtcgagcgcatgggcaagctgagcgagattgagcaagatcgcgaactgacccggctttccgagcagatcgacggattgcggcagacggctgtggaagccgcccgcgaaatgcgagaggtggccagcaccgccctctatggtgccaggctggatcgtatcccgtctgccgaagcacagcaggccctccagcctctaatcgatgcgtcggctgacgctgcgcgaggcgtggaggtggactggaagtcggtgatggactccctggctgccagcggcgctgttcccgattcactcaagcgcaagctgctggacatggcggctggtcaggcagaggcaggccgtactgctaccgagctggggcagcgtcatgcggaactcaaggcacgcctggagggttcgactgccgccatcaatgagaacagcgatgcactgagtaaagggtcggacaaggcagccgagtatatccagtccctgcgcctggccatcgccgacctggaagatccatcggtcctgggcaaggccggccgtcgcctccagcagttcggggccgacctcaatgccgagcagagtgccgaaatactccgcctggagaccctgaaggccaataccgaaaaggcggcccaggcccgcgaggatgcacggcgcaaggctgaatccagtgcgcgacaacaagcctccacggctgagcagttggcgaagagccaggaaggctatgttgcggggctggaaaagcaagcccgcaccctgggtctcaccagcgcagaggtgcgggcctacgagctggccgagaagggtttgaccggagccctccaagctcgggcagcggcagcacttgccgccctcgcggcggacgagaagaagcggcaagccgacgccactgcgcgcaccaacgccggactggaggccgaatatctgcgggcgaccggccgcaccgttgacgcggggctgctggagattcggacgaaatttgacgcgatgcgtcgtgacttcgaaaaggcgggcaacgacgccggcctggcctggatcgacaagctaatccccgtcgccgaggccaaggtccgcctggatgacgtcaagcagcagatggacgatttgctggccgaccagcaacgggccgagtcgtccgttaacgtccagcaggatgccggcatcatcaacgaaatggacgcccggcagcgcatcctggacattcaccgagcgacctacgagaagctccagcagattcggccgatcctagagcagatggcccgccagcctggcgaggtcggccgagccgctgccgaatcgctcgcccaactggacgccgaggcggcgcgactccagcagaccacgacgctgctcgaaaccaccctacgggacggcctcaccagcggctttaccgacgccatcaaagggctcgcttccgggaccatggacttgcgcgacgccatcacgtcgctgggtgaagctgtactcaatgccttggtgaacatggcggcgcagaacctcgcgcagtcgttgtccagcggcatcatggggctgtttggtggcggccagcaggacaccagcatgactaccggcgcggcggctgtgaccgcgtcggccggtgccctatcgactgcgggcgcctcgctgctgaccggggccgctgctatccagacggccgctgcgtcgctggcagccgccaatggcgtccaagggctgggcgctgctgcgggtggtgcgggtgcggcaggagcggcagcgggcggcggcagttggtggtcctccatcgccggcgtgttcggtttcgccaccggcggccacatcaagggaccaggaacaggcacaagcgacagtatcccgattctggcatccaacgacgagtttatgacccgcgccgcagttgtacgacagcctggcgccctggcatttctcgaacagttcaaccgctacggcatggccgcgctggccggctgggcgaaccctgtccgtcacgcaaccggcggacagatcggcattcccgctcccaatctgccggctcccgtccgtggcggcgcgaacctgcccgagccctccaaaaacttcagtacctcggtcgctaactcgatctacctgcacgccgttcaggaccccgaccagatggcggccgaaatgtgggccggcaagggcggcgaccattacatcgtctggctgaacaagaaccgccaggccgtcaagcaaatactcggaaactaggaattcatggctactgaaatcggcaccgccacgaaccaccagaacctggtcgagcgcctcgtccagttcctcaccgcgaacccagacctggtcgcggctgggcaggcctacgagaaggttttcgacaacaccatccccgcgtccggcacggccatcgccgtgcgccaggtgaccctgcgcgccccgggcctgggcggcaccgacagcatctacatggggattcagagctacggcgataccgccctggactactacaaccttcgcctgatgggcggcacggcgttcaatcctggagcaatcccgcctggcggcgactactggaccgcgtttgccaactacagtccgcgggttcaggcgctgctgtggaaccagcccatgccgtactggttcttcgccaacggccgacgcttctgggtcgtcgtgaaagtctcgacgatctacgagtcggccggcgccggcttcatcctgccaccctgtccgccgtcgcagtatccgtacccgcttgccgtcgtgggctcctaccgtggtgacgttgcaactcgctggtcagacgtcagcgaccggcacagaggcatcagcagcccctacgagcgtagctgctatctccgcgatcccgccgggcgctggctcggtttcactgtcgcaggccgttcaagcaacgagtccgactacaacaatcggaccctgctgccgcttggctgcggtcgctatgcgggtggtagcgacactgtgatcaaccagctccgcgactctttcagcaagttcccgctgaaagctttgcagttcgtcacccgcgaaaccgaggggcgccgctatctgggcgatttcgacggcgccttctacgtgccgacgctcaactccggcgccgaagacgtgattgtcgaggacggtgtggaccacgtcgtttttcaaaccgcttggcgtagcggtaacccttggctctacgcgatcaggaaggactgaaatggcttacttcacaggaacagcgaacaacccggccgacttgctcgccaagctgcgcgtccacgccgagtcgctcggctgggtcaccgaccgcgcctcggcatcggaatggctttgtcacaacgccgacggctactggtcgttcaacgccggttccaatcaatggcagctcgcgggcaatacggggttcgacgacgggcttgcgtggaatgcgcagcccggcaactcggtgcagaacaacccgtattcgtcgaaagaagcaaccatagcgcagctcagcgccgggccattcacgcgctatcacctgttcgccaccgctgcctatctgcacctgcacgtcgaaatcgctgccggtcagtttcgtccagtgatgatcggctccctcaacaagcgtggcgtcggctatacgggcggccagtatgtttgcggctcgttcctctacagctctggccaggcgctcacaaacaactggtcatcgcatccattcgatggttaccacattcgatacagcggcggcggcagcatgctgcggctagacagcctcgacggtggcccatcgccggagtggttgccgttcgactacacaacgaacgtctcccggcgcgtcgtcggccccggtcgcggaaactacagcagtcagtaccatcccgacgtggggctgatcgacgcgagcgcaaacgagctgaacagctcgaccacccctgtgccctgcgccatctatgcgttcggcgctcagcagcgctcgcggtacgtgggcgaggtgccggactttggcatatgcaacatggcgttcctcgcgcctggcgatccgctggtgatcggcagcgacacttggcgcgtctatccgttgctccaacgcggaagcgctaccgatttcggcaacaccagcgcctgggtcggctactgcttccgggtgcttgagtaatggcgacgtttccggggttccaggtgccaaagccgctcgtggggatcgttgccggcatcacgccgaatatcgacgccctggagctgaaccaggacatcagcctggcagcggtcgcggcctcgacctgggccggcgcctacgcggcgcatcagccggtagaggtgatccattcgacgtaccaggctgtccaccaaagcgctctggaagagaactactacaaccgcctgtggctgatccctacgaccatggagctgggcaacgtcgtcagcacccaggtacgaccggcatcagtctggaacgcttatttcagtccgcgcacgctgaccgccatcgagcgggaagatgcagacggcatcacgctatccggccaggcgtcgccgccgctgggttttgccgccctggaggaacgcacttggaccgtcagcattggcacggacggcccgcccgtcgtcaatgcgcggatcgtctggacgctccagggcgagccggacctggtcctggtcatcaccggcaatcgcatcatcgcctggaccttcgcgccggactggggcgacagcatcgtcgagcgcctgagcgcctcgacaaatatcctgcaaagcgaatcagccgtgacccagcgccgggctatgcgcctggcgccgcgccgggagttcgaagcgaacatgtacgcggtagaccgcgagcggcagctcctggacatgacgctgtttggctggggcgcgcgaatttgggcgctgccgatttggcctgatatccaactgctccaagaaccgctggcggccggctcgctgaacattccgtgcgacacggtcggcctcgacttccgcgacggcggtctggcgatgctgcgcggcgaggacgccttcacctatgaagtcgtcgaggtcaaggcagtgaccgccgccggcctggacctggtccgccccgtccaggccacctgggtaactggctcgcgactgtacccggtgcgcaccgcgcagctgaccgaacagcccacgctgacccggctgaccgataccgcgcagtctgcgcgggtgtcgttcctgataatggagcccagcgcctggcccgaggtaatgccggcgacgacctacagggggcggccagtgctggagcagcgcccggacgaaagcgaagacctcacctccagctatcagcgcctgctgtccaccctggacaacggcagcgcgattccccgcgtgaccgacgtcgccgggatggcgctgcccgtcatcggtcatcgctggatcggcatgggccgagccgagcggtcggcgttccgcagcctggtctatgcgctgcgaggccagcagaagccgctatgggtgccgacccacgccgacgacctgaccctagtcgccaccgtctcgcagctgtccactgcgctggacgtgcgcaatatcggctatgcccgtttcgccaatgggcgaccgggtcgtcgcgatatccgcatcgagctgtacgacggcaccgtctatcaccgccgcattctcaccagcaccgagctggacgccgacaccgagcgcttggccatcgacgccgccctgggccgcctggtcgagccgaccgatgtagcgcgcatctgtttcatggcgctctgtagcgccgccagcgacgtggtcgagattgagcacgtcaccgatagcgagggcgtcgcaaccgccgcgctgacattcaaaggggttcgtgacgatgagttttaacagccgcgaaagctcgctcgcggatgggcagccggtgcggctgtaccagttcagccgtggcgcgatccgctggagctacaacagcagcgaccgggacatcacctaccagaaccagattttccgcaccgtgccgggcggcatcaccgacaacgggatcatctgttccggcgacccgcagtccgatcagttcatcatcaccgcgccggccgacctcgatgtcgcgctgctgtacaaggccaaatcgccgagtgatgccatcgatctggtcgtctacgacatgcactacggcgatgtcgaggcagcggtttcctgggtgggggagattggcgacgtggactggccgaccgtggacagcagtcgcataacgtgcgtgtccgaagacgagctgatggaccagccaggcttgatcgataccagttgccgcacctgcacggcgaccttgggcgaccaccgctgcaaggtaaacctcattccgtatcgagtgacgctgacaccgcagagcgtgtccgcgtgggtgatttccagcggagtggtcgccggctatgccgacggctggtttaccggtggctatgtggagtggcaggtggacggcgacaactacgaccgccgctacatcgagcggcacgccggggccgatctgcacatcctgggcggcaccgagggcgtcccggcgggggggcaactgcgggtctatccaggctgcgatctgctcgatgaaacctgcgccggaaagttcgacaacatcctgaatttccggggctttaacaagatgcaaggcaagtcgccattcgatggcgaccaggtctggtgaggtaggccatggacccgatcacaatcaatctcgtcattctggctgcgtcgttcatcctatccagagccttggcgccgaagccgcaaaagcccaagccaacagcgtttgaagacatcgatttcccgcgctgcgacgagggcgacgaactggccgccgtgttcggtcagtgctggaggaagtcctggatggtgctgaccgtaggcaactaccgaacgaaggcgatcaagacaaaggggagcaagaaatgatcgttacggctcagcacttacatacggtcccgacctggaccactcggcagggctactgccatcgccaggcgcgggagttcttcaagcgccatcacctcgactggatggcgttcttacgggacggcatcgaggccgatcagttgattgcgaccggcgacgcgctcgcgctcaagctggttgagcacgcacgccaggaggtggctgatgggcgctaaacccaaggctcaaacggtcggctttcgatacttcttcgacatccatttcaccctaggcaagaaaatcgacgagctgtgcgcgctccgggcaagcggaaaaaccgcgtggaaaggatcgatcactactaacggtcaggtacgcatcaacgccccgaaactgttcggcggcgacaagggcgaaggtgggctcgatggaacgttggatatcctgttcggcgaagaagaccagggtgtcctgccgcgcctggcggccatgctcggcggcctggtgccggcgttccgtggcgtaaccacagggttctattccggcttggtaacctccatgaacccctacccgaagacatgggaatttttggtccggggaggaaaccgcttgtgggacggcaatccctggtatcccgaaaagcagttcatctggctagcggacggtcagatcaaggcgatgaacccggcgcacatcctttatctcgtctacaccggccgggacttccggggactggcccgcacgcgaatggacgaggcgagctggcgggccgctgctgacaagctgtatgccgagggtttcgggctgtgctttgaatggaccaggtccgacacgttcgccaacttctgcgagacggtgaaatcgcatatcggcgctgaggtttacccgaaccgtcagacgggacagatcagcatccggctcctgcgggacgactataacgtcgcagacctgccgctgttcgacgaggacagcggcctcctggaaatcactcaggagaagaccggctcgacctccctggcgccgagccagcttatcgtgaaatacatcgaccagatcgacggggcgcagcgccaaatcatcgtcaacaacaacgcggtcgctgcgtcgcaggggcggcgctcgtctgaggaaatcgagttcctgggcgtgcctaccggggagctggccgggcgagtcggtgagcgggaaatgcgtctgaagacaaccggcctgaagcgctataagggcgtgttcgaccgccgcgcccgtagcctgaaccctggccagccgttccgcatccgttcgacccggcgcggcatccctgaaaccgtcgttcgggtcggccggatcgaggacaacttcctcggcgacggcaagatcaccctgaccgtcgtccaggatcagttcaatctgccggcgacaaccggcgtggcgccgccaccaccgggctggattccgcccgaccggacgcctcgggcgatcactgtgcgccgcctgatcgaggcaccctatcgcgaactggccggcgtgatcgatccggcaaatctccagctcctggacgtgagcgcgtcctacttggccgcgctggccgaggcgccgaccagcctgtcgcagagctacacactgaccgaccgcgtcggcagctctggcgcgttcgttgatcgcggaaccggcgactggtgcccgaccggactactcgccgccgagctgccgctggcggccggtccgaacgtcgtcacgttgacgaacgccagccggctggaggacgtcactgtcggccaggccgcagtcgtggacgacgagatagtccgggtcgatgcggtcaactacgccagcggcacggtcaccctcgcgcgcggctgcgccgataccgtaccggccaagcatctggccggggctcgggtctggttctacgacacgttcgaagctgtggacgaaacggtctacagccagggcgtgacgctccaggcccggctgctgacgaacaccagcgagggccaactggccccggcgctggccgccaccgacagcctcaccctgaccgggcgccaaggtaagccgtatccgcccggccagttccgcatcaacggcagcgcgtacccaacgaaagtctacggggcgctgtcggtgagctgggcgaagcgcgaccggatcggccaggccgaccagttgatcgataccacggtcggcaacatcggacccgaagatggggcgacggttacgctcctggtctacagcggtacgacgctgaagcgtacctatgccggtctcacatccagtaactggtcctatccgctggccgaagacatggcggatggcccgctccaggacgtgcgccttgtcctgcgcagtgtccgcgacggcatcgattcttggcagcagcacgacatcacgattgaacgccacggcctcggtttccggcttggcgaagaactaggaggcgtatccgcatgagcctgacaatggggccgaacactggcttactgatcaacggcgcccccggtgaggggcattacagcgaactgatccgcatgttgcgctgggatgacttcctgcgccaaccggtcgtaaaggggcgggtcgcaacgctgccgacttccggccaggccgagggcgacacttacattttcaccggggccggggcgaaccagaaccgcttggcccgctggtgggcgactggtgcgtcaacgccaatctgggagtacatgccgccacggctgggctggcgtgtccaggtcgcaaacgagacaaccccggcaggccaggtcaagacctacgagtattccggcagcgcctggactgagctggtgggcggaatggccgacgcgccgagcgacgggaagcgctatgcccgactaaacaacgcgtgggcaggcttggggactgctgccgtcgccgatattcttgggccggtctctcaggctggcggtgtgccaactggtgcgatctacgagggcggcagtaacgcgaacggaagttacgtcaggctcgcagacggaacgcaaatttgctccagcagccttttaacgtttactgcgggttcaacgtcggtgggtgcgtcttggacgtttccggccagctttgtgtcgccgtcgctgatgtttggcaccgttgtagcatcgggagccggcgcagactatgaccccggcgtcgctgcgaggaacctgggagctgtttacttcaatgcgtcaacaaactctgctgcactggggtttctttgcatctcgtctgcatcgttcaccgctggcgcccaaactcgaaataaccgtgctgtcgcaattgggaggtggttctgatgatcatcacgttgtcgccgtatgtcgcgctgcccggcagcgatgaacatctgatgctgagcaggactggcgatgtactcaccgtgaacggccagtcgttcgatttcacaccgctcccggagggcggcgagttgccggccgaggctatcgggtcggagtggttcgctggccccgtcgttcgccgtgaggggcgtctagagttcagcctgcggctgccgctggctgacggcgctagtgcagccgctcgctttcctgaaccaatgctgatcgaggccgacggccctgtggagttgccgcaatgactattgactggagcatgttgaagtcacccgaagaccagcaggttgagcagcgggaggccatcagagcgcagcgccgccaggcctatcgcaccgagtccgacccgctgcgcctggaggccgagtttgacgccatcaccgctggcaccaagccggacctggcggcatgggttgcagctgtccaggcgatcaaagcgcggtatccactacctgaataggtagttgtgatggcgttctcgtttttgccacgttccgacagtctgatgtcgagtagtagataggaaccttgggatggacgaggtactgaggcaaaggttgcgggctgaactactggaagtggggtttctcaaccagtgctgccttgatctcatggaaagcatggaggctgagttcagtctcactaaggaccagcgcgagtgcattgagcagctcagccaattcctacgggagggcatcggcaaactgaccgctctgtctgaacgggtagccgacggcgatatcgtcgtcctgtgctgatcttttgaaattcttttgccgctggcgaaacggttagggcgcgtcatttattgcgcaaatcggcgccaaatttcgcgccgcgctaca

SEQ ID NO: 15 - DNA, 49139 bp, synthetic construct
  source 1..49139: mol_type = other DNA
tgcgcaagccagttgcagctggcttgcgcgtatagcaatacgtggagacctgagtatgagttacagagagagcattcgcaagtccgtgcgctttgaggtgttcaagcgcgacaacttcacttgccagtactgcggcgccaaggcgcctgacgtggtcctgcatgtcgatcacatcaacccggtgagcaagggcggcgacaacgagatcatcaacctggtgaccgcctgcctgccctgcaatctcggcaagtcggatcgcctgctgtcggacacctcaatgctggatcgtcagcgggcccagttggaagacctgaacgagcgccgcgagcagctggaaatgatgctggcctggcgcgatgagctccagtctttcggtgaagagaccgtacagctgattgccgatcgcatcaccgcgcgcatggtcggccactcggtcaacgagcacggcaagacggtaatccgcaaatggatcaagaagttctccgtcgaggagatcctggacgccctggacatcgccgccgacaagctcagcactgcgcccgatcaggaggaagtgctggagtgcttcgatgccattcctcgcatttgcgtcacccggcgccttcccgaagcaaagcagaaaatgctctacgccagaggaatcctgcgccgccggatttatgtcaacgaagctcacgtcatgccgctgatggccaaggccatcgaggcgggtctcgaggtggaagagctgatcgaatttgcgaaacaagtgaagaactggaccgaattccgggcagagatggaggaaatcgcaaatggctagggcccgcaacatcaaacccggaatcatggcaaacgaagacctagcagagctagatcctctcgctcgcctgctgttcatctacctctggatgttggccgatcgggaagggcgccttgaggatcgcccgaaacggatcaaggccgaggcacttccctacgacaacgtagacgctgacttgatgctggatgatctggccaaggcagggttcatccatcgctatgaggctgccggggtcaagctgattcaggttcttaactttgccaagcatcagacacctcatgtccgtgagcaggccagttctctcccgggcgttgacgcagaacacccaaagagagaacaaggcacaaccaaggaagtgcctggtcacaaccaaggctgtgctgagcaatcgccaagatcgcctgattctctgattccggattctctgattccagaggaagagcatgtcgacgctgacgcctcgacccattccgctccgcagcaagcagcagagcaagagcctggctccggccagaccgcacagctgttccagattgatcgcatcccttacgagaagatccgcgacctgtacaaccagatcctcggtggaaagctcaagcgctgcatgggagtgacggaggctcaccggaagcacatccgcgccgcgtacaacctcaagctcgatggcgggttcccggtccgtgacggtggactgtcgttttgggaagggctgttcaacgacgttctggattgccccttcatgctgggcaacaacaaccgggggtggcgcgcagacttcgagttcctgacaaccgccagcaagatccagcgcttcatggagggcaagtacgatgccgcatgagcgtcctctggtagcgatggaagctgagcagggtgtgcttggcgcgctgatgaagaaaccggaactgtgcgaggttgttggggctttcctttccccgaccgacttcagccatgccgacaactcggtgatctacagcctgatccttgcctgtcattcgaaggccatcgtgcctgacccgctttctctggcggaggctaggtcggagcttccaagtggcgcctttacgcttgcatacgccaacgatctatggcgcgaggttgcaagcacagctagcgccgaaaacttcgccaggattgtcgtcgagcgtgcaaaggctcgggagctgtacgaagcgggcgaacggatcatgaacatcgcccttcagagagggaaaatcccggaccaggtggctgaagcgcagagcatcgttctcgatctcaacgcccaggacgagactcctgatgtggtgacactgcgcgaggcaatgctcccagtcttcgacgaaatggaagttcgctggaagggaactcagtcggtcggactgaagttcaacctgccagacctcgatgccgttatccagggattgcgtcccggcaacctggcaatcatcgctggtcggcctggcacgggtaagacggttctcggggtggggattgctgacgaaattgccgttcgcaaccggggcgccgcgttgatcttctcgctggagatgtctcaagccgaacttgcaaagcgctcgctcgcatcgctttctggtgtttcgcaagcggcgatcgactcaggcaaagcgctggagtgccaggactctattgcgcgcatgactgccgcagtggaccaagtctccaggggtgatgtgcgaatttgcgacaagggaggactgactttcagtcggatctgctccatcgcccgattccagcatcgagcaaagccgctgagcctgatcgtcatcgactatctcgggcttatcacctcagatccgagtcaccgtcatcagaaccgaaaccaagaacttggcgccataagccgagggctcaaggctctcgccaaagagcttggcattccaattgtcgcgcttgctcagctcaatcggagcatcgaaacccgggccgacgccaagccaaaaatgagcgacctgcgcgattccggcgagatcgaacaagacgccgacgtgatcatcatggctcaccgggatatgagcactgagcgtggacagaacggtatcaccgagcttgatgtcgtgaagtgtcgacacgcaaagccgggcttctgcctgttgcagttccagggtgagttcgcgcgcttcgtcagttgcgcccaggaccgggaagagcagcaggagcagacggttcgtccgcagcgtccttccgcgcgatcaatggtagctgacttcaagccgcgaggtgcccaatgaaacgctccttgaccgtaatcgtaggcgccaagcgcttcacgatgattctgatggaggactgcgacccgctcgcggtcgtgaagagcatttggccgcaggggagggttgaggcatgaagaccttcgaactgatccgcatggaaggcctgcgcacctacggtcgccagattgaggccaatacctggcgcgaagccgagatgcaatgccgcgacggcgagatcgtaaacggcgaactgatcggtgtgtacgactgtgacccggtaactgaggccgtctgcactgcgcgcaatgacgtgatgattgatagcttgggggtgtgctgtggctgaccgcactttccgcatccaaggcgctgccggcatccgtccggctttcgtcgcggcctggaacctcatccaggggctgatgaaagaagcacagggtggctacgagctggttctacgccctctcaagtcgaagcgctccattgagcagaacaagcggtactggtcccttctgcgcgagctggccgccgtcgcctgggtcgacaaccgccagttcgacgatcaggtctggcacgaacagttcaagcgctggttcatcggctgcgaggacgtgaagttgccggacggctcgaccgagttgcgcggcatcagcaccacgaagctgaccgtagacgagtttggaatctacatgaccaagatcgaagcgtgggccgccgagcaagggtggccgctgatgatgcaggaggtcgcatgagcaagttcaaggcgggcgatctcgctcttaatctgcaagacatccccagctgcatcagtgcgggagtggtagtcgagttgatgtctcgacttgcccctggtgatctgtttgccgaagacggccagacctttcaggtgattcggccagcttggtgggtgctccatgaaggagaccggctctacatacctgaacggtatctcatgcccctgcgcggcgacttccagcccgagcagcagaaggcgaagggggtggaggcatgagcaggcggcaggttgcaaaaattctggtgggccagcttctggtcatcgcactcatcatctacacgcagacctctgcggccatcagcccatggattgtctcaatggttgggacggccaccctatggcttggctacttcgcgggagaagagctatgagccgcagcttgttcttctgcgccatgcggagagttcctgttcggccaagagcgctcattgtcctgatgatcatgatcgcctttggctgggtgccgcttgtggtggccgtatgcgaggcagtcggcgaaggggttcgggcctgccggcaggaatcgtccaggctctacggcgacttcagcaaagctttcaccgactgctggaaagccttggtttcgggggagcctcaatgagcctatccgccagccagcccaaaccgaagaaatgccagaaccctgcatgcggccaggagttcacccctcgcttcagcagcacgcaaaaggtctgctcgccggcctgcgccctgtccatcaaggacaagcacgccaagccggcgcggaaggctatcgccgaccgagagcggcgggagatcaaggttcggaaggagaggctgaagagtaaggcggatcacctgcgcgaggctcagcaggcattcaacgaattcattcgcctgcgcgacgccgaccagccgtgcatcagttgtggccgccaccacgatgggcagtaccacgccgggcactaccgcacggttgccgccagcccagagcttcgcttcgagccgctcaacgtccacaagcagtgcgccccatgcaacaaccataagtcaggcgacatcgtgaactaccggatcaacctggtgcgcaagatcggcgccgagaacgtggagtggctggaaggccctcatgagcccctgaaactgaccatcgaagaaatcaaagcgctgaaggcccagttccgggcctgggtgcgcgaactgaagagggcaacggcatgaccaaagaaactctgaccatcgttctcttcagcatagggagcggtctcatcggttatgcgatcggtattgctgccgcctggctgggaaactggttcgccgacggttatcacccgctgctgctgtcgaacatggtcagcacaccaggtgctgaggatggtgagcgcgccaacgaataccccgattatctggagcctccgagaggctgtttcggcatgtgctgtgctggatgtgatgctcgctcgcaggtcaactccaggagcaaaacagtcagcgaacagacagaccaatcttacgttttaaacgccgtgctcagcgctcaaggggatgaatgatgatctacaccagcattcggtcggcagtcgtctctgccttggcggcggaaaccatcgacaacactgcaaagcaagcctggcagaagctctaccagccagggtatgccgagagtgagggtttagctgggctgatcaggggctcgaacacgtcaggcatcaagcgcatcgatgctgattgctgggtgcacgcccggctgcacagtcagctcaagcctaggcactggaacgcgcttgtggcgaagtacagcacccaccgcgagaagaagaaggccgcaatcgaggcgcttatccccctgatcgccaccccggcgccgcgcagattcctcggaatggcagtctatacctgggctatccccaagctgaagggggcagaaggcaagcgctctaccgacatgatcattctcgacgccgtgttctaccacatgaacaactgggaatctgaaggccgccccgaacagacgaggcgacgctggaggtcaggaattcacagtgtgctgaacgaaatgctcaaggaggcagagctcgatgcgggtgaaatcctgatggaggagggcatcatcgtcggagaggctgcgtaggacttgcaattagtgagcgtttgagcgaatatttccccatcctgccgatcttgcgcgttatgaggatcggtagctctgaagccctggcaaatgccggggctttttcgtttccggggtatggatgaatctcgagcatcgcataaggcgctggcttcttcaggctgggcgacgtggcaagccgatccacgcaattctcatccaccccaacgacatccaatctgcaagaaagatctgccggtttgtgccagtgaaggtgctcggcattgaagtacgccggtatggcgcaacagggagcgctgctgatttgtaatcagagggttgcgggttcgactcctgctgccggcaccacactacaaggcccaggcaatgacctgggcttttctgcatctggagtaagcaaatggacccgatgacgaccgttggcggaggtctcttcgccaagtacagcgtcgctattgccgggttctgggggtctattctgtcccttggattcctgagcggcctgaaccgctggcaagccgcgctcgctgtagcaaccggattcgggtgctcaacctattggactgctccggttgccgcatggctttcgcgtgagtacgagattccactcgatgacgcatttctgagtggtgtcgcattcaccattggtttgctggcgatgaatatcatccccggcctgaaggcggcagtaacggcaatcacagagcggttccttcctacgagaggaacctgatcatgatcatgtcgattctggcggcgctggatgcgctgctgtgtgtgcttgtcgttgtagctgctctggagttcctgcgcaccgtccagctgtctgggcagccgctattgggtatctccttctacctggtggcaggtggtgcattcggaatcctgtacggaatcatgaagggcgcaccggttaatccattttcggtgatcctccatgctgggctcgtactttacgcctggtcccggcgccggcagatattcggaagcgactggtcgtggaactgaagcgacctaaccctccagagacgatcgggcagttcgcggaaggcgaagattgggcggacgcctttgtccccgctcaggatgttctggcttgggcgaagtcagtgttaatcgatccgaacggaatcctgggcaatgaagaccacgcccacctacaagacgctcctctcgctttcctatgggctgcctccagcttcaccaagcaggggaggacggtactgggtcagtgcgaagaggtgacgttccgctgtggagcctggcagaagggtaggcaggaacagcagatgatccgttggttcggatacctgccgaggtttctgatcaccctggctgctgactactgctcccagtgctccgacgcggagttctgcgcattggtcgagcatgagctctaccacatctgccaagagcacaaccaatatggcgagcccaagttcaccgaggagggctttccaaagctgaagctccgcgggcatgacgtcgaggagttcgtcggcgtggtgaggcggtacggcccaagcaaggacgtgcagtatctcatcgacgctgctagcaggcctccagaggtggccaaaattaacatttcgagagcctgcggtacgtgcctgctgaagtcggcatagccacgacaggcccatgacaggaagaaaaacgatggcaaccctgaacagcgacgtgaaggcgttcatcgttcaggcgctggcctgtttcgatacgccatcccaggttgcggaatcggtcaagaaggaattcggcatcgaggtcagtcggcagcagatcgagtcgcacgacccgaacaaggtgtgcagcaagggccttgccgcgaagtggcggatcctcttcgaggacacccgcaagcgcttccgcgaggagatcgccgacatcccgatcgccaaccgcgcctaccgactgagggcattgggtcggatggctgagcgcgccgagggcatgcgaaacatggccctggctgcccagctttacgagcaggccgccaaggagtcgggtggcatgtacagcaacaagcaccagctcgagcactctggtcctggcggaggtccgatcccgacaatgccgaccaccatccagcttgtggcgccaggccatgaccacggcgaagattgaacttccgccaaagctgataccagtcttctcaggccctgcccggtaccgcggcgcccatggtggacgaggcagtgccaaaacgcgcacgttcgccaagatgacggcagtaagggcgtacatgtacgcggaggctggaatcagtggcgtgatcctcggggcgcgcgagtacatgaactcgcttgaagagtcctccatggaggaaatcaagcaggcaattcgatccgagccatggctggacgcgtactttgacattggtgagaagtacattcggaccaagaatcgccgaatttcgtatgtgttctgcggattgcgccataacctcgacagcatcaagtcgaaggccagaatcctgatcgcctgggttgacgaggctgaaaacgtcagcgaaacggcgtggataaagctcctgccgacggttcgtgagaacgactcggaggtctggattacctggaacccggagcgcgatggaagcgccaccgacacccggttccggaagaacatgccggcaggcgcaaaaatcgtcgagatgaactacacggacaatccgtggtttcccgatgtgctcgatcaggagcgcctgaacgaccggcagacgctggacgaccagacctatgcctggatctgggatggcgcctaccgcgagaacagcgacgctcagatccttgctggcaagtaccgggtggccgagttcgagcctggtcccgattgggatggcccttactacggcatcgactgggggttcagccaggacccgactgtcggcgtcaaatgctggatttacgaccgcaggctttggattgagcacgaagccggaaaggttggacttgagaacgacgatatcgctgagtacatgatcaggcgcttgccagggatcgaacgacatgcagtccgagccgactcggccaggccggagacgatcagccacgtcaggagtaaagggaaagatggcagtcgtgcatgtctgcccaggatcgaaggtgtcgagaaatggaaaggcagcgtcgaggacggcattgcccaccttcgcagctatgtcgagatcgtgatccatgagcgatgcacgaaaaccctccgcgaggccaggctatacagctacaaggtagaccggcagaccggggatgtgcttaccgatatcgtcgacaagaacaaccactactgggacgccacacgctacgcgttgggcccgctgatcaagcgccgcggcgcggtcggtatgctgctaccaggagcccgctgatggccatcttcatcctcacggagcgcgcaaccagccgctccatggtggtccgtgctcgctgcacgtcctgcgcccgcaccgtggcggtcgagaacgctggcgctgaagggacgatggtatggcgcgaccccaacctctcttctgtcgaactggtccgcgagacggacaagccaggcctcatcctgaaatcggactgaccatgactgacaaactcgacctcgcggtcaatcacgcgatgagcagtgctgtcgcgcgtgcgcgaatgagcctgctgaaccagggcatcggccatgacgccaagcggccgcaggcatggtgcgagtatggtttccctcaggaaatcacgttcaacgacctgtacaccatgtaccggcggggcggtattgcccatggcgcggtcgagaagatcgtcaccacgtgctggaagacaaatccgcaggtcatcgagggcgacgatcaggaccgctccaaggacgaaaccgagtgggagaggaagaacaagccgttgatcgcaggcggcaggttctggcgggctgtctccgaagccgaccggcgccgcttggtgggtcggtattccgggttgctcctgcacatcagggatagccagccgtgggatatgcctgtcacgggaaaggtcaatggcctggcgaaggtcaccccggcctgggctgggtgccttaagccgaagtcgttcgacgaaaagctagatagcgagacctacgggcagcccaccatgtgggaatacaccgaggcctcccaagccgggcgccctggcctggtgcgggatatccatccggatcgggtgtttatcctcggcgactggaccggcgatgcaatcggcttcctggagcctgcctacaactccttcatcagccttgagaaggtcgagggaggcagtggcgaatcgttcctcaagaacgccgcacgtcagctcctgctgaacttcgacaaggagattcagctcggcgagatcgccagcacctacggcgtgacgatcgatgcgctcaacgaacgcttcaacgaggcggcgcgtcagttaaaccgcggcaacgatgtcctgcttccaacccagggggcgaccgtcacgcagatggtgtccgccgtttcggaccccagcccaacctacaacgtcaacctgcaaaccgccgccgccggggtcgacatcccgaccaagattctggtgggcatgcagaccggcgagcgggcgagcagtgaggaccagaagtaccacaacgccagatgccaggcgcgccgggtgcaagaactgacgttcgagatcaacgacctgttcgggcacctgatgcgcatcggcgtggtccctctgaaggccgagttcacggcaatctgggatgacctcaccgttccaaccaaggccgagcgcctggccaactccaagaccatgagcgagatcaacagcgccgcaatcggcactggcgagccggtattcaccgcggaggagatccgcgaagaggctggctacgacccgctcgtgggcggtgacccgctgcctgataccgaaccggaggatgaagatgccgcgcgcaccgatcctaccggcgagcagcagtgacccgaccggggtagatcgactggaaaggggcgcaatgcgcgagttcgacaggcgcatgcggaaaatccgggatggctatgtcgctgccttggaccgaatcccggcccagccggtggtgaatgagcagtacacctaccgtctcgaccaggcccttctctccgcgatcttcgccgacaccaacctgatggtcgacgagatactgcaggagggcggggagcgcgacctctggttcttcgaatcctatgtcggggttgcctacatccgcggtaccgcacagacgcatgccaacctggcgcagcaatcgcctgcataccgcgccggccgggaatcgctggatgtcctgcttcgatccgacgcctaccgcgcgcggatggcactgcttcgcgcccgggagttcgaggagatgaagggcttgtccggccaagtcaaggccgacatggcgcgcattctcgccgagggcatggggcgcgggaagaatccccgcgaaatcgcacgggacctgaccgcacagaccggcatcgaggcgcgtcgcggccatcgcatcgcacgcaccgaagtcacaaccgctctccgaagggctcgctgggacgagaaagacgctgctgaggccgactacggcgttcagtcgaagctgatgcatatgtcggccctgtcccccagcaccagggcaacccatgcggccaggcacgccaggctctacacctcggacgaggtgagggactggtacagccgagacggaaactcgatcaactgcaagtgcagccaggtcgaggtactggtcgatgacgaagggaatccggttgtcccggccatcgtcgagcgcgcgcgccgcaactaccaagtcatgaaagccaaagggcgcgggccctgggcgaaagaggattgagccatgcccatgcaggtcaacatcaccacccaggtcaacagcgccagcattcggcgtgagacacacaacgggcgcgaacacctggttctgccgagctacaccctgccggccggcgtgatcatgaacggtggtctctacaccgccgagcagatcgacaagcactacccaggcctggagggaacgctggcgccgctcgggcacccgatggtcgacgggaagttcgtgtctgcgttctcgcctgaggggatcaacgccgcccacgtcggcgcctggaaccgcaacgtgaagaagtccggcaaccgggtctacatggagaagtgggtcgacgtcgagtttgccaagtccacggagggcggccgtgaactgttgcagcgcgtcgaagcgctggagaagggggaggacgtccccccgatccataccagcgttgccgcattcctcaatcgcatcgagccgaacgaaagccagcgtgcccagggcgcggagtgggtcgccgacatccagagcatggatcacgacgcgatcctgctgcacgaagtaggggcggccactcctgagcagggcgtcggcctgatggtaaacgccgaccaggctgtcccgcttcagccgaattccggcgctctggttggcgagtcctaccgggagcgggagcagcgtctcgatcgcgccgcaaaggagcgattcgcctccgggcccgaccagtacgcatgggttgccgacttcaccgattctcaggctgtgatcagccgcaatggcggtgtgaccgaggtgtacggctacaaggtcgaggcagggaagatcgtcttcgacgaatccggccagcccgttgtcaggcaagagtcctgggtcgccatggtggccaacagcatcaagaacattttcacccatcgtcaggctcggcctgatcaacctgagaaggagggcgacatgcccctgacccccgaagaaaaggccgaaatcgtgaaggaaatcggcaccaacacctccagcgccatcaaggaactggcggacactatcatcaagcctctggccgacaaggtcgacggcctggtcgccaatcacaaggcgctggccgacacgctgaccgccaaccagcgcgccgaggaagacagcatgcgcgaagcggtcaaggccaagtttggcgaggtcatcgccaacagcctggccggcgacgcgctcaaggaactgttcaagcagtgcggcgaatccgctccactgggcgccaatgctgccaccgacaaaggcggcctcaccgccgatatcgccaacctgccgaaggagtaagccatgtctcgctatcgtcgcgtgaacatcgacggcaagtcgctgttcaagaccgaaacccgcaagaccgccgcggcactcctgcccggcacgttcgccgtgatcaatggcagcgacctgttcgcccaggcaagcgccagcgttggccgcctctacgtcatcgactgcgctcaccacgaaggactcaacatccgcgatgcggttcccgccggccattcggccgtgggcaactacgtcgaagagggtcgcgaactcgccgtgctgtgcccggccggcacctacaagaaagacacgccgatcaaactcggcaccagcggccagggtgccatcgcgtcgagcgataccgacacggtcctcgggtacagccaggacgatgcagtcatcgcctccggcgaaaccgacttcatccgcatccgcttccgtgtcggcagtgtcgccgccccggcgccctaataggagtacggacacatgttcctcacccagcaagcaaccgccgcccatcctcgcctgatgggccactaccaggagttgcaggccaatcgcaacatctggaacaaccagaacgccgctatgatcgcccgccaccgcggcgccatgacccccgaaatgctggcctgcaacgcgctcgccggcctgggtcgtgagttctgggccgaggtcgacgcccagatcatccagtaccgcaaccaggaaaccggcatggagatcgtcaacgatctcctgcaggtgcagaccgtgcttccgatcggcaagaccgccaagctctacaacgtggtcggcgacatcgccgatgatgtgtcggtgagcatcgacggccaggccccgtactccttcgatcacaccgagtacaactccgatggcgaccccattccggtgttcaccgccggctacggtgtcaactggcgccatgccgccggcatgaacaccgtcggcatcgacctggttctggactcgcaggctgcgaagctccgcaagttcaacaagcggatcgttgcctacaccctggacggcgccaccaacatccaggtcgagaactacccggctcagggtctgcgcaatcaccgcaacaccatcaaggtcaacctgggctccggcgccggcggcgcgaacatcgacctgaccaccgccacgccgcagcagatcatcgacttcttcaccaaaggcgcattcggccaagctgcgcgtgccaacaaggtggacgcctacgatgttctctgggtttccccggaaatcaacgccaacctgtcccagccctacatgatcaccatgggcggcggtgccaacgcggtggtggccggcaccgtgctcgatgcggtcatgcgcttcatcccggcgcgcgcggttcgccagaccttcgccctgtcgggcaacgagttcctgggctatcagcgccgccgcgacgtggtcaccccgctggtcggcatggctaccggtgttatcccgctgccgcgcccgctgccgcaggtcaactacaacttccagatcatgagcgccatgggcatccaggtgaagaaggacgacgaaggtctgtccggcgtgatctacggcgccaacctggcgtaaggagaacgacatgcccaaatacgaggtgatcaagccctggaacggcgtttccaagggtcaggtgctggagctcgaatcacttgccgctgcgctcctgccgaacgtgcgcgaggttggcgcactcaggagcggaagcctgaccttggacgtttcggcccaggtcgacgaagcggccaggcaagctctcgccgaagcgcgtgtatccgtcgatgccatgatcgacgaagccaaggcccaggccggtaccctgaccccggccattccggacggtagcgagcgccgcgagctgatcaaagcgcgcctgaaggagctgaagatcgagttcgatggccgccagggcgaggaagcgcttgccgccctgctgccggagggcgaactggcgaagctgttcccggccaagtgaccggtgcgtgacgagaggccgcctgcgggcggcttcgtcgtttctggcctcagcgatggggtcgcttcttctggagaatgaaatgtttggcaatctgatcgactcggacatcccggcaattccgaaggctccgcccgctcccatggagttcccggcctcgttcggggctagcgatgacttcaggctctgcgatgctatccggaacaccgtggatgctgcgcaagacgcccaaggtatgacgcttcggattcttcaacgacacctcctccgtctgtgcaacctgcaggtcgagcaactggagggatgtggtgatgatcacagttgagcaggcccggcagtatctgcagagccagggcatcgacaacgtgcccgatttcatactcgcggcgtggatcgagcaattgcaggagatccagagttgcctggatgcccactacccggcatcgaccgcgctgttgatccaggcctacctgctggcgctgtttgcgctggcccaggccgacaagtacatcagcagccagacggccccatccggcgcttctcgatcgttccgctaccaggcctttgctgatcgctggaaggcgcagttggccctgctgaacgccctggacaagcacggatgtgtgacggggctgattcccccgaacccaacccagaccgcacacggcggtctttggatcgcgcgaggcggctgcatgtgtggtgactcatgagcacgacggcgaattggagttacaccaacacggcgacggttcggccattcctgcacttcgacctttcgacccaggaggccgtttacggccctgagtacgaaatcgcctgcacctggaccgccaagagcgagcagatgcgggaggagggcgggcaatctggagcgcggggggctgagttcgtatcgcgccaccagatattcaccgaggaccgccggccgaagtacctggacctgatccagttcgacggatccaacggctgggaagagattcgctcggtgacgaactgggacatgtccttcttcggtgaacagccggactttctgctggtgacctgacatggcaatccaaggaatcgaccgcgtccggcggaatcttcgtgtggctgtcgaaaacatcgccggcggtgtttccgagcgcgcagtttacgaggtactgagccagggcgccgcaatggcgcagaccatgacgccgatcgacacgtcgaatttgatcaatagtcagactgcaccccagatcagtaatgggactgctggggtggaagggcggattggatatacagcagcctacgcggcagcggtccatgatgcgccaggaactctcgccggacagccaagggcggatttcggaaagacagcggacggaaccgcctttggaggcggtactggagttgggaactactgggatccaaatgcagagccagagtttctcactaaggggttcgatcagattgaatctgcaatcccatcaattctccgcaggatctaccgcgtatgaccccctacgacgccttccaggattggctggcttcgatcctgggcgagggctaccagtacagccgtgggatgtgggtcgaccacccgtcgctcgactcggcattcatcgcagcgatccagcaaaccggcggccccccgactcaggtcgacattcgtcgcctgcggttcaaggtgatcctcctcggcccgaagggcgtccggaaacatgttgtcgacgtcggcaactcaatcgagaccctggcgcaggtagcgcttggtgacagcgtcccctgtggcgccgcatctgttcgggcaatcggcgagccgatcgggcctggatacaccaccgaaaaccgggcctggtacagcctggaccttgaagttctctattaatcaggaggccagacatggcttgcaagaagctcaaatttccgggccgcgacgtcgtgctcgagtattacatcgggtgcggcgatgcgctgccggcggagaatgactggcgccgttttgggtcgctccgcacgaaggaattcaccgtcgagtgggacaccatcgacgcgactgattccgactcggttggcgcactgcgggagaacctggccagtttccagacgctgaccatttccggtgacggtaccgtgaaggcctccggtgccggcgcgcagaacctgatcgacctgacgaagcatgtcgtgaagccggacgcgaccggcggacagcctgttgtctggatgcgcatgaccttcccggacctgaccttcaccgcattcatgctcatcagcaacctcagtcgctccgcgccgtacgacgatgtcaccacctacagcttcgaggcttcggcgaccgcttccgacttcggcctgatcgtcgaggatacccccgacgcggatgcgccggacccgaccagcattcaggtcgtgccggagaccctctcgcttaccgttggcgaaggcttcaacttcgagggcgtcgtgctgcctgttggcgctccgcaaggcctgcgctggacttccagtgcgccgaccgtggccgcagtgaacacggttaccggcgaggtgagcgcgctgtcggccggtaccgccacgatcaccgccgcttccagcgtcgccccgggcgtcaccgataccgcaaccgtcacggtcatcccgctggtgcagggcatcaccgtctcgccgacatctgtctcgatcgccgaaggtgccacccagcaactgaccgccgctgtatctccgactggcgcggctcctggcctggtctacgaaagtgcggcgccggcgattgctaccgtgagctctaccggcctggttaccggcgttgatgtgggcaccaccacggtgaaaatcaccagtgcggcgcggccgtcggtgagcgtgacagttccggtaaccgtcactgcgccgtgatcctcaccgagatcggtgagataggcgtacacacggcctcgggggagttctttctcctgcggccgtccctgtacgccatgacccagctcggtacgccggccgagattgtcgacgtcttcgcgcgcgtcatgagcgacccgatcactgagaagcatcaggcggaccagttcgcggacgccctggccgtggtggtggcctgtagtgagcaggacctgtccgacgtgtttggctactacgaccaggatcttgtctaccggccaggaactgcggacgtcgagcaccttgtgcctctcgcgcgctgcctgctgaagcacggcgtcacaggagcgcttccgccgcttccccggcgccacgacgaagagccgaactactcgggggagttcgttgcgcgggagtacgtcgcgacggcgatagcgcacctggggctgagcgagcgcgaagcttggtccatgaccatgaccggcctgatcggcgccctgcgcgcgaaataccccccaaccgaatcgaacgctccgggcgccagagccccgaccgcggcagagcatgacgcgacgatggagtggttcgacaagatcgaggccaagcgcaaggcgcgggcgaaaggagcaccctgatggctgagaatgtcggcagcatctattacaccgtcgaggcggatacctctggccttgtaaacggcacgaatgctgctgaccgttcattggatcagatgcaggcaaccatgcggcgtgctgatagcgaggcggcacgtctcaacacgactgtcaccaagctttcgtcggctattaagacgatcatcgcggcgtcagcgctccgcgagatggccagcatggtccagtcctatcaggagatggctgacagggttcgtctggcgtctgcaagccaggaagagtatgaaaacgtacaggccagactgctccgtaccgccaacgggacataccgagcgctctccgaggcgcaggaactctacatccgcacttctgcaggcctgaaagctctcggatacgacacaacgtctgcactggatgtgatggattcgctgtcgtatgcattcgtgaccaatgcgaccaaggcggatgcagcagaggcagcgatcagccagttctccaaggcaatcaacaccggcaaggtttcggctgaccaatgggaaacaatctccagcgcagttccgtctgttattgaggatatcggcgccgctgcaggtaagacgggggcggaagtcaggagtcttggtgcgcaggggcaattaacggcgcaaatgctcaccgagggtctacgtaagtccttggaagagaactcaaaggcagccgccggcatgtccaataacctgaccgatgcaggggtcaggattcggactgcatttactcaagtccttgtttcgctggaagaccagactggcgcccttcaaaccttcaccaatggtcttatttcggctgctgatgcgcttcttgagttcgggcttgactcggaaaaaatggcagcatttctcgacactgcaacagtcgcagcagcttctctggcctctgttgtggctgggcgtctagttacctccctgtatgcagcaggtgcggcccaagtgcaaagattgcgggcaacgcttgagcagatagcagctgatcggaatgctgctataggtgcactgaggcgggcagaggcagagaaggccgccgccgccgcggctgtcgctctggctcaggcggacttgaatgctgccaggggttcaaatgcccacgcaacagctctaaacgcgctgctggccgctaaagaacgcgacttggccgccacaagagcgctaacggctgctcaagcaacgctgaatggtgtagcaaccaccgggacggtggtgatgggtggacttcgatcggcaatggcgttcctcggcggaccgcttggggttgttctgctggcagcaaccgcgatcgcaacatttgcaacgaatgcacgggaggcgaaagagcctacggaccttctaaccctgtccgttgaaaaacttggacaggcacagctgaaggttgcacaactggacatcgacaagcgaatccaagcagtgagcgataagctcaaactgcttggggaaaactatgcgttcgcggcaaaagaagcccaaggctctggtcgaagggccaatcgatatgctgaagatgccgtgcgtatccagggcgcggtcgaggagcttacgcaggagcttgaccagttacagaaaaagcgttcagacgtcgacgcagccctagataaaaagagttcatccccatctggtaatggcccggatcgccaggcaaacccggaggatacaaaggctctccagaatcttcgcgacgaggctgaactatctgctctcgcgggtgaagaacgggcgaagcttgccgcgcgcaaaaagctcagtgctgatgccacaaaagaggagatcgcggaggcggagcgtctcgctgtccagatattccgcaacagcgaagcgcggaagcaagagaagaagtcagcctctgataccgcctctacggtcaaaaagtcgatggaggatcagcgtcgcgctgccttggacaatgagaagactatcggagacctttcccagcaactggcacaggctggactgaagggaaaggaactggcagaagctggggcgcaatctcgccttaatccattcgccacgccggagcaggtcgcccaggtccgcgcgctcgccgcagctctgtacgaagcgcaacaggtcgaagccaacaagcagttgctggggcaaatggaccctatcgccggcgaagaccagcgctaccagaccgaactggagaatctgaaaaagctgaacgaggccaagttgctcgaggaccagcgctacctggaactcaaggcgcaggccgagcaacagcacgatgccacgatgaagcaactggaggaggagcgattccgccgccaggctgccggcaacgagatgatcatggcaacgctggatcaggtgcagcaggccggcacgaacgctctgactgggctgataaccggggcgaacaacggtgccgatgccatgcggcaactggccggcgccatgctgaaccaggtcgttggcgccctcgtcaaggtcggcatcgaacaggcgaagaacttcatcatggggcagagcatgcaagcgaccgcaaccgcccagggcattgctcaggccggggcgttggctggcgcatatgccccagctgcagctgcggcctctgtggcctcatttggcggcgctgcgacggcaggccttgctgcaatggcagcagcaatcccagcgatgctaggcctcttcggaggacgccaatatggcggaggcgtccaggcaaatggcctgtaccgaatcaacgagaacggcgcgccagaggtattccaggctgcgaatggccggcagtacatgctgccgaatacgcgaggcgaggtgatcagcaacggcgacgccaccgcgcagggctcgccgcagatcagcctgcagatcatcaacaacggtcctccggtttccgccaccgccaccatggacgggaacaacctgcgggtaactctcgatgcggtcgagcaggactttgccaacaaggtttcgtccggccaggggctttacccgaaagcaatcgaaggcgcatatggattcaagagggcagggcgatgatcaaatggcctgatggccttcccttcccgctcagggaggggtacggcttcaagacggtagagccaatggccaggaccgtcctccagagcggccgtgcacgctaccgacggaacttcagcaatgtgccggtcaacctggaggtttcctggctgttcaccgctgagcaggcgcgtctgttcaaggggtggtaccgagacgtcctgaaagacggcgtcaagtggttcgagtgcgatttgcgtacggaagagggaatcgttccgtgcaacctgcacttcgaggggatctacgacggtggctatctcgtcgggcgcgaccactggcgcttcaacgcgaccgtcgtgatgcgagagcgctcgatcatcgatcctgggtgggctgagattctgcccgagtacatcctcctcgctgacatcttcgacatcgcgatgaacagggagtggcctcgacatggcgacggctcttgagcggttctatgcctcaggcggtgaggacctgcagctcgccacgatcgagttgtcatgcccggcgtggccggagcctattctcatctgccagggctatgacgacctaacctgcatgaccgaagacgggcggctgctgacgttcatcgctggtgcgatcgatgtatcgattccgaagcgagacaacagcggaaaccagaacgttggattcgcgatcgacaacgcgaccggattcgcccagcagcgtatcaacgaagcgctggaggctggcgagtatgtcaccctgatcctgcggatgtacctggagagcgatctcacagcgcccgctgagcggccataccgcatgagggtcaagacgccgggtttcgagggtctcactgttcaggtcgaggccggttactacgacctcatcaataccgccgcgctgcgccacatctacaacgtcagcgagttctccggactcaaatactggccttgatcccatgccgaacagatacctcaccgccatctataccgagggcgggcgggcactgccgtgcctggactgctggggcctgacgctcatagcgcgggttgagctgttcggactgccgatgctgaccgacttcgatggtgtcacgcgactcaccccggtttcgatgcagcgggcgtgcgatacggagatccagcgcgcgctcgagcaatgcgagccaggacctggggtcatcgccgcggcctatagagggcggctgctcgatcacgtaggtctgctggtcgaggtggatggacgcctgcggattctcgaaatcaacccgggaagcggggtgtcgctcaccccgctccagatgttctccgacaaatattccaaggtggtcttctaccgtgatcgaaatctacccatcgctccttgacggagaaccgctggagcggcatccgatcggtcgcaggatgacgattcatgcctggctgaccgcgaattctcctgggtaccgctgccacgatgtccacccgttctccatcggtgttgtccccgccgaggttgcgctctgcggtgacctgaccgacaagcagaaaaaggcgcatgaggagttcgtccaccccggcgagtgggccgagcgcatcatcgaccgcggcgacattgtgaggatctacaagctcccgcgcgggactgatccgttcacgattactgcggcccttttcaagggggcgcaatcggtttttcggatgctcatgcctcaattgcccggcatgccgacgaaccccgggcagggcgcgtcgctctctgaaaccagcgcgcgcgggaacaaggtaaaactcggcgatgcgatccgcgaagttgctggccgtcgtctgatttatcccgactacatcctgccgcccaggaagtatttcgccggtccgcgtgagcagtggaccgaaatgctgttgtgcattggccgtggtcggttccagatcgccgaaggtgcagcgaaaatcggtgaaacgtcgttcctggcactgggcgctgatgcctctttccagattttcgaaccagggcagaacgtcagcgggcacccggcatcggtctggtggcacctggttgaggaagttggtgcgagctcaactggtaatgccggcctggacctgaccgagagctccaatctcacgccgaacccgtcggcaactacgttcacgttttccggaacgaacatcatcatttctgccggagccgggtcgttcccctctgacttggttgcggggacgatcctccgggttgaggcgatgtacccctattcggttaacgatggcggcgggacgaatcgcgacgtcgtgacgggggatatcgctcagctcgggctggatgttggcgatgagatcgaggttgttggcaccaacggcggcctctacatcgtaaacgacatcacctccacgtcgatgacgctcaactacagcaacggttctccggcgaatgcgctccagaccgggtccggcagcgccgcaatcggcccgcgcggactgcgctatcggatcacggcgtacagcgcgcagcaactcacagtcgagcggctgaccagtgccggcggtgtagatgtggactggccaggattcaccgctctcaattcgtctacgtctcgcgtcacgatcgatccgactagcctcgaagggggctggcgcgggccattccctgcatgccctgtatcggagaagaccaacttcgtcgagatcgacgtgttttgcccggaaggcctgtgcggtgtaggcagggaagggcagatctaccagatccgcacctattacgacatccagtggcgagacatggccatcggcggcgcatggacgacggtcagtaagaaccatgctggcagttctctcgaccagcagggttttacggacggcatctcgctgccgtacatgatgcggcccgagtttcgcatcagaaaagtgttcgtcaaccagggcggcaactcaacatccgagtaccgagaccgcactcagtggtacgggatgcgcgcgcgcctccaggctccgtcgtcctacgccggcgtcactacaatggctgttcgatatcggtcgtctgaccgtatcgcggcgcagacagaaagccgcgtctcggtagaggctacccgcatgctaccgactcggcagaacggtgcatggacacccgagatagcaacgcgagacatcgtcccattcctctgctacatcgcgaaggaacgcggctacaccgatgcggatctcgatcttgaggaactcgatcggctggacgcaatctggaaggcccgcggcgacacgtttgacatgatctacgaggacggcaaggtcacggtcgcgcaggtcatggacgatgtgcttgccgccgggtatgcggagaagaccattaagcgcggcgtgatctccgcagcccgagacgaaccaaggaccacattcgggcacatgtactcgccgcagaacatggatggtccgctgaggatcagcatcagcgcgccgtctgaggacgactacgacggcgtcgatgtagagttcgtcaatgccaacggctggatcgaagataccgtccagtgccgactgcccggcgatgttggcaggaaggtcgagaagatcacggctgtcggtgtcacaaaccgcgatcgcgcctggcgctacgggatgcgccgccggatggctcagcgataccggagaactgagtattcgttcgataccggcctagacgcgctgaacagcgagttctgggattatgtggcccttgccggcgatgttcccggccctggcctggcgcagagcgcatacctgaaatcgttcgttatctctggaaactcggtcctgatcgagtccagcgagccgctcgactggtcactgctgaactcgccagcgctctacctgcggcgcccaggcggaacggtttccggtggatatccggcgtcgaggatcgacgactaccggctgagcattcccagcatcgatttcgtccctgatgtttcgtgggaaatcgaaccgccgcacctgctgctgggaaatccatacccggtgctgatcagttccatcgatcccaacggaaataccgcggcatctgttcgtgcggtgaactattctgaaagagtatacgattatgacgattcatttgcgcctgagtaatccaatttggcccccttctttaggttgtcttctgcccaaagaggttgaagatttgtatagtgattcagcctgattacctcctcgttagaggatgcagaggaaagcgggatcttgtggtcaatatgccacaaatcccgattttcccaagtcattccgggcagaaaaagagtctctatgtgcaatcgtaacgtatcccaatcgcatccaagtatctctgctgtggctgatgattttcctatgccctgtctttttagtactgttgatattctagagcgaatattgcaccttaatctaaatattggatctatgcttcttcgagttttcatatagctgttggctctagagttctctgtttctttgtttttcctgtagtaatttcttcttttttcaataagtttttgtgggttttcttcttttcttttcttccatatttctgcatgccttccttgaattttggatgcccaagactttgcatgagcctttaccctatcttgattcttcaatttccatgattttgagtattcttttagtctctctgagttattaagataatatgtcttgcttttcagtctgattttttcacgattttgttcgcgccattctcttgttctggagaggattttttcataattttgtttctcatattctttctgctttgatcggattttttcgtaattcaattctctgtatttttttcgtttttcgtttacgcatgacttgcattgagagtggagtccatcctttctttgcttattttttatgaactctgatacgtgcagttcctcgttgcagctgctgcatgtttttttgcttgtcaattcaatctcctattcttgtgttgttagcttggacctgccgagctacgcatctaagaatactgcaaagctatagattaacctggacaaccatacacaacctagcccgccatagagcgggctttttcatgcttggagaatttgcatgactacgtacgccaccagcaatccgcttggctccaaagacccgcgcgacttgtacgacaacgccgagaacttcgacgcggcgatgaacgaccgggtaaacaccacgtggaatgatcgtttcggcgttagtcgcccaacgatgaaagggtatgaggaacagttcaacggctggctggacgcccaaggcttcgaacccggagtcctggagtacgtcgacggctcaccgctgaccgtagaccgtccgacccaactgatccagcgcgacggaaacctctacagcgtcaagcgtcctgcatcgttccccgtcaatctgaccgggaactgggcgacggaccagagcctgcttgttatccaagtagaccaagggttcccgcaagaaatcggtcgcggcgtacgccgggttgactcggttgccgacctccgggccatcgcagggcgattcgccggggatgccgcgctggttgtcggatactacgcggaaaccccgggggtcggcggcggagagttccactgggattcaacctcgatagaggacgacaacggcggctcgatcatccaggcaaccggtatcaccactggccgatggaagcgcgatataacgcacggcgtgtgggccgaatggttcggcgctcgcaatgatggtactgatgctgcgggaactactgctgcggtgtgggctgcaatcatcgcactccggcacgacccggagacaatcgtgcagtacatcggcggtcccactgtcacagcgtatgcatccgggcgactgaacttcggtaacggggtctttgcactccagcctgatagtttcgatattacccaggacctcggcctgaccatcgtcgggcagggattcagaggtaagaaccaggcgatgaaggcggctactactctggtagtgagaggtacaagctctggcttcttcttcaggcactatgggaatggcggcaggaatctaacattcaacaacattgatgttgtgtatgatgacagccaattcagcggcgatatcatagaaaccacctcttctcccggccttactctgcaaagggtgcgggttggctgttatggtggatttcttgccagtcgtctcaccaccgcgagaagctgcatacgggcgacgtttgatgaattcatcaggtgcgaggatgtcgttttagatggggctcaatatgggttctactctgatgggacgataaacgttccagggctttcattcggcggctggggtgtgacttttctgaattgcacattttacgacttcgcgaagtccatggttctgcatgctggaaatcgcacaaggcacagccttaacattattgcgagctactttaaccccatcaatacatcccccgagcgctgccatgatatagataatgtcgagggactgattatcgatggttgccagcacactcctagcactggaagccagccttcacaggaatggtttagggttattggtagtactggcaggatttcctgtaacgcctttgccggactttcctcaaaacttggaaccattggtggggcgaatccgtctgctgttgagtggtcgaataaccgggtttcttgccagggcggcctaaccataaccggtggagttgttcgcggtggcgggaatgagtacagcaatgccgaccactctgtagatgtcgctccggttgcaattgtatctttagacatcgggcctgacattcataaagccggcgtcactggttactcatataggatatcggcagatagctcgatgctgagtgggagagttaactactcattcgaacaggataattccaatagtaaatactatagcgcctctactagggtagggatgtcaaactgcgatagcaggttcataactcttgctactgctggaaccaaactgtcgccttataacgctgggcgcacgtacaatgtgactgttgcaggtacgcagaccttgccaaccccgatcccaggggctgcgccaatacgcattctaaagtccggcgcaaatgctctgacgattgcaaccacctctggaacaaacttcctgatcggtgcctccgggtcaaggaccagtgcagtggcgacctctactgaggtaggttctctcatagagtttgagccgttaacgtctacggcatgggttggcagagtgctatcaggcacttggtcatttacctgacagtttcggagatggggacacaaggattcctatccttgtgtttctttctacgatagtcactattacgatatccggtctgtacctatcaaccagatcggcaattactttagggctagaacgctgatgatgcagttgtagggtttctgagaacgtggcggccataaatggggatatagcagatccgaaagagtctcgaagccacagaacacgcttgttgttaagcgcgccctctgatcggaccaatagtggcttaacgggggctgtaacttgaacattgtctcccgagtagactttctccatgctttcgaagtctatttggctaacatggattttacgtatggaactgtccgacagatccacctctgcatccgtgatgtacggacgtatcctttggaatgcagaaaggtcgccgcctccccgtttccttataatcacagcctctggttttggttcttcaggtatagatatatctggggagttagattttatacgcttcgccagtgcataaaaagaaacccaagctcctagtgtattccagtgagtgtctgtcttgtagtataaaggtgcggtggatctagattttatattaataagttcattttttggatatacaaaaatatctggagattttctgtatatgtgctgggcaatgcttgtaccggaaggtgcagcccagtcaggaaggttctcggggtatatcgtagacttgtcagggccaattaaaacatagtagcccctaacgccatttgacgaaaaccattcacgccatccgtcagaaacgtttttgataatatctgtttttgcagtgtcggagtccgtgactccgactcgttttgcggttacagagttttcgaagaaatcgccgaggaacatccatccgtctcttccaataataaccttttcaggactaatggatattcctagcttgtagaaaatcatcccgatgtagggtagtgtaaaatccatgttgtaggaaaggtccttccaccctactatagtttctggaagtggtttgtttgagctaatcgcttgctcaatgtttacggcaggagctattcctagaacagcgatagaaatgaatatgaatgaatatattttccctttcacttctataatccttagaaattgaaatataggaatacagtgcttgttgattgtagtgtagagtacattgccaagcagaatagtattgacatgtatattgcttttaaatttccgatccttccggtcgttgaaagctcgaatgagtttttctgtgaaattatcaaaaatgctgctgcaatcattccatagcacagcgagttcgcaacaacaccgattggcagaaattgtaaaagcttgtcggaaattacccctgcccacgcaagatcgcttgtcggtatttcagccaggctttccgatgagatagatctaatatcaatcatccctccaaggattgacatggcttcctgcatggatgtggctcggaaaaatacccaggttatatttacgaatagaaatgtcacaacccaagccaaaggtcttggcatagacattccgagatttttccacattctgtggatgacaagcgctccaccatgcagcgccccccatatcacaaacatccagcttgctccatgccataggccaccaagaacaaacgttgccattaggttgaagtaaactctggcggaagaacagcggtttccacctaacgggatgtaaaggtagtctcgcagatagcggcttagggtcatgtgccaacgccgccagaaatcttgaatatcaagcgccttgtagggcgagttgaagtttattgggagccaaatgttaaagagaagggccgcgcctatggccatgtcgcagtaaccgctaaagtcaaagtatagttggaatgtgtaggaaaggcttgtcgcccatgatctgaagaaatcatgattggcaccgctcgaaaatcctgcatctgcccagacagagaatgtgtcagcgatcataactttcttgaataggccgatgctgaatataaacagtccagtaagaatatttctatagcgtactgcccatgtccatttcgacttgaattgacccatcatttccttgtggtggagtattgggccggcaattagatgcgggaagaatgtaacgaataaagcgtaatttattaggtcgtattcttttgcttcgcctctgtagctatccaccaagaatgcaatttgagtgaatgtgtagaagctaataccaagaggcaagattatttcatgtagcgcaaattctgatccggccgcagcattcaggttctcaataaaaaagttcgcatatttaaagtatccaagcagagccagattcgcagtaatgcttaatgctagtattgtttttctgtatccaccaatggataaattctttgaggtcggggagatcgcgcaccctactgcaaagttgaataaaattgaccctatcaggagtggtatatagtcaacgctccagtatccatagaagaaaacactggctaatactagccatattttccccaatgagatcatccttagcttgtttagtccaaaataaacaaagaacactattggcaagtaggccagtatgaaagcagcggaactgaagatcattatgccttcctgttcgttccctgatgagggaaggtttgttagtgctgtggccacatcgagggcggcgcagatcatacccaattggagcggaacatgcccatcactgagcagcagttgctgcatatcctcccgaacgccggctcgagggccggcgtttttgttggtgcgctgaaccgcgggatgacgcgcttcggtatcacgtcgcctgtgcgcgcggcgacgttcctcgcccaggtcggccacgaaagcggccagttgacccgcttggtggagaacctcaactacagtgcccgtggcctggctgcgacctggccgagccggtacctcggcgccgacggccagcccaacgccctggcgcagcgcctggcgcgcaacccccgagccatcgccaacaacgcctacgcctcgcgcaacggcaatggcgacgaggcatcgggcgacggctggcggtaccgcgggcgcgggctgctgcagatcaccggccgggcgaactaccgcgccgccggcgacgggctgggccagccgctggagcaggaacccgagcttctcgagcaaccggagtgggcggcgatctcggcggcctggtggtgggccagtcacggcttgaacgacctggccgaccgcggcgagttcgccgccatcactcggcgcatcaacggcggcacgaacggccaggcggagcgcctggcgctgtgggagcgggcgaagagggtgctgtcgtgatctccgcccgcgttctatcggtcgcgctggcctgcctgctactgctcggcctcggcgccgccggcggtgtctggctcggcgcgcggcactaccggccgcagctcgatgctgcgctggcggatctggtcgcctgccgtgcctcccggggagagttggagtccgcagtggcggagcaggtccggcaggttgccgcgctgcgcgtggtcggcgaacagcgggcccgggatgccgcgctggctgtggatcggggacgacagcaggccgcggagcagtatgccgcggcacagcgcctgctgagccagcgaaccgccggcgagcagtgtgcggccgccgaggcggtcattgatcaggagttgggcctatgaaactgcaggcgtggcgaaagactgcaggtgcagcgattttcggcaggtgcagccgaaaggcgcaggtggtgcaggtgctggggttggtgttcgcgctggcgggatgcgccggccaggtcgagcctgagccgcgcacggtgcgcgtagaagtgccggtggcggtgccgtgccgggtgccggcggtggaggttcccgcatgggccacggcggggctgcgaaaaggcgacgatctccagaccaaggtccgtgcgctgctggccgagcggcggcagcggatcgggtatgaagcccaactgctggctgccaacagagcatgccagtaggagtagactacggccttttcctacggagcttggtgatgctggtcattcgattcaagggctggtcggtgaaactcgaccaccaggtgggcagcgctgggaagttcggcatctggtcgttccacggttcggagagcagctacgtgccggacatggagacgattctccggcatgcagcgatccggccggcggagccgaaagaaggcgggcggtagggcccggcgtagcggcttacgaggcggagcgctgatcctgtaccagtttttgtaccaatcgatgcgaattctggcgaatcatggcgcctgaaagccttgattctactgctctccagcgcgctagctatcgccaaaaaaatcgcatggtgatgttagctgtagatatcaaggcattgtcctgcggggctttgcgggatggttacgcgccttcctctgcttcctgtaccaattccgtaccagttttaaccctggtctgtagcttctccaactcgctccaatccgaggcggagttcagccacttggcataggtcgatagcagcatctgcacgctgtggcctagctgtccagcgataaacgcagggttcatgccagccatcaggcacatggtcgcgtatgtgtggcgggtgtcatactgccggcgccttcggatggatagagcatcaagcgcggcgtggaagtgctttatggtaacacttggctccttgatccacagcccgcctttgctgggcgggaatacgaacgggctgaccgcgaactccgagactgatgcgacgcgcctcaggcgcgcaatccgcttggcctctaccagggcattcaatgctcgatcattgagcagcacgtcgcgctcatgcttggtctttacgcgttcctcgatcccgcgatctatgacgatccggcacacatgaatacgtcgtgcctcttcgtctacctcgtcccatcgaagggcgaacgcctctccaggccgaagaccagtgaagaacaggaattcgtacagtgcggcgtagatccttgagtacttcccaagggtcgcgtacaggtgctggatgatgcgttctgcctcgtcccgggtgaatggatctaccagtttcttagacacccgaggcttctcaaggggcgccatcgggttcttcttgatcagaccgtccttcacagcggaatctaggatcgtcgacagcttgaacatcgcgtttcgcttcacgcctggcgacgtccactcgatgctgctgatgattcggcgcaagagggtaggggtgatctgatcaagccgggctactgctagatgtggcatccagtattggttgaggatgctcttgtagttcttgcgtgtcccaagcacgatctctcggctgtctagccagagttgagcatgctcaccgaacagggggatttggctgctgaccgattccgcaatcgcagacccggggaagaactctgcataccgggcttcatccatgatgcccagcttgattgcctggactacctgatctctaagaccggatgcagtcttaatccctttttgcgtcgcgggataggggagtgtttcgcacttccttgttccgttccacatgaagcggatacggatagagttgccgatgacttccaccccggtgggcatacccaaaggctttcgagccattcgtcgtatctccgtcgactgtagattattttcccgttgaccttgttccagacgccttctggaatctgtccctttgaccgtctggtttgtagggcgcggtaggttatcccaagcagcgccgccatgacctgttcgggcaccaaaaaattagcgcaagaagacaaaaatcaccttgcgctaatgctctgttacagtcacgcagatggcgggtcgttcgccaggcactccagggcgaactggacggtatacggcgcggggcggtagccctccttgatgtcctcgctcaggtaatagcgcatcaccctgtcactgaggccgagcagctcggctgcgcgccgctggctgatgccggctttcttgagcagcccgcgcaggtagcgcgggtctgggttgtggttagaggcgtcaggcttcataactcagatgcgcgcgccagcaagcagatcgatcgcttcggccgccacctgttgaggcagctcaatgccggggaagtgtgtttcgcccccgagacgacggtagctaaaccatggatggcgggcggcgaaatcgtcgtgaagtgcgtcgtactccccgatcttgggatgtgagaacacgtgccggatcgcgcacggttccgccagagcctccatgcgccgcatcggcgatccccaggttcggtaggcctcgtcaatcacccggccagcacgagcccacatgtcaaaaccgtgaccgccgctgtcgtatcgcacgtgatccagcaccgcttgattggtggtccccgccagccacgactgaacgaggccatcacgcccttccttccagcgctctggatcctggataccgtgcagcgcggcaacgaactcccgcggtgctggcgtcatgatgagatcgaggatcatcacggccgggacccgctgagcgccgagccgatcagcgatctcgagcgccgcccatccaccgtgcgcgtgggcgattggtacgaaactgtccacctcaagcgcatccagcaggccgatcgtgtctgccgccatctcgtcaataccgaagtcgccaactagattccgatcgggcccatgcccgcgccaacatacgcggaccgtccgctgcgctgcccgtagatacggcagcatgccgtcatacgcgcgaagatcgtgcgcccaaccgctcagcgtgacgaacaccgggcctggttcatgcccctggtcatcgaaggcgatctgcacgccattgacagtctttgtggtgatcataactcagctctcgaagtaccgacgtggattatccaccagcatggtgttgatctgatcctcggtgacgccgcgctcgagcagcgtgggaatgacctgatcgctgatgtgggtgaagttccagttcggtactgcggccgccttggcctcactcgagaaccagtcgatgaagcacgaggcatcatgtgccagaaccattttctcggcatagccacggcgggccagttccacgacagtgttcacccgctcctcgaacggcagcagaacatcgagaccgaaacggtccatcccgagtagcgaacccgcatcggcaagtgcacacaggtagtccaggtcggtcgaatcacccgagtgcccgatgacgaccttgctcagatctgcaccttcctcggccagaaccttctgcgcaacgaggcccgattccgtgtgcgggttcgtgtgaaccgtgatcggtaccccggtttcgacctgcgcctgaccgaccgctcgcatcacacgctcgacaccgggagtcagaccaggttcttcgatggcgcacttgaggaatgacgcgcggatgtctgtgccggcaatgccgtccttgatgtccttcacaaatagatcaaccataggctcgcgcacgtcgaacagcaaacctggaccggtgtaatggaattggaacggaatgtcgttgtacgtgtagacgccggtggcgacgatgatgttgagatcgacctgctcgttgatccgcgcaatacgcgggatgtagcgaccgagtccgatgaccgtgggatcgacgatcgtgctgatccctcgcgacttcagttcggacagcttggtcaccgcatcggctactcgagcctcctcgtcccaaggctccgggtagtcgggatagttctgacgcatctcctcccccagaacgaagacatgctcgtgcatcaacacctttcccagatcggctgtgtccaccggcccacgaacggtttgtactgaactcatggcttctatccttcttggcgcctcgccgttgtggctggcatgacgttagattaggcacattgtgcctaattcgcaataggcacaatgtgccgcttgtccgaaagtggccattgtcttcgtactcgatttgctctgcggtactcatagacaatacctctccgccccagctattgccggggagggcatgatggtaggatttagacgcccagccgggttagctcagggagagctagtggcgcccggctgggttacttgatgagttcggctgggacgttgatggtttcgcccagcttcgctcgaacgatggcgcggcaggctgctattaggtgggttggacctgccgatgctgcatcagctggcatatcgcagccgcaggctgtgaagaatcgcagcggttcgccatgccagtcgctaccgatccactcgaattcaaagcggtgcttttcaatcagtggtccgccttgagcccatgagtccgaaggttcgtatcgctcgacttcttcagtaatcgagcgagggccaaaggtgcagccatatttgcagcagtgaatgccgcctctcacgtcataacggtactgtccaatgtcatggacaatgacctcttcgccttcagccattgcaacggcccaattaagcgctgccccctcaagatcccagatcttcacttctacggtttcgctcatagttggtcctccgggggggcggatacggttgggttcgttggggttattcgcccgctgctttggagatcaggtgcatgagcatttcgcgcagttgctcgcgctctagcacctgtccggttttcgcgtactcgtcggcctggcgcaggatcgcgtcgatctcgatgttgaacatcggcgagagcacgtctggctcgcactgctcgagcagcaactggattgcgcgggtcgggtgcgccatcgtgatcccgagccagttgtaggccgaggcagtgcggtagtagcgaaggccggcgatctcatgccgctgaggcgggcggaagggtttcgtgcgcatatgcaatccgggtaggttgagcctacattttccagattgctgtatatgcgtacagtggttggcgatgggtggctatgcctgctccgacaggtactgcaactcccaggtcgggtggaacttccttggcttgctttcgccgtcgagcttgatcatgaggtgggcgcccttggcgcttgtgattgtccctcgctcttcggtgccgcgccctcggtaaatgacttggccgccgcgcttgcatggaacggcataggccttgcggatgaactccatgctcattgcgtccctccctcctgctcgcccagcaggtcgcgcaggtcgttcgcaatctcaagcatcttcttcgcgcgtgtcgtggctgctttcgtgcctgccggaacgttttcgcagttccaatcggactctcggcggcactcccgctctatgcgtcgcagcaagtcctcggcgaccggcacatgaccatccgggaccatgtagagtgccttggtcctgcgctcggttctctcccttgatacatgcccgcaacgaccagcgagcgatcgactgatccctaattcgctgatgaacccgacgagggacagcttatcagccattgccgttctccttgccctggttgagcaggacgcgaaggtctgccgttatccggtagcattcagtcgggaacgaggtagaccaggcgcatgcgcagtactcttctgggccgcggcatggctcgttcatcacctgcttggcgatcagtccatggcgttcagcgctttcctgtatgcctgccccatcgaagcttccgccatcgagggctccgcagatgatctcgcgcgcgaacttggccatcccctgcacaagcccctcgctgaccgtcataccgttgatgcgcgccagttcgtcgaggcaggcgttccagccgctattacgatttagccctgggacgccggcatttagaagcttccgctccggcacaaccaccacccttgcgcgcagtgtcgcgagttcggcgcgaagctcctcgatctccatctccatgccgccgcactgctggcgggcagcatctccctttgccgctgcgtcctcggccatggctagtttggcgactagggcgtcgtagtcggaggccaggacgacctcataccccattactgcctgctcgccctgggtcaaagagcgcatgctcggcacgtcgaaccgcttcacctcactcatgacctacctccttgctggctgctcggcgcttcttcatgatctctgctacgccgtcggggtacgtgatagccacggccccggctgcgagagctgctgacttcttcgacaggcagatatcgaagtgctccttgatggtcccggcatgctgaatccacttccgctgaacaccgatcttgtctgccattgcgagcagttcctcggtcgtgtccgcgagcatgtgacacatcttcatgcggccaaaggttgcgttcatgtcgtcgacgtaaacggccatcacaccccctccttgccgggcgcggcggccttccgaagtgcggcgttcaatgctctttccatcgatttgaacggggactcgcccggtcggaaagcgtcaagggcagccacgatcatttcgccagtaaccttcagcacgctgtgctgagccgagctgccgggcacgtcggcgagtatggaaagcagttggcgctcagccgtaattcgggtgtcgtggtccttgtcgctcatcatgttgagaagcggctcaatcggaaccagcttccagccctccggcacgctgtgctgagccttggcgaccgctagcgcctcgttgagccggaacccttcgtgcacccagtccgtcaacttcccttccagctccgcgaccctggccagggcgacttccagccgcttagcgttttcgtcgcgctcgtacatcactttcatgcacttttcgaagctgccaacagggtcacctttggactcactcaggcgctcgacttcgaccagggcggcgtcgcgctctttacgcatttcatcccagtccgcgaggcgctgctctgcctgctctgcccacgaatcgcgatccgcccgcagctccccgacgatgcggtcgtgctgttcgaataggtcagcggctttctcggcgtactcgacgatggaaacgtcgcaccctgtatcgcggccttcggcatcctcgaagcgcagatcaacgttgtcgccgtcgatgtcttcagcgtccatagcgccgatgttgcgcaggacgaacgcgacttctgctacctccggccgctcctcttcccctaccaggtcggtcccccacttcgctacaggcacttcgaaccggtcgttggctacatcaatggcggcacgcagggttggggccggagagggttgagtctgcgctggggagggttgcgccagggcggcgcgggccatccaccccttcttgttttcccgtatggagtggtggttttcgttcagatcatacttgtcttcaattccatactccttgcaggcccaggctaggaacttctccagctcatccccgcctgcctgctctaccggtgccttgttcagttccttgctcacaatcccttctcctgccgctcaatagcagcgatgaattcgacaatctctgtgctgaggtccatggcgccaatgctgttgtggaccccgacgtagcggtttgcgcgcttcagaaggagcaccgctgtgcgcaggccggagtcacgcttggtcttcgccttgacttccatcatccacctccgggtagacctgaacgccctcggcgccctgggcctggttgatcgctatctgcctcaccgctctcgcgaatagcagaatgtcgtctggggtcatgagctggctttcttcgggccagccggtgaccgtcacaccgccagggcggtgatgcgctgttagctggtgcatggggttattcctgttcggggagagggagtcgcggcgctaacgatgcccgaacctgatgccgtgctcggcggcgatcttgcggacagtagcgcggtcaaggtccattgcgtctgcggtggcggagatagtcatccccttgtctgcgcagtaacggactgtttgcgatagcagcctgcgattctctcggcggttgctttcgaacgcagcgtgcgcggcgtcggtctgccctggcttagcttttcgtgccgacctaccgttccactggacgtccttgtctcccgacatgccgattgggatggatgcgatctttccgccgctggctaggaacgcatctacctggctggctatttcgtctcgatgcaagtcctggctcatgctgccacccctagcaccttttccatgcgctcctcgagcagttcgtagaaggtctttactcgctcggacagcttgcgtatgtaggcctcatcgcggtggacgcgcaccatgcaaagcggcatgcctggccagtagccgaggaagtcgatccactcgcgctccgaaacccaaaggcctccatagcactgagccgcgtgctcggaaggcagctcgcctgcgatgatcacgctaaccagcttttccggtaccttggttttcacctctatcaggccgttgtcgccgaccagtccatccggcgaatagccgatcccgtggttcagaatgatcccggcctgctggatctgatctggctcggtatctgtgcgcaggcagtacaagtcgcgcacaaccggctcaagcttgtgacccctggcgctgctaccgttaccacgccatggctcggcctctgctccggtgatccgctcaccaattagacggtccatgtaagtgaaggcgccaacgccgaaccctgcctggcctttgccgttaaccatcaacacgtccagttcggagcaggttgcgattccaagacgcgcgtcaagccactcctgggagccctgctccaggtccttgaagatctgcatgattcactcctgggagcgcttggcgcgctcgcgagccttggtaagccgtgccagtgccgcatcgaagtcggcggatgggacaccctcagcagagccgtacatagcatcgaaggcttcttgcgtgtcctgaaggcattgggagagaagggttttcagttgctgcgcctgagcttgggtaatgagcttctttggcggcacagccgcgttgccgtcgtcgtcctcgccgcgagtggtgatgttcagcagtgcggacagcacgtaacgcttgccgtagctgaccgatgatccaagagactgaacggcgttcttgctgccacttgtgtctagcggaacgagcatcgtcgtctgctctcggtgtccggcgcagtgcatcagaattccagtaaccgaaacgccagtctgaacagtctcgacgcggaagctcactgcgaaaccgaaccgctgcatgatcggcttcacgatgtcgttgatgtcttcgaaggtcgcgtagttgctgcgcttttggccgttgacggtgatagcgccacgctcggcaatgctcggcaattcgctttgcatggcggccatggatgcgttgaactcagcctctgcgctgcgggactgcatccgttcgtgcatggccataagccgctccatcttctcgatgtcgcacgcagggtcagcagcggcacgctggatcacttgaaggattgttgccgactcaccagcttggattacggcagcaccttcctgccgctgtgcaatggagttgctcatgatgggcctcagtagttgattgtgatgtgaggaaccttgcgctgagcgatcagtgtgatcgcctgcttggcgcattcctcgggcatgccgccggcgatcagggccgccagggcttcgttgttgatggctttcttgtgggccttgtcggcttctcgggctgctgcctcgcgctcgatcctggcttgctcgtctgcctgccgttggcgctctgcggcagcggcttcttcggcgcgccgctgtgcatcacgctcagcctgctcggcgcgttgctgtgcttccaacttctcgcgctccgccttctcggcagcgagtcgcagttccagttcccggcgctcggcggcagcctttgcctcggtttcgcggcgagcggcggcttcgcgttcttcctgggcgcgtcgttccgctgcaaggcgctcggcctcggctgcttcgcgggcaatgcgctcctcgcgctctttctgctcgcgtgctgctgcttcggcgcgcaggcgttccagttcggcctgctcggcttcgaacttctcacgggcaaccagggcttctcggagagcgatcaaagccttatctttggcgcgagcagcctctgcctcgaactcttcccaggcttcacttatggccaggccttccaaccaagcgatgttggctttgagttcattagagtccagatcgcggcattccaggcgaaggtttatcttgtcgatctcgccctgatgacgcgcaacccgcgccgcttcagcctcttcccactcggtcaacggactgcgcacttcggcctgccaggaatccaacaggtcgcgcatccgcttacgctcggcatcgatcttcttcggaacttccttcagctcagcgaccaattccttgcccacgttgtccagcgccgtcttggagcgggcgaccttgtaggcgatggaagcgatggcatcgcggcccttgcgggttgaaacgtccggcacgaagccgtcgatttcctcgcgaatcttggccaggaacgggtcaaggccattggctgccgagtagacttgcagagcggtttctttggctggtacttcgaccagttggttttctgcggacatgaatgatcctcgccgcgcatgcgcagccagtgaagggaggggttattggccagtggccgtagattctgcggtgatgatcccgccccagatcgggccggctgcgagaatgaacaggtacagcaggccgccgaagaggctgcctagccagattgctgtgcgtctggtgttcatagccctgccacctcaacaaacgccacggcgaacatgaacacgctgcccacaaaaaagccgccgaagatcaggacttgggcggcctctttcaggtctatggtgatggtcatggcgtgctctccattgcttcatcaacagctttgtctacggccttcccgaaaagccagttagacacctgatcgccacagtcatcggtaagcgacaccatcggatagaccccgtctgcgtccgccgacttgtcccgcaaccaccgatagcgcttagcatcagcctcagcagcgcgcaggcgagcgatcaggccaagtatctcctctgctggagtgttgatatttacatccgtcaacactggctcgttacagcagacttcctcgcgcgcgctcatgtattcggccccggatttgaaattgccacaacagacgaatgccctcttgtggcagtactcttccaactccgccaattgctcatcactgatcgattgcacgataggggttgtcatttcccttcctcctggcggcggtagccggcgtcaaatagcgcgtaaagcgtagggtactgatatggaactccttgaattgacatagccatatcaccgactgccttctcccgctcctcggcggcgatctgctcaggggttcggagcgggcggaaagcaggaagagatccgaatttcaaaacggcatatgacccgtactgcccctttcttttgccttcgcaccaacggaatacgacacggccctcgtcgtgagcgagtatcttggctcgaaagtacgcaatatcggcgccgtcccagatggcctcggcctcaatgccaatcggaggaaagccttggccgtcccatgaggtaggcacaagccgcggaacggaatcttcaatgagggacttgccttcttctgggttgcaatacctcatccaaaagggagggcagaagtacatcggtatctcgccatccttcagccacgggtaggcgagtttttggttgtagtgcgtcgcaccctctggtgccttgttccagtcaatgctcatactcgtctctccctaaccagtcgttcagcgttctcgatcagcgttgcttcgaatgcgcggaaccagatgcgttgtgccagttccaggtcgcctcggcgcactgcaagcagtagctgcgtcatcgggcactctttgccgtctacctcggcgagccactcgggcacgaatccagcaaagccgtagaccgtgaactccggcccgataaagggcctctctttccggtcatggaacggcacgcaatcaccgtcctcgcagttcaggagcttcccgacttgctcagtgacatactctcggtcgccgtcatcgtctggcggcagcgcgttgtcccagcgctcctgggcgtatttcaatgcagtgttcatttctcacctcagtcggtgtaggcgatgtacttgaactggcctttctcttcgttgaagtactcgaagcggccgccaaacgtcccgatcacggctttttcaacctcggcgcgcgaagtgccgatggggaaaactcccttcttgatcattgacgcgcccgaatgcggttcccatgtccagtcgattttggttgggtcaagcacccgaggcttgctttcgaggaaagccccatatccaccaatgtctaggatgatcgtgtgaatctcgcgcacacagagcggatcgtccgccgcgcgccaaccgcagtcaggacagcacatgtccgcgctcgtatgcgctgcacacggagggctaatatggcaactgcaattctcgaccctctccagctcaatcactccctcgcagccgccgcggttgcagatggagccttcctcgtatccgagttctttcatgtctcacctcgcgttcgcgtgcatgcggcagcgttccgaatcgctgtcgtcatacaggcgaaaaaatgcccggacttgccgggctaatgagcggtagggtggggatggccggagtttcaccggcggcttaattggtcactgccaataagctattaccgctattcgcatgcgatacttatccccattgaagggtggcgtccttgccggggaagtcagtcggctggaggcgctgggagtggcatccagtgcgttgggcgccagttgaaaattgatgaatgtattggatcaaaccaatcccacccagcgttcagggggccatcaccgcgctgccatgtcgcatagccgatactcccctccgtgtactttcgcatgtgagtttctctcacgccgtaatctgggcaataaccaagaaacttggtgccatcctttggagcgctatcaatcgttttccactcgctcatcttgcctccagtgtgtgtattcgccagggcgcggttaggcggttggtttgactggtcgaactgaaacaacaacccaagcatcatttccaataacaaatacacaggaagcttcttcgtaggggccgtcgtagaggttgccgtccgaaccttcttgcccgaaatcgatcttaccgttcatatcggcgattccatcccaaagcgggccagtagtcagcgcatgcgatgcccattccggggcgctcttccagtcgatatttacgctgttctccagcggaagctctggactcggcatccagtatttgaccttgtaacattggctttcgcctttacgttggcaccatgcgcctaaccattcgccttctccctcgtaagttgctccttctatttcatatcgcccacataccgggatcatgatcaggcatttgtcgccaacgtttggtagatgatcactacacttgatccactcactcatctatcacctcaccaataaatagtcagaaacagaacaacgaacagcgctgcgaactcgccaaggtctggcatggattcctctcttcccgtatcagggcaaatggattgcatcccgctgctagccaaggcttgcagggacgactttcatcgcttcagcgacaatcgagtgaactccttgtgagtcaaccgtggcgaaccccttttcggcgtggtcccactgctcatcctcgtctccggggaagttgctgcacgccactgaacagacgccaagcccgtcgggcttgaagtagaggcgcacctccgggccgtcatccccgcgatcaagcatcacgagcacctggcccaggtcttcgaactcaaacagcttcgcgaactgcttcattggtattcctcggtttggtttcccagatgcccctcggaggaagggcatcgaggaaatcggtattgctcccgcgttcgcctactgggcttctacaacccgcgggtgttgctgtcctcaccactgccgatagcagctcggactcgatgtgtttggccttgggcttccctcgctgcgccttcaatcggcttacggagcaggtcatggggactaggggtgatctcgagggttcgctgcagcccggcggcctggtgaagtgggcagctgatcgcgaggcgccgacccgtgtcgtcggctgggcttagtgcttcatgggatggttcctcctctggtgatggggtggagaactctccggtatggagcaggtcgatccctcttcggggcctggaaccgacttccctcggtccgtggtatccggcgagcctccggcttgttgccgcgttgttctgcggcgttgaggtgagtatgagactgctcatatttactgtcaatgagtattcccatatttttttatgaggtgactcatcggaggtttctcaggacgaaaaaaagcccgcgctaagcgggctcgttgggttgctggaggggcttaggaaccgattccgccgccacgccagataacgcggccgatgatcggtagatcatgaactgacgtttcgcttgcgatttcgtctgggtatgcggttttgtcagggttgtcgcttcgaatgagccaagcaccagttagctgttgattcaggcgcttgatgctgacgccgccgtctggtcgcctgatgacgtacacctgcttatcctggggctctatcttggccacgtcgaagagaaccacatcgccttcgaatatgtagggctccatgctgtcgccctctgcgtagatcacgaagaggttctctggtttggagttgacccgcttcagccaatctcgcttgaacaccaaaccttcagtggtctcaacgtgatcattgaaatatccatcgccgcactcgccgcgagcagtgtattggggaatcagggcgtagtccttttcgctcggggctcctggtggaacctcttcattgttgttcatgtttccacgcccggcggctagccatagtgcgcttacgccacaagcggcagccaactgagcaatatatgccgacccctgcgacttcccctgctcaaggttggaaattgaggtttggtccaggccgactcgttgagctaattgagcctgggtgagtttggcgtgcttgcgcgcggccttgatgcggtctttgagttccatccgaaaagtatcaggggcgttcccatatccttgcaaatgagtattcccctgggataccttatgagtattcccataaggagggatgctatgaccaccatctacaaagagctcgtcgcccattttgggactcaagacgagaccgccgcgaagctcggcgttgaccaaagcactgtgtctggatgggtccggggaaagcacgggatgtctcctgttgttgcgaagcgggctcaggttctgaccgacgggaaattcaagaaagaggacctgtgtccggctttcccgtgggaagtgctgtcggcggttgcctgacatgacagccagccaattaaacgccgagcaggaagcaagggcccgcacgttcttaggcgtctccttgcatggggatgatccgactgcaatagcccgcacgttccagacttggagcgcgatgctcgagcgctgctacatccctggatccatgagtggaaagcactaccttgggcgcggaataggcgtctgtgagcgctggttcgtcttctccaacttcgtgagagacatggggcttcgcccgaaggggacgactctcgaccgagtcgacaatgatggcgattacctcccagaaaactgccgctgggcaacccgccagcagcaggcgagaaacacccgtagaaacaaaatggttggcgatgtacttcaagtcgacgccgccattgcatcaggtgttctggcgtcgaccatctcccgtcgcatggcttctggctactcagcagaagaagccattgataactcaaagatcaccaaagtgaagctcactgcagagatggcgagagcgatcaaggatcgcctgaaaaccggtgatacccagtccaagattgctgcctgcttcggtgtctctcgccagatgatctccggaatagcctccggtcgatattggaggtctgcatgaacagcatggaaacccgcgctagaaaaaattacagcctcatcgtgcagcgacttgcatcggttggaaatgcgccggttgcgcatgcagtcggttgcgacgagtcgacgatcagccggatgaagccggagaagttcttggagttcgcccggatcttggctgtgctggacctgaaggtcgtaggcaacgagatgaagtgcttcaacgagaaggagatcgccgcgatcttgcacctggcgaagtcgaagctttccgaggtcgagagcgtcgagcagttggagtgggactgatgcgaaagcgcctcacgaataccgactacgccgcaatggctaacgctgctgaagagctggcgggtatgggttcgagtgagtggaggcgcagatacaacaaagccctgcgcgactactacagggctttgtcggtgcccc

SEQ ID NO: 16 - DNA, 48914 bp, synthetic construct
  source 1..48914: mol_type = other DNA
tgcgcaagccagttgcagctggcttgcgcgtatagcaatacgtggagacctgagtatgagttacagagagagcattcgcaagtccgtgcgctttgaggtgttcaagcgcgacaacttcacttgccagtactgcggcgccaaggcgcctgacgtggtcctgcatgtcgatcacatcaacccggtgagcaagggcggcgacaacgagatcatcaacctggtgaccgcctgcctgccctgcaatctcggcaagtcggatcgcctgctgtcggacacctcaatgctggatcgtcagcgggcccagttggaagacctgaacgagcgccgcgagcagctggaaatgatgctggcctggcgcgatgagctccagtctttcggtgaagagaccgtacagctgattgccgatcgcatcaccgcgcgcatggtcggccactcggtcaacgagcacggcaagacggtaatccgcaaatggatcaagaagttctccgtcgaggagatcctggacgccctggacatcgccgccgacaagctcagcactgcgcccgatcaggaggaagtgctggagtgcttcgatgccattcctcgcatttgcgtcacccggcgccttcccgaagcaaagcagaaaatgctctacgccagaggaatcctgcgccgccggatttatgtcaacgaagctcacgtcatgccgctgatggccaaggccatcgaggcgggtctcgaggtggaagagctgatcgaatttgcgaaacaagtgaagaactggaccgaattccgggcagagatggaggaaatcgcaaatggctagggcccgcaacatcaaacccggaatcatggcaaacgaagacctagcagagctagatcctctcgctcgcctgctgttcatctacctctggatgttggccgatcgggaagggcgccttgaggatcgcccgaaacggatcaaggccgaggcacttccctacgacaacgtagacgctgacttgatgctggatgatctggccaaggcagggttcatccatcgctatgaggctgccggggtcaagctgattcaggttcttaactttgccaagcatcagacacctcatgtccgtgagcaggccagttctctcccgggcgttgacgcagaacacccaaagagagaacaaggcacaaccaaggaagtgcctggtcacaaccaaggctgtgctgagcaatcgccaagatcgcctgattctctgattccggattctctgattccagaggaagagcatgtcgacgctgacgcctcgacccattccgctccgcagcaagcagcagagcaagagcctggctccggccagaccgcacagctgttccagattgatcgcatcccttacgagaagatccgcgacctgtacaaccagatcctcggtggaaagctcaagcgctgcatgggagtgacggaggctcaccggaagcacatccgcgccgcgtacaacctcaagctcgatggcgggttcccggtccgtgacggtggactgtcgttttgggaagggctgttcaacgacgttctggattgccccttcatgctgggcaacaacaaccgggggtggcgcgcagacttcgagttcctgacaaccgccagcaagatccagcgcttcatggagggcaagtacgatgccgcatgagcgtcctctggtagcgatggaagctgagcagggtgtgcttggcgcgctgatgaagaaaccggaactgtgcgaggttgttggggctttcctttccccgaccgacttcagccatgccgacaactcggtgatctacagcctgatccttgcctgtcattcgaaggccatcgtgcctgacccgctttctctggcggaggctaggtcggagcttccaagtggcgcctttacgcttgcatacgccaacgatctatggcgcgaggttgcaagcacagctagcgccgaaaacttcgccaggattgtcgtcgagcgtgcaaaggctcgggagctgtacgaagcgggcgaacggatcatgaacatcgcccttcagagagggaaaatcccggaccaggtggctgaagcgcagagcatcgttctcgatctcaacgcccaggacgagactcctgatgtggtgacactgcgcgaggcaatgctcccagtcttcgacgaaatggaagttcgctggaagggaactcagtcggtcggactgaagttcaacctgccagacctcgatgccgttatccagggattgcgtcccggcaacctggcaatcatcgctggtcggcctggcacgggtaagacggttctcggggtggggattgctgacgaaattgccgttcgcaaccggggcgccgcgttgatcttctcgctggagatgtctcaagccgaacttgcaaagcgctcgctcgcatcgctttctggtgtttcgcaagcggcgatcgactcaggcaaagcgctggagtgccaggactctattgcgcgcatgactgccgcagtggaccaagtctccaggggtgatgtgcgaatttgcgacaagggaggactgactttcagtcggatctgctccatcgcccgattccagcatcgagcaaagccgctgagcctgatcgtcatcgactatctcgggcttatcacctcagatccgagtcaccgtcatcagaaccgaaaccaagaacttggcgccataagccgagggctcaaggctctcgccaaagagcttggcattccaattgtcgcgcttgctcagctcaatcggagcatcgaaacccgggccgacgccaagccaaaaatgagcgacctgcgcgattccggcgagatcgaacaagacgccgacgtgatcatcatggctcaccgggatatgagcactgagcgtggacagaacggtatcaccgagcttgatgtcgtgaagtgtcgacacgcaaagccgggcttctgcctgttgcagttccagggtgagttcgcgcgcttcgtcagttgcgcccaggaccgggaagagcagcaggagcagacggttcgtccgcagcgtccttccgcgcgatcaatggtagctgacttcaagccgcgaggtgcccaatgaaacgctccttgaccgtaatcgtaggcgccaagcgcttcacgatgattctgatggaggactgcgacccgctcgcggtcgtgaagagcatttggccgcaggggagggttgaggcatgaagaccttcgaactgatccgcatggaaggcctgcgcacctacggtcgccagattgaggccaatacctggcgcgaagccgagatgcaatgccgcgacggcgagatcgtaaacggcgaactgatcggtgtgtacgactgtgacccggtaactgaggccgtctgcactgcgcgcaatgacgtgatgattgatagcttgggggtgtgctgtggctgaccgcactttccgcatccaaggcgctgccggcatccgtccggctttcgtcgcggcctggaacctcatccaggggctgatgaaagaagcacagggtggctacgagctggttctacgccctctcaagtcgaagcgctccattgagcagaacaagcggtactggtcccttctgcgcgagctggccgccgtcgcctgggtcgacaaccgccagttcgacgatcaggtctggcacgaacagttcaagcgctggttcatcggctgcgaggacgtgaagttgccggacggctcgaccgagttgcgcggcatcagcaccacgaagctgaccgtagacgagtttggaatctacatgaccaagatcgaagcgtgggccgccgagcaagggtggccgctgatgatgcaggaggtcgcatgagcaagttcaaggcgggcgatctcgctcttaatctgcaagacatccccagctgcatcagtgcgggagtggtagtcgagttgatgtctcgacttgcccctggtgatctgtttgccgaagacggccagacctttcaggtgattcggccagcttggtgggtgctccatgaaggagaccggctctacatacctgaacggtatctcatgcccctgcgcggcgacttccagcccgagcagcagaaggcgaagggggtggaggcatgagcaggcggcaggttgcaaaaattctggtgggccagcttctggtcatcgcactcatcatctacacgcagacctctgcggccatcagcccatggattgtctcaatggttgggacggccaccctatggcttggctacttcgcgggagaagagctatgagccgcagcttgttcttctgcgccatgcggagagttcctgttcggccaagagcgctcattgtcctgatgatcatgatcgcctttggctgggtgccgcttgtggtggccgtatgcgaggcagtcggcgaaggggttcgggcctgccggcaggaatcgtccaggctctacggcgacttcagcaaagctttcaccgactgctggaaagccttggtttcgggggagcctcaatgagcctatccgccagccagcccaaaccgaagaaatgccagaaccctgcatgcggccaggagttcacccctcgcttcagcagcacgcaaaaggtctgctcgccggcctgcgccctgtccatcaaggacaagcacgccaagccggcgcggaaggctatcgccgaccgagagcggcgggagatcaaggttcggaaggagaggctgaagagtaaggcggatcacctgcgcgaggctcagcaggcattcaacgaattcattcgcctgcgcgacgccgaccagccgtgcatcagttgtggccgccaccacgatgggcagtaccacgccgggcactaccgcacggttgccgccagcccagagcttcgcttcgagccgctcaacgtccacaagcagtgcgccccatgcaacaaccataagtcaggcgacatcgtgaactaccggatcaacctggtgcgcaagatcggcgccgagaacgtggagtggctggaaggccctcatgagcccctgaaactgaccatcgaagaaatcaaagcgctgaaggcccagttccgggcctgggtgcgcgaactgaagagggcaacggcatgaccaaagaaactctgaccatcgttctcttcagcatagggagcggtctcatcggttatgcgatcggtattgctgccgcctggctgggaaactggttcgccgacggttatcacccgctgctgctgtcgaacatggtcagcacaccaggtgctgaggatggtgagcgcgccaacgaataccccgattatctggagcctccgagaggctgtttcggcatgtgctgtgctggatgtgatgctcgctcgcaggtcaactccaggagcaaaacagtcagcgaacagacagaccaatcttacgttttaaacgccgtgctcagcgctcaaggggatgaatgatgatctacaccagcattcggtcggcagtcgtctctgccttggcggcggaaaccatcgacaacactgcaaagcaagcctggcagaagctctaccagccagggtatgccgagagtgagggtttagctgggctgatcaggggctcgaacacgtcaggcatcaagcgcatcgatgctgattgctgggtgcacgcccggctgcacagtcagctcaagcctaggcactggaacgcgcttgtggcgaagtacagcacccaccgcgagaagaagaaggccgcaatcgaggcgcttatccccctgatcgccaccccggcgccgcgcagattcctcggaatggcagtctatacctgggctatccccaagctgaagggggcagaaggcaagcgctctaccgacatgatcattctcgacgccgtgttctaccacatgaacaactgggaatctgaaggccgccccgaacagacgaggcgacgctggaggtcaggaattcacagtgtgctgaacgaaatgctcaaggaggcagagctcgatgcgggtgaaatcctgatggaggagggcatcatcgtcggagaggctgcgtaggacttgcaattagtgagcgtttgagcgaatatttccccatcctgccgatcttgcgcgttatgaggatcggtagctctgaagccctggcaaatgccggggctttttcgtttccggggtatggatgaatctcgagcatcgcataaggcgctggcttcttcaggctgggcgacgtggcaagccgatccacgcaattctcatccaccccaacgacatccaatctgcaagaaagatctgccggtttgtgccagtgaaggtgctcggcattgaagtacgccggtatggcgcaacagggagcgctgctgatttgtaatcagagggttgcgggttcgactcctgctgccggcaccacactacaaggcccaggcaatgacctgggcttttctgcatctggagtaagcaaatggacccgatgacgaccgttggcggaggtctcttcgccaagtacagcgtcgctattgccgggttctgggggtctattctgtcccttggattcctgagcggcctgaaccgctggcaagccgcgctcgctgtagcaaccggattcgggtgctcaacctattggactgctccggttgccgcatggctttcgcgtgagtacgagattccactcgatgacgcatttctgagtggtgtcgcattcaccattggtttgctggcgatgaatatcatccccggcctgaaggcggcagtaacggcaatcacagagcggttccttcctacgagaggaacctgatcatgatcatgtcgattctggcggcgctggatgcgctgctgtgtgtgcttgtcgttgtagctgctctggagttcctgcgcaccgtccagctgtctgggcagccgctattgggtatctccttctacctggtggcaggtggtgcattcggaatcctgtacggaatcatgaagggcgcaccggttaatccattttcggtgatcctccatgctgggctcgtactttacgcctggtcccggcgccggcagatattcggaagcgactggtcgtggaactgaagcgacctaaccctccagagacgatcgggcagttcgcggaaggcgaagattgggcggacgcctttgtccccgctcaggatgttctggcttgggcgaagtcagtgttaatcgatccgaacggaatcctgggcaatgaagaccacgcccacctacaagacgctcctctcgctttcctatgggctgcctccagcttcaccaagcaggggaggacggtactgggtcagtgcgaagaggtgacgttccgctgtggagcctggcagaagggtaggcaggaacagcagatgatccgttggttcggatacctgccgaggtttctgatcaccctggctgctgactactgctcccagtgctccgacgcggagttctgcgcattggtcgagcatgagctctaccacatctgccaagagcacaaccaatatggcgagcccaagttcaccgaggagggctttccaaagctgaagctccgcgggcatgacgtcgaggagttcgtcggcgtggtgaggcggtacggcccaagcaaggacgtgcagtatctcatcgacgctgctagcaggcctccagaggtggccaaaattaacatttcgagagcctgcggtacgtgcctgctgaagtcggcatagccacgacaggcccatgacaggaagaaaaacgatggcaaccctgaacagcgacgtgaaggcgttcatcgttcaggcgctggcctgtttcgatacgccatcccaggttgcggaatcggtcaagaaggaattcggcatcgaggtcagtcggcagcagatcgagtcgcacgacccgaacaaggtgtgcagcaagggccttgccgcgaagtggcggatcctcttcgaggacacccgcaagcgcttccgcgaggagatcgccgacatcccgatcgccaaccgcgcctaccgactgagggcattgggtcggatggctgagcgcgccgagggcatgcgaaacatggccctggctgcccagctttacgagcaggccgccaaggagtcgggtggcatgtacagcaacaagcaccagctcgagcactctggtcctggcggaggtccgatcccgacaatgccgaccaccatccagcttgtggcgccaggccatgaccacggcgaagattgaacttccgccaaagctgataccagtcttctcaggccctgcccggtaccgcggcgcccatggtggacgaggcagtgccaaaacgcgcacgttcgccaagatgacggcagtaagggcgtacatgtacgcggaggctggaatcagtggcgtgatcctcggggcgcgcgagtacatgaactcgcttgaagagtcctccatggaggaaatcaagcaggcaattcgatccgagccatggctggacgcgtactttgacattggtgagaagtacattcggaccaagaatcgccgaatttcgtatgtgttctgcggattgcgccataacctcgacagcatcaagtcgaaggccagaatcctgatcgcctgggttgacgaggctgaaaacgtcagcgaaacggcgtggataaagctcctgccgacggttcgtgagaacgactcggaggtctggattacctggaacccggagcgcgatggaagcgccaccgacacccggttccggaagaacatgccggcaggcgcaaaaatcgtcgagatgaactacacggacaatccgtggtttcccgatgtgctcgatcaggagcgcctgaacgaccggcagacgctggacgaccagacctatgcctggatctgggatggcgcctaccgcgagaacagcgacgctcagatccttgctggcaagtaccgggtggccgagttcgagcctggtcccgattgggatggcccttactacggcatcgactgggggttcagccaggacccgactgtcggcgtcaaatgctggatttacgaccgcaggctttggattgagcacgaagccggaaaggttggacttgagaacgacgatatcgctgagtacatgatcaggcgcttgccagggatcgaacgacatgcagtccgagccgactcggccaggccggagacgatcagccacgtcaggagtaaagggaaagatggcagtcgtgcatgtctgcccaggatcgaaggtgtcgagaaatggaaaggcagcgtcgaggacggcattgcccaccttcgcagctatgtcgagatcgtgatccatgagcgatgcacgaaaaccctccgcgaggccaggctatacagctacaaggtagaccggcagaccggggatgtgcttaccgatatcgtcgacaagaacaaccactactgggacgccacacgctacgcgttgggcccgctgatcaagcgccgcggcgcggtcggtatgctgctaccaggagcccgctgatggccatcttcatcctcacggagcgcgcaaccagccgctccatggtggtccgtgctcgctgcacgtcctgcgcccgcaccgtggcggtcgagaacgctggcgctgaagggacgatggtatggcgcgaccccaacctctcttctgtcgaactggtccgcgagacggacaagccaggcctcatcctgaaatcggactgaccatgactgacaaactcgacctcgcggtcaatcacgcgatgagcagtgctgtcgcgcgtgcgcgaatgagcctgctgaaccagggcatcggccatgacgccaagcggccgcaggcatggtgcgagtatggtttccctcaggaaatcacgttcaacgacctgtacaccatgtaccggcggggcggtattgcccatggcgcggtcgagaagatcgtcaccacgtgctggaagacaaatccgcaggtcatcgagggcgacgatcaggaccgctccaaggacgaaaccgagtgggagaggaagaacaagccgttgatcgcaggcggcaggttctggcgggctgtctccgaagccgaccggcgccgcttggtgggtcggtattccgggttgctcctgcacatcagggatagccagccgtgggatatgcctgtcacgggaaaggtcaatggcctggcgaaggtcaccccggcctgggctgggtgccttaagccgaagtcgttcgacgaaaagctagatagcgagacctacgggcagcccaccatgtgggaatacaccgaggcctcccaagccgggcgccctggcctggtgcgggatatccatccggatcgggtgtttatcctcggcgactggaccggcgatgcaatcggcttcctggagcctgcctacaactccttcatcagccttgagaaggtcgagggaggcagtggcgaatcgttcctcaagaacgccgcacgtcagctcctgctgaacttcgacaaggagattcagctcggcgagatcgccagcacctacggcgtgacgatcgatgcgctcaacgaacgcttcaacgaggcggcgcgtcagttaaaccgcggcaacgatgtcctgcttccaacccagggggcgaccgtcacgcagatggtgtccgccgtttcggaccccagcccaacctacaacgtcaacctgcaaaccgccgccgccggggtcgacatcccgaccaagattctggtgggcatgcagaccggcgagcgggcgagcagtgaggaccagaagtaccacaacgccagatgccaggcgcgccgggtgcaagaactgacgttcgagatcaacgacctgttcgggcacctgatgcgcatcggcgtggtccctctgaaggccgagttcacggcaatctgggatgacctcaccgttccaaccaaggccgagcgcctggccaactccaagaccatgagcgagatcaacagcgccgcaatcggcactggcgagccggtattcaccgcggaggagatccgcgaagaggctggctacgacccgctcgtgggcggtgacccgctgcctgataccgaaccggaggatgaagatgccgcgcgcaccgatcctaccggcgagcagcagtgacccgaccggggtagatcgactggaaaggggcgcaatgcgcgagttcgacaggcgcatgcggaaaatccgggatggctatgtcgctgccttggaccgaatcccggcccagccggtggtgaatgagcagtacacctaccgtctcgaccaggcccttctctccgcgatcttcgccgacaccaacctgatggtcgacgagatactgcaggagggcggggagcgcgacctctggttcttcgaatcctatgtcggggttgcctacatccgcggtaccgcacagacgcatgccaacctggcgcagcaatcgcctgcataccgcgccggccgggaatcgctggatgtcctgcttcgatccgacgcctaccgcgcgcggatggcactgcttcgcgcccgggagttcgaggagatgaagggcttgtccggccaagtcaaggccgacatggcgcgcattctcgccgagggcatggggcgcgggaagaatccccgcgaaatcgcacgggacctgaccgcacagaccggcatcgaggcgcgtcgcggccatcgcatcgcacgcaccgaagtcacaaccgctctccgaagggctcgctgggacgagaaagacgctgctgaggccgactacggcgttcagtcgaagctgatgcatatgtcggccctgtcccccagcaccagggcaacccatgcggccaggcacgccaggctctacacctcggacgaggtgagggactggtacagccgagacggaaactcgatcaactgcaagtgcagccaggtcgaggtactggtcgatgacgaagggaatccggttgtcccggccatcgtcgagcgcgcgcgccgcaactaccaagtcatgaaagccaaagggcgcgggccctgggcgaaagaggattgagccatgcccatgcaggtcaacatcaccacccaggtcaacagcgccagcattcggcgtgagacacacaacgggcgcgaacacctggttctgccgagctacaccctgccggccggcgtgatcatgaacggtggtctctacaccgccgagcagatcgacaagcactacccaggcctggagggaacgctggcgccgctcgggcacccgatggtcgacgggaagttcgtgtctgcgttctcgcctgaggggatcaacgccgcccacgtcggcgcctggaaccgcaacgtgaagaagtccggcaaccgggtctacatggagaagtgggtcgacgtcgagtttgccaagtccacggagggcggccgtgaactgttgcagcgcgtcgaagcgctggagaagggggaggacgtccccccgatccataccagcgttgccgcattcctcaatcgcatcgagccgaacgaaagccagcgtgcccagggcgcggagtgggtcgccgacatccagagcatggatcacgacgcgatcctgctgcacgaagtaggggcggccactcctgagcagggcgtcggcctgatggtaaacgccgaccaggctgtcccgcttcagccgaattccggcgctctggttggcgagtcctaccgggagcgggagcagcgtctcgatcgcgccgcaaaggagcgattcgcctccgggcccgaccagtacgcatgggttgccgacttcaccgattctcaggctgtgatcagccgcaatggcggtgtgaccgaggtgtacggctacaaggtcgaggcagggaagatcgtcttcgacgaatccggccagcccgttgtcaggcaagagtcctgggtcgccatggtggccaacagcatcaagaacattttcacccatcgtcaggctcggcctgatcaacctgagaaggagggcgacatgcccctgacccccgaagaaaaggccgaaatcgtgaaggaaatcggcaccaacacctccagcgccatcaaggaactggcggacactatcatcaagcctctggccgacaaggtcgacggcctggtcgccaatcacaaggcgctggccgacacgctgaccgccaaccagcgcgccgaggaagacagcatgcgcgaagcggtcaaggccaagtttggcgaggtcatcgccaacagcctggccggcgacgcgctcaaggaactgttcaagcagtgcggcgaatccgctccactgggcgccaatgctgccaccgacaaaggcggcctcaccgccgatatcgccaacctgccgaaggagtaagccatgtctcgctatcgtcgcgtgaacatcgacggcaagtcgctgttcaagaccgaaacccgcaagaccgccgcggcactcctgcccggcacgttcgccgtgatcaatggcagcgacctgttcgcccaggcaagcgccagcgttggccgcctctacgtcatcgactgcgctcaccacgaaggactcaacatccgcgatgcggttcccgccggccattcggccgtgggcaactacgtcgaagagggtcgcgaactcgccgtgctgtgcccggccggcacctacaagaaagacacgccgatcaaactcggcaccagcggccagggtgccatcgcgtcgagcgataccgacacggtcctcgggtacagccaggacgatgcagtcatcgcctccggcgaaaccgacttcatccgcatccgcttccgtgtcggcagtgtcgccgccccggcgccctaataggagtacggacacatgttcctcacccagcaagcaaccgccgcccatcctcgcctgatgggccactaccaggagttgcaggccaatcgcaacatctggaacaaccagaacgccgctatgatcgcccgccaccgcggcgccatgacccccgaaatgctggcctgcaacgcgctcgccggcctgggtcgtgagttctgggccgaggtcgacgcccagatcatccagtaccgcaaccaggaaaccggcatggagatcgtcaacgatctcctgcaggtgcagaccgtgcttccgatcggcaagaccgccaagctctacaacgtggtcggcgacatcgccgatgatgtgtcggtgagcatcgacggccaggccccgtactccttcgatcacaccgagtacaactccgatggcgaccccattccggtgttcaccgccggctacggtgtcaactggcgccatgccgccggcatgaacaccgtcggcatcgacctggttctggactcgcaggctgcgaagctccgcaagttcaacaagcggatcgttgcctacaccctggacggcgccaccaacatccaggtcgagaactacccggctcagggtctgcgcaatcaccgcaacaccatcaaggtcaacctgggctccggcgccggcggcgcgaacatcgacctgaccaccgccacgccgcagcagatcatcgacttcttcaccaaaggcgcattcggccaagctgcgcgtgccaacaaggtggacgcctacgatgttctctgggtttccccggaaatcaacgccaacctgtcccagccctacatgatcaccatgggcggcggtgccaacgcggtggtggccggcaccgtgctcgatgcggtcatgcgcttcatcccggcgcgcgcggttcgccagaccttcgccctgtcgggcaacgagttcctgggctatcagcgccgccgcgacgtggtcaccccgctggtcggcatggctaccggtgttatcccgctgccgcgcccgctgccgcaggtcaactacaacttccagatcatgagcgccatgggcatccaggtgaagaaggacgacgaaggtctgtccggcgtgatctacggcgccaacctggcgtaaggagaacgacatgcccaaatacgaggtgatcaagccctggaacggcgtttccaagggtcaggtgctggagctcgaatcacttgccgctgcgctcctgccgaacgtgcgcgaggttggcgcactcaggagcggaagcctgaccttggacgtttcggcccaggtcgacgaagcggccaggcaagctctcgccgaagcgcgtgtatccgtcgatgccatgatcgacgaagccaaggcccaggccggtaccctgaccccggccattccggacggtagcgagcgccgcgagctgatcaaagcgcgcctgaaggagctgaagatcgagttcgatggccgccagggcgaggaagcgcttgccgccctgctgccggagggcgaactggcgaagctgttcccggccaagtgaccggtgcgtgacgagaggccgcctgcgggcggcttcgtcgtttctggcctcagcgatggggtcgcttcttctggagaatgaaatgtttggcaatctgatcgactcggacatcccggcaattccgaaggctccgcccgctcccatggagttcccggcctcgttcggggctagcgatgacttcaggctctgcgatgctatccggaacaccgtggatgctgcgcaagacgcccaaggtatgacgcttcggattcttcaacgacacctcctccgtctgtgcaacctgcaggtcgagcaactggagggatgtggtgatgatcacagttgagcaggcccggcagtatctgcagagccagggcatcgacaacgtgcccgatttcatactcgcggcgtggatcgagcaattgcaggagatccagagttgcctggatgcccactacccggcatcgaccgcgctgttgatccaggcctacctgctggcgctgtttgcgctggcccaggccgacaagtacatcagcagccagacggccccatccggcgcttctcgatcgttccgctaccaggcctttgctgatcgctggaaggcgcagttggccctgctgaacgccctggacaagcacggatgtgtgacggggctgattcccccgaacccaacccagaccgcacacggcggtctttggatcgcgcgaggcggctgcatgtgtggtgactcatgagcacgacggcgaattggagttacaccaacacggcgacggttcggccattcctgcacttcgacctttcgacccaggaggccgtttacggccctgagtacgaaatcgcctgcacctggaccgccaagagcgagcagatgcgggaggagggcgggcaatctggagcgcggggggctgagttcgtatcgcgccaccagatattcaccgaggaccgccggccgaagtacctggacctgatccagttcgacggatccaacggctgggaagagattcgctcggtgacgaactgggacatgtccttcttcggtgaacagccggactttctgctggtgacctgacatggcaatccaaggaatcgaccgcgtccggcggaatcttcgtgtggctgtcgaaaacatcgccggcggtgtttccgagcgcgcagtttacgaggtactgagccagggcgccgcaatggcgcagaccatgacgccgatcgacacgtcgaatttgatcaatagtcagactgcaccccagatcagtaatgggactgctggggtggaagggcggattggatatacagcagcctacgcggcagcggtccatgatgcgccaggaactctcgccggacagccaagggcggatttcggaaagacagcggacggaaccgcctttggaggcggtactggagttgggaactactgggatccaaatgcagagccagagtttctcactaaggggttcgatcagattgaatctgcaatcccatcaattctccgcaggatctaccgcgtatgaccccctacgacgccttccaggattggctggcttcgatcctgggcgagggctaccagtacagccgtgggatgtgggtcgaccacccgtcgctcgactcggcattcatcgcagcgatccagcaaaccggcggccccccgactcaggtcgacattcgtcgcctgcggttcaaggtgatcctcctcggcccgaagggcgtccggaaacatgttgtcgacgtcggcaactcaatcgagaccctggcgcaggtagcgcttggtgacagcgtcccctgtggcgccgcatctgttcgggcaatcggcgagccgatcgggcctggatacaccaccgaaaaccgggcctggtacagcctggaccttgaagttctctattaatcaggaggccagacatggcttgcaagaagctcaaatttccgggccgcgacgtcgtgctcgagtattacatcgggtgcggcgatgcgctgccggcggagaatgactggcgccgttttgggtcgctccgcacgaaggaattcaccgtcgagtgggacaccatcgacgcgactgattccgactcggttggcgcactgcgggagaacctggccagtttccagacgctgaccatttccggtgacggtaccgtgaaggcctccggtgccggcgcgcagaacctgatcgacctgacgaagcatgtcgtgaagccggacgcgaccggcggacagcctgttgtctggatgcgcatgaccttcccggacctgaccttcaccgcattcatgctcatcagcaacctcagtcgctccgcgccgtacgacgatgtcaccacctacagcttcgaggcttcggcgaccgcttccgacttcggcctgatcgtcgaggatacccccgacgcggatgcgccggacccgaccagcattcaggtcgtgccggagaccctctcgcttaccgttggcgaaggcttcaacttcgagggcgtcgtgctgcctgttggcgctccgcaaggcctgcgctggacttccagtgcgccgaccgtggccgcagtgaacacggttaccggcgaggtgagcgcgctgtcggccggtaccgccacgatcaccgccgcttccagcgtcgccccgggcgtcaccgataccgcaaccgtcacggtcatcccgctggtgcagggcatcaccgtctcgccgacatctgtctcgatcgccgaaggtgccacccagcaactgaccgccgctgtatctccgactggcgcggctcctggcctggtctacgaaagtgcggcgccggcgattgctaccgtgagctctaccggcctggttaccggcgttgatgtgggcaccaccacggtgaaaatcaccagtgcggcgcggccgtcggtgagcgtgacagttccggtaaccgtcactgcgccgtgatcctcaccgagatcggtgagataggcgtacacacggcctcgggggagttctttctcctgcggccgtccctgtacgccatgacccagctcggtacgccggccgagattgtcgacgtcttcgcgcgcgtcatgagcgacccgatcactgagaagcatcaggcggaccagttcgcggacgccctggccgtggtggtggcctgtagtgagcaggacctgtccgacgtgtttggctactacgaccaggatcttgtctaccggccaggaactgcggacgtcgagcaccttgtgcctctcgcgcgctgcctgctgaagcacggcgtcacaggagcgcttccgccgcttccccggcgccacgacgaagagccgaactactcgggggagttcgttgcgcgggagtacgtcgcgacggcgatagcgcacctggggctgagcgagcgcgaagcttggtccatgaccatgaccggcctgatcggcgccctgcgcgcgaaataccccccaaccgaatcgaacgctccgggcgccagagccccgaccgcggcagagcatgacgcgacgatggagtggttcgacaagatcgaggccaagcgcaaggcgcgggcgaaaggagcaccctgatggctgagaatgtcggcagcatctattacaccgtcgaggcggatacctctggccttgtaaacggcacgaatgctgctgaccgttcattggatcagatgcaggcaaccatgcggcgtgctgatagcgaggcggcacgtctcaacacgactgtcaccaagctttcgtcggctattaagacgatcatcgcggcgtcagcgctccgcgagatggccagcatggtccagtcctatcaggagatggctgacagggttcgtctggcgtctgcaagccaggaagagtatgaaaacgtacaggccagactgctccgtaccgccaacgggacataccgagcgctctccgaggcgcaggaactctacatccgcacttctgcaggcctgaaagctctcggatacgacacaacgtctgcactggatgtgatggattcgctgtcgtatgcattcgtgaccaatgcgaccaaggcggatgcagcagaggcagcgatcagccagttctccaaggcaatcaacaccggcaaggtttcggctgaccaatgggaaacaatctccagcgcagttccgtctgttattgaggatatcggcgccgctgcaggtaagacgggggcggaagtcaggagtcttggtgcgcaggggcaattaacggcgcaaatgctcaccgagggtctacgtaagtccttggaagagaactcaaaggcagccgccggcatgtccaataacctgaccgatgcaggggtcaggattcggactgcatttactcaagtccttgtttcgctggaagaccagactggcgcccttcaaaccttcaccaatggtcttatttcggctgctgatgcgcttcttgagttcgggcttgactcggaaaaaatggcagcatttctcgacactgcaacagtcgcagcagcttctctggcctctgttgtggctgggcgtctagttacctccctgtatgcagcaggtgcggcccaagtgcaaagattgcgggcaacgcttgagcagatagcagctgatcggaatgctgctataggtgcactgaggcgggcagaggcagagaaggccgccgccgccgcggctgtcgctctggctcaggcggacttgaatgctgccaggggttcaaatgcccacgcaacagctctaaacgcgctgctggccgctaaagaacgcgacttggccgccacaagagcgctaacggctgctcaagcaacgctgaatggtgtagcaaccaccgggacggtggtgatgggtggacttcgatcggcaatggcgttcctcggcggaccgcttggggttgttctgctggcagcaaccgcgatcgcaacatttgcaacgaatgcacgggaggcgaaagagcctacggaccttctaaccctgtccgttgaaaaacttggacaggcacagctgaaggttgcacaactggacatcgacaagcgaatccaagcagtgagcgataagctcaaactgcttggggaaaactatgcgttcgcggcaaaagaagcccaaggctctggtcgaagggccaatcgatatgctgaagatgccgtgcgtatccagggcgcggtcgaggagcttacgcaggagcttgaccagttacagaaaaagcgttcagacgtcgacgcagccctagataaaaagagttcatccccatctggtaatggcccggatcgccaggcaaacccggaggatacaaaggctctccagaatcttcgcgacgaggctgaactatctgctctcgcgggtgaagaacgggcgaagcttgccgcgcgcaaaaagctcagtgctgatgccacaaaagaggagatcgcggaggcggagcgtctcgctgtccagatattccgcaacagcgaagcgcggaagcaagagaagaagtcagcctctgataccgcctctacggtcaaaaagtcgatggaggatcagcgtcgcgctgccttggacaatgagaagactatcggagacctttcccagcaactggcacaggctggactgaagggaaaggaactggcagaagctggggcgcaatctcgccttaatccattcgccacgccggagcaggtcgcccaggtccgcgcgctcgccgcagctctgtacgaagcgcaacaggtcgaagccaacaagcagttgctggggcaaatggaccctatcgccggcgaagaccagcgctaccagaccgaactggagaatctgaaaaagctgaacgaggccaagttgctcgaggaccagcgctacctggaactcaaggcgcaggccgagcaacagcacgatgccacgatgaagcaactggaggaggagcgattccgccgccaggctgccggcaacgagatgatcatggcaacgctggatcaggtgcagcaggccggcacgaacgctctgactgggctgataaccggggcgaacaacggtgccgatgccatgcggcaactggccggcgccatgctgaaccaggtcgttggcgccctcgtcaaggtcggcatcgaacaggcgaagaacttcatcatggggcagagcatgcaagcgaccgcaaccgcccagggcattgctcaggccggggcgttggctggcgcatatgccccagctgcagctgcggcctctgtggcctcatttggcggcgctgcgacggcaggccttgctgcaatggcagcagcaatcccagcgatgctaggcctcttcggaggacgccaatatggcggaggcgtccaggcaaatggcctgtaccgaatcaacgagaacggcgcgccagaggtattccaggctgcgaatggccggcagtacatgctgccgaatacgcgaggcgaggtgatcagcaacggcgacgccaccgcgcagggctcgccgcagatcagcctgcagatcatcaacaacggtcctccggtttccgccaccgccaccatggacgggaacaacctgcgggtaactctcgatgcggtcgagcaggactttgccaacaaggtttcgtccggccaggggctttacccgaaagcaatcgaaggcgcatatggattcaagagggcagggcgatgatcaaatggcctgatggccttcccttcccgctcagggaggggtacggcttcaagacggtagagccaatggccaggaccgtcctccagagcggccgtgcacgctaccgacggaacttcagcaatgtgccggtcaacctggaggtttcctggctgttcaccgctgagcaggcgcgtctgttcaaggggtggtaccgagacgtcctgaaagacggcgtcaagtggttcgagtgcgatttgcgtacggaagagggaatcgttccgtgcaacctgcacttcgaggggatctacgacggtggctatctcgtcgggcgcgaccactggcgcttcaacgcgaccgtcgtgatgcgagagcgctcgatcatcgatcctgggtgggctgagattctgcccgagtacatcctcctcgctgacatcttcgacatcgcgatgaacagggagtggcctcgacatggcgacggctcttgagcggttctatgcctcaggcggtgaggacctgcagctcgccacgatcgagttgtcatgcccggcgtggccggagcctattctcatctgccagggctatgacgacctaacctgcatgaccgaagacgggcggctgctgacgttcatcgctggtgcgatcgatgtatcgattccgaagcgagacaacagcggaaaccagaacgttggattcgcgatcgacaacgcgaccggattcgcccagcagcgtatcaacgaagcgctggaggctggcgagtatgtcaccctgatcctgcggatgtacctggagagcgatctcacagcgcccgctgagcggccataccgcatgagggtcaagacgccgggtttcgagggtctcactgttcaggtcgaggccggttactacgacctcatcaataccgccgcgctgcgccacatctacaacgtcagcgagttctccggactcaaatactggccttgatcccatgccgaacagatacctcaccgccatctataccgagggcgggcgggcactgccgtgcctggactgctggggcctgacgctcatagcgcgggttgagctgttcggactgccgatgctgaccgacttcgatggtgtcacgcgactcaccccggtttcgatgcagcgggcgtgcgatacggagatccagcgcgcgctcgagcaatgcgagccaggacctggggtcatcgccgcggcctatagagggcggctgctcgatcacgtaggtctgctggtcgaggtggatggacgcctgcggattctcgaaatcaacccgggaagcggggtgtcgctcaccccgctccagatgttctccgacaaatattccaaggtggtcttctaccgtgatcgaaatctacccatcgctccttgacggagaaccgctggagcggcatccgatcggtcgcaggatgacgattcatgcctggctgaccgcgaattctcctgggtaccgctgccacgatgtccacccgttctccatcggtgttgtccccgccgaggttgcgctctgcggtgacctgaccgacaagcagaaaaaggcgcatgaggagttcgtccaccccggcgagtgggccgagcgcatcatcgaccgcggcgacattgtgaggatctacaagctcccgcgcgggactgatccgttcacgattactgcggcccttttcaagggggcgcaatcggtttttcggatgctcatgcctcaattgcccggcatgccgacgaaccccgggcagggcgcgtcgctctctgaaaccagcgcgcgcgggaacaaggtaaaactcggcgatgcgatccgcgaagttgctggccgtcgtctgatttatcccgactacatcctgccgcccaggaagtatttcgccggtccgcgtgagcagtggaccgaaatgctgttgtgcattggccgtggtcggttccagatcgccgaaggtgcagcgaaaatcggtgaaacgtcgttcctggcactgggcgctgatgcctctttccagattttcgaaccagggcagaacgtcagcgggcacccggcatcggtctggtggcacctggttgaggaagttggtgcgagctcaactggtaatgccggcctggacctgaccgagagctccaatctcacgccgaacccgtcggcaactacgttcacgttttccggaacgaacatcatcatttctgccggagccgggtcgttcccctctgacttggttgcggggacgatcctccgggttgaggcgatgtacccctattcggttaacgatggcggcgggacgaatcgcgacgtcgtgacgggggatatcgctcagctcgggctggatgttggcgatgagatcgaggttgttggcaccaacggcggcctctacatcgtaaacgacatcacctccacgtcgatgacgctcaactacagcaacggttctccggcgaatgcgctccagaccgggtccggcagcgccgcaatcggcccgcgcggactgcgctatcggatcacggcgtacagcgcgcagcaactcacagtcgagcggctgaccagtgccggcggtgtagatgtggactggccaggattcaccgctctcaattcgtctacgtctcgcgtcacgatcgatccgactagcctcgaagggggctggcgcgggccattccctgcatgccctgtatcggagaagaccaacttcgtcgagatcgacgtgttttgcccggaaggcctgtgcggtgtaggcagggaagggcagatctaccagatccgcacctattacgacatccagtggcgagacatggccatcggcggcgcatggacgacggtcagtaagaaccatgctggcagttctctcgaccagcagggttttacggacggcatctcgctgccgtacatgatgcggcccgagtttcgcatcagaaaagtgttcgtcaaccagggcggcaactcaacatccgagtaccgagaccgcactcagtggtacgggatgcgcgcgcgcctccaggctccgtcgtcctacgccggcgtcactacaatggctgttcgatatcggtcgtctgaccgtatcgcggcgcagacagaaagccgcgtctcggtagaggctacccgcatgctaccgactcggcagaacggtgcatggacacccgagatagcaacgcgagacatcgtcccattcctctgctacatcgcgaaggaacgcggctacaccgatgcggatctcgatcttgaggaactcgatcggctggacgcaatctggaaggcccgcggcgacacgtttgacatgatctacgaggacggcaaggtcacggtcgcgcaggtcatggacgatgtgcttgccgccgggtatgcggagaagaccattaagcgcggcgtgatctccgcagcccgagacgaaccaaggaccacattcgggcacatgtactcgccgcagaacatggatggtccgctgaggatcagcatcagcgcgccgtctgaggacgactacgacggcgtcgatgtagagttcgtcaatgccaacggctggatcgaagataccgtccagtgccgactgcccggcgatgttggcaggaaggtcgagaagatcacggctgtcggtgtcacaaaccgcgatcgcgcctggcgctacgggatgcgccgccggatggctcagcgataccggagaactgagtattcgttcgataccggcctagacgcgctgaacagcgagttctgggattatgtggcccttgccggcgatgttcccggccctggcctggcgcagagcgcatacctgaaatcgttcgttatctctggaaactcggtcctgatcgagtccagcgagccgctcgactggtcactgctgaactcgccagcgctctacctgcggcgcccaggcggaacggtttccggtggatatccggcgtcgaggatcgacgactaccggctgagcattcccagcatcgatttcgtccctgatgtttcgtgggaaatcgaaccgccgcacctgctgctgggaaatccatacccggtgctgatcagttccatcgatcccaacggaaataccgcggcatctgttcgtgcggtgaactattctgaaagagtatacgattatgacgattcatttgcgcctgagtaatccaatttggcccccttctttaggttgtcttctgcccaaagaggttgaagatttgtatagtgattcagcctgattacctcctcgttagaggatgcagaggaaagcgggatcttgtggtcaatatgccacaaatcccgattttcccaagtcattccgggcagaaaaagagtctctatgtgcaatcgtaacgtatcccaatcgcatccaagtatctctgctgtggctgatgattttcctatgccctgtctttttagtactgttgatattctagagcgaatattgcaccttaatctaaatattggatctatgcttcttcgagttttcatatagctgttggctctagagttctctgtttctttgtttttcctgtagtaatttcttcttttttcaataagtttttgtgggttttcttcttttcttttcttccatatttctgcatgccttccttgaattttggatgcccaagactttgcatgagcctttaccctatcttgattcttcaatttccatgattttgagtattcttttagtctctctgagttattaagataatatgtcttgcttttcagtctgattttttcacgattttgttcgcgccattctcttgttctggagaggattttttcataattttgtttctcatattctttctgctttgatcggattttttcgtaattcaattctctgtatttttttcgtttttcgtttacgcatgacttgcattgagagtggagtccatcctttctttgcttattttttatgaactctgatacgtgcagttcctcgttgcagctgctgcatgtttttttgcttgtcaattcaatctcctattcttgtgttgttagcttggacctgccgagctacgcatctaagaatactgcaaagctatagattaacctggacaaccatacacaacctagcccgccatagagcgggctttttcatgcttggagaatttgcatgactacgtacgccaccagcaatccgcttggctccaaagacccgcgcgacttgtacgacaacgccgagaacttcgacgcggcgatgaacgaccgggtaaacaccacgtggaatgatcgtttcggcgttagtcgcccaacgatgaaagggtatgaggaacagttcaacggctggctggacgcccaaggcttcgaacccggagtcctggagtacgtcgacggctcaccgctgaccgtagaccgtccgacccaactgatccagcgcgacggaaacctctacagcgtcaagcgtcctgcatcgttccccgtcaatctgaccgggaactgggcgacggaccagagcctgcttgttatccaagtagaccaagggttcccgcaagaaatcggtcgcggcgtacgccgggttgactcggttgccgacctccgggccatcgcagggcgattcgccggggatgccgcgctggttgtcggatactacgcggaaaccccgggggtcggcggcggagagttccactgggattcaacctcgatagaggacgacaacggcggctcgatcatccaggcaaccggtatcaccactggccgatggaagcgcgatataacgcacggcgtgtgggccgaatggttcggcgctcgcaatgatggtactgatgctgcgggaactactgctgcggtgtgggctgcaatcatcgcactccggcacgacccggagacaatcgtgcagtacatcggcggtcccactgtcacagcgtatgcatccgggcgactgaacttcggtaacggggtctttgcactccagcctgatagtttcgatattacccaggacctcggcctgaccatcgtcgggcagggattcagaggtaagaaccaggcgatgaaggcggctactactctggtagtgagaggtacaagctctggcttcttcttcaggcactatgggaatggcggcaggaatctaacattcaacaacattgatgttgtgtatgatgacagccaattcagcggcgatatcatagaaaccacctcttctcccggccttactctgcaaagggtgcgggttggctgttatggtggatttcttgccagtcgtctcaccaccgcgagaagctgcatacgggcgacgtttgatgaattcatcaggtgcgaggatgtcgttttagatggggctcaatatgggttctactctgatgggacgataaacgttccagggctttcattcggcggctggggtgtgacttttctgaattgcacattttacgacttcgcgaagtccatggttctgcatgctggaaatcgcacaaggcacagccttaacattattgcgagctactttaaccccatcaatacatcccccgagcgctgccatgatatagataatgtcgagggactgattatcgatggttgccagcacactcctagcactggaagccagccttcacaggaatggtttagggttattggtagtactggcaggatttcctgtaacgcctttgccggactttcctcaaaacttggaaccattggtggggcgaatccgtctgctgttgagtggtcgaataaccgggtttcttgccagggcggcctaaccataaccggtggagttgttcgcggtggcgggaatgagtacagcaatgccgaccactctgtagatgtcgctccggttgcaattgtatctttagacatcgggcctgacattcataaagccggcgtcactggttactcatataggatatcggcagatagctcgatgctgagtgggagagttaactactcattcgaacaggataattccaatagtaaatactatagcgcctctactagggtagggatgtcaaactgcgatagcaggttcataactcttgctactgctggaaccaaactgtcgccttataacgctgggcgcacgtacaatgtgactgttgcaggtacgcagaccttgccaaccccgatcccaggggctgcgccaatacgcattctaaagtccggcgcaaatgctctgacgattgcaaccacctctggaacaaacttcctgatcggtgcctccgggtcaaggaccagtgcagtggcgacctctactgaggtaggttctctcatagagtttgagccgttaacgtctacggcatgggttggcagagtgctatcaggcacttggtcatttacctgacagtttcggagatggggacacaaggattcctatccttgtgtttctttctacgatagtcactattacgatatccggtctgtacctatcaaccagatcggcaattactttagggctagaacgctgatgatgcagttgtagggtttctgagaacgtggcggccataaatggggatatagcagatccgaaagagtctcgaagccacagaacacgcttgttgttaagcgcgccctctgatcggaccaatagtggcttaacgggggctgtaacttgaacattgtctcccgagtagactttctccatgctttcgaagtctatttggctaacatggattttacgtatggaactgtccgacagatccacctctgcatccgtgatgtacggacgtatcctttggaatgcagaaaggtcgccgcctccccgtttccttataatcacagcctctggttttggttcttcaggtatagatatatctggggagttagattttatacgcttcgccagtgcataaaaagaaacccaagctcctagtgtattccagtgagtgtctgtcttgtagtataaaggtgcggtggatctagattttatattaataagttcattttttggatatacaaaaatatctggagattttctgtatatgtgctgggcaatgcttgtaccggaaggtgcagcccagtcaggaaggttctcggggtatatcgtagacttgtcagggccaattaaaacatagtagcccctaacgccatttgacgaaaaccattcacgccatccgtcagaaacgtttttgataatatctgtttttgcagtgtcggagtccgtgactccgactcgttttgcggttacagagttttcgaagaaatcgccgaggaacatccatccgtctcttccaataataaccttttcaggactaatggatattcctagcttgtagaaaatcatcccgatgtagggtagtgtaaaatccatgttgtaggaaaggtccttccaccctactatagtttctggaagtggtttgtttgagctaatcgcttgctcaatgtttacggcaggagctattcctagaacagcgatagaaatgaatatgaatgaatatattttccctttcacttctataatccttagaaattgaaatataggaatacagtgcttgttgattgtagtgtagagtacattgccaagcagaatagtattgacatgtatattgcttttaaatttccgatccttccggtcgttgaaagctcgaatgagtttttctgtgaaattatcaaaaatgctgctgcaatcattccatagcacagcgagttcgcaacaacaccgattggcagaaattgtaaaagcttgtcggaaattacccctgcccacgcaagatcgcttgtcggtatttcagccaggctttccgatgagatagatctaatatcaatcatccctccaaggattgacatggcttcctgcatggatgtggctcggaaaaatacccaggttatatttacgaatagaaatgtcacaacccaagccaaaggtcttggcatagacattccgagatttttccacattctgtggatgacaagcgctccaccatgcagcgccccccatatcacaaacatccagcttgctccatgccataggccaccaagaacaaacgttgccattaggttgaagtaaactctggcggaagaacagcggtttccacctaacgggatgtaaaggtagtctcgcagatagcggcttagggtcatgtgccaacgccgccagaaatcttgaatatcaagcgccttgtagggcgagttgaagtttattgggagccaaatgttaaagagaagggccgcgcctatggccatgtcgcagtaaccgctaaagtcaaagtatagttggaatgtgtaggaaaggcttgtcgcccatgatctgaagaaatcatgattggcaccgctcgaaaatcctgcatctgcccagacagagaatgtgtcagcgatcataactttcttgaataggccgatgctgaatataaacagtccagtaagaatatttctatagcgtactgcccatgtccatttcgacttgaattgacccatcatttccttgtggtggagtattgggccggcaattagatgcgggaagaatgtaacgaataaagcgtaatttattaggtcgtattcttttgcttcgcctctgtagctatccaccaagaatgcaatttgagtgaatgtgtagaagctaataccaagaggcaagattatttcatgtagcgcaaattctgatccggccgcagcattcaggttctcaataaaaaagttcgcatatttaaagtatccaagcagagccagattcgcagtaatgcttaatgctagtattgtttttctgtatccaccaatggataaattctttgaggtcggggagatcgcgcaccctactgcaaagttgaataaaattgaccctatcaggagtggtatatagtcaacgctccagtatccatagaagaaaacactggctaatactagccatattttccccaatgagatcatccttagcttgtttagtccaaaataaacaaagaacactattggcaagtaggccagtatgaaagcagcggaactgaagatcattatgccttcctgttcgttccctgatgagggaaggtttgttagtgctgtggccacatcgagggcggcgcagatcatacccaattggagcggaacatgcccatcactgagcagcagttgctgcatatcctcccgaacgccggctcgagggccggcgtttttgttggtgcgctgaaccgcgggatgacgcgcttcggtatcacgtcgcctgtgcgcgcggcgacgttcctcgcccaggtcggccacgaaagcggccagttgacccgcttggtggagaacctcaactacagtgcccgtggcctggctgcgacctggccgagccggtacctcggcgccgacggccagcccaacgccctggcgcagcgcctggcgcgcaacccccgagccatcgccaacaacgcctacgcctcgcgcaacggcaatggcgacgaggcatcgggcgacggctggcggtaccgcgggcgcgggctgctgcagatcaccggccgggcgaactaccgcgccgccggcgacgggctgggccagccgctggagcaggaacccgagcttctcgagcaaccggagtgggcggcgatctcggcggcctggtggtgggccagtcacggcttgaacgacctggccgaccgcggcgagttcgccgccatcactcggcgcatcaacggcggcacgaacggccaggcggagcgcctggcgctgtgggagcgggcgaagagggtgctgtcgtgatctccgcccgcgttctatcggtcgcgctggcctgcctgctactgctcggcctcggcgccgccggcggtgtctggctcggcgcgcggcactaccggccgcagctcgatgctgcgctggcggatctggtcgcctgccgtgcctcccggggagagttggagtccgcagtggcggagcaggtccggcaggttgccgcgctgcgcgtggtcggcgaacagcgggcccgggatgccgcgctggctgtggatcggggacgacagcaggccgcggagcagtatgccgcggcacagcgcctgctgagccagcgaaccgccggcgagcagtgtgcggccgccgaggcggtcattgatcaggagttgggcctatgaaactgcaggcgtggcgaaagactgcaggtgcagcgattttcggcaggtgcagccgaaaggcgcaggtggtgcaggtgctggggttggtgttcgcgctggcgggatgcgccggccaggtcgagcctgagccgcgcacggtgcgcgtagaagtgccggtggcggtgccgtgccgggtgccggcggtggaggttcccgcatgggccacggcggggctgcgaaaaggcgacgatctccagaccaaggtccgtgcgctgctggccgagcggcggcagcggatcgggtatgaagcccaactgctggctgccaacagagcatgccagtaggagtagactacggccttttcctacggagcttggtgatgctggtcattcgattcaagggctggtcggtgaaactcgaccaccaggtgggcagcgctgggaagttcggcatctggtcgttccacggttcggagagcagctacgtgccggacatggagacgattctccggcatgcagcgatccggccggcggagccgaaagaaggcgggcggtagggcccggcgtagcggcttacgaggcggagcgctgatcctgtaccagtttttgtaccaatcgatgcgaattctggcgaatcatggcgcctgaaagccttgattctactgctctccagcgcgctagctatcgccaaaaaaatcgcatggtgatgttagctgtagatatcaaggcattgtcctgcggggctttgcgggatggttacgcgccttcctctgcttcctgtaccaattccgtaccagttttaaccctggtctgtagcttctccaactcgctccaatccgaggcggagttcagccacttggcataggtcgatagcagcatctgcacgctgtggcctagctgtccagcgataaacgcagggttcatgccagccatcaggcacatggtcgcgtatgtgtggcgggtgtcatactgccggcgccttcggatggatagagcatcaagcgcggcgtggaagtgctttatggtaacacttggctccttgatccacagcccgcctttgctgggcgggaatacgaacgggctgaccgcgaactccgagactgatgcgacgcgcctcaggcgcgcaatccgcttggcctctaccagggcattcaatgctcgatcattgagcagcacgtcgcgctcatgcttggtctttacgcgttcctcgatcccgcgatctatgacgatccggcacacatgaatacgtcgtgcctcttcgtctacctcgtcccatcgaagggcgaacgcctctccaggccgaagaccagtgaagaacaggaattcgtacagtgcggcgtagatccttgagtacttcccaagggtcgcgtacaggtgctggatgatgcgttctgcctcgtcccgggtgaatggatctaccagtttcttagacacccgaggcttctcaaggggcgccatcgggttcttcttgatcagaccgtccttcacagcggaatctaggatcgtcgacagcttgaacatcgcgtttcgcttcacgcctggcgacgtccactcgatgctgctgatgattcggcgcaagagggtaggggtgatctgatcaagccgggctactgctagatgtggcatccagtattggttgaggatgctcttgtagttcttgcgtgtcccaagcacgatctctcggctgtctagccagagttgagcatgctcaccgaacagggggatttggctgctgaccgattccgcaatcgcagacccggggaagaactctgcataccgggcttcatccatgatgcccagcttgattgcctggactacctgatctctaagaccggatgcagtcttaatccctttttgcgtcgcgggataggggagtgtttcgcacttccttgttccgttccacatgaagcggatacggatagagttgccgatgacttccaccccggtgggcatacccaaaggctttcgagccattcgtcgtatctccgtcgactgtagattattttcccgttgaccttgttccagacgccttctggaatctgtccctttgaccgtctggtttgtagggcgcggtaggttatcccaagcagcgccgccatgacctgttcgggcaccaaaaaattagcgcaagaagacaaaaatcaccttgcgctaatgctctgttacagtcagatgcgcgcgccagcaagcagatcgatcgcttcggccgccacctgttgaggcagctcaatgccggggaagtgtgtttcgcccccgagacgacggtagctaaaccatggatggcgggcggcgaaatcgtcgtgaagtgcgtcgtactccccgatcttgggatgtgagaacacgtgccggatcgcgcacggttccgccagagcctccatgcgccgcatcggcgatccccaggttcggtaggcctcgtcaatcacccggccagcacgagcccacatgtcaaaaccgtgaccgccgctgtcgtatcgcacgtgatccagcaccgcttgattggtggtccccgccagccacgactgaacgaggccatcacgcccttccttccagcgctctggatcctggataccgtgcagcgcggcaacgaactcccgcggtgctggcgtcatgatgagatcgaggatcatcacggccgggacccgctgagcgccgagccgatcagcgatctcgagcgccgcccatccaccgtgcgcgtgggcgattggtacgaaactgtccacctcaagcgcatccagcaggccgatcgtgtctgccgccatctcgtcaataccgaagtcgccaactagattccgatcgggcccatgcccgcgccaacatacgcggaccgtccgctgcgctgcccgtagatacggcagcatgccgtcatacgcgcgaagatcgtgcgcccaaccgctcagcgtgacgaacaccgggcctggttcatgcccctggtcatcgaaggcgatctgcacgccattgacagtctttgtggtgatcataactcagctctcgaagtaccgacgtggattatccaccagcatggtgttgatctgatcctcggtgacgccgcgctcgagcagcgtgggaatgacctgatcgctgatgtgggtgaagttccagttcggtactgcggccgccttggcctcactcgagaaccagtcgatgaagcacgaggcatcatgtgccagaaccattttctcggcatagccacggcgggccagttccacgacagtgttcacccgctcctcgaacggcagcagaacatcgagaccgaaacggtccatcccgagtagcgaacccgcatcggcaagtgcacacaggtagtccaggtcggtcgaatcacccgagtgcccgatgacgaccttgctcagatctgcaccttcctcggccagaaccttctgcgcaacgaggcccgattccgtgtgcgggttcgtgtgaaccgtgatcggtaccccggtttcgacctgcgcctgaccgaccgctcgcatcacacgctcgacaccgggagtcagaccaggttcttcgatggcgcacttgaggaatgacgcgcggatgtctgtgccggcaatgccgtccttgatgtccttcacaaatagatcaaccataggctcgcgcacgtcgaacagcaaacctggaccggtgtaatggaattggaacggaatgtcgttgtacgtgtagacgccggtggcgacgatgatgttgagatcgacctgctcgttgatccgcgcaatacgcgggatgtagcgaccgagtccgatgaccgtgggatcgacgatcgtgctgatccctcgcgacttcagttcggacagcttggtcaccgcatcggctactcgagcctcctcgtcccaaggctccgggtagtcgggatagttctgacgcatctcctcccccagaacgaagacatgctcgtgcatcaacacctttcccagatcggctgtgtccaccggcccacgaacggtttgtactgaactcatggtttgaatccttgttggcgcctcgccgttgtggctggcatgacgttagattaggcacattgtgcctaattcgcaataggcacagtgtgccgcttgtccgaaagtggccattgtcttcgtactcgatttgctctgcggtactcatagacaatacctctccgccccagctattgccggggagggcatgatggtaggatttagacgcccagccgggttagctcagggagagctagtggcgcccggctgggttacttgatgagttcggctgggacgttgatggtttcgcccagcttcgctcgaacgatggcgcggcaggctgctattaggtgggttggacctgccgatgctgcatcagctggcatatcgcagccgcaggctgtgaagaatcgcagcggttcgccatgccagtcgctaccgatccactcgaattcaaagcggtgcttttcaatcagtggtccgccttgagcccatgagtccgaaggttcgtatcgctcgacttcttcagtaatcgagcgagggccaaaggtgcagccatatttgcagcagtgaatgccgcctctcacgtcataacggtactgtccaatgtcatggacaatgacctcttcgccttcagccattgcaacggcccaattaagcgctgccccctcaagatcccagatcttcacttctacggtttcgctcatagttggtcctccgggggggcggatacggttgggttcgttggggttattcgcccgctgctttggagatcaggtgcatgagcatttcgcgcagttgctcgcgctctagcacctgtccggttttcgcgtactcgtcggcctggcgcaggatcgcgtcgatctcgatgttgaacatcggcgagagcacgtctggctcgcactgctcgagcagcaactggattgcgcgggtcgggtgcgccatcgtgatcccgagccagttgtaggccgaggcagtgcggtagtagcgaaggccggcgatctcatgccgctgaggcgggcggaagggtttcgtgcgcatatgcaatccgggtaggttgagcctacattttccagattgctgtatatgcgtacagtggttggcgatgggtggctatgcctgctccgacaggtactgcaactcccaggtcgggtggaacttccttggcttgctttcgccgtcgagcttgatcatgaggtgggcgcccttggcgcttgtgattgtccctcgctcttcggtgccgcgccctcggtaaatgacttggccgccgcgcttgcatggaacggcataggccttgcggatgaactccatgctcattgcgtccctccctcctgctcgcccagcaggtcgcgcaggtcgttcgcaatctcaagcatcttcttcgcgcgtgtcgtggctgctttcgtgcctgccggaacgttttcgcagttccaatcggactctcggcggcactcccgctctatgcgtcgcagcaagtcctcggcgaccggcacatgaccatccgggaccatgtagagtgccttggtcctgcgctcggttctctcccttgatacatgcccgcaacgaccagcgagcgatcgactgatccctaattcgctgatgaacccgacgagggacagcttatcagccattgccgttctccttgccctggttgagcaggacgcgaaggtctgccgttatccggtagcattcagtcgggaacgaggtagaccaggcgcatgcgcagtactcttctgggccgcggcatggctcgttcatcacctgcttggcgatcagtccatggcgttcagcgctttcctgtatgcctgccccatcgaagcttccgccatcgagggctccgcagatgatctcgcgcgcgaacttggccatcccctgcacaagcccctcgctgaccgtcataccgttgatgcgcgccagttcgtcgaggcaggcgttccagccgctattacgatttagccctgggacgccggcatttagaagcttccgctccggcacaaccaccacccttgcgcgcagtgtcgcgagttcggcgcgaagctcctcgatctccatctccatgccgccgcactgctggcgggcagcatctccctttgccgctgcgtcctcggccatggctagtttggcgactagggcgtcgtagtcggaggccaggacgacctcataccccattactgcctgctcgccctgggtcaaagagcgcatgctcggcacgtcgaaccgcttcacctcactcatgacctacctccttgctggctgctcggcgcttcttcatgatctctgctacgccgtcggggtacgtgatagccacggccccggctgcgagagctgctgacttcttcgacaggcagatatcgaagtgctccttgatggtcccggcatgctgaatccacttccgctgaacaccgatcttgtctgccattgcgagcagttcctcggtcgtgtccgcgagcatgtgacacatcttcatgcggccaaaggttgcgttcatgtcgtcgacgtaaacggccatcacaccccctccttgccgggcgcggcggccttccgaagtgcggcgttcaatgctctttccatcgatttgaacggggactcgcccggtcggaaagcgtcaagggcagccacgatcatttcgccagtaaccttcagcacgctgtgctgagccgagctgccgggcacgtcggcgagtatggaaagcagttggcgctcagccgtaattcgggtgtcgtggtccttgtcgctcatcatgttgagaagcggctcaatcggaaccagcttccagccctccggcacgctgtgctgagccttggcgaccgctagcgcctcgttgagccggaacccttcgtgcacccagtccgtcaacttcccttccagctccgcgaccctggccagggcgacttccagccgcttagcgttttcgtcgcgctcgtacatcactttcatgcacttttcgaagctgccaacagggtcacctttggactcactcaggcgctcgacttcgaccagggcggcgtcgcgctctttacgcatttcatcccagtccgcgaggcgctgctctgcctgctctgcccacgaatcgcgatccgcccgcagctccccgacgatgcggtcgtgctgttcgaataggtcagcggctttctcggcgtactcgacgatggaaacgtcgcaccctgtatcgcggccttcggcatcctcgaagcgcagatcaacgttgtcgccgtcgatgtcttcagcgtccatagcgccgatgttgcgcaggacgaacgcgacttctgctacctccggccgctcctcttcccctaccaggtcggtcccccacttcgctacaggcacttcgaaccggtcgttggctacatcaatggcggcacgcagggttggggccggagagggttgagtctgcgctggggagggttgcgccagggcggcgcgggccatccaccccttcttgttttcccgtatggagtggtggttttcgttcagatcatacttgtcttcaattccatactccttgcaggcccaggctaggaacttctccagctcatccccgcctgcctgctctaccggtgccttgttcagttccttgctcacaatcccttctcctgccgctcaatagcagcgatgaattcgacaatctctgtgctgaggtccatggcgccaatgctgttgtggaccccgacgtagcggtttgcgcgcttcagaaggagcaccgctgtgcgcaggccggagtcacgcttggtcttcgccttgacttccatcatccacctccgggtagacctgaacgccctcggcgccctgggcctggttgatcgctatctgcctcaccgctctcgcgaatagcagaatgtcgtctggggtcatgagctggctttcttcgggccagccggtgaccgtcacaccgccagggcggtgatgcgctgttagctggtgcatggggttattcctgttcggggagagggagtcgcggcgctaacgatgcccgaacctgatgccgtgctcggcggcgatcttgcggacagtagcgcggtcaaggtccattgcgtctgcggtggcggagatagtcatccccttgtctgcgcagtaacggactgtttgcgatagcagcctgcgattctctcggcggttgctttcgaacgcagcgtgcgcggcgtcggtctgccctggcttagcttttcgtgccgacctaccgttccactggacgtccttgtctcccgacatgccgattgggatggatgcgatctttccgccgctggctaggaacgcatctacctggctggctatttcgtctcgatgcaagtcctggctcatgctgccacccctagcaccttttccatgcgctcctcgagcagttcgtagaaggtctttactcgctcggacagcttgcgtatgtaggcctcatcgcggtggacgcgcaccatgcaaagcggcatgcctggccagtagccgaggaagtcgatccactcgcgctccgaaacccaaaggcctccatagcactgagccgcgtgctcggaaggcagctcgcctgcgatgatcacgctaaccagcttttccggtaccttggttttcacctctatcaggccgttgtcgccgaccagtccatccggcgaatagccgatcccgtggttcagaatgatcccggcctgctggatctgatctggctcggtatctgtgcgcaggcagtacaagtcgcgcacaaccggctcaagcttgtgacccctggcgctgctaccgttaccacgccatggctcggcctctgctccggtgatccgctcaccaattagacggtccatgtaagtgaaggcgccaacgccgaaccctgcctggcctttgccgttaaccatcaacacgtccagttcggagcaggttgcgattccaagacgcgcgtcaagccactcctgggagccctgctccaggtccttgaagatctgcatgattcactcctgggagcgcttggcgcgctcgcgagccttggtaagccgtgccagtgccgcatcgaagtcggcggatgggacaccctcagcagagccgtacatagcatcgaaggcttcttgcgtgtcctgaaggcattgggagagaagggttttcagttgctgcgcctgagcttgggtaatgagcttctttggcggcacagccgcgttgccgtcgtcgtcctcgccgcgagtggtgatgttcagcagtgcggacagcacgtaacgcttgccgtagctgaccgatgatccaagagactgaacggcgttcttgctgccacttgtgtctagcggaacgagcatcgtcgtctgctctcggtgtccggcgcagtgcatcagaattccagtaaccgaaacgccagtctgaacagtctcgacgcggaagctcactgcgaaaccgaaccgctgcatgatcggcttcacgatgtcgttgatgtcttcgaaggtcgcgtagttgctgcgcttttggccgttgacggtgatagcgccacgctcggcaatgctcggcaattcgctttgcatggcggccatggatgcgttgaactcagcctctgcgctgcgggactgcatccgttcgtgcatggccataagccgctccatcttctcgatgtcgcacgcagggtcagcagcggcacgctggatcacttgaaggattgttgccgactcaccagcttggattacggcagcaccttcctgccgctgtgcaatggagttgctcatgatgggcctcagtagttgattgtgatgtgaggaaccttgcgctgagcgatcagtgtgatcgcctgcttggcgcattcctcgggcatgccgccggcgatcagggccgccagggcttcgttgttgatggctttcttgtgggccttgtcggcttctcgggctgctgcctcgcgctcgatcctggcttgctcgtctgcctgccgttggcgctctgcggcagcggcttcttcggcgcgccgctgtgcatcacgctcagcctgctcggcgcgttgctgtgcttccaacttctcgcgctccgccttctcggcagcgagtcgcagttccagttcccggcgctcggcggcagcctttgcctcggtttcgcggcgagcggcggcttcgcgttcttcctgggcgcgtcgttccgctgcaaggcgctcggcctcggctgcttcgcgggcaatgcgctcctcgcgctctttctgctcgcgtgctgctgcttcggcgcgcaggcgttccagttcggcctgctcggcttcgaacttctcacgggcaaccagggcttctcggagagcgatcaaagccttatctttggcgcgagcagcctctgcctcgaactcttcccaggcttcacttatggccaggccttccaaccaagcgatgttggctttgagttcattagagtccagatcgcggcattccaggcgaaggtttatcttgtcgatctcgccctgatgacgcgcaacccgcgccgcttcagcctcttcccactcggtcaacggactgcgcacttcggcctgccaggaatccaacaggtcgcgcatccgcttacgctcggcatcgatcttcttcggaacttccttcagctcagcgaccaattccttgcccacgttgtccagcgccgtcttggagcgggcgaccttgtaggcgatggaagcgatggcatcgcggcccttgcgggttgaaacgtccggcacgaagccgtcgatttcctcgcgaatcttggccaggaacgggtcaaggccattggctgccgagtagacttgcagagcggtttctttggctggtacttcgaccagttggttttctgcggacatgaatgatcctcgccgcgcatgcgcagccagtgaagggaggggttattggccagtggccgtagattctgcggtgatgatcccgccccagatcgggccggctgcgagaatgaacaggtacagcaggccgccgaagaggctgcctagccagattgctgtgcgtctggtgttcatagccctgccacctcaacaaacgccacggcgaacatgaacacgctgcccacaaaaaagccgccgaagatcaggacttgggcggcctctttcaggtctatggtgatggtcatggcgtgctctccattgcttcatcaacagctttgtctacggccttcccgaaaagccagttagacacctgatcgccacagtcatcggtaagcgacaccatcggatagaccccgtctgcgtccgccgacttgtcccgcaaccaccgatagcgcttagcatcagcctcagcagcgcgcaggcgagcgatcaggccaagtatctcctctgctggagtgttgatatttacatccgtcaacactggctcgttacagcagacttcctcgcgcgcgctcatgtattcggccccggatttgaaattgccacaacagacgaatgccctcttgtggcagtactcttccaactccgccaattgctcatcactgatcgattgcacgataggggttgtcatttcccttcctcctggcggcggtagccggcgtcaaatagcgcgtaaagcgtagggtactgatatggaactccttgaattgacatagccatatcaccgactgccttctcccgctcctcggcggcgatctgctcaggggttcggagcgggcggaaagcaggaagagatccgaatttcaaaacggcatatgacccgtactgcccctttcttttgccttcgcaccaacggaatacgacacggccctcgtcgtgagcgagtatcttggctcgaaagtacgcaatatcggcgccgtcccagatggcctcggcctcaatgccaatcggaggaaagccttggccgtcccatgaggtaggcacaagccgcggaacggaatcttcaatgagggacttgccttcttctgggttgcaatacctcatccaaaagggagggcagaagtacatcggtatctcgccatccttcagccacgggtaggcgagtttttggttgtagtgcgtcgcaccctctggtgccttgttccagtcaatgctcatactcgtctctccctaaccagtcgttcagcgttctcgatcagcgttgcttcgaatgcgcggaaccagatgcgttgtgccagttccaggtcgcctcggcgcactgcaagcagtagctgcgtcatcgggcactctttgccgtctacctcggcgagccactcgggcacgaatccagcaaagccgtagaccgtgaactccggcccgataaagggcctctctttccggtcatggaacggcacgcaatcaccgtcctcgcagttcaggagcttcccgacttgctcagtgacatactctcggtcgccgtcatcgtctggcggcagcgcgttgtcccagcgctcctgggcgtatttcaatgcagtgttcatttctcacctcagtcggtgtaggcgatgtacttgaactggcctttctcttcgttgaagtactcgaagcggccgccaaacgtcccgatcacggctttttcaacctcggcgcgcgaagtgccgatggggaaaactcccttcttgatcattgacgcgcccgaatgcggttcccatgtccagtcgattttggttgggtcaagcacccgaggcttgctttcgaggaaagccccatatccaccaatgtctaggatgatcgtgtgaatctcgcgcacacagagcggatcgtccgccgcgcgccaaccgcagtcaggacagcacatgtccgcgctcgtatgcgctgcacacggagggctaatatggcaactgcaattctcgaccctctccagctcaatcactccctcgcagccgccgcggttgcagatggagccttcctcgtatccgagttctttcatgtctcacctcgcgttcgcgtgcatgcggcagcgttccgaatcgctgtcgtcatacaggcgaaaaaatgcccggacttgccgggctaatgagcggtagggtggggatggccggagtttcaccggcggcttaattggtcactgccaataagctattaccgctattcgcatgcgatacttatccccattgaagggtggcgtccttgccggggaagtcagtcggctggaggcgctgggagtggcatccagtgcgttgggcgccagttgaaaattgatgaatgtattggatcaaaccaatcccacccagcgttcagggggccatcaccgcgctgccatgtcgcatagccgatactcccctccgtgtactttcgcatgtgagtttctctcacgccgtaatctgggcaataaccaagaaacttggtgccatcctttggagcgctatcaatcgttttccactcgctcatcttgcctccagtgtgtgtattcgccagggcgcggttaggcggttggtttgactggtcgaactgaaacaacaacccaagcatcatttccaataacaaatacacaggaagcttcttcgtaggggccgtcgtagaggttgccgtccgaaccttcttgcccgaaatcgatcttaccgttcatatcggcgattccatcccaaagcgggccagtagtcagcgcatgcgatgcccattccggggcgctcttccagtcgatatttacgctgttctccagcggaagctctggactcggcatccagtatttgaccttgtaacattggctttcgcctttacgttggcaccatgcgcctaaccattcgccttctccctcgtaagttgctccttctatttcatatcgcccacataccgggatcatgatcaggcatttgtcgccaacgtttggtagatgatcactacacttgatccactcactcatctatcacctcaccaataaatagtcagaaacagaacaacgaacagcgctgcgaactcgccaaggtctggcatggattcctctcttcccgtatcagggcaaatggattgcatcccgctgctagccaaggcttgcagggacgactttcatcgcttcagcgacaatcgagtgaactccttgtgagtcaaccgtggcgaaccccttttcggcgtggtcccactgctcatcctcgtctccggggaagttgctgcacgccactgaacagacgccaagcccgtcgggcttgaagtagaggcgcacctccgggccgtcatccccgcgatcaagcatcacgagcacctggcccaggtcttcgaactcaaacagcttcgcgaactgcttcattggtattcctcggtttggtttcccagatgcccctcggaggaagggcatcgaggaaatcggtattgctcccgcgttcgcctactgggcttctacaacccgcgggtgttgctgtcctcaccactgccgatagcagctcggactcgatgtgtttggccttgggcttccctcgctgcgccttcaatcggcttacggagcaggtcatggggactaggggtgatctcgagggttcgctgcagcccggcggcctggtgaagtgggcagctgatcgcgaggcgccgacccgtgtcgtcggctgggcttagtgcttcatgggatggttcctcctctggtgatggggtggagaactctccggtatggagcaggtcgatccctcttcggggcctggaaccgacttccctcggtccgtggtatccggcgagcctccggcttgttgccgcgttgttctgcggcgttgaggtgagtatgagactgctcatatttactgtcaatgagtattcccatatttttttatgaggtgactcatcggaggtttctcaggacgaaaaaaagcccgcgctaagcgggctcgttgggttgctggaggggcttaggaaccgattccgccgccacgccagataacgcggccgatgatcggtagatcatgaactgacgtttcgcttgcgatttcgtctgggtatgcggttttgtcagggttgtcgcttcgaatgagccaagcaccagttagctgttgattcaggcgcttgatgctgacgccgccgtctggtcgcctgatgacgtacacctgcttatcctggggctctatcttggccacgtcgaagagaaccacatcgccttcgaatatgtagggctccatgctgtcgccctctgcgtagatcacgaagaggttctctggtttggagttgacccgcttcagccaatctcgcttgaacaccaaaccttcagtggtctcaacgtgatcattgaaatatccatcgccgcactcgccgcgagcagtgtattggggaatcagggcgtagtccttttcgctcggggctcctggtggaacctcttcattgttgttcatgtttccacgcccggcggctagccatagtgcgcttacgccacaagcggcagccaactgagcaatatatgccgacccctgcgacttcccctgctcaaggttggaaattgaggtttggtccaggccgactcgttgagctaattgagcctgggtgagtttggcgtgcttgcgcgcggccttgatgcggtctttgagttccatccgaaaagtatcaggggcgttcccatatccttgcaaatgagtattcccctgggataccttatgagtattcccataaggagggatgctatgaccaccatctacaaagagctcgtcgcccattttgggactcaagacgagaccgccgcgaagctcggcgttgaccaaagcactgtgtctggatgggtccggggaaagcacgggatgtctcctgttgttgcgaagcgggctcaggttctgaccgacgggaaattcaagaaagaggacctgtgtccggctttcccgtgggaagtgctgtcggcggttgcctgacatgacagccagccaattaaacgccgagcaggaagcaagggcccgcacgttcttaggcgtctccttgcatggggatgatccgactgcaatagcccgcacgttccagacttggagcgcgatgctcgagcgctgctacatccctggatccatgagtggaaagcactaccttgggcgcggaataggcgtctgtgagcgctggttcgtcttctccaacttcgtgagagacatggggcttcgcccgaaggggacgactctcgaccgagtcgacaatgatggcgattacctcccagaaaactgccgctgggcaacccgccagcagcaggcgagaaacacccgtagaaacaaaatggttggcgatgtacttcaagtcgacgccgccattgcatcaggtgttctggcgtcgaccatctcccgtcgcatggcttctggctactcagcagaagaagccattgataactcaaagatcaccaaagtgaagctcactgcagagatggcgagagcgatcaaggatcgcctgaaaaccggtgatacccagtccaagattgctgcctgcttcggtgtctctcgccagatgatctccggaatagcctccggtcgatattggaggtctgcatgaacagcatggaaacccgcgctagaaaaaattacagcctcatcgtgcagcgacttgcatcggttggaaatgcgccggttgcgcatgcagtcggttgcgacgagtcgacgatcagccggatgaagccggagaagttcttggagttcgcccggatcttggctgtgctggacctgaaggtcgtaggcaacgagatgaagtgcttcaacgagaaggagatcgccgcgatcttgcacctggcgaagtcgaagctttccgaggtcgagagcgtcgagcagttggagtgggactgatgcgaaagcgcctcacgaataccgactacgccgcaatggctaacgctgctgaagagctggcgggtatgggttcgagtgagtggaggcgcagatacaacaaagccctgcgcgactactacagggctttgtcggtgcccc